European Patent Application EP 4 335 870 A1, published March 13, 2024. Title: PEPTIDE THERAPEUTICS AGAINST SARS-COV-2 SPIKE PROTEIN. Applicant: NantCell, Inc. Application EP. The sequence listing filed with the application follows.

SEQUENCE LISTING (245 sequences)

SEQ ID NO: 1 - protein, 327 aa, synthetic construct
  REGION 1..327: note = Receptor binding domain of SARS-CoV-2 Spike, fused to anendosomal targeting sequence
MLLLPFQLLAVLFPGGNSERVQPTESIVRFPNITNLCPFGEVFNATRFASVYAWNRKRISNCVADYSVLYNSASFSTFKCYGVSPTKLNDLCFTNVYADSFVIRGDEVRQIAPGQTGKIADYNYKLPDDFTGCVIAWNSNNLDSKVGGNYNYLYRLFRKSNLKPFERDISTEIYQAGSTPCNGVEGFNCYFPLQSYGFQPTNGVGYQPYRVVVLSFELLHAPATVCGPKKSTNLVKNKCVNFNFNGLTGTGVLTESNKKFLPFQQFGRDIADTTDAVRDPQTLEILDITPCSMLIPIAVGGALAGLVLIVLIAYLIGKKHCSYQDIL

SEQ ID NO: 2 - protein, 516 aa, synthetic construct
  REGION 1..516: note = SARS-CoV-2 N protein, fused to endosomal targeting sequence
MLLLPFQLLAVLFPGGNSEDYKDDDDKGGGSGGGSGGGSGGGSMSDNGPQNQRNAPRITFGGPSDSTGSNQNGERSGARSKQRRPQGLPNNTASWFTALTQHGKEDLKFPRGQGVPINTNSSPDDQIGYYRRATRRIRGGDGKMKDLSPRWYFYYLGTGPEAGLPYGANKDGIIWVATEGALNTPKDHIGTRNPANNAAIVLQLPQGTTLPKGFYAEGSRGGSQASSRSSSRSRNSSRNSTPGSSRGTSPARMAGNGGDAALALLLLDRLNQLESKMSGKGQQQQGQTVTKKSAAEASKKPRQKRTATKAYNVTQAFGRRGPEQTQGNFGDQELIRQGTDYKHWPQIAQFAPSASAFFGMSRIGMEVTPSGTWLTYTGAIKLDDKDPNFKDQVILLNKHIDAYKTFPPTEPKKDKKKKADETQALPQRQKKQQTVTLLPAADLDDFSKQLQQSMSSADSTQAGPGPGNLVPMVATVGPGPGMLIPIAVGGALAGLVLIVLIAYLIGKKHCSYQDIL

SEQ ID NO: 3 - protein, 6 aa, synthetic construct
  REGION 1..6: note = Anti-Spike Group 1, CDR-H1
SSYTMH

SEQ ID NO: 4 - protein, 10 aa, synthetic construct
  REGION 1..10: note = Anti-Spike Group 1, CDR-H2
AISGSGGSTY

SEQ ID NO: 5 - protein, 7 aa, synthetic construct
  REGION 1..7: note = Anti-Spike Group 1, CDR-H3
DLFDFWG

SEQ ID NO: 6 - protein, 6 aa, synthetic construct
  REGION 1..6: note = Anti-Spike Group 1, CDR-L3
DYGFPL

SEQ ID NO: 7 - protein, 6 aa, synthetic construct
  REGION 1..6: note = Anti-Spike Group 2, CDR-H1
SNYAMH

SEQ ID NO: 8 - protein, 10 aa, synthetic construct
  REGION 1..10: note = Anti-Spike Group 2, CDR-H2
AISGNGGSTG

SEQ ID NO: 9 - protein, 8 aa, synthetic construct
  REGION 1..8: note = Anti-Spike Group 2, CDR-H3
DRWYVKNA

SEQ ID NO: 10 - protein, 6 aa, synthetic construct
  REGION 1..6: note = Anti-Spike Group 2, CDR-L3
LDGTPF

SEQ ID NO: 11 - protein, 6 aa, synthetic construct
  REGION 1..6: note = Anti-Spike Group 3, CDR-H1
SSYAMH

SEQ ID NO: 12 - protein, 10 aa, synthetic construct
  REGION 1..10: note = Anti-Spike Group 3, CDR-H2
AIYGNGGSTD

SEQ ID NO: 13 - protein, 8 aa, synthetic construct
  REGION 1..8: note = Anti-Spike Group 3, CDR-H3
DRYMLWMA

SEQ ID NO: 14 - protein, 6 aa, synthetic construct
  REGION 1..6: note = Anti-Spike Group 3, CDR-L3
DTDDPL

SEQ ID NO: 15 - protein, 6 aa, synthetic construct
  REGION 1..6: note = Anti-Spike Group 4, CDR-H1
SSYAMS

SEQ ID NO: 16 - protein, 10 aa, synthetic construct
  REGION 1..10: note = Anti-Spike Group 4, CDR-H2
IISGSGGSTY

SEQ ID NO: 17 - protein, 8 aa, synthetic construct
  REGION 1..8: note = Anti-Spike Group 4, CDR-H3
DLYGLWNA

SEQ ID NO: 18 - protein, 6 aa, synthetic construct
  REGION 1..6: note = Anti-Spike Group 4, CDR-L3
DSADPR

SEQ ID NO: 19 - protein, 6 aa, synthetic construct
  REGION 1..6: note = Anti-Spike Group 5, CDR-H1
SSYAMS

SEQ ID NO: 20 - protein, 10 aa, synthetic construct
  REGION 1..10: note = Anti-Spike Group 5, CDR-H2
AIRGSGGSTY

SEQ ID NO: 21 - protein, 8 aa, synthetic construct
  REGION 1..8: note = Anti-Spike Group 5, CDR-H3
DRWCRCIA

SEQ ID NO: 22 - protein, 6 aa, synthetic construct
  REGION 1..6: note = Anti-Spike Group 5, CDR-L3
VAANPY

SEQ ID NO: 23 - protein, 6 aa, synthetic construct
  REGION 1..6: note = Anti-Spike Group 6, CDR-H1
SSYAMS

SEQ ID NO: 24 - protein, 10 aa, synthetic construct
  REGION 1..10: note = Anti-Spike Group 6, CDR-H2
AISGSGGSTN

SEQ ID NO: 25 - protein, 8 aa, synthetic construct
  REGION 1..8: note = Anti-Spike Group 6, CDR-H3
DLWGLAFA

SEQ ID NO: 26 - protein, 6 aa, synthetic construct
  REGION 1..6: note = Anti-Spike Group 6, CDR-L3
DSSNPW

SEQ ID NO: 27 - protein, 6 aa, synthetic construct
  REGION 1..6: note = Anti-Spike Group 7, CDR-H1
SSYYMH

SEQ ID NO: 28 - protein, 10 aa, synthetic construct
  REGION 1..10: note = Anti-Spike Group 7, CDR-H2
AISGSGGYTY

SEQ ID NO: 29 - protein, 9 aa, synthetic construct
  REGION 1..9: note = Anti-Spike Group 7, CDR-H3
DRDHAYDWG

SEQ ID NO: 30 - protein, 6 aa, synthetic construct
  REGION 1..6: note = Anti-Spike Group 7, CDR-L3
WADWPL

SEQ ID NO: 31 - protein, 6 aa, synthetic construct
  REGION 1..6: note = Anti-Spike Group 8, CDR-H1
SSYAMH

SEQ ID NO: 32 - protein, 10 aa, synthetic construct
  REGION 1..10: note = Anti-Spike Group 8, CDR-H2
AISWSGRSTY

SEQ ID NO: 33 - protein, 9 aa, synthetic construct
  REGION 1..9: note = Anti-Spike Group 8, CDR-H3
DLSSNWGCG

SEQ ID NO: 34 - protein, 6 aa, synthetic construct
  REGION 1..6: note = Anti-Spike Group 8, CDR-L3
SADTPF

SEQ ID NO: 35 - protein, 6 aa, synthetic construct
  REGION 1..6: note = Anti-Spike Group 9, CDR-H1
SSYAMT

SEQ ID NO: 36 - protein, 10 aa, synthetic construct
  REGION 1..10: note = Anti-Spike Group 9, CDR-H2
YISGSGGGTY

SEQ ID NO: 37 - protein, 9 aa, synthetic construct
  REGION 1..9: note = Anti-Spike Group 9, CDR-H3
DRWASGWLA

SEQ ID NO: 38 - protein, 6 aa, synthetic construct
  REGION 1..6: note = Anti-Spike Group 9, CDR-L3
AYAYPL

SEQ ID NO: 39 - protein, 6 aa, synthetic construct
  REGION 1..6: note = Anti-Spike Group 10, CDR-H1
SSYYMH

SEQ ID NO: 40 - protein, 10 aa, synthetic construct
  REGION 1..10: note = Anti-Spike Group 10, CDR-H2
AISGSGGYTY

SEQ ID NO: 41 - protein, 9 aa, synthetic construct
  REGION 1..9: note = Anti-Spike Group 10, CDR-H3
DLWGSGFFA

SEQ ID NO: 42 - protein, 6 aa, synthetic construct
  REGION 1..6: note = Anti-Spike Group 10, CDR-L3
DAGTPL

SEQ ID NO: 43 - protein, 6 aa, synthetic construct
  REGION 1..6: note = Anti-Spike Group 11, CDR-H1
SSYAMS

SEQ ID NO: 44 - protein, 10 aa, synthetic construct
  REGION 1..10: note = Anti-Spike Group 11, CDR-H2
LISGSGGSTY

SEQ ID NO: 45 - protein, 9 aa, synthetic construct
  REGION 1..9: note = Anti-Spike Group 11, CDR-H3
DLWGSGFFA

SEQ ID NO: 46 - protein, 6 aa, synthetic construct
  REGION 1..6: note = Anti-Spike Group 11, CDR-L3
DAGTPL

SEQ ID NO: 47 - protein, 6 aa, synthetic construct
  REGION 1..6: note = Anti-Spike Group 12, CDR-H1
SSYAMH

SEQ ID NO: 48 - protein, 10 aa, synthetic construct
  REGION 1..10: note = Anti-Spike Group 12, CDR-H2
LISGSGGSTD

SEQ ID NO: 49 - protein, 9 aa, synthetic construct
  REGION 1..9: note = Anti-Spike Group 12, CDR-H3
DLVVPYGPG

SEQ ID NO: 50 - protein, 6 aa, synthetic construct
  REGION 1..6: note = Anti-Spike Group 12, CDR-L3
STDGPL

SEQ ID NO: 51 - protein, 6 aa, synthetic construct
  REGION 1..6: note = Anti-Spike Group 13, CDR-H1
SSYAMS

SEQ ID NO: 52 - protein, 10 aa, synthetic construct
  REGION 1..10: note = Anti-Spike Group 13, CDR-H2
AISGSGGSTS

SEQ ID NO: 53 - protein, 9 aa, synthetic construct
  REGION 1..9: note = Anti-Spike Group 13, CDR-H3
DLFMEFMWA

SEQ ID NO: 54 - protein, 6 aa, synthetic construct
  REGION 1..6: note = Anti-Spike Group 13, CDR-L3
WANLPY

SEQ ID NO: 55 - protein, 6 aa, synthetic construct
  REGION 1..6: note = Anti-Spike Group 14, CDR-H1
SSYAMT

SEQ ID NO: 56 - protein, 10 aa, synthetic construct
  REGION 1..10: note = Anti-Spike Group 14, CDR-H2
AISGSGGSTY

SEQ ID NO: 57 - protein, 10 aa, synthetic construct
  REGION 1..10: note = Anti-Spike Group 14, CDR-H3
DRWWDSLWVG

SEQ ID NO: 58 - protein, 6 aa, synthetic construct
  REGION 1..6: note = Anti-Spike Group 14, CDR-L3
TDDNPF

SEQ ID NO: 59 - protein, 6 aa, synthetic construct
  REGION 1..6: note = Anti-Spike Group 15, CDR-H1
SSYAMS

SEQ ID NO: 60 - protein, 10 aa, synthetic construct
  REGION 1..10: note = Anti-Spike Group 15, CDR-H2
AISNSGGETY

SEQ ID NO: 61 - protein, 10 aa, synthetic construct
  REGION 1..10: note = Anti-Spike Group 15, CDR-H3
DLWVENLWWG

SEQ ID NO: 62 - protein, 6 aa, synthetic construct
  REGION 1..6: note = Anti-Spike Group 15, CDR-L3
TDDIPF

SEQ ID NO: 63 - protein, 6 aa, synthetic construct
  REGION 1..6: note = Anti-Spike Group 16, CDR-H1
SSYTMH

SEQ ID NO: 64 - protein, 10 aa, synthetic construct
  REGION 1..10: note = Anti-Spike Group 16, CDR-H2
AISGSGGYTY

SEQ ID NO: 65 - protein, 10 aa, synthetic construct
  REGION 1..10: note = Anti-Spike Group 16, CDR-H3
DRDLLWMGWA

SEQ ID NO: 66 - protein, 6 aa, synthetic construct
  REGION 1..6: note = Anti-Spike Group 16, CDR-L3
YANWPL

SEQ ID NO: 67 - protein, 6 aa, synthetic construct
  REGION 1..6: note = Anti-Spike Group 17, CDR-H1
SSYAMH

SEQ ID NO: 68 - protein, 10 aa, synthetic construct
  REGION 1..10: note = Anti-Spike Group 17, CDR-H2
AIWGSGSNTY

SEQ ID NO: 69 - protein, 11 aa, synthetic construct
  REGION 1..11: note = Anti-Spike Group 17, CDR-H3
GRDLAAFTKTA

SEQ ID NO: 70 - protein, 6 aa, synthetic construct
  REGION 1..6: note = Anti-Spike Group 17, CDR-L3
HDALPW

SEQ ID NO: 71 - protein, 6 aa, synthetic construct
  REGION 1..6: note = Anti-Spike Group 18, CDR-H1
NSYAMH

SEQ ID NO: 72 - protein, 10 aa, synthetic construct
  REGION 1..10: note = Anti-Spike Group 18, CDR-H2
AISGSGGRTY

SEQ ID NO: 73 - protein, 12 aa, synthetic construct
  REGION 1..12: note = Anti-Spike Group 18, CDR-H3
DLRSSWVFYTLA

SEQ ID NO: 74 - protein, 6 aa, synthetic construct
  REGION 1..6: note = Anti-Spike Group 18, CDR-L3
GYTIPL

SEQ ID NO: 75 - protein, 6 aa, synthetic construct
  REGION 1..6: note = Anti-Spike Group 19, CDR-H1
SNYAMH

SEQ ID NO: 76 - protein, 10 aa, synthetic construct
  REGION 1..10: note = Anti-Spike Group 19, CDR-H2
AISGSGGSTY

SEQ ID NO: 77 - protein, 13 aa, synthetic construct
  REGION 1..13: note = Anti-Spike Group 19, CDR-H3
DLSFWLTYHLASA

SEQ ID NO: 78 - protein, 6 aa, synthetic construct
  REGION 1..6: note = Anti-Spike Group 19, CDR-L3
SYSDPL

SEQ ID NO: 79 - protein, 6 aa, synthetic construct
  REGION 1..6: note = Anti-Spike Group 20, CDR-H1
SSYAMH

SEQ ID NO: 80 - protein, 10 aa, synthetic construct
  REGION 1..10: note = Anti-Spike Group 20, CDR-H2
AIDGNGGYTY

SEQ ID NO: 81 - protein, 13 aa, synthetic construct
  REGION 1..13: note = Anti-Spike Group 20, CDR-H3
GRVSASWYGADVG

SEQ ID NO: 82 - protein, 6 aa, synthetic construct
  REGION 1..6: note = Anti-Spike Group 20, CDR-L3
SYGIPL

SEQ ID NO: 83 - protein, 6 aa, synthetic construct
  REGION 1..6: note = Anti-RBD Group 1, CDR-H1
NSYAMH

SEQ ID NO: 84 - protein, 10 aa, synthetic construct
  REGION 1..10: note = Anti-RBD Group 1, CDR-H2
AISGNGGSTY

SEQ ID NO: 85 - protein, 8 aa, synthetic construct
  REGION 1..8: note = Anti-RBD Group 1, CDR-H3
DRCFAIWG

SEQ ID NO: 86 - protein, 6 aa, synthetic construct
  REGION 1..6: note = Anti-RBD Group 1, CDR-L3
YDDHPF

SEQ ID NO: 87 - protein, 6 aa, synthetic construct
  REGION 1..6: note = Anti-RBD Group 2, CDR-H1
SSYAMN

SEQ ID NO: 88 - protein, 10 aa, synthetic construct
  REGION 1..10: note = Anti-RBD Group 2, CDR-H2
AISGSGGSTY

SEQ ID NO: 89 - protein, 8 aa, synthetic construct
  REGION 1..8: note = Anti-RBD Group 2, CDR-H3
GRVWVWVA

SEQ ID NO: 90 - protein, 6 aa, synthetic construct
  REGION 1..6: note = Anti-RBD Group 2, CDR-L3
WDALPR

SEQ ID NO: 91 - protein, 6 aa, synthetic construct
  REGION 1..6: note = Anti-RBD Group 3, CDR-H1
GSYAMH

SEQ ID NO: 92 - protein, 10 aa, synthetic construct
  REGION 1..10: note = Anti-RBD Group 3, CDR-H2
GISGSGGYTY

SEQ ID NO: 93 - protein, 8 aa, synthetic construct
  REGION 1..8: note = Anti-RBD Group 3, CDR-H3
DRLNMFLA

SEQ ID NO: 94 - protein, 6 aa, synthetic construct
  REGION 1..6: note = Anti-RBD Group 3, CDR-L3
DAGTPL

SEQ ID NO: 95 - protein, 6 aa, synthetic construct
  REGION 1..6: note = Anti-RBD Group 4, CDR-H1
SSYAMN

SEQ ID NO: 96 - protein, 10 aa, synthetic construct
  REGION 1..10: note = Anti-RBD Group 4, CDR-H2
AISGGGGNTY

SEQ ID NO: 97 - protein, 8 aa, synthetic construct
  REGION 1..8: note = Anti-RBD Group 4, CDR-H3
DLRCRPGA

SEQ ID NO: 98 - protein, 6 aa, synthetic construct
  REGION 1..6: note = Anti-RBD Group 4, CDR-L3
LYSDPY

SEQ ID NO: 99 - protein, 6 aa, synthetic construct
  REGION 1..6: note = Anti-RBD Group 5, CDR-H1
SSYAMS

SEQ ID NO: 100 - protein, 10 aa, synthetic construct
  REGION 1..10: note = Anti-RBD Group 5, CDR-H2
LISGSGGSTY

SEQ ID NO: 101 - protein, 9 aa, synthetic construct
  REGION 1..9: note = Anti-RBD Group 5, CDR-H3
DLWGSGFFA

SEQ ID NO: 102 - protein, 6 aa, synthetic construct
  REGION 1..6: note = Anti-RBD Group 5, CDR-L3
DAGTPL

SEQ ID NO: 103 - protein, 6 aa, synthetic construct
  REGION 1..6: note = Anti-RBD Group 6, CDR-H1
SAYAMH

SEQ ID NO: 104 - protein, 10 aa, synthetic construct
  REGION 1..10: note = Anti-RBD Group 6, CDR-H2
AIWGSGGSTY

SEQ ID NO: 105 - protein, 9 aa, synthetic construct
  REGION 1..9: note = Anti-RBD Group 6, CDR-H3
DLWMAMWFG

SEQ ID NO: 106 - protein, 6 aa, synthetic construct
  REGION 1..6: note = Anti-RBD Group 6, CDR-L3
RSTYPL

SEQ ID NO: 107 - protein, 6 aa, synthetic construct
  REGION 1..6: note = Anti-RBD Group 7, CDR-H1
SNYAMH

SEQ ID NO: 108 - protein, 10 aa, synthetic construct
  REGION 1..10: note = Anti-RBD Group 7, CDR-H2
AISWSGGSTY

SEQ ID NO: 109 - protein, 9 aa, synthetic construct
  REGION 1..9: note = Anti-RBD Group 7, CDR-H3
DRFYIVLLG

SEQ ID NO: 110 - protein, 6 aa, synthetic construct
  REGION 1..6: note = Anti-RBD Group 7, CDR-L3
RDAGPF

SEQ ID NO: 111 - protein, 6 aa, synthetic construct
  REGION 1..6: note = Anti-RBD Group 8, CDR-H1
SSYAMS

SEQ ID NO: 112 - protein, 10 aa, synthetic construct
  REGION 1..10: note = Anti-RBD Group 8, CDR-H2
AISSSGGSTN

SEQ ID NO: 113 - protein, 10 aa, synthetic construct
  REGION 1..10: note = Anti-RBD Group 8, CDR-H3
DLWSERVWFG

SEQ ID NO: 114 - protein, 6 aa, synthetic construct
  REGION 1..6: note = Anti-RBD Group 8, CDR-L3
VDNAPY

SEQ ID NO: 115 - protein, 6 aa, synthetic construct
  REGION 1..6: note = Anti-RBD Group 9, CDR-H1
SSYAMH

SEQ ID NO: 116 - protein, 10 aa, synthetic construct
  REGION 1..10: note = Anti-RBD Group 9, CDR-H2
AIWGSGSNTY

SEQ ID NO: 117 - protein, 11 aa, synthetic construct
  REGION 1..11: note = Anti-RBD Group 9, CDR-H3
GRDLAAFTKTA

SEQ ID NO: 118 - protein, 6 aa, synthetic construct
  REGION 1..6: note = Anti-RBD Group 9, CDR-L3
HDALPW

SEQ ID NO: 119 - protein, 6 aa, synthetic construct
  REGION 1..6: note = Anti-RBD Group 10, CDR-H1
SSYAMN

SEQ ID NO: 120 - protein, 10 aa, synthetic construct
  REGION 1..10: note = Anti-RBD Group 10, CDR-H2
AISGSGGSTY

SEQ ID NO: 121 - protein, 12 aa, synthetic construct
  REGION 1..12: note = Anti-RBD Group 10, CDR-H3
DLLWTSKAVWWG

SEQ ID NO: 122 - protein, 6 aa, synthetic construct
  REGION 1..6: note = Anti-RBD Group 10, CDR-L3
SATMPW

SEQ ID NO: 123 - protein, 6 aa, synthetic construct
  REGION 1..6: note = Anti-RBD Group 11, CDR-H1
SSYAMT

SEQ ID NO: 124 - protein, 10 aa, synthetic construct
  REGION 1..10: note = Anti-RBD Group 11, CDR-H2
AIDGNGGSTS

SEQ ID NO: 125 - protein, 12 aa, synthetic construct
  REGION 1..12: note = Anti-RBD Group 11, CDR-H3
DLGFMTIVAFAA

SEQ ID NO: 126 - protein, 6 aa, synthetic construct
  REGION 1..6: note = Anti-RBD Group 11, CDR-L3
SYDRPW

SEQ ID NO: 127 - protein, 29 aa, Homo sapiens
EVQLVESGGGLVQPGGSLRLSCAASGFTF

SEQ ID NO: 128 - protein, 14 aa, Homo sapiens
WVRQAPGKGLEWVS

SEQ ID NO: 129 - protein, 39 aa, Homo sapiens
YADSVKGRFTISRDNSKNTLYLQMNSLRAEDTAVYYCAR

SEQ ID NO: 130 - protein, 14 aa, Homo sapiens
FDVWGQGTLVTVSS

SEQ ID NO: 131 - protein, 90 aa, Homo sapiens
DIQMTQSPSSLSASVGDRVTITCQASQDISNYLNWYQQKPGKAPKLLIYDASNLETGVPSRFSGSGSGTDFTFTISSLQPEDIATYYCQQ

SEQ ID NO: 132 - protein, 11 aa, Homo sapiens
TFGQGTKVEIK

SEQ ID NO: 133 - protein, 419 aa, SARS CoV
MSDNGPQNQRNAPRITFGGPSDSTGSNQNGERSGARSKQRRPQGLPNNTASWFTALTQHGKEDLKFPRGQGVPINTNSSPDDQIGYYRRATRRIRGGDGKMKDLSPRWYFYYLGTGPEAGLPYGANKDGIIWVATEGALNTPKDHIGTRNPANNAAIVLQLPQGTTLPKGFYAEGSRGGSQASSRSSSRSRNSSRNSTPGSSRGTSPARMAGNGGDAALALLLLDRLNQLESKMSGKGQQQQGQTVTKKSAAEASKKPRQKRTATKAYNVTQAFGRRGPEQTQGNFGDQELIRQGTDYKHWPQIAQFAPSASAFFGMSRIGMEVTPSGTWLTYTGAIKLDDKDPNFKDQVILLNKHIDAYKTFPPTEPKKDKKKKADETQALPQRQKKQQTVTLLPAADLDDFSKQLQQSMSSADSTQA

SEQ ID NO: 134 - protein, 422 aa, SARS CoV-2
MSDNGPQSNQRSAPRITFGGPTDSTDNNQNGGRNGARPKQRRPQGLPNNTASWFTALTQHGKEELRFPRGQGVPINTNSGPDDQIGYYRRATRRVRGGDGKMKELSPRWYFYYLGTGPEASLPYGANKEGIVWVATEGALNTPKDHIGTRNPNNNAATVLQLPQGTTLPKGFYAEGSRGGSQASSRSSSRSRGNSRNSTPGSSRGNSPARMASGGGETALALLLLDRLNQLESKVSGKGQQQQGQTVTKKSAAEASKKPRQKRTATKQYNVTQAFGRRGPEQTQGNFGDQDLIRQGTDYKHWPQIAQFAPSASAFFGMSRIGMEVTPSGTWLTYHGAIKLDDKDPQFKDNVILLNKHIDAYKTFPPTEPKKDKKKKTDEAQPLPQRQKKQPTVTLLPAADMDDFSRQLQNSMSGASADSTQA

SEQ ID NO: 135 - protein, 805 aa, Homo sapiens [sequence omitted]

SEQ ID NO: 136 - protein, 805 aa, synthetic construct
  REGION 1..805: note = Q24 mutant ACE2
  MUTAGEN 24: note = The sequence here can be Ala, Arg, Asn, Asp, Cys, Glu, Gly, His,Ile, Lys, Leu, Met, Phe, Pro, Ser, Thr, Trp, Tyr, or Val.
MSSSSWLLLSLVAVTAAQSTIEEXAKTFLDKFNHEAEDLFYQSSLASWNYNTNITEENVQNMNNAGDKWSAFLKEQSTLAQMYPLQEIQNLTVKLQLQALQQNGSSVLSEDKSKRLNTILNTMSTIYSTGKVCNPDNPQECLLLEPGLNEIMANSLDYNERLWAWESWRSEVGKQLRPLYEEYVVLKNEMARANHYEDYGDYWRGDYEVNGVDGYDYSRGQLIEDVEHTFEEIKPLYEHLHAYVRAKLMNAYPSYISPIGCLPAHLLGDMWGRFWTNLYSLTVPFGQKPNIDVTDAMVDQAWDAQRIFKEAEKFFVSVGLPNMTQGFWENSMLTDPGNVQKAVCHPTAWDLGKGDFRILMCTKVTMDDFLTAHHEMGHIQYDMAYAAQPFLLRNGANEGFHEAVGEIMSLSAATPKHLKSIGLLSPDFQEDNETEINFLLKQALTIVGTLPFTYMLEKWRWMVFKGEIPKDQWMKKWWEMKREIVGVVEPVPHDETYCDPASLFHVSNDYSFIRYYTRTLYQFQFQEALCQAAKHEGPLHKCDISNSTEAGQKLFNMLRLGKSEPWTLALENVVGAKNMNVRPLLNYFEPLFTWLKDQNKNSFVGWSTDWSPYADQSIKVRISLKSALGDKAYEWNDNEMYLFRSSVAYAMRQYFLKVKNQMILFGEEDVRVANLKPRISFNFFVTAPKNVSDIIPRTEVEKAIRMSRSRINDAFRLNDNSLEFLGIQPTLGPPNQPPVSIWLIVFGVVMGVIVVGIVILIFTGIRDRKKKNKARSGENPYASIDISKGENNPGFQNTDDVQTSF

SEQ ID NO: 137 - protein, 805 aa, synthetic construct
  REGION 1..805: note = T27 mutant ACE2
  MUTAGEN 27: note = The sequence here can be Ala, Arg, Asn, Asp, Cys, Gln, Glu, Gly,His, Ile, Lys, Leu, Met, Phe, Pro, Ser, Trp, Tyr, or Val.
MSSSSWLLLSLVAVTAAQSTIEEQAKXFLDKFNHEAEDLFYQSSLASWNYNTNITEENVQNMNNAGDKWSAFLKEQSTLAQMYPLQEIQNLTVKLQLQALQQNGSSVLSEDKSKRLNTILNTMSTIYSTGKVCNPDNPQECLLLEPGLNEIMANSLDYNERLWAWESWRSEVGKQLRPLYEEYVVLKNEMARANHYEDYGDYWRGDYEVNGVDGYDYSRGQLIEDVEHTFEEIKPLYEHLHAYVRAKLMNAYPSYISPIGCLPAHLLGDMWGRFWTNLYSLTVPFGQKPNIDVTDAMVDQAWDAQRIFKEAEKFFVSVGLPNMTQGFWENSMLTDPGNVQKAVCHPTAWDLGKGDFRILMCTKVTMDDFLTAHHEMGHIQYDMAYAAQPFLLRNGANEGFHEAVGEIMSLSAATPKHLKSIGLLSPDFQEDNETEINFLLKQALTIVGTLPFTYMLEKWRWMVFKGEIPKDQWMKKWWEMKREIVGVVEPVPHDETYCDPASLFHVSNDYSFIRYYTRTLYQFQFQEALCQAAKHEGPLHKCDISNSTEAGQKLFNMLRLGKSEPWTLALENVVGAKNMNVRPLLNYFEPLFTWLKDQNKNSFVGWSTDWSPYADQSIKVRISLKSALGDKAYEWNDNEMYLFRSSVAYAMRQYFLKVKNQMILFGEEDVRVANLKPRISFNFFVTAPKNVSDIIPRTEVEKAIRMSRSRINDAFRLNDNSLEFLGIQPTLGPPNQPPVSIWLIVFGVVMGVIVVGIVILIFTGIRDRKKKNKARSGENPYASIDISKGENNPGFQNTDDVQTSF

SEQ ID NO: 138 - protein, 805 aa, synthetic construct
  REGION 1..805: note = D30 mutant ACE2
  MUTAGEN 30: note = The sequence here can be Ala, Arg, Asn, Cys, Gln, Glu, Gly, His,Ile, Lys, Leu, Met, Phe, Pro, Ser, Thr, Trp, Tyr, or Val.
MSSSSWLLLSLVAVTAAQSTIEEQAKTFLXKFNHEAEDLFYQSSLASWNYNTNITEENVQNMNNAGDKWSAFLKEQSTLAQMYPLQEIQNLTVKLQLQALQQNGSSVLSEDKSKRLNTILNTMSTIYSTGKVCNPDNPQECLLLEPGLNEIMANSLDYNERLWAWESWRSEVGKQLRPLYEEYVVLKNEMARANHYEDYGDYWRGDYEVNGVDGYDYSRGQLIEDVEHTFEEIKPLYEHLHAYVRAKLMNAYPSYISPIGCLPAHLLGDMWGRFWTNLYSLTVPFGQKPNIDVTDAMVDQAWDAQRIFKEAEKFFVSVGLPNMTQGFWENSMLTDPGNVQKAVCHPTAWDLGKGDFRILMCTKVTMDDFLTAHHEMGHIQYDMAYAAQPFLLRNGANEGFHEAVGEIMSLSAATPKHLKSIGLLSPDFQEDNETEINFLLKQALTIVGTLPFTYMLEKWRWMVFKGEIPKDQWMKKWWEMKREIVGVVEPVPHDETYCDPASLFHVSNDYSFIRYYTRTLYQFQFQEALCQAAKHEGPLHKCDISNSTEAGQKLFNMLRLGKSEPWTLALENVVGAKNMNVRPLLNYFEPLFTWLKDQNKNSFVGWSTDWSPYADQSIKVRISLKSALGDKAYEWNDNEMYLFRSSVAYAMRQYFLKVKNQMILFGEEDVRVANLKPRISFNFFVTAPKNVSDIIPRTEVEKAIRMSRSRINDAFRLNDNSLEFLGIQPTLGPPNQPPVSIWLIVFGVVMGVIVVGIVILIFTGIRDRKKKNKARSGENPYASIDISKGENNPGFQNTDDVQTSF

SEQ ID NO: 139 - protein, 805 aa, synthetic construct
  REGION 1..805: note = H34 mutant ACE2
  MUTAGEN 34: note = The sequence here can be Ala, Arg, Asn, Asp, Cys, Gln, Glu, Gly,Ile, Lys, Leu, Met, Phe, Pro, Ser, Thr, Trp, Tyr, or Val.
MSSSSWLLLSLVAVTAAQSTIEEQAKTFLDKFNXEAEDLFYQSSLASWNYNTNITEENVQNMNNAGDKWSAFLKEQSTLAQMYPLQEIQNLTVKLQLQALQQNGSSVLSEDKSKRLNTILNTMSTIYSTGKVCNPDNPQECLLLEPGLNEIMANSLDYNERLWAWESWRSEVGKQLRPLYEEYVVLKNEMARANHYEDYGDYWRGDYEVNGVDGYDYSRGQLIEDVEHTFEEIKPLYEHLHAYVRAKLMNAYPSYISPIGCLPAHLLGDMWGRFWTNLYSLTVPFGQKPNIDVTDAMVDQAWDAQRIFKEAEKFFVSVGLPNMTQGFWENSMLTDPGNVQKAVCHPTAWDLGKGDFRILMCTKVTMDDFLTAHHEMGHIQYDMAYAAQPFLLRNGANEGFHEAVGEIMSLSAATPKHLKSIGLLSPDFQEDNETEINFLLKQALTIVGTLPFTYMLEKWRWMVFKGEIPKDQWMKKWWEMKREIVGVVEPVPHDETYCDPASLFHVSNDYSFIRYYTRTLYQFQFQEALCQAAKHEGPLHKCDISNSTEAGQKLFNMLRLGKSEPWTLALENVVGAKNMNVRPLLNYFEPLFTWLKDQNKNSFVGWSTDWSPYADQSIKVRISLKSALGDKAYEWNDNEMYLFRSSVAYAMRQYFLKVKNQMILFGEEDVRVANLKPRISFNFFVTAPKNVSDIIPRTEVEKAIRMSRSRINDAFRLNDNSLEFLGIQPTLGPPNQPPVSIWLIVFGVVMGVIVVGIVILIFTGIRDRKKKNKARSGENPYASIDISKGENNPGFQNTDDVQTSF

SEQ ID NO: 140 - protein, 805 aa, synthetic construct
  REGION 1..805: note = E35 mutant ACE2
  MUTAGEN 35: note = The sequence here can be Ala, Arg, Asn, Asp, Cys, Gln, Gly, His,Ile, Lys, Leu, Met, Phe, Pro, Ser, Thr, Trp, Tyr, or Val.
MSSSSWLLLSLVAVTAAQSTIEEQAKTFLDKFNHXAEDLFYQSSLASWNYNTNITEENVQNMNNAGDKWSAFLKEQSTLAQMYPLQEIQNLTVKLQLQALQQNGSSVLSEDKSKRLNTILNTMSTIYSTGKVCNPDNPQECLLLEPGLNEIMANSLDYNERLWAWESWRSEVGKQLRPLYEEYVVLKNEMARANHYEDYGDYWRGDYEVNGVDGYDYSRGQLIEDVEHTFEEIKPLYEHLHAYVRAKLMNAYPSYISPIGCLPAHLLGDMWGRFWTNLYSLTVPFGQKPNIDVTDAMVDQAWDAQRIFKEAEKFFVSVGLPNMTQGFWENSMLTDPGNVQKAVCHPTAWDLGKGDFRILMCTKVTMDDFLTAHHEMGHIQYDMAYAAQPFLLRNGANEGFHEAVGEIMSLSAATPKHLKSIGLLSPDFQEDNETEINFLLKQALTIVGTLPFTYMLEKWRWMVFKGEIPKDQWMKKWWEMKREIVGVVEPVPHDETYCDPASLFHVSNDYSFIRYYTRTLYQFQFQEALCQAAKHEGPLHKCDISNSTEAGQKLFNMLRLGKSEPWTLALENVVGAKNMNVRPLLNYFEPLFTWLKDQNKNSFVGWSTDWSPYADQSIKVRISLKSALGDKAYEWNDNEMYLFRSSVAYAMRQYFLKVKNQMILFGEEDVRVANLKPRISFNFFVTAPKNVSDIIPRTEVEKAIRMSRSRINDAFRLNDNSLEFLGIQPTLGPPNQPPVSIWLIVFGVVMGVIVVGIVILIFTGIRDRKKKNKARSGENPYASIDISKGENNPGFQNTDDVQTSF

SEQ ID NO: 141 - protein, 805 aa, synthetic construct
  REGION 1..805: note = D38 mutant ACE2
  MUTAGEN 38: note = The sequence here can be Ala, Arg, Asn, Cys, Gln, Glu, Gly, His,Ile, Lys, Leu, Met, Phe, Pro, Ser, Thr, Trp, Tyr, or Val.
MSSSSWLLLSLVAVTAAQSTIEEQAKTFLDKFNHEAEXLFYQSSLASWNYNTNITEENVQNMNNAGDKWSAFLKEQSTLAQMYPLQEIQNLTVKLQLQALQQNGSSVLSEDKSKRLNTILNTMSTIYSTGKVCNPDNPQECLLLEPGLNEIMANSLDYNERLWAWESWRSEVGKQLRPLYEEYVVLKNEMARANHYEDYGDYWRGDYEVNGVDGYDYSRGQLIEDVEHTFEEIKPLYEHLHAYVRAKLMNAYPSYISPIGCLPAHLLGDMWGRFWTNLYSLTVPFGQKPNIDVTDAMVDQAWDAQRIFKEAEKFFVSVGLPNMTQGFWENSMLTDPGNVQKAVCHPTAWDLGKGDFRILMCTKVTMDDFLTAHHEMGHIQYDMAYAAQPFLLRNGANEGFHEAVGEIMSLSAATPKHLKSIGLLSPDFQEDNETEINFLLKQALTIVGTLPFTYMLEKWRWMVFKGEIPKDQWMKKWWEMKREIVGVVEPVPHDETYCDPASLFHVSNDYSFIRYYTRTLYQFQFQEALCQAAKHEGPLHKCDISNSTEAGQKLFNMLRLGKSEPWTLALENVVGAKNMNVRPLLNYFEPLFTWLKDQNKNSFVGWSTDWSPYADQSIKVRISLKSALGDKAYEWNDNEMYLFRSSVAYAMRQYFLKVKNQMILFGEEDVRVANLKPRISFNFFVTAPKNVSDIIPRTEVEKAIRMSRSRINDAFRLNDNSLEFLGIQPTLGPPNQPPVSIWLIVFGVVMGVIVVGIVILIFTGIRDRKKKNKARSGENPYASIDISKGENNPGFQNTDDVQTSF

SEQ ID NO: 142 - protein, 805 aa, synthetic construct
  REGION 1..805: note = Y41 mutant ACE2
  MUTAGEN 41: note = The sequence here can be Ala, Arg, Asn, Asp, Cys, Gln, Glu, Gly,His, Ile, Lys, Leu, Met, Phe, Pro, Ser, Thr, Trp, or Val.
MSSSSWLLLSLVAVTAAQSTIEEQAKTFLDKFNHEAEDLFXQSSLASWNYNTNITEENVQNMNNAGDKWSAFLKEQSTLAQMYPLQEIQNLTVKLQLQALQQNGSSVLSEDKSKRLNTILNTMSTIYSTGKVCNPDNPQECLLLEPGLNEIMANSLDYNERLWAWESWRSEVGKQLRPLYEEYVVLKNEMARANHYEDYGDYWRGDYEVNGVDGYDYSRGQLIEDVEHTFEEIKPLYEHLHAYVRAKLMNAYPSYISPIGCLPAHLLGDMWGRFWTNLYSLTVPFGQKPNIDVTDAMVDQAWDAQRIFKEAEKFFVSVGLPNMTQGFWENSMLTDPGNVQKAVCHPTAWDLGKGDFRILMCTKVTMDDFLTAHHEMGHIQYDMAYAAQPFLLRNGANEGFHEAVGEIMSLSAATPKHLKSIGLLSPDFQEDNETEINFLLKQALTIVGTLPFTYMLEKWRWMVFKGEIPKDQWMKKWWEMKREIVGVVEPVPHDETYCDPASLFHVSNDYSFIRYYTRTLYQFQFQEALCQAAKHEGPLHKCDISNSTEAGQKLFNMLRLGKSEPWTLALENVVGAKNMNVRPLLNYFEPLFTWLKDQNKNSFVGWSTDWSPYADQSIKVRISLKSALGDKAYEWNDNEMYLFRSSVAYAMRQYFLKVKNQMILFGEEDVRVANLKPRISFNFFVTAPKNVSDIIPRTEVEKAIRMSRSRINDAFRLNDNSLEFLGIQPTLGPPNQPPVSIWLIVFGVVMGVIVVGIVILIFTGIRDRKKKNKARSGENPYASIDISKGENNPGFQNTDDVQTSF

SEQ ID NO: 143 - protein, 805 aa, synthetic construct
  REGION 1..805: note = D355 mutant ACE2
  MUTAGEN 355: note = The sequence here can be Ala, Arg, Asn, Cys, Gln, Glu, Gly, His,Ile, Lys, Leu, Met, Phe, Pro, Ser, Thr, Trp, Tyr, or Val.
MSSSSWLLLSLVAVTAAQSTIEEQAKTFLDKFNHEAEDLFYQSSLASWNYNTNITEENVQNMNNAGDKWSAFLKEQSTLAQMYPLQEIQNLTVKLQLQALQQNGSSVLSEDKSKRLNTILNTMSTIYSTGKVCNPDNPQECLLLEPGLNEIMANSLDYNERLWAWESWRSEVGKQLRPLYEEYVVLKNEMARANHYEDYGDYWRGDYEVNGVDGYDYSRGQLIEDVEHTFEEIKPLYEHLHAYVRAKLMNAYPSYISPIGCLPAHLLGDMWGRFWTNLYSLTVPFGQKPNIDVTDAMVDQAWDAQRIFKEAEKFFVSVGLPNMTQGFWENSMLTDPGNVQKAVCHPTAWDLGKGXFRILMCTKVTMDDFLTAHHEMGHIQYDMAYAAQPFLLRNGANEGFHEAVGEIMSLSAATPKHLKSIGLLSPDFQEDNETEINFLLKQALTIVGTLPFTYMLEKWRWMVFKGEIPKDQWMKKWWEMKREIVGVVEPVPHDETYCDPASLFHVSNDYSFIRYYTRTLYQFQFQEALCQAAKHEGPLHKCDISNSTEAGQKLFNMLRLGKSEPWTLALENVVGAKNMNVRPLLNYFEPLFTWLKDQNKNSFVGWSTDWSPYADQSIKVRISLKSALGDKAYEWNDNEMYLFRSSVAYAMRQYFLKVKNQMILFGEEDVRVANLKPRISFNFFVTAPKNVSDIIPRTEVEKAIRMSRSRINDAFRLNDNSLEFLGIQPTLGPPNQPPVSIWLIVFGVVMGVIVVGIVILIFTGIRDRKKKNKARSGENPYASIDISKGENNPGFQNTDDVQTSF

SEQ ID NO: 144 - protein, 805 aa, synthetic construct
  REGION 1..805: note = Mutant ACE2
  MUTAGEN 24: note = The sequence here can be Ala, Arg, Asn, Asp, Cys, Glu, Gly, His,Ile, Lys, Leu, Met, Phe, Pro, Ser, Thr, Trp, Tyr, or Val.
  MUTAGEN 27: note = The sequence here can be Ala, Arg, Asn, Asp, Cys, Gln, Glu, Gly,His, Ile, Lys, Leu, Met, Phe, Pro, Ser, Trp, Tyr, or Val.
  MUTAGEN 30: note = The sequence here can be Ala, Arg, Asn, Cys, Gln, Glu, Gly, His,Ile, Lys, Leu, Met, Phe, Pro, Ser, Thr, Trp, Tyr, or Val.
  MUTAGEN 34: note = The sequence here can be Ala, Arg, Asn, Asp, Cys, Gln, Glu, Gly,Ile, Lys, Leu, Met, Phe, Pro, Ser, Thr, Trp, Tyr, or Val.
  MUTAGEN 35: note = The sequence here can be Ala, Arg, Asn, Asp, Cys, Gln, Gly, His,Ile, Lys, Leu, Met, Phe, Pro, Ser, Thr, Trp, Tyr, or Val.
  MUTAGEN 38: note = The sequence here can be Ala, Arg, Asn, Cys, Gln, Glu, Gly, His,Ile, Lys, Leu, Met, Phe, Pro, Ser, Thr, Trp, Tyr, or Val.
  MUTAGEN 41: note = The sequence here can be Ala, Arg, Asn, Asp, Cys, Gln, Glu, Gly,His, Ile, Lys, Leu, Met, Phe, Pro, Ser, Thr, Trp, or Val.
  MUTAGEN 273: note = The sequence here can be Ala, Asn, Asp, Cys, Gln, Glu, Gly, His,Ile, Lys, Leu, Met, Phe, Pro, Ser, Thr, Trp, Tyr, or Val.
  MUTAGEN 345: note = The sequence here can be Ala, Arg, Asn, Asp, Cys, Gln, Glu, Gly,Ile, Lys, Leu, Met, Phe, Pro, Ser, Thr, Trp, Tyr, or Val.
  MUTAGEN 355: note = The sequence here can be Ala, Arg, Asn, Cys, Gln, Glu, Gly, His,Ile, Lys, Leu, Met, Phe, Pro, Ser, Thr, Trp, Tyr, or Val.
  MUTAGEN 374: note = The sequence here can be Ala, Arg, Asn, Asp, Cys, Gln, Glu, Gly,Ile, Lys, Leu, Met, Phe, Pro, Ser, Thr, Trp, Tyr, or Val.
  MUTAGEN 378: note = The sequence here can be Ala, Arg, Asn, Asp, Cys, Gln, Glu, Gly,Ile, Lys, Leu, Met, Phe, Pro, Ser, Thr, Trp, Tyr, or Val.
  MUTAGEN 505: note = The sequence here can be Ala, Arg, Asn, Asp, Cys, Gln, Glu, Gly,Ile, Lys, Leu, Met, Phe, Pro, Ser, Thr, Trp, Tyr, or Val.
MSSSSWLLLSLVAVTAAQSTIEEXAKXFLXKFNXXAEXLFXQSSLASWNYNTNITEENVQNMNNAGDKWSAFLKEQSTLAQMYPLQEIQNLTVKLQLQALQQNGSSVLSEDKSKRLNTILNTMSTIYSTGKVCNPDNPQECLLLEPGLNEIMANSLDYNERLWAWESWRSEVGKQLRPLYEEYVVLKNEMARANHYEDYGDYWRGDYEVNGVDGYDYSRGQLIEDVEHTFEEIKPLYEHLHAYVRAKLMNAYPSYISPIGCLPAHLLGDMWGXFWTNLYSLTVPFGQKPNIDVTDAMVDQAWDAQRIFKEAEKFFVSVGLPNMTQGFWENSMLTDPGNVQKAVCXPTAWDLGKGXFRILMCTKVTMDDFLTAHXEMGXIQYDMAYAAQPFLLRNGANEGFHEAVGEIMSLSAATPKHLKSIGLLSPDFQEDNETEINFLLKQALTIVGTLPFTYMLEKWRWMVFKGEIPKDQWMKKWWEMKREIVGVVEPVPHDETYCDPASLFXVSNDYSFIRYYTRTLYQFQFQEALCQAAKHEGPLHKCDISNSTEAGQKLFNMLRLGKSEPWTLALENVVGAKNMNVRPLLNYFEPLFTWLKDQNKNSFVGWSTDWSPYADQSIKVRISLKSALGDKAYEWNDNEMYLFRSSVAYAMRQYFLKVKNQMILFGEEDVRVANLKPRISFNFFVTAPKNVSDIIPRTEVEKAIRMSRSRINDAFRLNDNSLEFLGIQPTLGPPNQPPVSIWLIVFGVVMGVIVVGIVILIFTGIRDRKKKNKARSGENPYASIDISKGENNPGFQNTDDVQTSF

SEQ ID NO: 145 - protein, 225 aa, Homo sapiens
THTCPPCPAPELLGGPSVFLFPPKPKDTLMISRTPEVTCVVVDVSHEDPQVKFNWYVDGVQVHNAKTKPREQQYNSTYRVVSVLTVLHQNWLDGKEYKCKVSNKALPAPIEKTISKAKGQPREPQVYTLPPSREEMTKNQVSLTCLVKGFYPSDIAVEWESNGQPENNYKTTPPVLDSDGSFFLYSKLTVDKSRWQQGNVFSCSVMHEALHNHYTQKSLSLSPGK

SEQ ID NO: 146 - protein, 275 aa, Homo sapiens
MDPKQTTLLCLGDFPMPFISAKSSPVIPLDGSVKIQCQAIREAYLTQLMIIKNSTYREIGRRLKFWNETDPEFVIDHMDANKAGRYQCQYRIGHYRFRYSDTLELVVTGLYGKPFLSADRGLVLMPGENISLTCSSAHIPFDRFSLAKEGELSLPQHQSGEHPANFSLGPVDLNVSGIYRCYGWYNRSPYLWSFPSNALELVVTDSIHQDYTTQNLIRMAVAGLVLVALLAILVENWHSHTALNKEASADVAEPSWSQQMCQPGLTFARTPSVCK

SEQ ID NO: 147 - protein, 594 aa, synthetic construct
  REGION 1..594: note = D30E ACE2 mutant
IEEQAKTFLEKFNHEAEDLFYQSSLASWNYNTNITEENVQNMNNAGDKWSAFLKEQSTLAQMYPLQEIQNLTVKLQLQALQQNGSSVLSEDKSKRLNTILNTMSTIYSTGKVCNPDNPQECLLLEPGLNEIMANSLDYNERLWAWESWRSEVGKQLRPLYEEYVVLKNEMARANHYEDYGDYWRGDYEVNGVDGYDYSRGQLIEDVEHTFEEIKPLYEHLHAYVRAKLMNAYPSYISPIGCLPAHLLGDMWGRFWTNLYSLTVPFGQKPNIDVTDAMVDQAWDAQRIFKEAEKFFVSVGLPNMTQGFWENSMLTDPGNVQKAVCHPTAWDLGKGDFRILMCTKVTMDDFLTAHHEMGHIQYDMAYAAQPFLLRNGANEGFHEAVGEIMSLSAATPKHLKSIGLLSPDFQEDNETEINFLLKQALTIVGTLPFTYMLEKWRWMVFKGEIPKDQWMKKWWEMKREIVGVVEPVPHDETYCDPASLFHVSNDYSFIRYYTRTLYQFQFQEALCQAAKHEGPLHKCDISNSTEAGQKLFNMLRLGKSEPWTLALENVVGAKNMNVRPLLNYFEPLFTWLKDQNKNSFVGWSTDWSPYA

SEQ ID NO: 148 - protein, 594 aa, synthetic construct
  REGION 1..594: note = D38M ACE2 mutant
IEEQAKTFLDKFNHEAMDLFYQSSLASWNYNTNITEENVQNMNNAGDKWSAFLKEQSTLAQMYPLQEIQNLTVKLQLQALQQNGSSVLSEDKSKRLNTILNTMSTIYSTGKVCNPDNPQECLLLEPGLNEIMANSLDYNERLWAWESWRSEVGKQLRPLYEEYVVLKNEMARANHYEDYGDYWRGDYEVNGVDGYDYSRGQLIEDVEHTFEEIKPLYEHLHAYVRAKLMNAYPSYISPIGCLPAHLLGDMWGRFWTNLYSLTVPFGQKPNIDVTDAMVDQAWDAQRIFKEAEKFFVSVGLPNMTQGFWENSMLTDPGNVQKAVCHPTAWDLGKGDFRILMCTKVTMDDFLTAHHEMGHIQYDMAYAAQPFLLRNGANEGFHEAVGEIMSLSAATPKHLKSIGLLSPDFQEDNETEINFLLKQALTIVGTLPFTYMLEKWRWMVFKGEIPKDQWMKKWWEMKREIVGVVEPVPHDETYCDPASLFHVSNDYSFIRYYTRTLYQFQFQEALCQAAKHEGPLHKCDISNSTEAGQKLFNMLRLGKSEPWTLALENVVGAKNMNVRPLLNYFEPLFTWLKDQNKNSFVGWSTDWSPYA

SEQ ID NO: 149 - protein, 594 aa, synthetic construct
  REGION 1..594: note = D38W ACE2 mutant
IEEQAKTFLDKFNHEAWDLFYQSSLASWNYNTNITEENVQNMNNAGDKWSAFLKEQSTLAQMYPLQEIQNLTVKLQLQALQQNGSSVLSEDKSKRLNTILNTMSTIYSTGKVCNPDNPQECLLLEPGLNEIMANSLDYNERLWAWESWRSEVGKQLRPLYEEYVVLKNEMARANHYEDYGDYWRGDYEVNGVDGYDYSRGQLIEDVEHTFEEIKPLYEHLHAYVRAKLMNAYPSYISPIGCLPAHLLGDMWGRFWTNLYSLTVPFGQKPNIDVTDAMVDQAWDAQRIFKEAEKFFVSVGLPNMTQGFWENSMLTDPGNVQKAVCHPTAWDLGKGDFRILMCTKVTMDDFLTAHHEMGHIQYDMAYAAQPFLLRNGANEGFHEAVGEIMSLSAATPKHLKSIGLLSPDFQEDNETEINFLLKQALTIVGTLPFTYMLEKWRWMVFKGEIPKDQWMKKWWEMKREIVGVVEPVPHDETYCDPASLFHVSNDYSFIRYYTRTLYQFQFQEALCQAAKHEGPLHKCDISNSTEAGQKLFNMLRLGKSEPWTLALENVVGAKNMNVRPLLNYFEPLFTWLKDQNKNSFVGWSTDWSPYA

SEQ ID NO: 150 - protein, 594 aa, synthetic construct
  REGION 1..594: note = D38Y ACE2 mutant
IEEQAKTFLDKFNHEAYDLFYQSSLASWNYNTNITEENVQNMNNAGDKWSAFLKEQSTLAQMYPLQEIQNLTVKLQLQALQQNGSSVLSEDKSKRLNTILNTMSTIYSTGKVCNPDNPQECLLLEPGLNEIMANSLDYNERLWAWESWRSEVGKQLRPLYEEYVVLKNEMARANHYEDYGDYWRGDYEVNGVDGYDYSRGQLIEDVEHTFEEIKPLYEHLHAYVRAKLMNAYPSYISPIGCLPAHLLGDMWGRFWTNLYSLTVPFGQKPNIDVTDAMVDQAWDAQRIFKEAEKFFVSVGLPNMTQGFWENSMLTDPGNVQKAVCHPTAWDLGKGDFRILMCTKVTMDDFLTAHHEMGHIQYDMAYAAQPFLLRNGANEGFHEAVGEIMSLSAATPKHLKSIGLLSPDFQEDNETEINFLLKQALTIVGTLPFTYMLEKWRWMVFKGEIPKDQWMKKWWEMKREIVGVVEPVPHDETYCDPASLFHVSNDYSFIRYYTRTLYQFQFQEALCQAAKHEGPLHKCDISNSTEAGQKLFNMLRLGKSEPWTLALENVVGAKNMNVRPLLNYFEPLFTWLKDQNKNSFVGWSTDWSPYA

SEQ ID NO: 151 - protein, 594 aa, synthetic construct
  REGION 1..594: note = H34E ACE2 mutant
IEEQAKTFLDKFNEEAEDLFYQSSLASWNYNTNITEENVQNMNNAGDKWSAFLKEQSTLAQMYPLQEIQNLTVKLQLQALQQNGSSVLSEDKSKRLNTILNTMSTIYSTGKVCNPDNPQECLLLEPGLNEIMANSLDYNERLWAWESWRSEVGKQLRPLYEEYVVLKNEMARANHYEDYGDYWRGDYEVNGVDGYDYSRGQLIEDVEHTFEEIKPLYEHLHAYVRAKLMNAYPSYISPIGCLPAHLLGDMWGRFWTNLYSLTVPFGQKPNIDVTDAMVDQAWDAQRIFKEAEKFFVSVGLPNMTQGFWENSMLTDPGNVQKAVCHPTAWDLGKGDFRILMCTKVTMDDFLTAHHEMGHIQYDMAYAAQPFLLRNGANEGFHEAVGEIMSLSAATPKHLKSIGLLSPDFQEDNETEINFLLKQALTIVGTLPFTYMLEKWRWMVFKGEIPKDQWMKKWWEMKREIVGVVEPVPHDETYCDPASLFHVSNDYSFIRYYTRTLYQFQFQEALCQAAKHEGPLHKCDISNSTEAGQKLFNMLRLGKSEPWTLALENVVGAKNMNVRPLLNYFEPLFTWLKDQNKNSFVGWSTDWSPYA

SEQ ID NO: 152 - protein, 594 aa, synthetic construct
  REGION 1..594: note = H34F ACE2 mutant
IEEQAKTFLDKFNFEAEDLFYQSSLASWNYNTNITEENVQNMNNAGDKWSAFLKEQSTLAQMYPLQEIQNLTVKLQLQALQQNGSSVLSEDKSKRLNTILNTMSTIYSTGKVCNPDNPQECLLLEPGLNEIMANSLDYNERLWAWESWRSEVGKQLRPLYEEYVVLKNEMARANHYEDYGDYWRGDYEVNGVDGYDYSRGQLIEDVEHTFEEIKPLYEHLHAYVRAKLMNAYPSYISPIGCLPAHLLGDMWGRFWTNLYSLTVPFGQKPNIDVTDAMVDQAWDAQRIFKEAEKFFVSVGLPNMTQGFWENSMLTDPGNVQKAVCHPTAWDLGKGDFRILMCTKVTMDDFLTAHHEMGHIQYDMAYAAQPFLLRNGANEGFHEAVGEIMSLSAATPKHLKSIGLLSPDFQEDNETEINFLLKQALTIVGTLPFTYMLEKWRWMVFKGEIPKDQWMKKWWEMKREIVGVVEPVPHDETYCDPASLFHVSNDYSFIRYYTRTLYQFQFQEALCQAAKHEGPLHKCDISNSTEAGQKLFNMLRLGKSEPWTLALENVVGAKNMNVRPLLNYFEPLFTWLKDQNKNSFVGWSTDWSPYA

SEQ ID NO: 153 - protein, 594 aa, synthetic construct
  REGION 1..594: note = H34K ACE2 mutant
IEEQAKTFLDKFNKEAEDLFYQSSLASWNYNTNITEENVQNMNNAGDKWSAFLKEQSTLAQMYPLQEIQNLTVKLQLQALQQNGSSVLSEDKSKRLNTILNTMSTIYSTGKVCNPDNPQECLLLEPGLNEIMANSLDYNERLWAWESWRSEVGKQLRPLYEEYVVLKNEMARANHYEDYGDYWRGDYEVNGVDGYDYSRGQLIEDVEHTFEEIKPLYEHLHAYVRAKLMNAYPSYISPIGCLPAHLLGDMWGRFWTNLYSLTVPFGQKPNIDVTDAMVDQAWDAQRIFKEAEKFFVSVGLPNMTQGFWENSMLTDPGNVQKAVCHPTAWDLGKGDFRILMCTKVTMDDFLTAHHEMGHIQYDMAYAAQPFLLRNGANEGFHEAVGEIMSLSAATPKHLKSIGLLSPDFQEDNETEINFLLKQALTIVGTLPFTYMLEKWRWMVFKGEIPKDQWMKKWWEMKREIVGVVEPVPHDETYCDPASLFHVSNDYSFIRYYTRTLYQFQFQEALCQAAKHEGPLHKCDISNSTEAGQKLFNMLRLGKSEPWTLALENVVGAKNMNVRPLLNYFEPLFTWLKDQNKNSFVGWSTDWSPYA

SEQ ID NO: 154 - protein, 594 aa, synthetic construct
  REGION 1..594: note = H34M ACE2 mutant
IEEQAKTFLDKFNMEAEDLFYQSSLASWNYNTNITEENVQNMNNAGDKWSAFLKEQSTLAQMYPLQEIQNLTVKLQLQALQQNGSSVLSEDKSKRLNTILNTMSTIYSTGKVCNPDNPQECLLLEPGLNEIMANSLDYNERLWAWESWRSEVGKQLRPLYEEYVVLKNEMARANHYEDYGDYWRGDYEVNGVDGYDYSRGQLIEDVEHTFEEIKPLYEHLHAYVRAKLMNAYPSYISPIGCLPAHLLGDMWGRFWTNLYSLTVPFGQKPNIDVTDAMVDQAWDAQRIFKEAEKFFVSVGLPNMTQGFWENSMLTDPGNVQKAVCHPTAWDLGKGDFRILMCTKVTMDDFLTAHHEMGHIQYDMAYAAQPFLLRNGANEGFHEAVGEIMSLSAATPKHLKSIGLLSPDFQEDNETEINFLLKQALTIVGTLPFTYMLEKWRWMVFKGEIPKDQWMKKWWEMKREIVGVVEPVPHDETYCDPASLFHVSNDYSFIRYYTRTLYQFQFQEALCQAAKHEGPLHKCDISNSTEAGQKLFNMLRLGKSEPWTLALENVVGAKNMNVRPLLNYFEPLFTWLKDQNKNSFVGWSTDWSPYA

SEQ ID NO: 155 - protein, 594 aa, synthetic construct
  REGION 1..594: note = H34W ACE2 mutant
IEEQAKTFLDKFNWEAEDLFYQSSLASWNYNTNITEENVQNMNNAGDKWSAFLKEQSTLAQMYPLQEIQNLTVKLQLQALQQNGSSVLSEDKSKRLNTILNTMSTIYSTGKVCNPDNPQECLLLEPGLNEIMANSLDYNERLWAWESWRSEVGKQLRPLYEEYVVLKNEMARANHYEDYGDYWRGDYEVNGVDGYDYSRGQLIEDVEHTFEEIKPLYEHLHAYVRAKLMNAYPSYISPIGCLPAHLLGDMWGRFWTNLYSLTVPFGQKPNIDVTDAMVDQAWDAQRIFKEAEKFFVSVGLPNMTQGFWENSMLTDPGNVQKAVCHPTAWDLGKGDFRILMCTKVTMDDFLTAHHEMGHIQYDMAYAAQPFLLRNGANEGFHEAVGEIMSLSAATPKHLKSIGLLSPDFQEDNETEINFLLKQALTIVGTLPFTYMLEKWRWMVFKGEIPKDQWMKKWWEMKREIVGVVEPVPHDETYCDPASLFHVSNDYSFIRYYTRTLYQFQFQEALCQAAKHEGPLHKCDISNSTEAGQKLFNMLRLGKSEPWTLALENVVGAKNMNVRPLLNYFEPLFTWLKDQNKNSFVGWSTDWSPYA

SEQ ID NO: 156 - protein, 594 aa, synthetic construct; identical to SEQ ID NO: 152
  REGION 1..594: note = H34Y ACE2 mutant

SEQ ID NO: 157 - protein, 594 aa, synthetic construct
  REGION 1..594: note = T27F ACE2 mutant
IEEQAKFFLDKFNHEAEDLFYQSSLASWNYNTNITEENVQNMNNAGDKWSAFLKEQSTLAQMYPLQEIQNLTVKLQLQALQQNGSSVLSEDKSKRLNTILNTMSTIYSTGKVCNPDNPQECLLLEPGLNEIMANSLDYNERLWAWESWRSEVGKQLRPLYEEYVVLKNEMARANHYEDYGDYWRGDYEVNGVDGYDYSRGQLIEDVEHTFEEIKPLYEHLHAYVRAKLMNAYPSYISPIGCLPAHLLGDMWGRFWTNLYSLTVPFGQKPNIDVTDAMVDQAWDAQRIFKEAEKFFVSVGLPNMTQGFWENSMLTDPGNVQKAVCHPTAWDLGKGDFRILMCTKVTMDDFLTAHHEMGHIQYDMAYAAQPFLLRNGANEGFHEAVGEIMSLSAATPKHLKSIGLLSPDFQEDNETEINFLLKQALTIVGTLPFTYMLEKWRWMVFKGEIPKDQWMKKWWEMKREIVGVVEPVPHDETYCDPASLFHVSNDYSFIRYYTRTLYQFQFQEALCQAAKHEGPLHKCDISNSTEAGQKLFNMLRLGKSEPWTLALENVVGAKNMNVRPLLNYFEPLFTWLKDQNKNSFVGWSTDWSPYA

SEQ ID NO: 158 - protein, 594 aa, synthetic construct
  REGION 1..594: note = T27W ACE2 mutant
IEEQAKWFLDKFNHEAEDLFYQSSLASWNYNTNITEENVQNMNNAGDKWSAFLKEQSTLAQMYPLQEIQNLTVKLQLQALQQNGSSVLSEDKSKRLNTILNTMSTIYSTGKVCNPDNPQECLLLEPGLNEIMANSLDYNERLWAWESWRSEVGKQLRPLYEEYVVLKNEMARANHYEDYGDYWRGDYEVNGVDGYDYSRGQLIEDVEHTFEEIKPLYEHLHAYVRAKLMNAYPSYISPIGCLPAHLLGDMWGRFWTNLYSLTVPFGQKPNIDVTDAMVDQAWDAQRIFKEAEKFFVSVGLPNMTQGFWENSMLTDPGNVQKAVCHPTAWDLGKGDFRILMCTKVTMDDFLTAHHEMGHIQYDMAYAAQPFLLRNGANEGFHEAVGEIMSLSAATPKHLKSIGLLSPDFQEDNETEINFLLKQALTIVGTLPFTYMLEKWRWMVFKGEIPKDQWMKKWWEMKREIVGVVEPVPHDETYCDPASLFHVSNDYSFIRYYTRTLYQFQFQEALCQAAKHEGPLHKCDISNSTEAGQKLFNMLRLGKSEPWTLALENVVGAKNMNVRPLLNYFEPLFTWLKDQNKNSFVGWSTDWSPYA

SEQ ID NO: 159 - protein, 594 aa, synthetic construct
  REGION 1..594: note = T27Y ACE2 mutant
IEEQAKYFLDKFNHEAEDLFYQSSLASWNYNTNITEENVQNMNNAGDKWSAFLKEQSTLAQMYPLQEIQNLTVKLQLQALQQNGSSVLSEDKSKRLNTILNTMSTIYSTGKVCNPDNPQECLLLEPGLNEIMANSLDYNERLWAWESWRSEVGKQLRPLYEEYVVLKNEMARANHYEDYGDYWRGDYEVNGVDGYDYSRGQLIEDVEHTFEEIKPLYEHLHAYVRAKLMNAYPSYISPIGCLPAHLLGDMWGRFWTNLYSLTVPFGQKPNIDVTDAMVDQAWDAQRIFKEAEKFFVSVGLPNMTQGFWENSMLTDPGNVQKAVCHPTAWDLGKGDFRILMCTKVTMDDFLTAHHEMGHIQYDMAYAAQPFLLRNGANEGFHEAVGEIMSLSAATPKHLKSIGLLSPDFQEDNETEINFLLKQALTIVGTLPFTYMLEKWRWMVFKGEIPKDQWMKKWWEMKREIVGVVEPVPHDETYCDPASLFHVSNDYSFIRYYTRTLYQFQFQEALCQAAKHEGPLHKCDISNSTEAGQKLFNMLRLGKSEPWTLALENVVGAKNMNVRPLLNYFEPLFTWLKDQNKNSFVGWSTDWSPYA

SEQ ID NO: 160 - protein, 595 aa, synthetic construct
  REGION 1..595: note = ACE2 mutant, Ala inserted at #30
IEEQAKTFLADKFNHEAEDLFYQSSLASWNYNTNITEENVQNMNNAGDKWSAFLKEQSTLAQMYPLQEIQNLTVKLQLQALQQNGSSVLSEDKSKRLNTILNTMSTIYSTGKVCNPDNPQECLLLEPGLNEIMANSLDYNERLWAWESWRSEVGKQLRPLYEEYVVLKNEMARANHYEDYGDYWRGDYEVNGVDGYDYSRGQLIEDVEHTFEEIKPLYEHLHAYVRAKLMNAYPSYISPIGCLPAHLLGDMWGRFWTNLYSLTVPFGQKPNIDVTDAMVDQAWDAQRIFKEAEKFFVSVGLPNMTQGFWENSMLTDPGNVQKAVCHPTAWDLGKGDFRILMCTKVTMDDFLTAHHEMGHIQYDMAYAAQPFLLRNGANEGFHEAVGEIMSLSAATPKHLKSIGLLSPDFQEDNETEINFLLKQALTIVGTLPFTYMLEKWRWMVFKGEIPKDQWMKKWWEMKREIVGVVEPVPHDETYCDPASLFHVSNDYSFIRYYTRTLYQFQFQEALCQAAKHEGPLHKCDISNSTEAGQKLFNMLRLGKSEPWTLALENVVGAKNMNVRPLLNYFEPLFTWLKDQNKNSFVGWSTDWSPYA

SEQ ID NO: 161 - protein, 595 aa, synthetic construct
  REGION 1..595: note = ACE2 mutant, Ala inserted at #31
IEEQAKTFLDAKFNHEAEDLFYQSSLASWNYNTNITEENVQNMNNAGDKWSAFLKEQSTLAQMYPLQEIQNLTVKLQLQALQQNGSSVLSEDKSKRLNTILNTMSTIYSTGKVCNPDNPQECLLLEPGLNEIMANSLDYNERLWAWESWRSEVGKQLRPLYEEYVVLKNEMARANHYEDYGDYWRGDYEVNGVDGYDYSRGQLIEDVEHTFEEIKPLYEHLHAYVRAKLMNAYPSYISPIGCLPAHLLGDMWGRFWTNLYSLTVPFGQKPNIDVTDAMVDQAWDAQRIFKEAEKFFVSVGLPNMTQGFWENSMLTDPGNVQKAVCHPTAWDLGKGDFRILMCTKVTMDDFLTAHHEMGHIQYDMAYAAQPFLLRNGANEGFHEAVGEIMSLSAATPKHLKSIGLLSPDFQEDNETEINFLLKQALTIVGTLPFTYMLEKWRWMVFKGEIPKDQWMKKWWEMKREIVGVVEPVPHDETYCDPASLFHVSNDYSFIRYYTRTLYQFQFQEALCQAAKHEGPLHKCDISNSTEAGQKLFNMLRLGKSEPWTLALENVVGAKNMNVRPLLNYFEPLFTWLKDQNKNSFVGWSTDWSPYA

SEQ ID NO: 162 - protein, 595 aa, synthetic construct
  REGION 1..595: note = ACE2 mutant, Ala inserted at #32
IEEQAKTFLDKAFNHEAEDLFYQSSLASWNYNTNITEENVQNMNNAGDKWSAFLKEQSTLAQMYPLQEIQNLTVKLQLQALQQNGSSVLSEDKSKRLNTILNTMSTIYSTGKVCNPDNPQECLLLEPGLNEIMANSLDYNERLWAWESWRSEVGKQLRPLYEEYVVLKNEMARANHYEDYGDYWRGDYEVNGVDGYDYSRGQLIEDVEHTFEEIKPLYEHLHAYVRAKLMNAYPSYISPIGCLPAHLLGDMWGRFWTNLYSLTVPFGQKPNIDVTDAMVDQAWDAQRIFKEAEKFFVSVGLPNMTQGFWENSMLTDPGNVQKAVCHPTAWDLGKGDFRILMCTKVTMDDFLTAHHEMGHIQYDMAYAAQPFLLRNGANEGFHEAVGEIMSLSAATPKHLKSIGLLSPDFQEDNETEINFLLKQALTIVGTLPFTYMLEKWRWMVFKGEIPKDQWMKKWWEMKREIVGVVEPVPHDETYCDPASLFHVSNDYSFIRYYTRTLYQFQFQEALCQAAKHEGPLHKCDISNSTEAGQKLFNMLRLGKSEPWTLALENVVGAKNMNVRPLLNYFEPLFTWLKDQNKNSFVGWSTDWSPYA

SEQ ID NO: 163 - protein, 595 aa, synthetic construct
  REGION 1..595: note = ACE2 mutant, Ala insertion at #33
IEEQAKTFLDKFANHEAEDLFYQSSLASWNYNTNITEENVQNMNNAGDKWSAFLKEQSTLAQMYPLQEIQNLTVKLQLQALQQNGSSVLSEDKSKRLNTILNTMSTIYSTGKVCNPDNPQECLLLEPGLNEIMANSLDYNERLWAWESWRSEVGKQLRPLYEEYVVLKNEMARANHYEDYGDYWRGDYEVNGVDGYDYSRGQLIEDVEHTFEEIKPLYEHLHAYVRAKLMNAYPSYISPIGCLPAHLLGDMWGRFWTNLYSLTVPFGQKPNIDVTDAMVDQAWDAQRIFKEAEKFFVSVGLPNMTQGFWENSMLTDPGNVQKAVCHPTAWDLGKGDFRILMCTKVTMDDFLTAHHEMGHIQYDMAYAAQPFLLRNGANEGFHEAVGEIMSLSAATPKHLKSIGLLSPDFQEDNETEINFLLKQALTIVGTLPFTYMLEKWRWMVFKGEIPKDQWMKKWWEMKREIVGVVEPVPHDETYCDPASLFHVSNDYSFIRYYTRTLYQFQFQEALCQAAKHEGPLHKCDISNSTEAGQKLFNMLRLGKSEPWTLALENVVGAKNMNVRPLLNYFEPLFTWLKDQNKNSFVGWSTDWSPYA

SEQ ID NO: 164 - protein, 595 aa, synthetic construct
  REGION 1..595: note = ACE2 mutant, Ala insertion at #34
IEEQAKTFLDKFNAHEAEDLFYQSSLASWNYNTNITEENVQNMNNAGDKWSAFLKEQSTLAQMYPLQEIQNLTVKLQLQALQQNGSSVLSEDKSKRLNTILNTMSTIYSTGKVCNPDNPQECLLLEPGLNEIMANSLDYNERLWAWESWRSEVGKQLRPLYEEYVVLKNEMARANHYEDYGDYWRGDYEVNGVDGYDYSRGQLIEDVEHTFEEIKPLYEHLHAYVRAKLMNAYPSYISPIGCLPAHLLGDMWGRFWTNLYSLTVPFGQKPNIDVTDAMVDQAWDAQRIFKEAEKFFVSVGLPNMTQGFWENSMLTDPGNVQKAVCHPTAWDLGKGDFRILMCTKVTMDDFLTAHHEMGHIQYDMAYAAQPFLLRNGANEGFHEAVGEIMSLSAATPKHLKSIGLLSPDFQEDNETEINFLLKQALTIVGTLPFTYMLEKWRWMVFKGEIPKDQWMKKWWEMKREIVGVVEPVPHDETYCDPASLFHVSNDYSFIRYYTRTLYQFQFQEALCQAAKHEGPLHKCDISNSTEAGQKLFNMLRLGKSEPWTLALENVVGAKNMNVRPLLNYFEPLFTWLKDQNKNSFVGWSTDWSPYA

SEQ ID NO: 165 - protein, 595 aa, synthetic construct
  REGION 1..595: note = ACE2 mutant, Ala insertion at #35
IEEQAKTFLDKFNHAEAEDLFYQSSLASWNYNTNITEENVQNMNNAGDKWSAFLKEQSTLAQMYPLQEIQNLTVKLQLQALQQNGSSVLSEDKSKRLNTILNTMSTIYSTGKVCNPDNPQECLLLEPGLNEIMANSLDYNERLWAWESWRSEVGKQLRPLYEEYVVLKNEMARANHYEDYGDYWRGDYEVNGVDGYDYSRGQLIEDVEHTFEEIKPLYEHLHAYVRAKLMNAYPSYISPIGCLPAHLLGDMWGRFWTNLYSLTVPFGQKPNIDVTDAMVDQAWDAQRIFKEAEKFFVSVGLPNMTQGFWENSMLTDPGNVQKAVCHPTAWDLGKGDFRILMCTKVTMDDFLTAHHEMGHIQYDMAYAAQPFLLRNGANEGFHEAVGEIMSLSAATPKHLKSIGLLSPDFQEDNETEINFLLKQALTIVGTLPFTYMLEKWRWMVFKGEIPKDQWMKKWWEMKREIVGVVEPVPHDETYCDPASLFHVSNDYSFIRYYTRTLYQFQFQEALCQAAKHEGPLHKCDISNSTEAGQKLFNMLRLGKSEPWTLALENVVGAKNMNVRPLLNYFEPLFTWLKDQNKNSFVGWSTDWSPYA

SEQ ID NO: 166 - protein, 595 aa, synthetic construct
  REGION 1..595: note = ACE2 mutant, Ala insertion at #36
IEEQAKTFLDKFNHEAAEDLFYQSSLASWNYNTNITEENVQNMNNAGDKWSAFLKEQSTLAQMYPLQEIQNLTVKLQLQALQQNGSSVLSEDKSKRLNTILNTMSTIYSTGKVCNPDNPQECLLLEPGLNEIMANSLDYNERLWAWESWRSEVGKQLRPLYEEYVVLKNEMARANHYEDYGDYWRGDYEVNGVDGYDYSRGQLIEDVEHTFEEIKPLYEHLHAYVRAKLMNAYPSYISPIGCLPAHLLGDMWGRFWTNLYSLTVPFGQKPNIDVTDAMVDQAWDAQRIFKEAEKFFVSVGLPNMTQGFWENSMLTDPGNVQKAVCHPTAWDLGKGDFRILMCTKVTMDDFLTAHHEMGHIQYDMAYAAQPFLLRNGANEGFHEAVGEIMSLSAATPKHLKSIGLLSPDFQEDNETEINFLLKQALTIVGTLPFTYMLEKWRWMVFKGEIPKDQWMKKWWEMKREIVGVVEPVPHDETYCDPASLFHVSNDYSFIRYYTRTLYQFQFQEALCQAAKHEGPLHKCDISNSTEAGQKLFNMLRLGKSEPWTLALENVVGAKNMNVRPLLNYFEPLFTWLKDQNKNSFVGWSTDWSPYA

SEQ ID NO: 167 - protein, 595 aa, synthetic construct
  REGION 1..595: note = ACE2 mutant, Ala insertion at #38
IEEQAKTFLDKFNHEAEADLFYQSSLASWNYNTNITEENVQNMNNAGDKWSAFLKEQSTLAQMYPLQEIQNLTVKLQLQALQQNGSSVLSEDKSKRLNTILNTMSTIYSTGKVCNPDNPQECLLLEPGLNEIMANSLDYNERLWAWESWRSEVGKQLRPLYEEYVVLKNEMARANHYEDYGDYWRGDYEVNGVDGYDYSRGQLIEDVEHTFEEIKPLYEHLHAYVRAKLMNAYPSYISPIGCLPAHLLGDMWGRFWTNLYSLTVPFGQKPNIDVTDAMVDQAWDAQRIFKEAEKFFVSVGLPNMTQGFWENSMLTDPGNVQKAVCHPTAWDLGKGDFRILMCTKVTMDDFLTAHHEMGHIQYDMAYAAQPFLLRNGANEGFHEAVGEIMSLSAATPKHLKSIGLLSPDFQEDNETEINFLLKQALTIVGTLPFTYMLEKWRWMVFKGEIPKDQWMKKWWEMKREIVGVVEPVPHDETYCDPASLFHVSNDYSFIRYYTRTLYQFQFQEALCQAAKHEGPLHKCDISNSTEAGQKLFNMLRLGKSEPWTLALENVVGAKNMNVRPLLNYFEPLFTWLKDQNKNSFVGWSTDWSPYA

SEQ ID NO: 168 - DNA, 3596 bp, Homo sapiens
  source 1..3596: mol_type = genomic DNA
ggcactcatacatacactctggcaatgaggacactgagctcgcttctgaaatttgacaagataaccactaaaatctctttgaattctatgttgttgtgatcccatggctacagaggatcaggagttgacatagatactctttggatttcataccatgtggaggctttcttacttccacgtgaccttgactgagttttgaatagcgcccaacccaagttcaaaggctgataagagagaaaatctcatgaggaggttttagtctagggaaagtcattcagtggatgtgatcttggctcacaggggacgatgtcaagctcttcctggctccttctcagccttgttgctgtaactgctgctcagtccaccattgaggaacaggccaagacatttttggacaagtttaaccacgaagccgaagacctgttctatcaaagttcacttgcttcttggaattataacaccaatattactgaagagaatgtccaaaacatgaataatgctggggacaaatggtctgcctttttaaaggaacagtccacacttgcccaaatgtatccactacaagaaattcagaatctcacagtcaagcttcagctgcaggctcttcagcaaaatgggtcttcagtgctctcagaagacaagagcaaacggttgaacacaattctaaatacaatgagcaccatctacagtactggaaaagtttgtaacccagataatccacaagaatgcttattacttgaaccaggtttgaatgaaataatggcaaacagtttagactacaatgagaggctctgggcttgggaaagctggagatctgaggtcggcaagcagctgaggccattatatgaagagtatgtggtcttgaaaaatgagatggcaagagcaaatcattatgaggactatggggattattggagaggagactatgaagtaaatggggtagatggctatgactacagccgcggccagttgattgaagatgtggaacatacctttgaagagattaaaccattatatgaacatcttcatgcctatgtgagggcaaagttgatgaatgcctatccttcctatatcagtccaattggatgcctccctgctcatttgcttggtgatatgtggggtagattttggacaaatctgtactctttgacagttccctttggacagaaaccaaacatagatgttactgatgcaatggtggaccaggcctgggatgcacagagaatattcaaggaggccgagaagttctttgtatctgttggtcttcctaatatgactcaaggattctgggaaaattccatgctaacggacccaggaaatgttcagaaagcagtctgccatcccacagcttgggacctggggaagggcgacttcaggatccttatgtgcacaaaggtgacaatggacgacttcctgacagctcatcatgagatggggcatatccagtatgatatggcatatgctgcacaaccttttctgctaagaaatggagctaatgaaggattccatgaagctgttggggaaatcatgtcactttctgcagccacacctaagcatttaaaatccattggtcttctgtcacccgattttcaagaagacaatgaaacagaaataaacttcctgctcaaacaagcactcacgattgttgggactctgccatttacttacatgttagagaagtggaggtggatggtctttaaaggggaaattcccaaagaccagtggatgaaaaagtggtgggagatgaagcgagagatagttggggtggtggaacctgtgccccatgatgaaacatactgtgaccccgcatctctgttccatgtttctaatgattactcattcattcgatattacacaaggaccctttaccaattccagtttcaagaagcactttgtcaagcagctaaacatgaaggccctctgcacaaatgtgacatctcaaactctacagaagctggacagaaactgttcaatatgctgaggcttggaaaatcagaaccctggaccctagcattggaaaatgttgtaggagcaaagaacatgaatgtaaggccactgctcaactactttgagcccttatttacctggctgaaagaccagaacaagaattcttttgtgggatggagtaccgactggagtccatatgcagaccaaagcatcaaagtgaggataagcctaaaatcagctcttggagataaagcatatgaatggaacgacaatgaaatgtacctgttccgatcatctgttgcatatgctatgaggcagtactttttaaaagtaaaaaatcagatgattctttttggggaggaggatgtgcgagtggctaatttgaaaccaagaatctcctttaatttctttgtcactgcacctaaaaatgtgtctgatatcattcctagaactgaagttgaaaaggccatcaggatgtcccggagccgtatcaatgatgctttccgtctgaatgacaacagcctagagtttctggggatacagccaacacttggacctcctaaccagccccctgtttccatatggctgattgtttttggagttgtgatgggagtgatagtggttggcattgtcatcctgatcttcactgggatcagagatcggaagaagaaaaataaagcaagaagtggagaaaatccttatgcctccatcgatattagcaaaggagaaaataatccaggattccaaaacactgatgatgttcagacctccttttagaaaaatctatgtttttcctcttgaggtgattttgttgtatgtaaatgttaatttcatggtatagaaaatataagatgataaagatatcattaaatgtcaaaactatgactctgttcagaaaaaaaattgtccaaagacaacatggccaaggagagagcatcttcattgacattgctttcagtatttatttctgtctctggatttgacttctgttctgtttcttaataaggattttgtattagagtatattagggaaagtgtgtatttggtctcacaggctgttcagggataatctaaatgtaaatgtctgttgaatttctgaagttgaaaacaaggatatatcattggagcaagtgttggatcttgtatggaatatggatggatcacttgtaaggacagtgcctgggaactggtgtagctgcaaggattgagaatggcatgcattagctcactttcatttaatccattgtcaaggatgacatgctttcttcacagtaactcagttcaagtactatggtgatttgcctacagtgatgtttggaatcgatcatgctttcttcaaggtgacaggtctaaagagagaagaatccagggaacaggtagaggacattgctttttcacttccaaggtgcttgatcaacatctccctgacaacacaaaactagagccaggggcctccgtgaactcccagagcatgcctgatagaaactcatttctactgttctctaactgtggagtgaatggaaattccaactgtatgttcaccctctgaagtgggtacccagtctcttaaatcttttgtatttgctcacagtgtttgagcagtgctgagcacaaagcagacactcaataaatgctagatttacacactc

SEQ ID NO: 169 - DNA, 696 bp, Homo sapiens
  source 1..696: mol_type = genomic DNA
gagcccaaatcttgtgacaaaactcacacatgcccaccgtgcccagcacctgaactcctggggggaccgtcagtcttcctcttccccccaaaacccaaggacaccctcatgatctcccggacccctgaggtcacatgcgtggtggtggacgtgagccacgaagaccctgaggtcaagttcaactggtacgtggacggcgtggaggtgcataatgccaagacaaagccgcgggaggagcagtacaacagcacgtaccgtgtggtcagcgtcctcaccgtcctgcaccaggactggctgaatggcaaggagtacaagtgcaaggtctccaacaaagccctcccagcccccatcgagaaaaccatctccaaagccaaagggcagccccgagaaccacaggtgtacaccctgcccccatcccgggaggagatgaccaagaaccaggtcagcctgacctgcctggtcaaaggcttctatcccagcgacatcgccgtggagtgggagagcaatgggcagccggagaacaactacaagaccacgcctcccgtgctggactccgacggctccttcttcctctatagcaagctcaccgtggacaagagcaggtggcagcaggggaacgtcttctcatgctccgtgatgcatgaggctctgcacaaccactacacgcagaagagcctctccctgtccccgggtaaa

SEQ ID NO: 170 - DNA, 2440 bp, Homo sapiens
  source 1..2440: mol_type = genomic DNA
atcctgctaatgtgcattgaaaggagagcaacggggctgaggccgtgtcagcacgatggaccccaaacagaccaccctcctgtgtcttggggactttcccatgcctttcatatctgccaaatcgagtcctgtgattcccttggatggatctgtgaaaatccagtgccaggccattcgtgaagcttacctgacccagctgatgatcataaaaaactccacgtaccgagagataggcagaagactgaagttttggaatgagactgatcctgagttcgtcattgaccacatggacgcaaacaaggcagggcgctatcagtgccaatataggatagggcactacaggttccggtacagtgacaccctggagctggtagtgacaggcttgtatggcaaacccttcctctctgcagatcggggtctggtgttgatgccaggagagaatatttccctcacgtgcagctcagcacacatcccatttgatagattttcactggccaaggagggagaactttctctgccacagcaccaaagtggggaacacccggccaacttctctttgggtcctgtggacctcaatgtctcagggatctacaggtgctacggttggtacaacaggagcccctacctgtggtccttccccagtaatgccttggagcttgtggtcacagactccatccaccaagattacacgacgcagaacttgatccgcatggccgtggcaggactggtcctcgtggctctcttggccatactggttgaaaattggcacagccatacggcactgaacaaggaagcctcggcagatgtggctgaaccgagctggagccaacagatgtgtcagccaggattgacctttgcacgaacaccaagtgtctgcaagtaaacacctggaggtgaaggcagagaggagccaggactgtggagtccgacaaagctacttgaaggacacaagagagaaaagctcactaagaagcttgaatctacttttttttttttttgagacagagtctggctctgtcacccaggctggagtgcagtggagcaatctcggctcattgaacctcttgggttcaagtgattcttgtgcctcagcctcccaagtagctggaattacaggcacataccactgcacccagctaatttttgtatttttagtagagatggggtttcactgtgttggccaggctggtctcgaactcctgacctcaggtgatccacccaccttggcctcccaaagtgctgagattataggcatgagccaccacgcctggccagatgcatgttcaaaccaatcaaatggtgttttcttatgcaggactgatcgatttgcacccacctttctgcacataagttatggttttccatcttatctgtcttctgattttttatatcctgtttaatttcttccttcattgttcttctctttttttatttattttatttatttttatttttatttttatttgagacagagtctcactctgttgcccaggctggagtgcagtggcacgatctcggctcactgcaacctctgcctcctgggttcaagtgattctcctgcctcggcctcccaagtagctgggattgcaggctcccaccatcacgcccagctacttttacagtatttttagtagagacggggtttcatcacattggccaagctggtctcaaacttctgacctcgtgatctgcccgcctcggcctcccaaagtgctgggattacagatgtgagccactgcgcccagccttctttttatatttttaaatgtgtcttccccaaatataaatggttggtaagcatgccaaatatattcaataacccccctcctttatttttttttgttgaagtgaggctctccctatgttgcctaagctggtcttgaactcctggtctcaagcaatcctcctacctcagcctcctgctgtgttcatctacaaattgataagagtgaaagtcataatcctacaggaggattaccctatttatttcacaaaccctatttctaccggattttcatacaaggaatacaggcatgtgtttcacctcattaatttattttttcacttagttttgatgatattcacatatattatcaagtgtgcaaacattaaattcttgtgtacaaaactcaaatggtcttccaaataattccccattcttttttcttataaactttcacagctttacccttgacagactttactcaaggaaatctaagttggtcatatgtggctctttcactgattgctatttacttcattgtccagtagcttatgtatgaaaatataattataaaatgtaagggtcctacttccagtgaaactgaagggacttaggcccacttttatcctttactgagagcttatctctacttgataaaatttctactgtattcttggcttaactcaggtcctgtgattaaaaaaaaaatgcaaagta

SEQ ID NO: 171 - DNA, 729 bp, Homo sapiens
  source 1..729: mol_type = genomic DNA
ccggccatggccgaggtgcagctgttggagtctgggggaggcttggtacagcctggggggtccctgagactctcctgtgcagcctctggattcacctttagcagctatgccatgagctgggtccgccaggctccagggaaggggctggagtgggtctcaactatttctagtaatggtggttatacatattacgcagactccgtgaagggcaggttcaccatctccagagacaattccaagaacacgctgtatctgcaaatgaacagcctgagagccgaggacacggccgtatattactgtgcgaaagcttattctgcttttgactactggggccagggaaccctggtcaccgtctcgagcggtggaggcggttcaggcggaggtggcagcggcggtggcgggtcgacggacatccagatgacccagtctccatcctccctgtctgcatctgtaggagacagagtcaccatcacttgccgggcaagtcagagcattagcagctatttaaattggtatcagcagaaaccagggaaagcccctaagctcctgatctatactgcatccactttgcaaagtggggtcccgtcaaggttcagtggcagtggatctgggacagatttcactctcaccatcagcagtctgcaacctgaagattttgcaacttactactgtcaacagacttctgctaatcctggtacgttcggccaagggaccaaggtggaaatcaaa

SEQ ID NO: 172 - DNA, 321 bp, Homo sapiens
  source 1..321: mol_type = genomic DNA
gacatccagttgacccagtctccatcctccctgtctgcatctgtaggagacagagtcaccatcacttgccaggcgagtcaggacattagcaactatttaaattggtatcagcagaaaccagggaaagcccctaagctcctgatctacgatgcatccaatttggaaacaggggtcccatcaaggttcagtggaagtggatctgggacagattttactttcaccatcagcagtctgcaacctgaagattttgcaacttactactgtcaacagagttacagttcaccttggacgttcggccaagggaccaaggtggaaatcaaa

SEQ ID NO: 173 - protein, 6 aa, synthetic construct
  REGION 1..6: note = Anti-Spike Group 21, CDR-H1
SSYAMS

SEQ ID NO: 174 - protein, 10 aa, synthetic construct
  REGION 1..10: note = Anti-Spike Group 21, CDR-H2
AISGSGGSTN

SEQ ID NO: 175 - protein, 8 aa, synthetic construct
  REGION 1..8: note = Anti-Spike Group 21, CDR-H3
DLWGLAFA

SEQ ID NO: 176 - protein, 6 aa, synthetic construct
  REGION 1..6: note = Anti-Spike Group 21, CDR-L3
DSSNPW

SEQ ID NO: 177 - protein, 6 aa, synthetic construct
  REGION 1..6: note = Anti-Spike Group 22, CDR-H1
SSYAMS

SEQ ID NO: 178 - protein, 10 aa, synthetic construct
  REGION 1..10: note = Anti-Spike Group 22, CDR-H2
SISGSGGSTD

SEQ ID NO: 179 - protein, 8 aa, synthetic construct
  REGION 1..8: note = Anti-Spike Group 22, CDR-H3
DLWGLAMA

SEQ ID NO: 180 - protein, 6 aa, synthetic construct
  REGION 1..6: note = Anti-Spike Group 22, CDR-L3
DNNVPL

SEQ ID NO: 181 - protein, 6 aa, synthetic construct
  REGION 1..6: note = Anti-Spike Group 23, CDR-H1
SSYAMH

SEQ ID NO: 182 - protein, 10 aa, synthetic construct
  REGION 1..10: note = Anti-Spike Group 23, CDR-H2
AISWSGRSTY

SEQ ID NO: 183 - protein, 9 aa, synthetic construct
  REGION 1..9: note = Anti-Spike Group 23, CDR-H3
DLSSNWGAG

SEQ ID NO: 184 - protein, 6 aa, synthetic construct
  REGION 1..6: note = Anti-Spike Group 23, CDR-L3
SADTPF

SEQ ID NO: 185 - protein, 6 aa, synthetic construct
  REGION 1..6: note = Anti-Spike Group 24, CDR-H1
SSYAMH

SEQ ID NO: 186 - protein, 10 aa, synthetic construct
  REGION 1..10: note = Anti-Spike Group 24, CDR-H2
AISWSGRSTY

SEQ ID NO: 187 - protein, 9 aa, synthetic construct
  REGION 1..9: note = Anti-Spike Group 24, CDR-H3
DLSSNWGSG

SEQ ID NO: 188 - protein, 6 aa, synthetic construct
  REGION 1..6: note = Anti-Spike Group 24, CDR-L3
SADTPF

SEQ ID NO: 189 - protein, 6 aa, synthetic construct
  REGION 1..6: note = Anti-Spike Group 25, CDR-H1
SSYAMH

SEQ ID NO: 190 - protein, 10 aa, synthetic construct
  REGION 1..10: note = Anti-Spike Group 25, CDR-H2
IISGSGGSTS

SEQ ID NO: 191 - protein, 9 aa, synthetic construct
  REGION 1..9: note = Anti-Spike Group 25, CDR-H3
DLCDCFAVA

SEQ ID NO: 192 - protein, 6 aa, synthetic construct
  REGION 1..6: note = Anti-Spike Group 25, CDR-L3
WAARPL

SEQ ID NO: 193 - protein, 6 aa, synthetic construct
  REGION 1..6: note = Anti-Spike Group 26, CDR-H1
SAYAMH

SEQ ID NO: 194 - protein, 10 aa, synthetic construct
  REGION 1..10: note = Anti-Spike Group 26, CDR-H2
AIWGSGGSTY

SEQ ID NO: 195 - protein, 9 aa, synthetic construct
  REGION 1..9: note = Anti-Spike Group 26, CDR-H3
DLWMAMWFG

SEQ ID NO: 196 - protein, 6 aa, synthetic construct
  REGION 1..6: note = Anti-Spike Group 26, CDR-L3
RSTYPL

SEQ ID NO: 197 - protein, 6 aa, synthetic construct
  REGION 1..6: note = Anti-Spike Group 27, CDR-H1
SSYAMS

SEQ ID NO: 198 - protein, 10 aa, synthetic construct
  REGION 1..10: note = Anti-Spike Group 27, CDR-H2
AISGSGGSTS

SEQ ID NO: 199 - protein, 10 aa, synthetic construct
  REGION 1..10: note = Anti-Spike Group 27, CDR-H3
DLIYDTVWWG

SEQ ID NO: 200 - protein, 6 aa, synthetic construct
  REGION 1..6: note = Anti-Spike Group 27, CDR-L3
DTNVPY

SEQ ID NO: 201 - protein, 805 aa, synthetic construct
  REGION 1..805: note = R273 mutant ACE2
  MUTAGEN 273: note = The sequence here can be Ala, Asn, Asp, Cys, Gln, Glu, Gly, His,Ile, Lys, Leu, Met, Phe, Pro, Ser, Thr, Trp, Tyr, or Val.
MSSSSWLLLSLVAVTAAQSTIEEQAKTFLDKFNHEAEDLFYQSSLASWNYNTNITEENVQNMNNAGDKWSAFLKEQSTLAQMYPLQEIQNLTVKLQLQALQQNGSSVLSEDKSKRLNTILNTMSTIYSTGKVCNPDNPQECLLLEPGLNEIMANSLDYNERLWAWESWRSEVGKQLRPLYEEYVVLKNEMARANHYEDYGDYWRGDYEVNGVDGYDYSRGQLIEDVEHTFEEIKPLYEHLHAYVRAKLMNAYPSYISPIGCLPAHLLGDMWGXFWTNLYSLTVPFGQKPNIDVTDAMVDQAWDAQRIFKEAEKFFVSVGLPNMTQGFWENSMLTDPGNVQKAVCHPTAWDLGKGDFRILMCTKVTMDDFLTAHHEMGHIQYDMAYAAQPFLLRNGANEGFHEAVGEIMSLSAATPKHLKSIGLLSPDFQEDNETEINFLLKQALTIVGTLPFTYMLEKWRWMVFKGEIPKDQWMKKWWEMKREIVGVVEPVPHDETYCDPASLFHVSNDYSFIRYYTRTLYQFQFQEALCQAAKHEGPLHKCDISNSTEAGQKLFNMLRLGKSEPWTLALENVVGAKNMNVRPLLNYFEPLFTWLKDQNKNSFVGWSTDWSPYADQSIKVRISLKSALGDKAYEWNDNEMYLFRSSVAYAMRQYFLKVKNQMILFGEEDVRVANLKPRISFNFFVTAPKNVSDIIPRTEVEKAIRMSRSRINDAFRLNDNSLEFLGIQPTLGPPNQPPVSIWLIVFGVVMGVIVVGIVILIFTGIRDRKKKNKARSGENPYASIDISKGENNPGFQNTDDVQTSF

SEQ ID NO: 202 - protein, 805 aa, synthetic construct
  REGION 1..805: note = H345 mutant ACE2
  MUTAGEN 345: note = The sequence here can be Ala, Arg, Asn, Asp, Cys, Gln, Glu, Gly,Ile, Lys, Leu, Met, Phe, Pro, Ser, Thr, Trp, Tyr, or Val.
MSSSSWLLLSLVAVTAAQSTIEEQAKTFLDKFNHEAEDLFYQSSLASWNYNTNITEENVQNMNNAGDKWSAFLKEQSTLAQMYPLQEIQNLTVKLQLQALQQNGSSVLSEDKSKRLNTILNTMSTIYSTGKVCNPDNPQECLLLEPGLNEIMANSLDYNERLWAWESWRSEVGKQLRPLYEEYVVLKNEMARANHYEDYGDYWRGDYEVNGVDGYDYSRGQLIEDVEHTFEEIKPLYEHLHAYVRAKLMNAYPSYISPIGCLPAHLLGDMWGRFWTNLYSLTVPFGQKPNIDVTDAMVDQAWDAQRIFKEAEKFFVSVGLPNMTQGFWENSMLTDPGNVQKAVCXPTAWDLGKGDFRILMCTKVTMDDFLTAHHEMGHIQYDMAYAAQPFLLRNGANEGFHEAVGEIMSLSAATPKHLKSIGLLSPDFQEDNETEINFLLKQALTIVGTLPFTYMLEKWRWMVFKGEIPKDQWMKKWWEMKREIVGVVEPVPHDETYCDPASLFHVSNDYSFIRYYTRTLYQFQFQEALCQAAKHEGPLHKCDISNSTEAGQKLFNMLRLGKSEPWTLALENVVGAKNMNVRPLLNYFEPLFTWLKDQNKNSFVGWSTDWSPYADQSIKVRISLKSALGDKAYEWNDNEMYLFRSSVAYAMRQYFLKVKNQMILFGEEDVRVANLKPRISFNFFVTAPKNVSDIIPRTEVEKAIRMSRSRINDAFRLNDNSLEFLGIQPTLGPPNQPPVSIWLIVFGVVMGVIVVGIVILIFTGIRDRKKKNKARSGENPYASIDISKGENNPGFQNTDDVQTSF

SEQ ID NO: 203 - protein, 805 aa, synthetic construct
  REGION 1..805: note = H374 mutant ACE2
  MUTAGEN 374: note = The sequence here can be Ala, Arg, Asn, Asp, Cys, Gln, Glu, Gly,Ile, Lys, Leu, Met, Phe, Pro, Ser, Thr, Trp, Tyr, or Val.
MSSSSWLLLSLVAVTAAQSTIEEQAKTFLDKFNHEAEDLFYQSSLASWNYNTNITEENVQNMNNAGDKWSAFLKEQSTLAQMYPLQEIQNLTVKLQLQALQQNGSSVLSEDKSKRLNTILNTMSTIYSTGKVCNPDNPQECLLLEPGLNEIMANSLDYNERLWAWESWRSEVGKQLRPLYEEYVVLKNEMARANHYEDYGDYWRGDYEVNGVDGYDYSRGQLIEDVEHTFEEIKPLYEHLHAYVRAKLMNAYPSYISPIGCLPAHLLGDMWGRFWTNLYSLTVPFGQKPNIDVTDAMVDQAWDAQRIFKEAEKFFVSVGLPNMTQGFWENSMLTDPGNVQKAVCHPTAWDLGKGDFRILMCTKVTMDDFLTAHXEMGHIQYDMAYAAQPFLLRNGANEGFHEAVGEIMSLSAATPKHLKSIGLLSPDFQEDNETEINFLLKQALTIVGTLPFTYMLEKWRWMVFKGEIPKDQWMKKWWEMKREIVGVVEPVPHDETYCDPASLFHVSNDYSFIRYYTRTLYQFQFQEALCQAAKHEGPLHKCDISNSTEAGQKLFNMLRLGKSEPWTLALENVVGAKNMNVRPLLNYFEPLFTWLKDQNKNSFVGWSTDWSPYADQSIKVRISLKSALGDKAYEWNDNEMYLFRSSVAYAMRQYFLKVKNQMILFGEEDVRVANLKPRISFNFFVTAPKNVSDIIPRTEVEKAIRMSRSRINDAFRLNDNSLEFLGIQPTLGPPNQPPVSIWLIVFGVVMGVIVVGIVILIFTGIRDRKKKNKARSGENPYASIDISKGENNPGFQNTDDVQTSF

SEQ ID NO: 204 - protein, 805 aa, synthetic construct
  REGION 1..805: note = H378 mutant ACE2
  MUTAGEN 378: note = The sequence here can be Ala, Arg, Asn, Asp, Cys, Gln, Glu, Gly,Ile, Lys, Leu, Met, Phe, Pro, Ser, Thr, Trp, Tyr, or Val.
MSSSSWLLLSLVAVTAAQSTIEEQAKTFLDKFNHEAEDLFYQSSLASWNYNTNITEENVQNMNNAGDKWSAFLKEQSTLAQMYPLQEIQNLTVKLQLQALQQNGSSVLSEDKSKRLNTILNTMSTIYSTGKVCNPDNPQECLLLEPGLNEIMANSLDYNERLWAWESWRSEVGKQLRPLYEEYVVLKNEMARANHYEDYGDYWRGDYEVNGVDGYDYSRGQLIEDVEHTFEEIKPLYEHLHAYVRAKLMNAYPSYISPIGCLPAHLLGDMWGRFWTNLYSLTVPFGQKPNIDVTDAMVDQAWDAQRIFKEAEKFFVSVGLPNMTQGFWENSMLTDPGNVQKAVCHPTAWDLGKGDFRILMCTKVTMDDFLTAHHEMGXIQYDMAYAAQPFLLRNGANEGFHEAVGEIMSLSAATPKHLKSIGLLSPDFQEDNETEINFLLKQALTIVGTLPFTYMLEKWRWMVFKGEIPKDQWMKKWWEMKREIVGVVEPVPHDETYCDPASLFHVSNDYSFIRYYTRTLYQFQFQEALCQAAKHEGPLHKCDISNSTEAGQKLFNMLRLGKSEPWTLALENVVGAKNMNVRPLLNYFEPLFTWLKDQNKNSFVGWSTDWSPYADQSIKVRISLKSALGDKAYEWNDNEMYLFRSSVAYAMRQYFLKVKNQMILFGEEDVRVANLKPRISFNFFVTAPKNVSDIIPRTEVEKAIRMSRSRINDAFRLNDNSLEFLGIQPTLGPPNQPPVSIWLIVFGVVMGVIVVGIVILIFTGIRDRKKKNKARSGENPYASIDISKGENNPGFQNTDDVQTSF

SEQ ID NO: 205 - protein, 805 aa, synthetic construct
  REGION 1..805: note = H505 mutant ACE2
  MUTAGEN 505: note = The sequence here can be Ala, Arg, Asn, Asp, Cys, Gln, Glu, Gly,Ile, Lys, Leu, Met, Phe, Pro, Ser, Thr, Trp, Tyr, or Val.
MSSSSWLLLSLVAVTAAQSTIEEQAKTFLDKFNHEAEDLFYQSSLASWNYNTNITEENVQNMNNAGDKWSAFLKEQSTLAQMYPLQEIQNLTVKLQLQALQQNGSSVLSEDKSKRLNTILNTMSTIYSTGKVCNPDNPQECLLLEPGLNEIMANSLDYNERLWAWESWRSEVGKQLRPLYEEYVVLKNEMARANHYEDYGDYWRGDYEVNGVDGYDYSRGQLIEDVEHTFEEIKPLYEHLHAYVRAKLMNAYPSYISPIGCLPAHLLGDMWGRFWTNLYSLTVPFGQKPNIDVTDAMVDQAWDAQRIFKEAEKFFVSVGLPNMTQGFWENSMLTDPGNVQKAVCHPTAWDLGKGDFRILMCTKVTMDDFLTAHHEMGHIQYDMAYAAQPFLLRNGANEGFHEAVGEIMSLSAATPKHLKSIGLLSPDFQEDNETEINFLLKQALTIVGTLPFTYMLEKWRWMVFKGEIPKDQWMKKWWEMKREIVGVVEPVPHDETYCDPASLFXVSNDYSFIRYYTRTLYQFQFQEALCQAAKHEGPLHKCDISNSTEAGQKLFNMLRLGKSEPWTLALENVVGAKNMNVRPLLNYFEPLFTWLKDQNKNSFVGWSTDWSPYADQSIKVRISLKSALGDKAYEWNDNEMYLFRSSVAYAMRQYFLKVKNQMILFGEEDVRVANLKPRISFNFFVTAPKNVSDIIPRTEVEKAIRMSRSRINDAFRLNDNSLEFLGIQPTLGPPNQPPVSIWLIVFGVVMGVIVVGIVILIFTGIRDRKKKNKARSGENPYASIDISKGENNPGFQNTDDVQTSF

SEQ ID NO: 206 - protein, 615 aa, synthetic construct
  REGION 1..615: note = T27Y H34A R273K ACE2 mutant
MSSSSWLLLSLVAVTAAQSTIEEQAKYFLDKFNAEAEDLFYQSSLASWNYNTNITEENVQNMNNAGDKWSAFLKEQSTLAQMYPLQEIQNLTVKLQLQALQQNGSSVLSEDKSKRLNTILNTMSTIYSTGKVCNPDNPQECLLLEPGLNEIMANSLDYNERLWAWESWRSEVGKQLRPLYEEYVVLKNEMARANHYEDYGDYWRGDYEVNGVDGYDYSRGQLIEDVEHTFEEIKPLYEHLHAYVRAKLMNAYPSYISPIGCLPAHLLGDMWGKFWTNLYSLTVPFGQKPNIDVTDAMVDQAWDAQRIFKEAEKFFVSVGLPNMTQGFWENSMLTDPGNVQKAVCHPTAWDLGKGDFRILMCTKVTMDDFLTAHHEMGHIQYDMAYAAQPFLLRNGANEGFHEAVGEIMSLSAATPKHLKSIGLLSPDFQEDNETEINFLLKQALTIVGTLPFTYMLEKWRWMVFKGEIPKDQWMKKWWEMKREIVGVVEPVPHDETYCDPASLFHVSNDYSFIRYYTRTLYQFQFQEALCQAAKHEGPLHKCDISNSTEAGQKLFNMLRLGKSEPWTLALENVVGAKNMNVRPLLNYFEPLFTWLKDQNKNSFVGWSTDWSPYAD

SEQ ID NO: 207 - protein, 615 aa, synthetic construct
  REGION 1..615: note = T27Y H34A R273L ACE2 mutant
MSSSSWLLLSLVAVTAAQSTIEEQAKYFLDKFNAEAEDLFYQSSLASWNYNTNITEENVQNMNNAGDKWSAFLKEQSTLAQMYPLQEIQNLTVKLQLQALQQNGSSVLSEDKSKRLNTILNTMSTIYSTGKVCNPDNPQECLLLEPGLNEIMANSLDYNERLWAWESWRSEVGKQLRPLYEEYVVLKNEMARANHYEDYGDYWRGDYEVNGVDGYDYSRGQLIEDVEHTFEEIKPLYEHLHAYVRAKLMNAYPSYISPIGCLPAHLLGDMWGLFWTNLYSLTVPFGQKPNIDVTDAMVDQAWDAQRIFKEAEKFFVSVGLPNMTQGFWENSMLTDPGNVQKAVCHPTAWDLGKGDFRILMCTKVTMDDFLTAHHEMGHIQYDMAYAAQPFLLRNGANEGFHEAVGEIMSLSAATPKHLKSIGLLSPDFQEDNETEINFLLKQALTIVGTLPFTYMLEKWRWMVFKGEIPKDQWMKKWWEMKREIVGVVEPVPHDETYCDPASLFHVSNDYSFIRYYTRTLYQFQFQEALCQAAKHEGPLHKCDISNSTEAGQKLFNMLRLGKSEPWTLALENVVGAKNMNVRPLLNYFEPLFTWLKDQNKNSFVGWSTDWSPYAD

SEQ ID NO: 208 - protein, 615 aa, synthetic construct
  REGION 1..615: note = T27Y H34A H505L ACE2 mutant
MSSSSWLLLSLVAVTAAQSTIEEQAKYFLDKFNAEAEDLFYQSSLASWNYNTNITEENVQNMNNAGDKWSAFLKEQSTLAQMYPLQEIQNLTVKLQLQALQQNGSSVLSEDKSKRLNTILNTMSTIYSTGKVCNPDNPQECLLLEPGLNEIMANSLDYNERLWAWESWRSEVGKQLRPLYEEYVVLKNEMARANHYEDYGDYWRGDYEVNGVDGYDYSRGQLIEDVEHTFEEIKPLYEHLHAYVRAKLMNAYPSYISPIGCLPAHLLGDMWGRFWTNLYSLTVPFGQKPNIDVTDAMVDQAWDAQRIFKEAEKFFVSVGLPNMTQGFWENSMLTDPGNVQKAVCHPTAWDLGKGDFRILMCTKVTMDDFLTAHHEMGHIQYDMAYAAQPFLLRNGANEGFHEAVGEIMSLSAATPKHLKSIGLLSPDFQEDNETEINFLLKQALTIVGTLPFTYMLEKWRWMVFKGEIPKDQWMKKWWEMKREIVGVVEPVPHDETYCDPASLFLVSNDYSFIRYYTRTLYQFQFQEALCQAAKHEGPLHKCDISNSTEAGQKLFNMLRLGKSEPWTLALENVVGAKNMNVRPLLNYFEPLFTWLKDQNKNSFVGWSTDWSPYAD

SEQ ID NO: 209 - protein, 615 aa, synthetic construct
  REGION 1..615: note = T27Y H34A H374N ACE2 mutant
MSSSSWLLLSLVAVTAAQSTIEEQAKYFLDKFNAEAEDLFYQSSLASWNYNTNITEENVQNMNNAGDKWSAFLKEQSTLAQMYPLQEIQNLTVKLQLQALQQNGSSVLSEDKSKRLNTILNTMSTIYSTGKVCNPDNPQECLLLEPGLNEIMANSLDYNERLWAWESWRSEVGKQLRPLYEEYVVLKNEMARANHYEDYGDYWRGDYEVNGVDGYDYSRGQLIEDVEHTFEEIKPLYEHLHAYVRAKLMNAYPSYISPIGCLPAHLLGDMWGRFWTNLYSLTVPFGQKPNIDVTDAMVDQAWDAQRIFKEAEKFFVSVGLPNMTQGFWENSMLTDPGNVQKAVCHPTAWDLGKGDFRILMCTKVTMDDFLTAHNEMGHIQYDMAYAAQPFLLRNGANEGFHEAVGEIMSLSAATPKHLKSIGLLSPDFQEDNETEINFLLKQALTIVGTLPFTYMLEKWRWMVFKGEIPKDQWMKKWWEMKREIVGVVEPVPHDETYCDPASLFHVSNDYSFIRYYTRTLYQFQFQEALCQAAKHEGPLHKCDISNSTEAGQKLFNMLRLGKSEPWTLALENVVGAKNMNVRPLLNYFEPLFTWLKDQNKNSFVGWSTDWSPYAD

SEQ ID NO: 210 - protein, 615 aa, synthetic construct
  REGION 1..615: note = T27Y H34A H378N ACE2 mutant
MSSSSWLLLSLVAVTAAQSTIEEQAKYFLDKFNAEAEDLFYQSSLASWNYNTNITEENVQNMNNAGDKWSAFLKEQSTLAQMYPLQEIQNLTVKLQLQALQQNGSSVLSEDKSKRLNTILNTMSTIYSTGKVCNPDNPQECLLLEPGLNEIMANSLDYNERLWAWESWRSEVGKQLRPLYEEYVVLKNEMARANHYEDYGDYWRGDYEVNGVDGYDYSRGQLIEDVEHTFEEIKPLYEHLHAYVRAKLMNAYPSYISPIGCLPAHLLGDMWGRFWTNLYSLTVPFGQKPNIDVTDAMVDQAWDAQRIFKEAEKFFVSVGLPNMTQGFWENSMLTDPGNVQKAVCHPTAWDLGKGDFRILMCTKVTMDDFLTAHHEMGNIQYDMAYAAQPFLLRNGANEGFHEAVGEIMSLSAATPKHLKSIGLLSPDFQEDNETEINFLLKQALTIVGTLPFTYMLEKWRWMVFKGEIPKDQWMKKWWEMKREIVGVVEPVPHDETYCDPASLFHVSNDYSFIRYYTRTLYQFQFQEALCQAAKHEGPLHKCDISNSTEAGQKLFNMLRLGKSEPWTLALENVVGAKNMNVRPLLNYFEPLFTWLKDQNKNSFVGWSTDWSPYAD

SEQ ID NO: 211 - protein, 614 aa, synthetic construct
  REGION 1..614: note = T27Y H34A H345A ACE2 mutant
MSSSSWLLLSLVAVTAAQSTIEEQAKYFLDKFNAEAEDLFYQSSLASWNYNTNITEENVQNMNNAGDKWSAFLKEQSTLAQMYPLQEIQNLTVKLQLQALQQNGSSVLSEDKSKRLNTILNTMSTIYSTGKVCNPDNPQECLLLEPGLNEIMANSLDYNERLWAWESWRSEVGKQLRPLYEEYVVLKNEMARANHYEDYGDYWRGDYEVNGVDGYDYSRGQLIEDVEHTFEEIKPLYEHLHAYVRAKLMNAYPSYISPIGCLPAHLLGDMWGRFWTNLYSLTVPFGQKPNIDVTDAMVDQAWDAQRIFKEAEKFFVSVGLPNMTQGFWENSMLTDPGNVQKAVCAPTAWDLGKGDFRILMCTKVTMDDFLTAHHEMGHIQYDMAYAAQPFLLRNGANEGFHEAVGEIMSLSAATPKHLKSIGLLSPDFQEDNETEINFLLKQALTIVGTLPFTYMLEKWRWMVFKGEIPKDQWMKKWWEMKREIVGVVEPVPHDETYCDPASLFHVSNDYSFIRYYTRTLYQFQFQEALCQAAKHEGPLHKCDISNSTEAGQKLFNMLRLGKSEPWTLALENVVGAKNMNVRPLLNYFEPLFTWLKDQNKNSFVGWSTDWSPYA

SEQ ID NO: 212 - protein, 615 aa, synthetic construct
  REGION 1..615: note = T27Y H34A R273Q ACE2 mutant
MSSSSWLLLSLVAVTAAQSTIEEQAKYFLDKFNAEAEDLFYQSSLASWNYNTNITEENVQNMNNAGDKWSAFLKEQSTLAQMYPLQEIQNLTVKLQLQALQQNGSSVLSEDKSKRLNTILNTMSTIYSTGKVCNPDNPQECLLLEPGLNEIMANSLDYNERLWAWESWRSEVGKQLRPLYEEYVVLKNEMARANHYEDYGDYWRGDYEVNGVDGYDYSRGQLIEDVEHTFEEIKPLYEHLHAYVRAKLMNAYPSYISPIGCLPAHLLGDMWGQFWTNLYSLTVPFGQKPNIDVTDAMVDQAWDAQRIFKEAEKFFVSVGLPNMTQGFWENSMLTDPGNVQKAVCHPTAWDLGKGDFRILMCTKVTMDDFLTAHHEMGHIQYDMAYAAQPFLLRNGANEGFHEAVGEIMSLSAATPKHLKSIGLLSPDFQEDNETEINFLLKQALTIVGTLPFTYMLEKWRWMVFKGEIPKDQWMKKWWEMKREIVGVVEPVPHDETYCDPASLFHVSNDYSFIRYYTRTLYQFQFQEALCQAAKHEGPLHKCDISNSTEAGQKLFNMLRLGKSEPWTLALENVVGAKNMNVRPLLNYFEPLFTWLKDQNKNSFVGWSTDWSPYAD

SEQ ID NO: 213 - DNA, 1845 bp, synthetic construct
  misc_feature 1..1845: note = CDS for T27Y H34A R273K ACE2 mutant
  source 1..1845: mol_type = other DNA
atgagcagcagtagttggcttctcttgagtttggtggcagtgacagcagcccagagtactatcgaggagcaggctaaatactttctggataagtttaacgccgaggccgaagacttgttctatcaatcttctctcgcttcatggaattacaatactaacatcactgaggagaacgtccagaatatgaacaatgctggcgacaaatggagcgccttcttgaaggagcagtctacccttgcacaaatgtatccactgcaggagatacagaaccttacagtaaagttgcagctccaggctctccagcagaacggatctagcgtgctttcagaggataaaagcaaaaggctgaacaccatacttaataccatgtccacaatttactctactggtaaagtatgtaaccccgacaaccctcaagaatgcctccttcttgagccaggcctcaatgagatcatggctaatagtctggactataatgaaagactgtgggcatgggagtcctggagatctgaagtagggaagcaactgaggcccctttatgaagagtacgtcgtacttaagaatgaaatggcccgcgctaaccactacgaggattacggcgattactggcgtggggactatgaagtaaatggtgtagatggatacgactatagtcgtgggcaattgattgaggatgtggagcacacttttgaggagataaaaccactctatgagcatcttcacgcatatgtgagagctaaactgatgaacgcctacccaagttacatcagtccaatcggatgtctcccagctcacctccttggcgacatgtggggaaagttctggaccaatctgtattccctcacagtccctttcgggcaaaagcctaatatagacgtgacagacgcaatggttgatcaggcttgggatgctcaaaggatttttaaggaagctgagaagttttttgtgtcagtcggtttgccaaatatgacacaaggcttctgggaaaatagcatgttgactgatcccggtaatgttcaaaaggctgtgtgtcaccctaccgcttgggaccttgggaaaggtgactttcgaatcttgatgtgtaccaaggtgacaatggatgactttcttacagcccatcatgaaatgggtcacatccagtatgatatggcttatgcagctcaacctttcctcttgagaaatggtgcaaatgaaggttttcatgaagctgtaggggaaataatgtccctgagtgctgcaaccccaaagcatctcaagagtatcggattgttgagcccagattttcaagaagataacgagaccgaaatcaacttccttctgaaacaagccctcacaatagttggtactcttccattcacatacatgctggagaaatggcgttggatggtttttaagggggagatacctaaagatcagtggatgaaaaagtggtgggagatgaagcgtgagatcgtaggggtcgtggagccagtgcctcatgatgagacttactgtgacccagcatcactcttccacgttagcaatgactattcatttatacgttattacactcgcactctttaccagtttcaatttcaggaggctctgtgtcaggctgccaagcatgagggaccccttcacaagtgtgatattagtaacagtactgaggcaggccaaaaactgttcaatatgttgaggcttggcaaaagcgagccatggactctcgccttggaaaatgttgtcggggctaaaaacatgaatgtacgccctctgcttaactattttgagcccctttttacatggctcaaggaccagaataagaactcctttgtcggctggtcaacagactggtctccctatgcagac

SEQ ID NO: 214 - DNA, 1845 bp, synthetic construct
  misc_feature 1..1845: note = CDS for T27Y H34A R273L ACE2 mutant
  source 1..1845: mol_type = other DNA
atgagcagcagtagttggcttctcttgagtttggtggcagtgacagcagcccagagtactatcgaggagcaggctaaatactttctggataagtttaacgccgaggccgaagacttgttctatcaatcttctctcgcttcatggaattacaatactaacatcactgaggagaacgtccagaatatgaacaatgctggcgacaaatggagcgccttcttgaaggagcagtctacccttgcacaaatgtatccactgcaggagatacagaaccttacagtaaagttgcagctccaggctctccagcagaacggatctagcgtgctttcagaggataaaagcaaaaggctgaacaccatacttaataccatgtccacaatttactctactggtaaagtatgtaaccccgacaaccctcaagaatgcctccttcttgagccaggcctcaatgagatcatggctaatagtctggactataatgaaagactgtgggcatgggagtcctggagatctgaagtagggaagcaactgaggcccctttatgaagagtacgtcgtacttaagaatgaaatggcccgcgctaaccactacgaggattacggcgattactggcgtggggactatgaagtaaatggtgtagatggatacgactatagtcgtgggcaattgattgaggatgtggagcacacttttgaggagataaaaccactctatgagcatcttcacgcatatgtgagagctaaactgatgaacgcctacccaagttacatcagtccaatcggatgtctcccagctcacctccttggcgacatgtggggactgttctggaccaatctgtattccctcacagtccctttcgggcaaaagcctaatatagacgtgacagacgcaatggttgatcaggcttgggatgctcaaaggatttttaaggaagctgagaagttttttgtgtcagtcggtttgccaaatatgacacaaggcttctgggaaaatagcatgttgactgatcccggtaatgttcaaaaggctgtgtgtcaccctaccgcttgggaccttgggaaaggtgactttcgaatcttgatgtgtaccaaggtgacaatggatgactttcttacagcccatcatgaaatgggtcacatccagtatgatatggcttatgcagctcaacctttcctcttgagaaatggtgcaaatgaaggttttcatgaagctgtaggggaaataatgtccctgagtgctgcaaccccaaagcatctcaagagtatcggattgttgagcccagattttcaagaagataacgagaccgaaatcaacttccttctgaaacaagccctcacaatagttggtactcttccattcacatacatgctggagaaatggcgttggatggtttttaagggggagatacctaaagatcagtggatgaaaaagtggtgggagatgaagcgtgagatcgtaggggtcgtggagccagtgcctcatgatgagacttactgtgacccagcatcactcttccacgttagcaatgactattcatttatacgttattacactcgcactctttaccagtttcaatttcaggaggctctgtgtcaggctgccaagcatgagggaccccttcacaagtgtgatattagtaacagtactgaggcaggccaaaaactgttcaatatgttgaggcttggcaaaagcgagccatggactctcgccttggaaaatgttgtcggggctaaaaacatgaatgtacgccctctgcttaactattttgagcccctttttacatggctcaaggaccagaataagaactcctttgtcggctggtcaacagactggtctccctatgcagac

SEQ ID NO: 215 - DNA, 1845 bp, synthetic construct
  misc_feature 1..1845: note = CDS for T27Y H34A H505L ACE2 mutant
  source 1..1845: mol_type = other DNA
atgagcagcagtagttggcttctcttgagtttggtggcagtgacagcagcccagagtactatcgaggagcaggctaaatactttctggataagtttaacgccgaggccgaagacttgttctatcaatcttctctcgcttcatggaattacaatactaacatcactgaggagaacgtccagaatatgaacaatgctggcgacaaatggagcgccttcttgaaggagcagtctacccttgcacaaatgtatccactgcaggagatacagaaccttacagtaaagttgcagctccaggctctccagcagaacggatctagcgtgctttcagaggataaaagcaaaaggctgaacaccatacttaataccatgtccacaatttactctactggtaaagtatgtaaccccgacaaccctcaagaatgcctccttcttgagccaggcctcaatgagatcatggctaatagtctggactataatgaaagactgtgggcatgggagtcctggagatctgaagtagggaagcaactgaggcccctttatgaagagtacgtcgtacttaagaatgaaatggcccgcgctaaccactacgaggattacggcgattactggcgtggggactatgaagtaaatggtgtagatggatacgactatagtcgtgggcaattgattgaggatgtggagcacacttttgaggagataaaaccactctatgagcatcttcacgcatatgtgagagctaaactgatgaacgcctacccaagttacatcagtccaatcggatgtctcccagctcacctccttggcgacatgtggggacgtttctggaccaatctgtattccctcacagtccctttcgggcaaaagcctaatatagacgtgacagacgcaatggttgatcaggcttgggatgctcaaaggatttttaaggaagctgagaagttttttgtgtcagtcggtttgccaaatatgacacaaggcttctgggaaaatagcatgttgactgatcccggtaatgttcaaaaggctgtgtgtcaccctaccgcttgggaccttgggaaaggtgactttcgaatcttgatgtgtaccaaggtgacaatggatgactttcttacagcccatcatgaaatgggtcacatccagtatgatatggcttatgcagctcaacctttcctcttgagaaatggtgcaaatgaaggttttcatgaagctgtaggggaaataatgtccctgagtgctgcaaccccaaagcatctcaagagtatcggattgttgagcccagattttcaagaagataacgagaccgaaatcaacttccttctgaaacaagccctcacaatagttggtactcttccattcacatacatgctggagaaatggcgttggatggtttttaagggggagatacctaaagatcagtggatgaaaaagtggtgggagatgaagcgtgagatcgtaggggtcgtggagccagtgcctcatgatgagacttactgtgacccagcatcactcttcctggttagcaatgactattcatttatacgttattacactcgcactctttaccagtttcaatttcaggaggctctgtgtcaggctgccaagcatgagggaccccttcacaagtgtgatattagtaacagtactgaggcaggccaaaaactgttcaatatgttgaggcttggcaaaagcgagccatggactctcgccttggaaaatgttgtcggggctaaaaacatgaatgtacgccctctgcttaactattttgagcccctttttacatggctcaaggaccagaataagaactcctttgtcggctggtcaacagactggtctccctatgcagac

SEQ ID NO: 216 - DNA, 1845 bp, synthetic construct
  misc_feature 1..1845: note = CDS for T27Y H34A H374N ACE2 mutant
  source 1..1845: mol_type = other DNA
atgagcagcagtagttggcttctcttgagtttggtggcagtgacagcagcccagagtactatcgaggagcaggctaaatactttctggataagtttaacgccgaggccgaagacttgttctatcaatcttctctcgcttcatggaattacaatactaacatcactgaggagaacgtccagaatatgaacaatgctggcgacaaatggagcgccttcttgaaggagcagtctacccttgcacaaatgtatccactgcaggagatacagaaccttacagtaaagttgcagctccaggctctccagcagaacggatctagcgtgctttcagaggataaaagcaaaaggctgaacaccatacttaataccatgtccacaatttactctactggtaaagtatgtaaccccgacaaccctcaagaatgcctccttcttgagccaggcctcaatgagatcatggctaatagtctggactataatgaaagactgtgggcatgggagtcctggagatctgaagtagggaagcaactgaggcccctttatgaagagtacgtcgtacttaagaatgaaatggcccgcgctaaccactacgaggattacggcgattactggcgtggggactatgaagtaaatggtgtagatggatacgactatagtcgtgggcaattgattgaggatgtggagcacacttttgaggagataaaaccactctatgagcatcttcacgcatatgtgagagctaaactgatgaacgcctacccaagttacatcagtccaatcggatgtctcccagctcacctccttggcgacatgtggggacgtttctggaccaatctgtattccctcacagtccctttcgggcaaaagcctaatatagacgtgacagacgcaatggttgatcaggcttgggatgctcaaaggatttttaaggaagctgagaagttttttgtgtcagtcggtttgccaaatatgacacaaggcttctgggaaaatagcatgttgactgatcccggtaatgttcaaaaggctgtgtgtcaccctaccgcttgggaccttgggaaaggtgactttcgaatcttgatgtgtaccaaggtgacaatggatgactttcttacagcccataatgaaatgggtcacatccagtatgatatggcttatgcagctcaacctttcctcttgagaaatggtgcaaatgaaggttttcatgaagctgtaggggaaataatgtccctgagtgctgcaaccccaaagcatctcaagagtatcggattgttgagcccagattttcaagaagataacgagaccgaaatcaacttccttctgaaacaagccctcacaatagttggtactcttccattcacatacatgctggagaaatggcgttggatggtttttaagggggagatacctaaagatcagtggatgaaaaagtggtgggagatgaagcgtgagatcgtaggggtcgtggagccagtgcctcatgatgagacttactgtgacccagcatcactcttccacgttagcaatgactattcatttatacgttattacactcgcactctttaccagtttcaatttcaggaggctctgtgtcaggctgccaagcatgagggaccccttcacaagtgtgatattagtaacagtactgaggcaggccaaaaactgttcaatatgttgaggcttggcaaaagcgagccatggactctcgccttggaaaatgttgtcggggctaaaaacatgaatgtacgccctctgcttaactattttgagcccctttttacatggctcaaggaccagaataagaactcctttgtcggctggtcaacagactggtctccctatgcagac

SEQ ID NO: 217 - DNA, 1845 bp, synthetic construct
  misc_feature 1..1845: note = CDS for T27Y H34A H378N ACE2 mutant
  source 1..1845: mol_type = other DNA
atgagcagcagtagttggcttctcttgagtttggtggcagtgacagcagcccagagtactatcgaggagcaggctaaatactttctggataagtttaacgccgaggccgaagacttgttctatcaatcttctctcgcttcatggaattacaatactaacatcactgaggagaacgtccagaatatgaacaatgctggcgacaaatggagcgccttcttgaaggagcagtctacccttgcacaaatgtatccactgcaggagatacagaaccttacagtaaagttgcagctccaggctctccagcagaacggatctagcgtgctttcagaggataaaagcaaaaggctgaacaccatacttaataccatgtccacaatttactctactggtaaagtatgtaaccccgacaaccctcaagaatgcctccttcttgagccaggcctcaatgagatcatggctaatagtctggactataatgaaagactgtgggcatgggagtcctggagatctgaagtagggaagcaactgaggcccctttatgaagagtacgtcgtacttaagaatgaaatggcccgcgctaaccactacgaggattacggcgattactggcgtggggactatgaagtaaatggtgtagatggatacgactatagtcgtgggcaattgattgaggatgtggagcacacttttgaggagataaaaccactctatgagcatcttcacgcatatgtgagagctaaactgatgaacgcctacccaagttacatcagtccaatcggatgtctcccagctcacctccttggcgacatgtggggacgtttctggaccaatctgtattccctcacagtccctttcgggcaaaagcctaatatagacgtgacagacgcaatggttgatcaggcttgggatgctcaaaggatttttaaggaagctgagaagttttttgtgtcagtcggtttgccaaatatgacacaaggcttctgggaaaatagcatgttgactgatcccggtaatgttcaaaaggctgtgtgtcaccctaccgcttgggaccttgggaaaggtgactttcgaatcttgatgtgtaccaaggtgacaatggatgactttcttacagcccatcatgaaatgggtaatatccagtatgatatggcttatgcagctcaacctttcctcttgagaaatggtgcaaatgaaggttttcatgaagctgtaggggaaataatgtccctgagtgctgcaaccccaaagcatctcaagagtatcggattgttgagcccagattttcaagaagataacgagaccgaaatcaacttccttctgaaacaagccctcacaatagttggtactcttccattcacatacatgctggagaaatggcgttggatggtttttaagggggagatacctaaagatcagtggatgaaaaagtggtgggagatgaagcgtgagatcgtaggggtcgtggagccagtgcctcatgatgagacttactgtgacccagcatcactcttccacgttagcaatgactattcatttatacgttattacactcgcactctttaccagtttcaatttcaggaggctctgtgtcaggctgccaagcatgagggaccccttcacaagtgtgatattagtaacagtactgaggcaggccaaaaactgttcaatatgttgaggcttggcaaaagcgagccatggactctcgccttggaaaatgttgtcggggctaaaaacatgaatgtacgccctctgcttaactattttgagcccctttttacatggctcaaggaccagaataagaactcctttgtcggctggtcaacagactggtctccctatgcagac

SEQ ID NO: 218 - DNA, 1845 bp, synthetic construct
  misc_feature 1..1845: note = CDS for T27Y H34A H345A ACE2 mutant
  source 1..1845: mol_type = other DNA
atgagcagcagtagttggcttctcttgagtttggtggcagtgacagcagcccagagtactatcgaggagcaggctaaatactttctggataagtttaacgccgaggccgaagacttgttctatcaatcttctctcgcttcatggaattacaatactaacatcactgaggagaacgtccagaatatgaacaatgctggcgacaaatggagcgccttcttgaaggagcagtctacccttgcacaaatgtatccactgcaggagatacagaaccttacagtaaagttgcagctccaggctctccagcagaacggatctagcgtgctttcagaggataaaagcaaaaggctgaacaccatacttaataccatgtccacaatttactctactggtaaagtatgtaaccccgacaaccctcaagaatgcctccttcttgagccaggcctcaatgagatcatggctaatagtctggactataatgaaagactgtgggcatgggagtcctggagatctgaagtagggaagcaactgaggcccctttatgaagagtacgtcgtacttaagaatgaaatggcccgcgctaaccactacgaggattacggcgattactggcgtggggactatgaagtaaatggtgtagatggatacgactatagtcgtgggcaattgattgaggatgtggagcacacttttgaggagataaaaccactctatgagcatcttcacgcatatgtgagagctaaactgatgaacgcctacccaagttacatcagtccaatcggatgtctcccagctcacctccttggcgacatgtggggacgtttctggaccaatctgtattccctcacagtccctttcgggcaaaagcctaatatagacgtgacagacgcaatggttgatcaggcttgggatgctcaaaggatttttaaggaagctgagaagttttttgtgtcagtcggtttgccaaatatgacacaaggcttctgggaaaatagcatgttgactgatcccggtaatgttcaaaaggctgtgtgtgcccctaccgcttgggaccttgggaaaggtgactttcgaatcttgatgtgtaccaaggtgacaatggatgactttcttacagcccatcatgaaatgggtcacatccagtatgatatggcttatgcagctcaacctttcctcttgagaaatggtgcaaatgaaggttttcatgaagctgtaggggaaataatgtccctgagtgctgcaaccccaaagcatctcaagagtatcggattgttgagcccagattttcaagaagataacgagaccgaaatcaacttccttctgaaacaagccctcacaatagttggtactcttccattcacatacatgctggagaaatggcgttggatggtttttaagggggagatacctaaagatcagtggatgaaaaagtggtgggagatgaagcgtgagatcgtaggggtcgtggagccagtgcctcatgatgagacttactgtgacccagcatcactcttccacgttagcaatgactattcatttatacgttattacactcgcactctttaccagtttcaatttcaggaggctctgtgtcaggctgccaagcatgagggaccccttcacaagtgtgatattagtaacagtactgaggcaggccaaaaactgttcaatatgttgaggcttggcaaaagcgagccatggactctcgccttggaaaatgttgtcggggctaaaaacatgaatgtacgccctctgcttaactattttgagcccctttttacatggctcaaggaccagaataagaactcctttgtcggctggtcaacagactggtctccctatgcagac

SEQ ID NO: 219 - DNA, 1845 bp, synthetic construct
  misc_feature 1..1845: note = CDS for T27Y H34A R273Q ACE2 mutant
  source 1..1845: mol_type = other DNA
atgagcagcagtagttggcttctcttgagtttggtggcagtgacagcagcccagagtactatcgaggagcaggctaaatactttctggataagtttaacgccgaggccgaagacttgttctatcaatcttctctcgcttcatggaattacaatactaacatcactgaggagaacgtccagaatatgaacaatgctggcgacaaatggagcgccttcttgaaggagcagtctacccttgcacaaatgtatccactgcaggagatacagaaccttacagtaaagttgcagctccaggctctccagcagaacggatctagcgtgctttcagaggataaaagcaaaaggctgaacaccatacttaataccatgtccacaatttactctactggtaaagtatgtaaccccgacaaccctcaagaatgcctccttcttgagccaggcctcaatgagatcatggctaatagtctggactataatgaaagactgtgggcatgggagtcctggagatctgaagtagggaagcaactgaggcccctttatgaagagtacgtcgtacttaagaatgaaatggcccgcgctaaccactacgaggattacggcgattactggcgtggggactatgaagtaaatggtgtagatggatacgactatagtcgtgggcaattgattgaggatgtggagcacacttttgaggagataaaaccactctatgagcatcttcacgcatatgtgagagctaaactgatgaacgcctacccaagttacatcagtccaatcggatgtctcccagctcacctccttggcgacatgtggggacagttctggaccaatctgtattccctcacagtccctttcgggcaaaagcctaatatagacgtgacagacgcaatggttgatcaggcttgggatgctcaaaggatttttaaggaagctgagaagttttttgtgtcagtcggtttgccaaatatgacacaaggcttctgggaaaatagcatgttgactgatcccggtaatgttcaaaaggctgtgtgtcaccctaccgcttgggaccttgggaaaggtgactttcgaatcttgatgtgtaccaaggtgacaatggatgactttcttacagcccatcatgaaatgggtcacatccagtatgatatggcttatgcagctcaacctttcctcttgagaaatggtgcaaatgaaggttttcatgaagctgtaggggaaataatgtccctgagtgctgcaaccccaaagcatctcaagagtatcggattgttgagcccagattttcaagaagataacgagaccgaaatcaacttccttctgaaacaagccctcacaatagttggtactcttccattcacatacatgctggagaaatggcgttggatggtttttaagggggagatacctaaagatcagtggatgaaaaagtggtgggagatgaagcgtgagatcgtaggggtcgtggagccagtgcctcatgatgagacttactgtgacccagcatcactcttccacgttagcaatgactattcatttatacgttattacactcgcactctttaccagtttcaatttcaggaggctctgtgtcaggctgccaagcatgagggaccccttcacaagtgtgatattagtaacagtactgaggcaggccaaaaactgttcaatatgttgaggcttggcaaaagcgagccatggactctcgccttggaaaatgttgtcggggctaaaaacatgaatgtacgccctctgcttaactattttgagcccctttttacatggctcaaggaccagaataagaactcctttgtcggctggtcaacagactggtctccctatgcagac

SEQ ID NO: 220 - DNA, 38496 bp, synthetic construct
  misc_feature 1..38496: note = vector for IgA against T27Y H34A R273K ACE2 mutant
  source 1..38496: mol_type = other DNA
tattattgatgatgttaattaacatgcatggatcctacgtctcgaccgatgcccttgagagccttcaacccagtcagctccttccggtgggcgcggggcatgactatcgtcgccgcacttatgactgtcttctttatcatgcaactcgtaggacaggtgccggcagcgctctgggtcattttcggcgaggaccgctttcgctggagcgcgacgatgatcggcctgtcgcttgcggtattcggaatcttgcacgccctcgctcaagccttcgtcactggtcccgccaccaaacgtttcggcgagaagcaggccattatcgccggcatggcggccgacgcgctgggctacgtcttgctggcgttcgcgacgcgaggctggatggccttccccattatgattcttctcgcttccggcggcatcgggatgcccgcgttgcaggccatgctgtccaggcaggtagatgacgaccatcagggacagcttcaaggatcgctcgcggctcttaccagcctaacttcgatcattggaccgctgatcgtcacggcgatttatgccgcctcggcgagcacatggaacgggttggcatggattgtaggcgccgccctataccttgtctgcctccccgcgttgcgtcgcggtgcatggagccgggccacctcgacctgaatggaagccggcggcacctcgctaacggattcaccactccaagaattggagccaatcaattcttgcggagaactgtgaatgcgcaaaccaacccttggcagaacatatccatcgcgtccgccatctccagcagccgcacgcggcgcatctcgggcagcgttgggtcctggccacgggtgcgcatgatcgtgctcctgtcgttgaggacccggctaggctggcggggttgccttactggttagcagaatgaatcaccgatacgcgagcgaacgtgaagcgactgctgctgcaaaacgtctgcgacctgagcaacaacatgaatggtcttcggtttccgtgtttcgtaaagtctggaaacgcggaagtcagcgccctgcaccattatgttccggatctgcatcgcaggatgctgctggctaccctgtggaacacctacatctgtattaacgaagcgctggcattgaccctgagtgatttttctctggtcccgccgcatccataccgccagttgtttaccctcacaacgttccagtaaccgggcatgttcatcatcagtaacccgtatcgtgagcatcctctctcgtttcatcggtatcattacccccatgaacagaaatcccccttacacggaggcatcagtgaccaaacaggaaaaaaccgcccttaacatggcccgctttatcagaagccagacattaacgcttctggagaaactcaacgagctggacgcggatgaacaggcagacatctgtgaatcgcttcacgaccacgctgatgagctttaccgcagctgcctcgcgcgtttcggtgatgacggtgaaaacctctgacacatgcagctcccggagacggtcacagcttgtctgtaagcggatgccgggagcagacaagcccgtcagggcgcgtcagcgggtgttggcgggtgtcggggcgcagccatgacccagtcacgtagcgatagcggagtgtatactggcttaactatgcggcatcagagcagattgtactgagagtgcaccatatgcggtgtgaaataccgcacagatgcgtaaggagaaaataccgcatcaggcgctcttccgcttcctcgctcactgactcgctgcgctcggtcgttcggctgcggcgagcggtatcagctcactcaaaggcggtaatacggttatccacagaatcaggggataacgcaggaaagaacatgtgagcaaaaggccagcaaaaggccaggaaccgtaaaaaggccgcgttgctggcgtttttccataggctccgcccccctgacgagcatcacaaaaatcgacgctcaagtcagaggtggcgaaacccgacaggactataaagataccaggcgtttccccctggaagctccctcgtgcgctctcctgttccgaccctgccgcttaccggatacctgtccgcctttctcccttcgggaagcgtggcgctttctcatagctcacgctgtaggtatctcagttcggtgtaggtcgttcgctccaagctgggctgtgtgcacgaaccccccgttcagcccgaccgctgcgccttatccggtaactatcgtcttgagtccaacccggtaagacacgacttatcgccactggcagcagccactggtaacaggattagcagagcgaggtatgtaggcggtgctacagagttcttgaagtggtggcctaactacggctacactagaaggacagtatttggtatctgcgctctgctgaagccagttaccttcggaaaaagagttggtagctcttgatccggcaaacaaaccaccgctggtagcggtggtttttttgtttgcaagcagcagattacgcgcagaaaaaaaggatctcaagaagatcctttgatcttttctacggggtctgacgctcagtggaacgaaaactcacgttaagggattttggtcatgagattatcaaaaaggatcttcacctagatccttttaaattaaaaatgaagttttaaatcaatctaaagtatatatgagtaaacttggtctgacagttaccaatgcttaatcagtgaggcacctatctcagcgatctgtctatttcgttcatccatagttgcctgactccccgtcgtgtagataactacgatacgggagggcttaccatctggccccagtgctgcaatgataccgcgagacccacgctcaccggctccagatttatcagcaataaaccagccagccggaagggccgagcgcagaagtggtcctgcaactttatccgcctccatccagtctattaattgttgccgggaagctagagtaagtagttcgccagttaatagtttgcgcaacgttgttgccattgctgcagccatgagattatcaaaaaggatcttcacctagatccttttcacgtagaaagccagtccgcagaaacggtgctgaccccggatgaatgtcagctactgggctatctggacaagggaaaacgcaagcgcaaagagaaagcaggtagcttgcagtgggcttacatggcgatagctagactgggcggttttatggacagcaagcgaaccggaattgccagctggggcgccctctggtaaggttgggaagccctgcaaagtaaactggatggctttcttgccgccaaggatctgatggcgcaggggatcaagctctgatcaagagacaggatgaggatcgtttcgcatgattgaacaagatggattgcacgcaggttctccggccgcttgggtggagaggctattcggctatgactgggcacaacagacaatcggctgctctgatgccgccgtgttccggctgtcagcgcaggggcgcccggttctttttgtcaagaccgacctgtccggtgccctgaatgaactgcaagacgaggcagcgcggctatcgtggctggccacgacgggcgttccttgcgcagctgtgctcgacgttgtcactgaagcgggaagggactggctgctattgggcgaagtgccggggcaggatctcctgtcatctcaccttgctcctgccgagaaagtatccatcatggctgatgcaatgcggcggctgcatacgcttgatccggctacctgcccattcgaccaccaagcgaaacatcgcatcgagcgagcacgtactcggatggaagccggtcttgtcgatcaggatgatctggacgaagagcatcaggggctcgcgccagccgaactgttcgccaggctcaaggcgagcatgcccgacggcgaggatctcgtcgtgacccatggcgatgcctgcttgccgaatatcatggtggaaaatggccgcttttctggattcatcgactgtggccggctgggtgtggcggaccgctatcaggacatagcgttggctacccgtgatattgctgaagagcttggcggcgaatgggctgaccgcttcctcgtgctttacggtatcgccgctcccgattcgcagcgcatcgccttctatcgccttcttgacgagttcttctgaattttgttaaaatttttgttaaatcagctcattttttaaccaataggccgaaatcggcaaaatcccttataaatcaaaagaatagaccgagatagggttgagtgttgttccagtttggaacaagagtccactattaaagaacgtggactccaacgtcaaagggcgaaaaaccgtctatcagggcgatggcccactacgtgaaccatcaccctaatcaagttttttggggtcgaggtgccgtaaagcactaaatcggaaccctaaagggagcccccgatttagagcttgacggggaaagccggcgaacgtggcgagaaaggaagggaagaaagcgaaaggagcgggcgctagggcgctggcaagtgtagcggtcacgctgcgcgtaaccaccacacccgccgcgcttaatgcgccgctacagggcgcgtccattcgccattcaggatcgaattaattcttaattaacatcatcaataatataccttattttggattgaagccaatatgataatgagggggtggagtttgtgacgtggcgcggggcgtgggaacggggcgggtgacgtagtagtgtggcggaagtgtgatgttgcaagtgtggcggaacacatgtaagcgacggatgtggcaaaagtgacgtttttggtgtgcgccggtgtacacaggaagtgacaattttcgcgcggttttaggcggatgttgtagtaaatttgggcgtaaccgagtaagatttggccattttcgcgggaaaactgaataagaggaagtgaaatctgaataattttgtgttactcatagcgcgtaatactgtaatagtaatcaattacggggtcattagttcatagcccatatatggagttccgcgttacataacttacggtaaatggcccgcctggctgaccgcccaacgacccccgcccattgacgtcaataatgacgtatgttcccatagtaacgccaatagggactttccattgacgtcaatgggtggagtatttacggtaaactgcccacttggcagtacatcaagtgtatcatatgccaagtacgccccctattgacgtcaatgacggtaaatggcccgcctggcattatgcccagtacatgaccttatgggactttcctacttggcagtacatctacgtattagtcatcgctattaccatggtgatgcggttttggcagtacatcaatgggcgtggatagcggtttgactcacggggatttccaagtctccaccccattgacgtcaatgggagtttgttttggcaccaaaatcaacgggactttccaaaatgtcgtaacaactccgccccattgacgcaaatgggcggtaggcgtgtacggtgggaggtctatataagcagagctggtttagtgaaccgtcagatccgctagagatctggtaccgtcgacgcggccgctcgagcctaagcttatgagcagcagtagttggcttctcttgagtttggtggcagtgacagcagcccagagtactatcgaggagcaggctaaatactttctggataagtttaacgccgaggccgaagacttgttctatcaatcttctctcgcttcatggaattacaatactaacatcactgaggagaacgtccagaatatgaacaatgctggcgacaaatggagcgccttcttgaaggagcagtctacccttgcacaaatgtatccactgcaggagatacagaaccttacagtaaagttgcagctccaggctctccagcagaacggatctagcgtgctttcagaggataaaagcaaaaggctgaacaccatacttaataccatgtccacaatttactctactggtaaagtatgtaaccccgacaaccctcaagaatgcctccttcttgagccaggcctcaatgagatcatggctaatagtctggactataatgaaagactgtgggcatgggagtcctggagatctgaagtagggaagcaactgaggcccctttatgaagagtacgtcgtacttaagaatgaaatggcccgcgctaaccactacgaggattacggcgattactggcgtggggactatgaagtaaatggtgtagatggatacgactatagtcgtgggcaattgattgaggatgtggagcacacttttgaggagataaaaccactctatgagcatcttcacgcatatgtgagagctaaactgatgaacgcctacccaagttacatcagtccaatcggatgtctcccagctcacctccttggcgacatgtggggaaagttctggaccaatctgtattccctcacagtccctttcgggcaaaagcctaatatagacgtgacagacgcaatggttgatcaggcttgggatgctcaaaggatttttaaggaagctgagaagttttttgtgtcagtcggtttgccaaatatgacacaaggcttctgggaaaatagcatgttgactgatcccggtaatgttcaaaaggctgtgtgtcaccctaccgcttgggaccttgggaaaggtgactttcgaatcttgatgtgtaccaaggtgacaatggatgactttcttacagcccatcatgaaatgggtcacatccagtatgatatggcttatgcagctcaacctttcctcttgagaaatggtgcaaatgaaggttttcatgaagctgtaggggaaataatgtccctgagtgctgcaaccccaaagcatctcaagagtatcggattgttgagcccagattttcaagaagataacgagaccgaaatcaacttccttctgaaacaagccctcacaatagttggtactcttccattcacatacatgctggagaaatggcgttggatggtttttaagggggagatacctaaagatcagtggatgaaaaagtggtgggagatgaagcgtgagatcgtaggggtcgtggagccagtgcctcatgatgagacttactgtgacccagcatcactcttccacgttagcaatgactattcatttatacgttattacactcgcactctttaccagtttcaatttcaggaggctctgtgtcaggctgccaagcatgagggaccccttcacaagtgtgatattagtaacagtactgaggcaggccaaaaactgttcaatatgttgaggcttggcaaaagcgagccatggactctcgccttggaaaatgttgtcggggctaaaaacatgaatgtacgccctctgcttaactattttgagcccctttttacatggctcaaggaccagaataagaactcctttgtcggctggtcaacagactggtctccctatgcagaccctagtactcctcctactccttctccatcaaccccaccaactccatcccctagctgctgtcacccaaggctgtctctgcaccgacctgcactcgaagaccttctgttgggctctgaagctaacctgacctgtactcttactggcttgcgcgatgctagcggcgtgactttcacctggacacctagtagcggtaaaagtgctgtacaaggacctcctgaacgcgacctgtgtggttgctactctgtgtcttctgtacttcccggctgtgccgagccctggaatcacgggaaaacctttacctgcaccgccgcttaccctgagtcaaaaactcccctcactgccacattgagtaagtcagggaatacattcaggccagaggttcatttgttgcctcctccatctgaagaacttgctttgaacgagctggtcactctgacctgcttggctaggggtttctcccccaaagatgtacttgtacggtggttgcagggcagccaagagttgccccgcgaaaagtatttgacctgggcctcaagacaagaacccagccaggggactaccacatttgccgtgaccagtattctgcgtgtagccgctgaagattggaagaaaggggatacattttcttgcatggtagggcatgaggcccttcccctcgctttcactcagaagacaatagacagactcgccggaaagcctactcacgtgaatgttagcgtagtcatggctgaggttgacggaacttgctactgagatatccgatccaccggatctagataactgatcataatcagccataccacatttgtagaggttttacttgctttaaaaaacctcccacacctccccctgaacctgaaacataaaatgaatgcaattgttgttgttaacttgtttattgcagcttataatggttacaaataaagcaatagcatcacaaatttcacaaataaagcatttttttcactgcattctagttgtggtttgtccaaactcatcaatgtatcttaggtttagtgaaccgtcagatccgctagcgttacataacttacggtaaatggcccgcctggctgaccgcccaacgacccccgcccattgacgtcaataatgacgtatgttcccatagtaacgccaatagggactttccattgacgtcaatgggtggagtatttacggtaaactgcccacttggcagtacatcaagtgtatcatatgccaagtacgccccctattgacgtcaatgacggtaaatggcccgcctggcattatgcccagtacatgaccttatgggactttcctacttggcagtacatctacgtattagtcatcgctattaccatggtgatgcggttttggcagtacatcaatgggcgtggatagcggtttgactcacggggatttccaagtctccaccccattgacgtcaatgggagtttgttttggcaccaaaatcaacgggactttccaaaatgtcgtaacaactccgccccattgacgcaaatgggcggtaggcgtgtacggtgggaggtctatataagcagagctggtttagtgaaccgtcagatccgctagagatctggtaccgtcgacgcggccgctcgagcctaagcttatgaagaaccatctgcttttctggggagtacttgccgttttcataaaagccgtacatgttaaagcacaagaggacgaacgcattgtgttggttgataataaatgcaaatgtgctcggataacatctcggatcattcgtagctcagaggaccccaatgaggatatagtagagcgaaacatcagaattatagtacccctgaacaacagagagaacataagtgatcccacaagtccattgcggacacgctttgtttaccatttgtctgatctgtgtaaaaaatgtgatccaacagaggtggaactcgacaatcagatcgtcaccgccacccagtctaacatctgcgatgaagattcagctacagagacatgctacacatacgaccggaacaagtgctatactgccgttgtgccactcgtttacggtggagaaacaaagatggttgaaactgcacttacaccagatgcctgctatccagattgagatatccgatccaccggatctagataactgatcataatcagccataccacatttgtagaggttttacttgctttaaaaaacctcccacacctccccctgaacctgaaacataaaatgaatgcaattgttgttgttaacttgtttattgcagcttataatggttacaaataaagcaatagcatcacaaatttcacaaataaagcatttttttcactgcattctagttgtggtttgtccaaactcatcaatgtatcttaacgcggatctgggcgtggttaagggtgggaaagaatatataaggtgggggtcttatgtagttttgtatctgttttgcagcagccgccgccgccatgagcaccaactcgtttgatggaagcattgtgagctcatatttgacaacgcgcatgcccccatgggccggggtgcgtcagaatgtgatgggctccagcattgatggtcgccccgtcctgcccgcaaactctactaccttgacctacgagaccgtgtctggaacgccgttggagactgcagcctccgccgccgcttcagccgctgcagccaccgcccgcgggattgtgactgactttgctttcctgagcccgcttgcaagcagtgcagcttcccgttcatccgcccgcgatgacaagttgacggctcttttggcacaattggattctttgacccgggaacttaatgtcgtttctcagcagctgttggatctgcgccagcaggtttctgccctgaaggcttcctcccctcccaatgcggtttaaaacataaataaaaaaccagactctgtttggatttggatcaagcaagtgtcttgctgtctttatttaggggttttgcgcgcgcggtaggcccgggaccagcggtctcggtcgttgagggtcctgtgtattttttccaggacgtggtaaaggtgactctggatgttcagatacatgggcataagcccgtctctggggtggaggtagcaccactgcagagcttcatgctgcggggtggtgttgtagatgatccagtcgtagcaggagcgctgggcgtggtgcctaaaaatgtctttcagtagcaagctgattgccaggggcaggcccttggtgtaagtgtttacaaagcggttaagctgggatgggtgcatacgtggggatatgagatgcatcttggactgtatttttaggttggctatgttcccagccatatccctccggggattcatgttgtgcagaaccaccagcacagtgtatccggtgcacttgggaaatttgtcatgtagcttagaaggaaatgcgtggaagaacttggagacgcccttgtgacctccaagattttccatgcattcgtccataatgatggcaatgggcccacgggcggcggcctgggcgaagatatttctgggatcactaacgtcatagttgtgttccaggatgagatcgtcataggccatttttacaaagcgcgggcggagggtgccagactgcggtataatggttccatccggcccaggggcgtagttaccctcacagatttgcatttcccacgctttgagttcagatggggggatcatgtctacctgcggggcgatgaagaaaacggtttccggggtaggggagatcagctgggaagaaagcaggttcctgagcagctgcgacttaccgcagccggtgggcccgtaaatcacacctattaccggctgcaactggtagttaagagagctgcagctgccgtcatccctgagcaggggggccacttcgttaagcatgtccctgactcgcatgttttccctgaccaaatccgccagaaggcgctcgccgcccagcgatagcagttcttgcaaggaagcaaagtttttcaacggtttgagaccgtccgccgtaggcatgcttttgagcgtttgaccaagcagttccaggcggtcccacagctcggtcacctgctctacggcatctcgatccagcatatctcctcgtttcgcgggttggggcggctttcgctgtacggcagtagtcggtgctcgtccagacgggccagggtcatgtctttccacgggcgcagggtcctcgtcagcgtagtctgggtcacggtgaaggggtgcgctccgggctgcgcgctggccagggtgcgcttgaggctggtcctgctggtgctgaagcgctgccggtcttcgccctgcgcgtcggccaggtagcatttgaccatggtgtcatagtccagcccctccgcggcgtggcccttggcgcgcagcttgcccttggaggaggcgccgcacgaggggcagtgcagacttttgagggcgtagagcttgggcgcgagaaataccgattccggggagtaggcatccgcgccgcaggccccgcagacggtctcgcattccacgagccaggtgagctctggccgttcggggtcaaaaaccaggtttcccccatgctttttgatgcgtttcttacctctggtttccatgagccggtgtccacgctcggtgacgaaaaggctgtccgtgtccccgtatacagacttgagaggcctgtcctcgagcggtgttccgcggtcctcctcgtatagaaactcggaccactctgagacaaaggctcgcgtccaggccagcacgaaggaggctaagtgggaggggtagcggtcgttgtccactagggggtccactcgctccagggtgtgaagacacatgtcgccctcttcggcatcaaggaaggtgattggtttgtaggtgtaggccacgtgaccgggtgttcctgaaggggggctataaaagggggtgggggcgcgttcgtcctcactctcttccgcatcgctgtctgcgagggccagctgttggggtgagtactccctctgaaaagcgggcatgacttctgcgctaagattgtcagtttccaaaaacgaggaggatttgatattcacctggcccgcggtgatgcctttgagggtggccgcatccatctggtcagaaaagacaatctttttgttgtcaagcttggtggcaaacgacccgtagagggcgttggacagcaacttggcgatggagcgcagggtttggtttttgtcgcgatcggcgcgctccttggccgcgatgtttagctgcacgtattcgcgcgcaacgcaccgccattcgggaaagacggtggtgcgctcgtcgggcaccaggtgcacgcgccaaccgcggttgtgcagggtgacaaggtcaacgctggtggctacctctccgcgtaggcgctcgttggtccagcagaggcggccgcccttgcgcgagcagaatggcggtagggggtctagctgcgtctcgtccggggggtctgcgtccacggtaaagaccccgggcagcaggcgcgcgtcgaagtagtctatcttgcatccttgcaagtctagcgcctgctgccatgcgcgggcggcaagcgcgcgctcgtatgggttgagtgggggaccccatggcatggggtgggtgagcgcggaggcgtacatgccgcaaatgtcgtaaacgtagaggggctctctgagtattccaagatatgtagggtagcatcttccaccgcggatgctggcgcgcacgtaatcgtatagttcgtgcgagggagcgaggaggtcgggaccgaggttgctacgggcgggctgctctgctcggaagactatctgcctgaagatggcatgtgagttggatgatatggttggacgctggaagacgttgaagctggcgtctgtgagacctaccgcgtcacgcacgaaggaggcgtaggagtcgcgcagcttgttgaccagctcggcggtgacctgcacgtctagggcgcagtagtccagggtttccttgatgatgtcatacttatcctgtcccttttttttccacagctcgcggttgaggacaaactcttcgcggtctttccagtactcttggatcggaaacccgtcggcctccgaacggtaagagcctagcatgtagaactggttgacggcctggtaggcgcagcatcccttttctacgggtagcgcgtatgcctgcgcggccttccggcatgaccagcatgaagggcacgagctgcttcccaaaggcccccatccaagtataggtctctacatcgtaggtgacaaagagacgctcggtgcgaggatgcgagccgatcgggaagaactggatctcccgccaccaattggaggagtggctattgatgtggtgaaagtagaagtccctgcgacgggccgaacactcgtgctggcttttgtaaaaacgtgcgcagtactggcagcggtgcacgggctgtacatcctgcacgaggttgacctgacgaccgcgcacaaggaagcagagtgggaatttgagcccctcgcctggcgggtttggctggtggtcttctacttcggctgcttgtccttgaccgtctggctgctcgaggggagttacggtggatcggaccaccacgccgcgcgagcccaaagtccagatgtccgcgcgcggcggtcggagcttgatgacaacatcgcgcagatgggagctgtccatggtctggagctcccgcggcgtcaggtcaggcgggagctcctgcaggtttacctcgcatagacgggtcagggcgcgggctagatccaggtgatacctaatttccaggggctggttggtggcggcgtcgatggcttgcaagaggccgcatccccgcggcgcgactacggtaccgcgcggcgggcggtgggccgcgggggtgtccttggatgatgcatctaaaagcggtgacgcgggcgagcccccggaggtagggggggctccggacccgccgggagagggggcaggggcacgtcggcgccgcgcgcgggcaggagctggtgctgcgcgcgtaggttgctggcgaacgcgacgacgcggcggttgatctcctgaatctggcgcctctgcgtgaagacgacgggcccggtgagcttgaacctgaaagagagttcgacagaatcaatttcggtgtcgttgacggcggcctggcgcaaaatctcctgcacgtctcctgagttgtcttgataggcgatctcggccatgaactgctcgatctcttcctcctggagatctccgcgtccggctcgctccacggtggcggcgaggtcgttggaaatgcgggccatgagctgcgagaaggcgttgaggcctccctcgttccagacgcggctgtagaccacgcccccttcggcatcgcgggcgcgcatgaccacctgcgcgagattgagctccacgtgccgggcgaagacggcgtagtttcgcaggcgctgaaagaggtagttgagggtggtggcggtgtgttctgccacgaagaagtacataacccagcgtcgcaacgtggattcgttgataattgttgtgtaggtactccgccgccgagggacctgagcgagtccgcatcgaccggatcggaaaacctctcgagaaaggcgtctaaccagtcacagtcgcaaggtaggctgagcaccgtggcgggcggcagcgggcggcggtcggggttgtttctggcggaggtgctgctgatgatgtaattaaagtaggcggtcttgagacggcggatggtcgacagaagcaccatgtccttgggtccggcctgctgaatgcgcaggcggtcggccatgccccaggcttcgttttgacatcggcgcaggtctttgtagtagtcttgcatgagcctttctaccggcacttcttcttctccttcctcttgtcctgcatctcttgcatctatcgctgcggcggcggcggagtttggccgtaggtggcgccctcttcctcccatgcgtgtgaccccgaagcccctcatcggctgaagcagggctaggtcggcgacaacgcgctcggctaatatggcctgctgcacctgcgtgagggtagactggaagtcatccatgtccacaaagcggtggtatgcgcccgtgttgatggtgtaagtgcagttggccataacggaccagttaacggtctggtgacccggctgcgagagctcggtgtacctgagacgcgagtaagccctcgagtcaaatacgtagtcgttgcaagtccgcaccaggtactggtatcccaccaaaaagtgcggcggcggctggcggtagaggggccagcgtagggtggccggggctccgggggcgagatcttccaacataaggcgatgatatccgtagatgtacctggacatccaggtgatgccggcggcggtggtggaggcgcgcggaaagtcgcggacgcggttccagatgttgcgcagcggcaaaaagtgctccatggtcgggacgctctggccggtcaggcgcgcgcaatcgttgacgctctagcgtgcaaaaggagagcctgtaagcgggcactcttccgtggtctggtggataaattcgcaagggtatcatggcggacgaccggggttcgagccccgtatccggccgtccgccgtgatccatgcggttaccgcccgcgtgtcgaacccaggtgtgcgacgtcagacaacgggggagtgctccttttggcttccttccaggcgcggcggctgctgcgctagcttttttggccactggccgcgcgcagcgtaagcggttaggctggaaagcgaaagcattaagtggctcgctccctgtagccggagggttattttccaagggttgagtcgcgggacccccggttcgagtctcggaccggccggactgcggcgaacgggggtttgcctccccgtcatgcaagaccccgcttgcaaattcctccggaaacagggacgagccccttttttgcttttcccagatgcatccggtgctgcggcagatgcgcccccctcctcagcagcggcaagagcaagagcagcggcagacatgcagggcaccctcccctcctcctaccgcgtcaggaggggcgacatccgcggttgacgcggcagcagatggtgattacgaacccccgcggcgccgggcccggcactacctggacttggaggagggcgagggcctggcgcggctaggagcgccctctcctgagcggcacccaagggtgcagctgaagcgtgatacgcgtgaggcgtacgtgccgcggcagaacctgtttcgcgaccgcgagggagaggagcccgaggagatgcgggatcgaaagttccacgcagggcgcgagctgcggcatggcctgaatcgcgagcggttgctgcgcgaggaggactttgagcccgacgcgcgaaccgggattagtcccgcgcgcgcacacgtggcggccgccgacctggtaaccgcatacgagcagacggtgaaccaggagattaactttcaaaaaagctttaacaaccacgtgcgtacgcttgtggcgcgcgaggaggtggctataggactgatgcatctgtgggactttgtaagcgcgctggagcaaaacccaaatagcaagccgctcatggcgcagctgttccttatagtgcagcacagcagggacaacgaggcattcagggatgcgctgctaaacatagtagagcccgagggccgctggctgctcgatttgataaacatcctgcagagcatagtggtgcaggagcgcagcttgagcctggctgacaaggtggccgccatcaactattccatgcttagcctgggcaagttttacgcccgcaagatataccataccccttacgttcccatagacaaggaggtaaagatcgaggggttctacatgcgcatggcgctgaaggtgcttaccttgagcgacgacctgggcgtttatcgcaacgagcgcatccacaaggccgtgagcgtgagccggcggcgcgagctcagcgaccgcgagctgatgcacagcctgcaaagggccctggctggcacgggcagcggcgatagagaggccgagtcctactttgacgcgggcgctgacctgcgctgggccccaagccgacgcgccctggaggcagctggggccggacctgggctggcggtggcacccgcgcgcgctggcaacgtcggcggcgtggaggaatatgacgaggacgatgagtacgagccagaggacggcgagtactaagcggtgatgtttctgatcagatgatgcaagacgcaacggacccggcggtgcgggcggcgctgcagagccagccgtccggccttaactccacggacgactggcgccaggtcatggaccgcatcatgtcgctgactgcgcgcaatcctgacgcgttccggcagcagccgcaggccaaccggctctccgcaattctggaagcggtggtcccggcgcgcgcaaaccccacgcacgagaaggtgctggcgatcgtaaacgcgctggccgaaaacagggccatccggcccgacgaggccggcctggtctacgacgcgctgcttcagcgcgtggctcgttacaacagcggcaacgtgcagaccaacctggaccggctggtgggggatgtgcgcgaggccgtggcgcagcgtgagcgcgcgcagcagcagggcaacctgggctccatggttgcactaaacgccttcctgagtacacagcccgccaacgtgccgcggggacaggaggactacaccaactttgtgagcgcactgcggctaatggtgactgagacaccgcaaagtgaggtgtaccagtctgggccagactattttttccagaccagtagacaaggcctgcagaccgtaaacctgagccaggctttcaaaaacttgcaggggctgtggggggtgcgggctcccacaggcgaccgcgcgaccgtgtctagcttgctgacgcccaactcgcgcctgttgctgctgctaatagcgcccttcacggacagtggcagcgtgtcccgggacacatacctaggtcacttgctgacactgtaccgcgaggccataggtcaggcgcatgtggacgagcatactttccaggagattacaagtgtcagccgcgcgctggggcaggaggacacgggcagcctggaggcaaccctaaactacctgctgaccaaccggcggcagaagatcccctcgttgcacagtttaaacagcgaggaggagcgcattttgcgctacgtgcagcagagcgtgagccttaacctgatgcgcgacggggtaacgcccagcgtggcgctggacatgaccgcgcgcaacatggaaccgggcatgtatgcctcaaaccggccgtttatcaaccgcctaatggactacttgcatcgcgcggccgccgtgaaccccgagtatttcaccaatgccatcttgaacccgcactggctaccgccccctggtttctacaccgggggattcgaggtgcccgagggtaacgatggattcctctgggacgacatagacgacagcgtgttttccccgcaaccgcagaccctgctagagttgcaacagcgcgagcaggcagaggcggcgctgcgaaaggaaagcttccgcaggccaagcagcttgtccgatctaggcgctgcggccccgcggtcagatgctagtagcccatttccaagcttgatagggtctcttaccagcactcgcaccacccgcccgcgcctgctgggcgaggaggagtacctaaacaactcgctgctgcagccgcagcgcgaaaaaaacctgcctccggcatttcccaacaacgggatagagagcctagtggacaagatgagtagatggaagacgtacgcgcaggagcacagggacgtgccaggcccgcgcccgcccacccgtcgtcaaaggcacgaccgtcagcggggtctggtgtgggaggacgatgactcggcagacgacagcagcgtcctggatttgggagggagtggcaacccgtttgcgcaccttcgccccaggctggggagaatgttttaaaaaaaaaaaagcatgatgcaaaataaaaaactcaccaaggccatggcaccgagcgttggttttcttgtattccccttagtatgcggcgcgcggcgatgtatgaggaaggtcctcctccctcctacgagagtgtggtgagcgcggcgccagtggcggcggcgctgggttctcccttcgatgctcccctggacccgccgtttgtgcctccgcggtacctgcggcctaccggggggagaaacagcatccgttactctgagttggcacccctattcgacaccacccgtgtgtacctggtggacaacaagtcaacggatgtggcatccctgaactaccagaacgaccacagcaactttctgaccacggtcattcaaaacaatgactacagcccgggggaggcaagcacacagaccatcaatcttgacgaccggtcgcactggggcggcgacctgaaaaccatcctgcataccaacatgccaaatgtgaacgagttcatgtttaccaataagtttaaggcgcgggtgatggtgtcgcgcttgcctactaaggacaatcaggtggagctgaaatacgagtgggtggagttcacgctgcccgagggcaactactccgagaccatgaccatagaccttatgaacaacgcgatcgtggagcactacttgaaagtgggcagacagaacggggttctggaaagcgacatcggggtaaagtttgacacccgcaacttcagactggggtttgaccccgtcactggtcttgtcatgcctggggtatatacaaacgaagccttccatccagacatcattttgctgccaggatgcggggtggacttcacccacagccgcctgagcaacttgttgggcatccgcaagcggcaacccttccaggagggctttaggatcacctacgatgatctggagggtggtaacattcccgcactgttggatgtggacgcctaccaggcgagcttgaaagatgacaccgaacagggcgggggtggcgcaggcggcagcaacagcagtggcagcggcgcggaagagaactccaacgcggcagccgcggcaatgcagccggtggaggacatgaacgatcatgccattcgcggcgacacctttgccacacgggctgaggagaagcgcgctgaggccgaagcagcggccgaagctgccgcccccgctgcgcaacccgaggtcgagaagcctcagaagaaaccggtgatcaaacccctgacagaggacagcaagaaacgcagttacaacctaataagcaatgacagcaccttcacccagtaccgcagctggtaccttgcatacaactacggcgaccctcagaccggaatccgctcatggaccctgctttgcactcctgacgtaacctgcggctcggagcaggtctactggtcgttgccagacatgatgcaagaccccgtgaccttccgctccacgcgccagatcagcaactttccggtggtgggcgccgagctgttgcccgtgcactccaagagcttctacaacgaccaggccgtctactcccaactcatccgccagtttacctctctgacccacgtgttcaatcgctttcccgagaaccagattttggcgcgcccgccagcccccaccatcaccaccgtcagtgaaaacgttcctgctctcacagatcacgggacgctaccgctgcgcaacagcatcggaggagtccagcgagtgaccattactgacgccagacgccgcacctgcccctacgtttacaaggccctgggcatagtctcgccgcgcgtcctatcgagccgcactttttgagcaagcatgtccatccttatatcgcccagcaataacacaggctggggcctgcgcttcccaagcaagatgtttggcggggccaagaagcgctccgaccaacacccagtgcgcgtgcgcgggcactaccgcgcgccctggggcgcgcacaaacgcggccgcactgggcgcaccaccgtcgatgacgccatcgacgcggtggtggaggaggcgcgcaactacacgcccacgccgccaccagtgtccacagtggacgcggccattcagaccgtggtgcgcggagcccggcgctatgctaaaatgaagagacggcggaggcgcgtagcacgtcgccaccgccgccgacccggcactgccgcccaacgcgcggcggcggccctgcttaaccgcgcacgtcgcaccggccgacgggcggccatgcgggccgctcgaaggctggccgcgggtattgtcactgtgccccccaggtccaggcgacgagcggccgccgcagcagccgcggccattagtgctatgactcagggtcgcaggggcaacgtgtattgggtgcgcgactcggttagcggcctgcgcgtgcccgtgcgcacccgccccccgcgcaactagattgcaagaaaaaactacttagactcgtactgttgtatgtatccagcggcggcggcgcgcaacgaagctatgtccaagcgcaaaatcaaagaagagatgctccaggtcatcgcgccggagatctatggccccccgaagaaggaagagcaggattacaagccccgaaagctaaagcgggtcaaaaagaaaaagaaagatgatgatgatgaacttgacgacgaggtggaactgctgcacgctaccgcgcccaggcgacgggtacagtggaaaggtcgacgcgtaaaacgtgttttgcgacccggcaccaccgtagtctttacgcccggtgagcgctccacccgcacctacaagcgcgtgtatgatgaggtgtacggcgacgaggacctgcttgagcaggccaacgagcgcctcggggagtttgcctacggaaagcggcataaggacatgctggcgttgccgctggacgagggcaacccaacacctagcctaaagcccgtaacactgcagcaggtgctgcccgcgcttgcaccgtccgaagaaaagcgcggcctaaagcgcgagtctggtgacttggcacccaccgtgcagctgatggtacccaagcgccagcgactggaagatgtcttggaaaaaatgaccgtggaacctgggctggagcccgaggtccgcgtgcggccaatcaagcaggtggcgccgggactgggcgtgcagaccgtggacgttcagatacccactaccagtagcaccagtattgccaccgccacagagggcatggagacacaaacgtccccggttgcctcagcggtggcggatgccgcggtgcaggcggtcgctgcggccgcgtccaagacctctacggaggtgcaaacggacccgtggatgtttcgcgtttcagccccccggcgcccgcgccgttcgaggaagtacggcgccgccagcgcgctactgcccgaatatgccctacatccttccattgcgcctacccccggctatcgtggctacacctaccgccccagaagacgagcaactacccgacgccgaaccaccactggaacccgccgccgccgtcgccgtcgccagcccgtgctggccccgatttccgtgcgcagggtggctcgcgaaggaggcaggaccctggtgctgccaacagcgcgctaccaccccagcatcgtttaaaagccggtctttgtggttcttgcagatatggccctcacctgccgcctccgtttcccggtgccgggattccgaggaagaatgcaccgtaggaggggcatggccggccacggcctgacgggcggcatgcgtcgtgcgcaccaccggcggcggcgcgcgtcgcaccgtcgcatgcgcggcggtatcctgcccctccttattccactgatcgccgcggcgattggcgccgtgcccggaattgcatccgtggccttgcaggcgcagagacactgattaaaaacaagttgcatgtggaaaaatcaaaataaaaagtctggactctcacgctcgcttggtcctgtaactattttgtagaatggaagacatcaactttgcgtctctggccccgcgacacggctcgcgcccgttcatgggaaactggcaagatatcggcaccagcaatatgagcggtggcgccttcagctggggctcgctgtggagcggcattaaaaatttcggttccaccgttaagaactatggcagcaaggcctggaacagcagcacaggccagatgctgagggataagttgaaagagcaaaatttccaacaaaaggtggtagatggcctggcctctggcattagcggggtggtggacctggccaaccaggcagtgcaaaataagattaacagtaagcttgatccccgccctcccgtagaggagcctccaccggccgtggagacagtgtctccagaggggcgtggcgaaaagcgtccgcgccccgacagggaagaaactctggtgacgcaaatagacgagcctccctcgtacgaggaggcactaaagcaaggcctgcccaccacccgtcccatcgcgcccatggctaccggagtgctgggccagcacacacccgtaacgctggacctgcctccccccgccgacacccagcagaaacctgtgctgccaggcccgaccgccgttgttgtaacccgtcctagccgcgcgtccctgcgccgcgccgccagcggtccgcgatcgttgcggcccgtagccagtggcaactggcaaagcacactgaacagcatcgtgggtctgggggtgcaatccctgaagcgccgacgatgcttctgatagctaacgtgtcgtatgtgtgtcatgtatgcgtccatgtcgccgccagaggagctgctgagccgccgcgcgcccgctttccaagatggctaccccttcgatgatgccgcagtggtcttacatgcacatctcgggccaggacgcctcggagtacctgagccccgggctggtgcagtttgcccgcgccaccgagacgtacttcagcctgaataacaagtttagaaaccccacggtggcgcctacgcacgacgtgaccacagaccggtcccagcgtttgacgctgcggttcatccctgtggaccgtgaggatactgcgtactcgtacaaggcgcggttcaccctagctgtgggtgataaccgtgtgctggacatggcttccacgtactttgacatccgcggcgtgctggacaggggccctacttttaagccctactctggcactgcctacaacgccctggctcccaagggtgccccaaatccttgcgaatgggatgaagctgctactgctcttgaaataaacctagaagaagaggacgatgacaacgaagacgaagtagacgagcaagctgagcagcaaaaaactcacgtatttgggcaggcgccttattctggtataaatattacaaaggagggtattcaaataggtgtcgaaggtcaaacacctaaatatgccgataaaacatttcaacctgaacctcaaataggagaatctcagtggtacgaaacagaaattaatcatgcagctgggagagtcctaaaaaagactaccccaatgaaaccatgttacggttcatatgcaaaacccacaaatgaaaatggagggcaaggcattcttgtaaagcaacaaaatggaaagctagaaagtcaagtggaaatgcaatttttctcaactactgaggcagccgcaggcaatggtgataacttgactcctaaagtggtattgtacagtgaagatgtagatatagaaaccccagacactcatatttcttacatgcccactattaaggaaggtaactcacgagaactaatgggccaacaatctatgcccaacaggcctaattacattgcttttagggacaattttattggtctaatgtattacaacagcacgggtaatatgggtgttctggcgggccaagcatcgcagttgaatgctgttgtagatttgcaagacagaaacacagagctttcataccagcttttgcttgattccattggtgatagaaccaggtacttttctatgtggaatcaggctgttgacagctatgatccagatgttagaattattgaaaatcatggaactgaagatgaacttccaaattactgctttccactgggaggtgtgattaatacagagactcttaccaaggtaaaacctaaaacaggtcaggaaaatggatgggaaaaagatgctacagaattttcagataaaaatgaaataagagttggaaataattttgccatggaaatcaatctaaatgccaacctgtggagaaatttcctgtactccaacatagcgctgtatttgcccgacaagctaaagtacagtccttccaacgtaaaaatttctgataacccaaacacctacgactacatgaacaagcgagtggtggctcccgggctagtggactgctacattaaccttggagcacgctggtcccttgactatatggacaacgtcaacccatttaaccaccaccgcaatgctggcctgcgctaccgctcaatgttgctgggcaatggtcgctatgtgcccttccacatccaggtgcctcagaagttctttgccattaaaaacctccttctcctgccgggctcatacacctacgagtggaacttcaggaaggatgttaacatggttctgcagagctccctaggaaatgacctaagggttgacggagccagcattaagtttgatagcatttgcctttacgccaccttcttccccatggcccacaacaccgcctccacgcttgaggccatgcttagaaacgacaccaacgaccagtcctttaacgactatctctccgccgccaacatgctctaccctatacccgccaacgctaccaacgtgcccatatccatcccctcccgcaactgggcggctttccgcggctgggccttcacgcgccttaagactaaggaaaccccatcactgggctcgggctacgacccttattacacctactctggctctataccctacctagatggaaccttttacctcaaccacacctttaagaaggtggccattacctttgactcttctgtcagctggcctggcaatgaccgcctgcttacccccaacgagtttgaaattaagcgctcagttgacggggagggttacaacgttgcccagtgtaacatgaccaaagactggttcctggtacaaatgctagctaactataacattggctaccagggcttctatatcccagagagctacaaggaccgcatgtactccttctttagaaacttccagcccatgagccgtcaggtggtggatgatactaaatacaaggactaccaacaggtgggcatcctacaccaacacaacaactctggatttgttggctaccttgcccccaccatgcgcgaaggacaggcctaccctgctaacttcccctatccgcttataggcaagaccgcagttgacagcattacccagaaaaagtttctttgcgatcgcaccctttggcgcatcccattctccagtaactttatgtccatgggcgcactcacagacctgggccaaaaccttctctacgccaactccgcccacgcgctagacatgacttttgaggtggatcccatggacgagcccacccttctttatgttttgtttgaagtctttgacgtggtccgtgtgcaccagccgcaccgcggcgtcatcgaaaccgtgtacctgcgcacgcccttctcggccggcaacgccacaacataaagaagcaagcaacatcaacaacagctgccgccatgggctccagtgagcaggaactgaaagccattgtcaaagatcttggttgtgggccatattttttgggcacctatgacaagcgctttccaggctttgtttctccacacaagctcgcctgcgccatagtcaatacggccggtcgcgagactgggggcgtacactggatggcctttgcctggaacccgcactcaaaaacatgctacctctttgagccctttggcttttctgaccagcgactcaagcaggtttaccagtttgagtacgagtcactcctgcgccgtagcgccattgcttcttcccccgaccgctgtataacgctggaaaagtccacccaaagcgtacaggggcccaactcggccgcctgtggactattctgctgcatgtttctccacgcctttgccaactggccccaaactcccatggatcacaaccccaccatgaaccttattaccggggtacccaactccatgctcaacagtccccaggtacagcccaccctgcgtcgcaaccaggaacagctctacagcttcctggagcgccactcgccctacttccgcagccacagtgcgcagattaggagcgccacttctttttgtcacttgaaaaacatgtaaaaataatgtactagagacactttcaataaaggcaaatgcttttatttgtacactctcgggtgattatttacccccacccttgccgtctgcgccgtttaaaaatcaaaggggttctgccgcgcatcgctatgcgccactggcagggacacgttgcgatactggtgtttagtgctccacttaaactcaggcacaaccatccgcggcagctcggtgaagttttcactccacaggctgcgcaccatcaccaacgcgtttagcaggtcgggcgccgatatcttgaagtcgcagttggggcctccgccctgcgcgcgcgagttgcgatacacagggttgcagcactggaacactatcagcgccgggtggtgcacgctggccagcacgctcttgtcggagatcagatccgcgtccaggtcctccgcgttgctcagggcgaacggagtcaactttggtagctgccttcccaaaaagggcgcgtgcccaggctttgagttgcactcgcaccgtagtggcatcaaaaggtgaccgtgcccggtctgggcgttaggatacagcgcctgcataaaagccttgatctgcttaaaagccacctgagcctttgcgccttcagagaagaacatgccgcaagacttgccggaaaactgattggccggacaggccgcgtcgtgcacgcagcaccttgcgtcggtgttggagatctgcaccacatttcggccccaccggttcttcacgatcttggccttgctagactgctccttcagcgcgcgctgcccgttttcgctcgtcacatccatttcaatcacgtgctccttatttatcataatgcttccgtgtagacacttaagctcgccttcgatctcagcgcagcggtgcagccacaacgcgcagcccgtgggctcgtgatgcttgtaggtcacctctgcaaacgactgcaggtacgcctgcaggaatcgccccatcatcgtcacaaaggtcttgttgctggtgaaggtcagctgcaacccgcggtgctcctcgttcagccaggtcttgcatacggccgccagagcttccacttggtcaggcagtagtttgaagttcgcctttagatcgttatccacgtggtacttgtccatcagcgcgcgcgcagcctccatgcccttctcccacgcagacacgatcggcacactcagcgggttcatcaccgtaatttcactttccgcttcgctgggctcttcctcttcctcttgcgtccgcataccacgcgccactgggtcgtcttcattcagccgccgcactgtgcgcttacctcctttgccatgcttgattagcaccggtgggttgctgaaacccaccatttgtagcgccacatcttctctttcttcctcgctgtccacgattacctctggtgatggcgggcgctcgggcttgggagaagggcgcttctttttcttcttgggcgcaatggccaaatccgccgccgaggtcgatggccgcgggctgggtgtgcgcggcaccagcgcgtcttgtgatgagtcttcctcgtcctcggactcgatacgccgcctcatccgcttttttgggggcgcccggggaggcggcggcgacggggacggggacgacacgtcctccatggttgggggacgtcgcgccgcaccgcgtccgcgctcgggggtggtttcgcgctgctcctcttcccgactggccatttccttctcctataggcagaaaaagatcatggagtcagtcgagaagaaggacagcctaaccgccccctctgagttcgccaccaccgcctccaccgatgccgccaacgcgcctaccaccttccccgtcgaggcacccccgcttgaggaggaggaagtgattatcgagcaggacccaggttttgtaagcgaagacgacgaggaccgctcagtaccaacagaggataaaaagcaagaccaggacaacgcagaggcaaacgaggaacaagtcgggcggggggacgaaaggcatggcgactacctagatgtgggagacgacgtgctgttgaagcatctgcagcgccagtgcgccattatctgcgacgcgttgcaagagcgcagcgatgtgcccctcgccatagcggatgtcagccttgcctacgaacgccacctattctcaccgcgcgtaccccccaaacgccaagaaaacggcacatgcgagcccaacccgcgcctcaacttctaccccgtatttgccgtgccagaggtgcttgccacctatcacatctttttccaaaactgcaagatacccctatcctgccgtgccaaccgcagccgagcggacaagcagctggccttgcggcagggcgctgtcatacctgatatcgcctcgctcaacgaagtgccaaaaatctttgagggtcttggacgcgacgagaagcgcgcggcaaacgctctgcaacaggaaaacagcgaaaatgaaagtcactctggagtgttggtggaactcgagggtgacaacgcgcgcctagccgtactaaaacgcagcatcgaggtcacccactttgcctacccggcacttaacctaccccccaaggtcatgagcacagtcatgagtgagctgatcgtgcgccgtgcgcagcccctggagagggatgcaaatttgcaagaacaaacagaggagggcctacccgcagttggcgacgagcagctagcgcgctggcttcaaacgcgcgagcctgccgacttggaggagcgacgcaaactaatgatggccgcagtgctcgttaccgtggagcttgagtgcatgcagcggttctttgctgacccggagatgcagcgcaagctagaggaaacattgcactacacctttcgacagggctacgtacgccaggcctgcaagatctccaacgtggagctctgcaacctggtctcctaccttggaattttgcacgaaaaccgccttgggcaaaacgtgcttcattccacgctcaagggcgaggcgcgccgcgactacgtccgcgactgcgtttacttatttctatgctacacctggcagacggccatgggcgtttggcagcagtgcttggaggagtgcaacctcaaggagctgcagaaactgctaaagcaaaacttgaaggacctatggacggccttcaacgagcgctccgtggccgcgcacctggcggacatcattttccccgaacgcctgcttaaaaccctgcaacagggtctgccagacttcaccagtcaaagcatgttgcagaactttaggaactttatcctagagcgctcaggaatcttgcccgccacctgctgtgcacttcctagcgactttgtgcccattaagtaccgcgaatgccctccgccgctttggggccactgctaccttctgcagctagccaactaccttgcctaccactctgacataatggaagacgtgagcggtgacggtctactggagtgtcactgtcgctgcaacctatgcaccccgcaccgctccctggtttgcaattcgcagctgcttaacgaaagtcaaattatcggtacctttgagctgcagggtccctcgcctgacgaaaagtccgcggctccggggttgaaactcactccggggctgtggacgtcggcttaccttcgcaaatttgtacctgaggactaccacgcccacgagattaggttctacgaagaccaatcccgcccgcctaatgcggagcttaccgcctgcgtcattacccagggccacattcttggccaattgcaagccatcaacaaagcccgccaagagtttctgctacgaaagggacggggggtttacttggacccccagtccggcgaggagctcaacccaatccccccgccgccgcagccctatcagcagcagccgcgggcccttgcttcccaggatggcacccaaaaagaagctgcagctgccgccgccacccacggacgaggaggaatactgggacagtcaggcagaggaggttttggacgaggaggaggaggacatgatggaagactgggagagcctagacgaggaagcttccgaggtcgaagaggtgtcagacgaaacaccgtcaccctcggtcgcattcccctcgccggcgccccagaaatcggcaaccggttccagcatggctacaacctccgctcctcaggcgccgccggcactgcccgttcgccgacccaaccgtagatgggacaccactggaaccagggccggtaagtccaagcagccgccgccgttagcccaagagcaacaacagcgccaaggctaccgctcatggcgcgggcacaagaacgccatagttgcttgcttgcaagactgtgggggcaacatctccttcgcccgccgctttcttctctaccatcacggcgtggccttcccccgtaacatcctgcattactaccgtcatctctacagcccatactgcaccggcggcagcggcagcaacagcagcggccacacagaagcaaaggcgaccggatagcaagactctgacaaagcccaagaaatccacagcggcggcagcagcaggaggaggagcgctgcgtctggcgcccaacgaacccgtatcgacccgcgagcttagaaacaggatttttcccactctgtatgctatatttcaacagagcaggggccaagaacaagagctgaaaataaaaaacaggtctctgcgatccctcacccgcagctgcctgtatcacaaaagcgaagatcagcttcggcgcacgctggaagacgcggaggctctcttcagtaaatactgcgcgctgactcttaaggactagtttcgcgccctttctcaaatttaagcgcgaaaactacgtcatctccagcggccacacccggcgccagcacctgttgtcagcgccattatgagcaaggaaattcccacgccctacatgtggagttaccagccacaaatgggacttgcggctggagctgcccaagactactcaacccgaataaactacatgagcgcgggaccccacatgatatcccgggtcaacggaatacgcgcccaccgaaaccgaattctcctggaacaggcggctattaccaccacacctcgtaataaccttaatccccgtagttggcccgctgccctggtgtaccaggaaagtcccgctcccaccactgtggtacttcccagagacgcccaggccgaagttcagatgactaactcaggggcgcagcttgcgggcggctttcgtcacagggtgcggtcgcccgggcagggtataactcacctgacaatcagagggcgaggtattcagctcaacgacgagtcggtgagctcctcgcttggtctccgtccggacgggacatttcagatcggcggcgccggccgctcttcattcacgcctcgtcaggcaatcctaactctgcagacctcgtcctctgagccgcgctctggaggcattggaactctgcaatttattgaggagtttgtgccatcggtctactttaaccccttctcgggacctcccggccactatccggatcaatttattcctaactttgacgcggtaaaggactcggcggacggctacgactgaatgttaagtggagaggcagagcaactgcgcctgaaacacctggtccactgtcgccgccacaagtgctttgcccgcgactccggtgagttttgctactttgaattgcccgaggatcatatcgagggcccggcgcacggcgtccggcttaccgcccagggagagcttgcccgtagcctgattcgggagtttacccagcgccccctgctagttgagcgggacaggggaccctgtgttctcactgtgatttgcaactgtcctaaccctggattacatcaagatcctctagttaatgtcaggtcgcctaagtcgattaactagagtacccggggatcttattccctttaactaataaaaaaaaataataaagcatcacttacttaaaatcagttagcaaatttctgtccagtttattcagcagcacctccttgccctcctcccagctctggtattgcagcttcctcctggctgcaaactttctccacaatctaaatggaatgtcagtttcctcctgttcctgtccatccgcacccactatcttcatgttgttgcagatgaagcgcgcaagaccgtctgaagataccttcaaccccgtgtatccatatgacacggaaaccggtcctccaactgtgccttttcttactcctccctttgtatcccccaatgggtttcaagagagtccccctggggtactctctttgcgcctatccgaacctctagttacctccaatggcatgcttgcgctcaaaatgggcaacggcctctctctggacgaggccggcaaccttacctcccaaaatgtaaccactgtgagcccacctctcaaaaaaaccaagtcaaacataaacctggaaatatctgcacccctcacagttacctcagaagccctaactgtggctgccgccgcacctctaatggtcgcgggcaacacactcaccatgcaatcacaggccccgctaaccgtgcacgactccaaacttagcattgccacccaaggacccctcacagtgtcagaaggaaagctagccctgcaaacatcaggccccctcaccaccaccgatagcagtacccttactatcactgcctcaccccctctaactactgccactggtagcttgggcattgacttgaaagagcccatttatacacaaaatggaaaactaggactaaagtacggggctcctttgcatgtaacagacgacctaaacactttgaccgtagcaactggtccaggtgtgactattaataatacttccttgcaaactaaagttactggagccttgggttttgattcacaaggcaatatgcaacttaatgtagcaggaggactaaggattgattctcaaaacagacgccttatacttgatgttagttatccgtttgatgctcaaaaccaactaaatctaagactaggacagggccctctttttataaactcagcccacaacttggatattaactacaacaaaggcctttacttgtttacagcttcaaacaattccaaaaagcttgaggttaacctaagcactgccaaggggttgatgtttgacgctacagccatagccattaatgcaggagatgggcttgaatttggttcacctaatgcaccaaacacaaatcccctcaaaacaaaaattggccatggcctagaatttgattcaaacaaggctatggttcctaaactaggaactggccttagttttgacagcacaggtgccattacagtaggaaacaaaaataatgataagctaactttgtggaccacaccagctccatctcctaactgtagactaaatgcagagaaagatgctaaactcactttggtcttaacaaaatgtggcagtcaaatacttgctacagtttcagttttggctgttaaaggcagtttggctccaatatctggaacagttcaaagtgctcatcttattataagatttgacgaaaatggagtgctactaaacaattccttcctggacccagaatattggaactttagaaatggagatcttactgaaggcacagcctatacaaacgctgttggatttatgcctaacctatcagcttatccaaaatctcacggtaaaactgccaaaagtaacattgtcagtcaagtttacttaaacggagacaaaactaaacctgtaacactaaccattacactaaacggtacacaggaaacaggagacacaactccaagtgcatactctatgtcattttcatgggactggtctggccacaactacattaatgaaatatttgccacatcctcttacactttttcatacattgcccaagaataaagaatcgtttgtgttatgtttcaacgtgtttatttttcaattgcagaaaatttcaagtcatttttcattcagtagtatagccccaccaccacatagcttatacagatcaccgtaccttaatcaaactcacagaaccctagtattcaacctgccacctccctcccaacacacagagtacacagtcctttctccccggctggccttaaaaagcatcatatcatgggtaacagacatattcttaggtgttatattccacacggtttcctgtcgagccaaacgctcatcagtgatattaataaactccccgggcagctcacttaagttcatgtcgctgtccagctgctgagccacaggctgctgtccaacttgcggttgcttaacgggcggcgaaggagaagtccacgcctacatgggggtagagtcataatcgtgcatcaggatagggcggtggtgctgcagcagcgcgcgaataaactgctgccgccgccgctccgtcctgcaggaatacaacatggcagtggtctcctcagcgatgattcgcaccgcccgcagcataaggcgccttgtcctccgggcacagcagcgcaccctgatctcacttaaatcagcacagtaactgcagcacagcaccacaatattgttcaaaatcccacagtgcaaggcgctgtatccaaagctcatggcggggaccacagaacccacgtggccatcataccacaagcgcaggtagattaagtggcgacccctcataaacacgctggacataaacattacctcttttggcatgttgtaattcaccacctcccggtaccatataaacctctgattaaacatggcgccatccaccaccatcctaaaccagctggccaaaacctgcccgccggctatacactgcagggaaccgggactggaacaatgacagtggagagcccaggactcgtaaccatggatcatcatgctcgtcatgatatcaatgttggcacaacacaggcacacgtgcatacacttcctcaggattacaagctcctcccgcgttagaaccatatcccagggaacaacccattcctgaatcagcgtaaatcccacactgcagggaagacctcgcacgtaactcacgttgtgcattgtcaaagtgttacattcgggcagcagcggatgatcctccagtatggtagcgcgggtttctgtctcaaaaggaggtagacgatccctactgtacggagtgcgccgagacaaccgagatcgtgttggtcgtagtgtcatgccaaatggaacgccggacgtagtcatatttcctgaagcaaaaccaggtgcgggcgtgacaaacagatctgcgtctccggtctcgccgcttagatcgctctgtgtagtagttgtagtatatccactctctcaaagcatccaggcgccccctggcttcgggttctatgtaaactccttcatgcgccgctgccctgataacatccaccaccgcagaataagccacacccagccaacctacacattcgttctgcgagtcacacacgggaggagcgggaagagctggaagaaccatgtttttttttttattccaaaagattatccaaaacctcaaaatgaagatctattaagtgaacgcgctcccctccggtggcgtggtcaaactctacagccaaagaacagataatggcatttgtaagatgttgcacaatggcttccaaaaggcaaacggccctcacgtccaagtggacgtaaaggctaaacccttcagggtgaatctcctctataaacattccagcaccttcaaccatgcccaaataattctcatctcgccaccttctcaatatatctctaagcaaatcccgaatattaagtccggccattgtaaaaatctgctccagagcgccctccaccttcagcctcaagcagcgaatcatgattgcaaaaattcaggttcctcacagacctgtataagattcaaaagcggaacattaacaaaaataccgcgatcccgtaggtcccttcgcagggccagctgaacataatcgtgcaggtctgcacggaccagcgcggccacttccccgccaggaaccatgacaaaagaacccacactgattatgacacgcatactcggagctatgctaaccagcgtagccccgatgtaagcttgttgcatgggcggcgatataaaatgcaaggtgctgctcaaaaaatcaggcaaagcctcgcgcaaaaaagaaagcacatcgtagtcatgctcatgcagataaaggcaggtaagctccggaaccaccacagaaaaagacaccatttttctctcaaacatgtctgcgggtttctgcataaacacaaaataaaataacaaaaaaacatttaaacattagaagcctgtcttacaacaggaaaaacaacccttataagcataagacggactacggccatgccggcgtgaccgtaaaaaaactggtcaccgtgattaaaaagcaccaccgacagctcctcggtcatgtccggagtcataatgtaagactcggtaaacacatcaggttgattcacatcggtcagtgctaaaaagcgaccgaaatagcccgggggaatacatacccgcaggcgtagagacaacattacagcccccataggaggtataacaaaattaataggagagaaaaacacataaacacctgaaaaaccctcctgcctaggcaaaatagcaccctcccgctccagaacaacatacagcgcttccacagcggcagccataacagtcagccttaccagtaaaaaagaaaacctattaaaaaaacaccactcgacacggcaccagctcaatcagtcacagtgtaaaaaagggccaagtgcagagcgagtatatataggactaaaaaatgacgtaacggttaaagtccacaaaaaacacccagaaaaccgcacgcgaacctacgcccagaaacgaaagccaaaaaacccacaacttcctcaaatcgtcacttccgttttcccacgttacgtcacttcccattttaagaaaactacaattcccaacacatacaagttactccgccctaaaacctacgtcacccgccccgttcccacgccccgcgccacgtcacaaactccaccccctcattatcatattggcttcaatccaaaataaggta

SEQ ID NO: 221 - DNA, 9701 bp, synthetic construct
  misc_feature 1..9701: note = vector for IgG1 against T27Y H34A R273K ACE2 mutant
  misc_feature 2929..2930: note = n is a, c, g, or t
  misc_feature 2934: note = n is a, c, g, or t
  source 1..9701: mol_type = other DNA
ggcgtaatctgctgcttgcaaacaaaaaaaccaccgctaccagcggtggtttgtttgccggatcaagagctaccaactctttttccgaaggtaactggcttcagcagagcgcagataccaaatactgtccttctagtgtagccgtagttaggccaccacttcaagaactctgtagcaccgcctacatacctcgctctgctgaagccagttaccagtggctgctgccagtggcgataagtcgtgtcttaccgggttggactcaagagatagttaccggataaggcgcagcggtcgggctgaacggggggttcgtgcacacagcccagcttggagcgaacgacctacaccgaactgagatacctacagcgtgagctatgagaaagcgccacgcttcccgaagggagaaaggcggacaggtatccggtaagcggcagggtcggaacaggagagcgcacgagggagcttccagggggaaacgcctggtatctttatagtcctgtcgggtttcgccacctctgacttgagcgtcgatttttgtgatgctcgtcaggggggcggagcctatggaaaaacgccagcaacgcaagctagagtttaaacttgacagatgagacaataaccctgataaatgcttcaataatattgaaaaaggaaaagtatgagtattcaacatttccgtgtcgcccttattcccttttttgcggcattttgccttcctgtttttgctcacccagaaacgctggtgaaagtaaaagatgcagaagatcacttgggtgcgcgagtgggttacatcgaactggatctcaacagcggtaagatccttgagagttttcgccccgaagaacgtttcccaatgatgagcacttttaaagttctgctatgtggcgcggtattatcccgtattgatgccgggcaagagcaactcggtcgccgcatacactattctcagaatgacttggttgaatactcaccagtcacagaaaagcatcttacggatggcatgacagtaagagaattatgcagtgctgccataaccatgagtgataacactgcggccaacttacttctgacaactatcggaggaccgaaggagctaaccgcttttttgcacaacatgggggatcatgtaactcgccttgatcgttgggaaccggagctgaatgaagccataccaaacgacgagcgtgacaccacgatgcctgtagcaatggcaacaacgttgcgaaaactattaactggcgaactacttactctagcttcccggcaacaactaatagactggatggaggcggataaagttgcaggaccacttctgcgctcggcacttccggctggctggtttattgctgataaatcaggagccggtgagcgtgggtcacgcggtatcattgcagcactggggccggatggtaagccctcccgtatcgtagttatctacactacggggagtcaggcaactatggatgaacgaaatagacagatcgctgagataggtgcctcactgattaagcattggtaaggataaatttctggtaaggaggacacgtatggaagtgggcaagttggggaagccgtatccgttgctgaatctggcatatgtgggagtataagacgcgcagcgtcgcatcaggcatttttttctgcgccaatgcaaaaaggccatccgtcaggatggcctttcggcataactagggccgccgatatttgaaaatatggcatattgaaaatgtcgccgatgtgagtttctgtgtaactgatatcgccatttttccaaaagtgatttttgggcatacgcgatatctggcgatagcgcttatatcgtttacgggggatggcgatagacgactttggtgacttgggcgattctgtgtgtcgcaaatatcgcagtttcgatataggtgacagacgatatgaggctatatcgccgatagaggcgacatcaagctggcacatggccaatgcatatcgatctatacattgaatcaatattggccattagccatattattcattggttatatagcataaatcaatattggctattggccattgcatacgttgtatccatatcataatatgtacatttatattggctcatgtccaacattaccgccatgttgacattgattattgactagttattaatagtaatcaattacggggtcattagttcatagcccatatatggagttccgcgttacataacttacggtaaatggcccgcctggctgaccgcccaacgacccccgcccattgacgtcaataatgacgtatgttcccatagtaacgccaatagggactttccattgacgtcaatgggtggagtatttacggtaaactgcccacttggcagtacatcaagtgtatcatatgccaagtacgccccctattgacgtcaatgacggtaaatggcccgcctggcattatgcccagtacatgaccttatgggactttcctacttggcagtacatctacgtattagtcatcgctattaccatggtgatgcggttttggcagtacatcaatgggcgtggatagcggtttgactcacggggatttccaagtctccaccccattgacgtcaatgggagtttgttttggcaccaaaatcaacgggactttccaaaatgtcgtaacaactccgccccattgacgcaaatgggcggtaggcgtgtacggtgggaggtctatataagcagagctcgtttagtgaaccgtcagatcgcctggagacgccatccacgctgttttgacctccatagaagacaccgggaccgatccagcctccgcggccgggaacggtgcattggaacgcggattccccgtgccaagagtgacgtaagtaccgcctatagagtctataggcccacccccttggcttcttatgcatgctatactgtttttggcttggggtctatacaccccccgnnttcntcatgttataggtgatggtatagcttagcctataggtgtgggttattgaccattattgaccactccccctattggtgacgatactttccattactaatccataacatggctctttgccacaactctctttattggctatatgccaatacactgtccttcagagactgacacggactctgtatttttacaggatggggtctcatttattatttacaaattcacatatacaacaccaccgtccccagtgcccgcagtttttattaaacataacgtgggatctccacgcgaatctcgggtacgtgttccggacatgggctcttctccggtagcggcggagcttctacatccgagccctgctcccatgcctccagcgactcatggtcgctcggcagctccttgctcctaacagtggaggccagacttaggcacagcacgatgcccaccaccaccagtgtgccgcacaaggccgtggcggtagggtatgtgtctgaaaatgagctcggggagcgggcttgcaccgctgacgcatttggaagacttaaggcagcggcagaagaagatgcaggcagctgagttgttgtgttctgataagagtcagaggtaactcccgttgcggtgctgttaacggtggagggcagtgtagtctgagcagtactcgttgctgccgcgcgcgccaccagacataatagctgacagactaacagactgttcctttccatgggtcttttctgcagtcaccgtccttgacacgaagctgctagcgccaccatgagcagcagtagttggcttctcttgagtttggtggcagtgacagcagcccagagtactatcgaggagcaggctaaatactttctggataagtttaacgccgaggccgaagacttgttctatcaatcttctctcgcttcatggaattacaatactaacatcactgaggagaacgtccagaatatgaacaatgctggcgacaaatggagcgccttcttgaaggagcagtctacccttgcacaaatgtatccactgcaggagatacagaaccttacagtaaagttgcagctccaggctctccagcagaacggatctagcgtgctttcagaggataaaagcaaaaggctgaacaccatacttaataccatgtccacaatttactctactggtaaagtatgtaaccccgacaaccctcaagaatgcctccttcttgagccaggcctcaatgagatcatggctaatagtctggactataatgaaagactgtgggcatgggagtcctggagatctgaagtagggaagcaactgaggcccctttatgaagagtacgtcgtacttaagaatgaaatggcccgcgctaaccactacgaggattacggcgattactggcgtggggactatgaagtaaatggtgtagatggatacgactatagtcgtgggcaattgattgaggatgtggagcacacttttgaggagataaaaccactctatgagcatcttcacgcatatgtgagagctaaactgatgaacgcctacccaagttacatcagtccaatcggatgtctcccagctcacctccttggcgacatgtggggaaagttctggaccaatctgtattccctcacagtccctttcgggcaaaagcctaatatagacgtgacagacgcaatggttgatcaggcttgggatgctcaaaggatttttaaggaagctgagaagttttttgtgtcagtcggtttgccaaatatgacacaaggcttctgggaaaatagcatgttgactgatcccggtaatgttcaaaaggctgtgtgtcaccctaccgcttgggaccttgggaaaggtgactttcgaatcttgatgtgtaccaaggtgacaatggatgactttcttacagcccatcatgaaatgggtcacatccagtatgatatggcttatgcagctcaacctttcctcttgagaaatggtgcaaatgaaggttttcatgaagctgtaggggaaataatgtccctgagtgctgcaaccccaaagcatctcaagagtatcggattgttgagcccagattttcaagaagataacgagaccgaaatcaacttccttctgaaacaagccctcacaatagttggtactcttccattcacatacatgctggagaaatggcgttggatggtttttaagggggagatacctaaagatcagtggatgaaaaagtggtgggagatgaagcgtgagatcgtaggggtcgtggagccagtgcctcatgatgagacttactgtgacccagcatcactcttccacgttagcaatgactattcatttatacgttattacactcgcactctttaccagtttcaatttcaggaggctctgtgtcaggctgccaagcatgagggaccccttcacaagtgtgatattagtaacagtactgaggcaggccaaaaactgttcaatatgttgaggcttggcaaaagcgagccatggactctcgccttggaaaatgttgtcggggctaaaaacatgaatgtacgccctctgcttaactattttgagcccctttttacatggctcaaggaccagaataagaactcctttgtcggctggtcaacagactggtctccctatgcagacaaaacacatacttgcccaccttgtcctgcaccagagctgctgggaggtccaagcgtgttcctgtttccacccaagcccaaagacacactgatgatttctcgaactccagaagtgacctgcgtggtcgtggacgtgagccacgaggatcccgaagtgaagttcaactggtacgtggatggcgtggaggtccataatgctaagactaaaccccgggaggaacagtacaacagcacttatagggtcgtgtccgtgctgaccgtcctgcatcaggattggctgaacgggaaggaatataagtgcaaagtgtctaataaggcactgcccgcccctatcgagaaaacaattagcaaggctaagggtcagcctagagaaccacaggtgtacactctgcctccaagtcgcgacgagctgaccaagaaccaggtgtcactgacatgtctggtcaaaggcttttatccctcagatatcgcagtggagtgggaaagcaatggacagcctgagaacaattacaagaccacaccccctgtgctggacagtgatggctcattctttctgtattctaagctgacagtggacaaaagtaggtggcagcagggaaacgtgttctcctgctctgtcatgcacgaagcactgcacaatcattatacccagaagagtctgtcactgagccctggcaaatgagcgataccgattctagaactagatcataatcagccataccacatttgtagaggttttacttgctttaaaaaacctcccacacctccccctgaacctgaaacataaaatgaatgcaattgttgttgttaacttgtttattgcagcttataatggttacaaataaagcaatagcatcacaaatttcacaaataaagcatttttttcactgcattctagttgtggtttgtccaaactcatcaatgtatcttaaggccgcaggtaagccagcccaggcctcgccctccagctcaaggcgggacaggtgccctagagtagcctgcatccagggacaggccccagccgggtgctgacacgtccacctccatctcttcctcaggtctgcccgggtggcatccctgtgacccctccccagtgcctctcctggtcgtggaaggtgctactccagtgcccaccagccttgtcctaataaaattaagttgcatcattttgtttgactaggtgtccttgtataatattatggggtggaggcgggtggtatggagcaaggggcccaagttaacttgtttattgcagcttataatggttacaaataaagcaatagcatcacaaatttcacaaataaagcatttttttcactgcattctagttgtggtttgtccaaactcatcaatgtatcttatcatgtctggatccgcttcaggcaccgggcttgcgggtcatgcaccaggtgcgcggtccttcgggcacctcgacgtcggcggtgacggtgaagccgagccgctcgtagaaggggaggttgcggggcgcggaggtctccaggaaggcgggcaccccggcgcgctcggccgcctccactccggggagcacgacggcgctgcccagacccttgccctggtggtcgggcgagacgccgacggtggccaggaaccacgcgggctccttgggccggtgcggcgccaggaggccttccatctgttgctgcgcggccagcctggaaccgctcaactcggccatgcgcgggccgatctcggcgaacaccgcccccgcttcgacgctctccggcgtggtccagaccgccaccgcggcgccgtcgtccgcgacccacaccttgccgatgtcgagcccgacgcgcgtgaggaagagttcttgcagctcggtgacccgctcgatgtggcggtccgggtcgacggtgtggcgcgtggcggggtagtcggcgaacgcggcggcgagggtgcgtacggcccgggggacgtcgtcgcgggtggcgaggcgcaccgtgggcttgtactcggtcatggtggcctgcagagtcgctctgtgttcgaggccacacgcgtcaccttaatatgcgaagtggacctgggaccgcgccgccccgactgcatctgcgtgttttcgccaatgacaagacgctgggcggggtttgtgtcatcatagaactaaagacatgcaaatatatttcttccggggacaccgccagcaaacgcgagcaacgggccacggggatgaagcagctgcgccactccctgaagatccatcgtctcctaacaagttacatcactcctgcccttcctcaccctcatctccatcacctccttcatctccgtcatctccgtcatcaccctccgcggcagccccttccaccataggtggaaaccagggaggcaaatctactccatcgtcaaagctgcacacagtcaccctgatattgcaggtaggagcgggctttgtcataacaaggtccttaatcgcatccttcaaaacctcagcaaatatatgagtttgtaaaaagaccatgaaataacagacaatggactcccttagcgggccaggttgtgggccgggtccaggggccattccaaaggggagacgactcaatggtgtaagacgacattgtggaatagcaagggcagttcctcgccttaggttgtaaagggaggtcttactacctccatatacgaacacaccggcgacccaagttccttcgtcggtagtcctttctacgtgactcctagccaggagagctcttaaaccttctgcaatgttctcaaatttcgggttggaacctccttgaccacgatgctttccaaaccaccctccttttttgcgcctgcctccatcaccctgacccccgctgcgcgggggcacgtcaggctcaccatctgggccgccttcttggtggtattcaaaataatcggcttcccctacagggtggaaaaatggccttctacctggagggggcctgcgcggtggagacccggatgatgatgactgactactgggactcctgggcctcttttctccacgtccacgacctctccccctggctctttcacgacttccccccctggctctttcacgtcctctaccccggcggcctccactacctcctcgaccccggcctccactacctcctcgaccccggcctccactgcctcctcgaccccggcctccacctcctgctcctgcccctcccgctcctgctcctgctcctgttccaccgtgggtccctttgcagccaatgcaacttggacgtttttggggtctccggacaccatctctatgtcttggccctgatcctgagccgcccggggctcctggtcttccgcctcctcgtcctcgtcctcttccccgtcctcgtccatgtgccatgatggcggcctgcagctgtgttcgaggccgcgcgtgtcaccttaatatgcgaagtggacctgggaccgcgccgccccgactgcatctgcgtgttcgagttcgccaatgacaagacgctgggcggggagatcccccttattaaccctaaacgggtagcatatgcttcccgggtagtagtatatactatccagactaaccctaattcaatagcatatgttacccaacgggaagcatatgctatcgaattagggttagtaaaagggtcctaaggaacagcgatctggatagcatatgctatcctaatctatatctgggtagcatatgctatcctaatctatatctgggtagcataggctatcctaatctatatctgggtagcatatgctatcctaatctatatctgggtagtatatgctatcctaatttatatctgggtagcataggctatcctaatctatatctgggtagcatatgctatcctaatctatatctgggtagtatatgctatcctaatctgtatccgggtagcatatgctatcctcatgcatatacagtcagcatatgatacccagtagtagagtgggagtgctatcctttgcatatgccgccacctcccaaggagatctgtcgacatcgatgggcgcgggtgtacactccgcccatcccgcccctaactccgcccagttccgcccattctccgcctcatggctgactaattttttttatttatgcagaggccgaggccgcctcggcctctgagctattccagaagtagtgaggaggcttttttggaggcctaggcttttgcaaaaagctaattc

SEQ ID NO: 222 - DNA, 38496 bp, synthetic construct
  misc_feature 1..38496: note = vector for IgA against T27Y H34A R273L ACE2 mutant
  source 1..38496: mol_type = other DNA
tattattgatgatgttaattaacatgcatggatcctacgtctcgaccgatgcccttgagagccttcaacccagtcagctccttccggtgggcgcggggcatgactatcgtcgccgcacttatgactgtcttctttatcatgcaactcgtaggacaggtgccggcagcgctctgggtcattttcggcgaggaccgctttcgctggagcgcgacgatgatcggcctgtcgcttgcggtattcggaatcttgcacgccctcgctcaagccttcgtcactggtcccgccaccaaacgtttcggcgagaagcaggccattatcgccggcatggcggccgacgcgctgggctacgtcttgctggcgttcgcgacgcgaggctggatggccttccccattatgattcttctcgcttccggcggcatcgggatgcccgcgttgcaggccatgctgtccaggcaggtagatgacgaccatcagggacagcttcaaggatcgctcgcggctcttaccagcctaacttcgatcattggaccgctgatcgtcacggcgatttatgccgcctcggcgagcacatggaacgggttggcatggattgtaggcgccgccctataccttgtctgcctccccgcgttgcgtcgcggtgcatggagccgggccacctcgacctgaatggaagccggcggcacctcgctaacggattcaccactccaagaattggagccaatcaattcttgcggagaactgtgaatgcgcaaaccaacccttggcagaacatatccatcgcgtccgccatctccagcagccgcacgcggcgcatctcgggcagcgttgggtcctggccacgggtgcgcatgatcgtgctcctgtcgttgaggacccggctaggctggcggggttgccttactggttagcagaatgaatcaccgatacgcgagcgaacgtgaagcgactgctgctgcaaaacgtctgcgacctgagcaacaacatgaatggtcttcggtttccgtgtttcgtaaagtctggaaacgcggaagtcagcgccctgcaccattatgttccggatctgcatcgcaggatgctgctggctaccctgtggaacacctacatctgtattaacgaagcgctggcattgaccctgagtgatttttctctggtcccgccgcatccataccgccagttgtttaccctcacaacgttccagtaaccgggcatgttcatcatcagtaacccgtatcgtgagcatcctctctcgtttcatcggtatcattacccccatgaacagaaatcccccttacacggaggcatcagtgaccaaacaggaaaaaaccgcccttaacatggcccgctttatcagaagccagacattaacgcttctggagaaactcaacgagctggacgcggatgaacaggcagacatctgtgaatcgcttcacgaccacgctgatgagctttaccgcagctgcctcgcgcgtttcggtgatgacggtgaaaacctctgacacatgcagctcccggagacggtcacagcttgtctgtaagcggatgccgggagcagacaagcccgtcagggcgcgtcagcgggtgttggcgggtgtcggggcgcagccatgacccagtcacgtagcgatagcggagtgtatactggcttaactatgcggcatcagagcagattgtactgagagtgcaccatatgcggtgtgaaataccgcacagatgcgtaaggagaaaataccgcatcaggcgctcttccgcttcctcgctcactgactcgctgcgctcggtcgttcggctgcggcgagcggtatcagctcactcaaaggcggtaatacggttatccacagaatcaggggataacgcaggaaagaacatgtgagcaaaaggccagcaaaaggccaggaaccgtaaaaaggccgcgttgctggcgtttttccataggctccgcccccctgacgagcatcacaaaaatcgacgctcaagtcagaggtggcgaaacccgacaggactataaagataccaggcgtttccccctggaagctccctcgtgcgctctcctgttccgaccctgccgcttaccggatacctgtccgcctttctcccttcgggaagcgtggcgctttctcatagctcacgctgtaggtatctcagttcggtgtaggtcgttcgctccaagctgggctgtgtgcacgaaccccccgttcagcccgaccgctgcgccttatccggtaactatcgtcttgagtccaacccggtaagacacgacttatcgccactggcagcagccactggtaacaggattagcagagcgaggtatgtaggcggtgctacagagttcttgaagtggtggcctaactacggctacactagaaggacagtatttggtatctgcgctctgctgaagccagttaccttcggaaaaagagttggtagctcttgatccggcaaacaaaccaccgctggtagcggtggtttttttgtttgcaagcagcagattacgcgcagaaaaaaaggatctcaagaagatcctttgatcttttctacggggtctgacgctcagtggaacgaaaactcacgttaagggattttggtcatgagattatcaaaaaggatcttcacctagatccttttaaattaaaaatgaagttttaaatcaatctaaagtatatatgagtaaacttggtctgacagttaccaatgcttaatcagtgaggcacctatctcagcgatctgtctatttcgttcatccatagttgcctgactccccgtcgtgtagataactacgatacgggagggcttaccatctggccccagtgctgcaatgataccgcgagacccacgctcaccggctccagatttatcagcaataaaccagccagccggaagggccgagcgcagaagtggtcctgcaactttatccgcctccatccagtctattaattgttgccgggaagctagagtaagtagttcgccagttaatagtttgcgcaacgttgttgccattgctgcagccatgagattatcaaaaaggatcttcacctagatccttttcacgtagaaagccagtccgcagaaacggtgctgaccccggatgaatgtcagctactgggctatctggacaagggaaaacgcaagcgcaaagagaaagcaggtagcttgcagtgggcttacatggcgatagctagactgggcggttttatggacagcaagcgaaccggaattgccagctggggcgccctctggtaaggttgggaagccctgcaaagtaaactggatggctttcttgccgccaaggatctgatggcgcaggggatcaagctctgatcaagagacaggatgaggatcgtttcgcatgattgaacaagatggattgcacgcaggttctccggccgcttgggtggagaggctattcggctatgactgggcacaacagacaatcggctgctctgatgccgccgtgttccggctgtcagcgcaggggcgcccggttctttttgtcaagaccgacctgtccggtgccctgaatgaactgcaagacgaggcagcgcggctatcgtggctggccacgacgggcgttccttgcgcagctgtgctcgacgttgtcactgaagcgggaagggactggctgctattgggcgaagtgccggggcaggatctcctgtcatctcaccttgctcctgccgagaaagtatccatcatggctgatgcaatgcggcggctgcatacgcttgatccggctacctgcccattcgaccaccaagcgaaacatcgcatcgagcgagcacgtactcggatggaagccggtcttgtcgatcaggatgatctggacgaagagcatcaggggctcgcgccagccgaactgttcgccaggctcaaggcgagcatgcccgacggcgaggatctcgtcgtgacccatggcgatgcctgcttgccgaatatcatggtggaaaatggccgcttttctggattcatcgactgtggccggctgggtgtggcggaccgctatcaggacatagcgttggctacccgtgatattgctgaagagcttggcggcgaatgggctgaccgcttcctcgtgctttacggtatcgccgctcccgattcgcagcgcatcgccttctatcgccttcttgacgagttcttctgaattttgttaaaatttttgttaaatcagctcattttttaaccaataggccgaaatcggcaaaatcccttataaatcaaaagaatagaccgagatagggttgagtgttgttccagtttggaacaagagtccactattaaagaacgtggactccaacgtcaaagggcgaaaaaccgtctatcagggcgatggcccactacgtgaaccatcaccctaatcaagttttttggggtcgaggtgccgtaaagcactaaatcggaaccctaaagggagcccccgatttagagcttgacggggaaagccggcgaacgtggcgagaaaggaagggaagaaagcgaaaggagcgggcgctagggcgctggcaagtgtagcggtcacgctgcgcgtaaccaccacacccgccgcgcttaatgcgccgctacagggcgcgtccattcgccattcaggatcgaattaattcttaattaacatcatcaataatataccttattttggattgaagccaatatgataatgagggggtggagtttgtgacgtggcgcggggcgtgggaacggggcgggtgacgtagtagtgtggcggaagtgtgatgttgcaagtgtggcggaacacatgtaagcgacggatgtggcaaaagtgacgtttttggtgtgcgccggtgtacacaggaagtgacaattttcgcgcggttttaggcggatgttgtagtaaatttgggcgtaaccgagtaagatttggccattttcgcgggaaaactgaataagaggaagtgaaatctgaataattttgtgttactcatagcgcgtaatactgtaatagtaatcaattacggggtcattagttcatagcccatatatggagttccgcgttacataacttacggtaaatggcccgcctggctgaccgcccaacgacccccgcccattgacgtcaataatgacgtatgttcccatagtaacgccaatagggactttccattgacgtcaatgggtggagtatttacggtaaactgcccacttggcagtacatcaagtgtatcatatgccaagtacgccccctattgacgtcaatgacggtaaatggcccgcctggcattatgcccagtacatgaccttatgggactttcctacttggcagtacatctacgtattagtcatcgctattaccatggtgatgcggttttggcagtacatcaatgggcgtggatagcggtttgactcacggggatttccaagtctccaccccattgacgtcaatgggagtttgttttggcaccaaaatcaacgggactttccaaaatgtcgtaacaactccgccccattgacgcaaatgggcggtaggcgtgtacggtgggaggtctatataagcagagctggtttagtgaaccgtcagatccgctagagatctggtaccgtcgacgcggccgctcgagcctaagcttatgagcagcagtagttggcttctcttgagtttggtggcagtgacagcagcccagagtactatcgaggagcaggctaaatactttctggataagtttaacgccgaggccgaagacttgttctatcaatcttctctcgcttcatggaattacaatactaacatcactgaggagaacgtccagaatatgaacaatgctggcgacaaatggagcgccttcttgaaggagcagtctacccttgcacaaatgtatccactgcaggagatacagaaccttacagtaaagttgcagctccaggctctccagcagaacggatctagcgtgctttcagaggataaaagcaaaaggctgaacaccatacttaataccatgtccacaatttactctactggtaaagtatgtaaccccgacaaccctcaagaatgcctccttcttgagccaggcctcaatgagatcatggctaatagtctggactataatgaaagactgtgggcatgggagtcctggagatctgaagtagggaagcaactgaggcccctttatgaagagtacgtcgtacttaagaatgaaatggcccgcgctaaccactacgaggattacggcgattactggcgtggggactatgaagtaaatggtgtagatggatacgactatagtcgtgggcaattgattgaggatgtggagcacacttttgaggagataaaaccactctatgagcatcttcacgcatatgtgagagctaaactgatgaacgcctacccaagttacatcagtccaatcggatgtctcccagctcacctccttggcgacatgtggggactgttctggaccaatctgtattccctcacagtccctttcgggcaaaagcctaatatagacgtgacagacgcaatggttgatcaggcttgggatgctcaaaggatttttaaggaagctgagaagttttttgtgtcagtcggtttgccaaatatgacacaaggcttctgggaaaatagcatgttgactgatcccggtaatgttcaaaaggctgtgtgtcaccctaccgcttgggaccttgggaaaggtgactttcgaatcttgatgtgtaccaaggtgacaatggatgactttcttacagcccatcatgaaatgggtcacatccagtatgatatggcttatgcagctcaacctttcctcttgagaaatggtgcaaatgaaggttttcatgaagctgtaggggaaataatgtccctgagtgctgcaaccccaaagcatctcaagagtatcggattgttgagcccagattttcaagaagataacgagaccgaaatcaacttccttctgaaacaagccctcacaatagttggtactcttccattcacatacatgctggagaaatggcgttggatggtttttaagggggagatacctaaagatcagtggatgaaaaagtggtgggagatgaagcgtgagatcgtaggggtcgtggagccagtgcctcatgatgagacttactgtgacccagcatcactcttccacgttagcaatgactattcatttatacgttattacactcgcactctttaccagtttcaatttcaggaggctctgtgtcaggctgccaagcatgagggaccccttcacaagtgtgatattagtaacagtactgaggcaggccaaaaactgttcaatatgttgaggcttggcaaaagcgagccatggactctcgccttggaaaatgttgtcggggctaaaaacatgaatgtacgccctctgcttaactattttgagcccctttttacatggctcaaggaccagaataagaactcctttgtcggctggtcaacagactggtctccctatgcagaccctagtactcctcctactccttctccatcaaccccaccaactccatcccctagctgctgtcacccaaggctgtctctgcaccgacctgcactcgaagaccttctgttgggctctgaagctaacctgacctgtactcttactggcttgcgcgatgctagcggcgtgactttcacctggacacctagtagcggtaaaagtgctgtacaaggacctcctgaacgcgacctgtgtggttgctactctgtgtcttctgtacttcccggctgtgccgagccctggaatcacgggaaaacctttacctgcaccgccgcttaccctgagtcaaaaactcccctcactgccacattgagtaagtcagggaatacattcaggccagaggttcatttgttgcctcctccatctgaagaacttgctttgaacgagctggtcactctgacctgcttggctaggggtttctcccccaaagatgtacttgtacggtggttgcagggcagccaagagttgccccgcgaaaagtatttgacctgggcctcaagacaagaacccagccaggggactaccacatttgccgtgaccagtattctgcgtgtagccgctgaagattggaagaaaggggatacattttcttgcatggtagggcatgaggcccttcccctcgctttcactcagaagacaatagacagactcgccggaaagcctactcacgtgaatgttagcgtagtcatggctgaggttgacggaacttgctactgagatatccgatccaccggatctagataactgatcataatcagccataccacatttgtagaggttttacttgctttaaaaaacctcccacacctccccctgaacctgaaacataaaatgaatgcaattgttgttgttaacttgtttattgcagcttataatggttacaaataaagcaatagcatcacaaatttcacaaataaagcatttttttcactgcattctagttgtggtttgtccaaactcatcaatgtatcttaggtttagtgaaccgtcagatccgctagcgttacataacttacggtaaatggcccgcctggctgaccgcccaacgacccccgcccattgacgtcaataatgacgtatgttcccatagtaacgccaatagggactttccattgacgtcaatgggtggagtatttacggtaaactgcccacttggcagtacatcaagtgtatcatatgccaagtacgccccctattgacgtcaatgacggtaaatggcccgcctggcattatgcccagtacatgaccttatgggactttcctacttggcagtacatctacgtattagtcatcgctattaccatggtgatgcggttttggcagtacatcaatgggcgtggatagcggtttgactcacggggatttccaagtctccaccccattgacgtcaatgggagtttgttttggcaccaaaatcaacgggactttccaaaatgtcgtaacaactccgccccattgacgcaaatgggcggtaggcgtgtacggtgggaggtctatataagcagagctggtttagtgaaccgtcagatccgctagagatctggtaccgtcgacgcggccgctcgagcctaagcttatgaagaaccatctgcttttctggggagtacttgccgttttcataaaagccgtacatgttaaagcacaagaggacgaacgcattgtgttggttgataataaatgcaaatgtgctcggataacatctcggatcattcgtagctcagaggaccccaatgaggatatagtagagcgaaacatcagaattatagtacccctgaacaacagagagaacataagtgatcccacaagtccattgcggacacgctttgtttaccatttgtctgatctgtgtaaaaaatgtgatccaacagaggtggaactcgacaatcagatcgtcaccgccacccagtctaacatctgcgatgaagattcagctacagagacatgctacacatacgaccggaacaagtgctatactgccgttgtgccactcgtttacggtggagaaacaaagatggttgaaactgcacttacaccagatgcctgctatccagattgagatatccgatccaccggatctagataactgatcataatcagccataccacatttgtagaggttttacttgctttaaaaaacctcccacacctccccctgaacctgaaacataaaatgaatgcaattgttgttgttaacttgtttattgcagcttataatggttacaaataaagcaatagcatcacaaatttcacaaataaagcatttttttcactgcattctagttgtggtttgtccaaactcatcaatgtatcttaacgcggatctgggcgtggttaagggtgggaaagaatatataaggtgggggtcttatgtagttttgtatctgttttgcagcagccgccgccgccatgagcaccaactcgtttgatggaagcattgtgagctcatatttgacaacgcgcatgcccccatgggccggggtgcgtcagaatgtgatgggctccagcattgatggtcgccccgtcctgcccgcaaactctactaccttgacctacgagaccgtgtctggaacgccgttggagactgcagcctccgccgccgcttcagccgctgcagccaccgcccgcgggattgtgactgactttgctttcctgagcccgcttgcaagcagtgcagcttcccgttcatccgcccgcgatgacaagttgacggctcttttggcacaattggattctttgacccgggaacttaatgtcgtttctcagcagctgttggatctgcgccagcaggtttctgccctgaaggcttcctcccctcccaatgcggtttaaaacataaataaaaaaccagactctgtttggatttggatcaagcaagtgtcttgctgtctttatttaggggttttgcgcgcgcggtaggcccgggaccagcggtctcggtcgttgagggtcctgtgtattttttccaggacgtggtaaaggtgactctggatgttcagatacatgggcataagcccgtctctggggtggaggtagcaccactgcagagcttcatgctgcggggtggtgttgtagatgatccagtcgtagcaggagcgctgggcgtggtgcctaaaaatgtctttcagtagcaagctgattgccaggggcaggcccttggtgtaagtgtttacaaagcggttaagctgggatgggtgcatacgtggggatatgagatgcatcttggactgtatttttaggttggctatgttcccagccatatccctccggggattcatgttgtgcagaaccaccagcacagtgtatccggtgcacttgggaaatttgtcatgtagcttagaaggaaatgcgtggaagaacttggagacgcccttgtgacctccaagattttccatgcattcgtccataatgatggcaatgggcccacgggcggcggcctgggcgaagatatttctgggatcactaacgtcatagttgtgttccaggatgagatcgtcataggccatttttacaaagcgcgggcggagggtgccagactgcggtataatggttccatccggcccaggggcgtagttaccctcacagatttgcatttcccacgctttgagttcagatggggggatcatgtctacctgcggggcgatgaagaaaacggtttccggggtaggggagatcagctgggaagaaagcaggttcctgagcagctgcgacttaccgcagccggtgggcccgtaaatcacacctattaccggctgcaactggtagttaagagagctgcagctgccgtcatccctgagcaggggggccacttcgttaagcatgtccctgactcgcatgttttccctgaccaaatccgccagaaggcgctcgccgcccagcgatagcagttcttgcaaggaagcaaagtttttcaacggtttgagaccgtccgccgtaggcatgcttttgagcgtttgaccaagcagttccaggcggtcccacagctcggtcacctgctctacggcatctcgatccagcatatctcctcgtttcgcgggttggggcggctttcgctgtacggcagtagtcggtgctcgtccagacgggccagggtcatgtctttccacgggcgcagggtcctcgtcagcgtagtctgggtcacggtgaaggggtgcgctccgggctgcgcgctggccagggtgcgcttgaggctggtcctgctggtgctgaagcgctgccggtcttcgccctgcgcgtcggccaggtagcatttgaccatggtgtcatagtccagcccctccgcggcgtggcccttggcgcgcagcttgcccttggaggaggcgccgcacgaggggcagtgcagacttttgagggcgtagagcttgggcgcgagaaataccgattccggggagtaggcatccgcgccgcaggccccgcagacggtctcgcattccacgagccaggtgagctctggccgttcggggtcaaaaaccaggtttcccccatgctttttgatgcgtttcttacctctggtttccatgagccggtgtccacgctcggtgacgaaaaggctgtccgtgtccccgtatacagacttgagaggcctgtcctcgagcggtgttccgcggtcctcctcgtatagaaactcggaccactctgagacaaaggctcgcgtccaggccagcacgaaggaggctaagtgggaggggtagcggtcgttgtccactagggggtccactcgctccagggtgtgaagacacatgtcgccctcttcggcatcaaggaaggtgattggtttgtaggtgtaggccacgtgaccgggtgttcctgaaggggggctataaaagggggtgggggcgcgttcgtcctcactctcttccgcatcgctgtctgcgagggccagctgttggggtgagtactccctctgaaaagcgggcatgacttctgcgctaagattgtcagtttccaaaaacgaggaggatttgatattcacctggcccgcggtgatgcctttgagggtggccgcatccatctggtcagaaaagacaatctttttgttgtcaagcttggtggcaaacgacccgtagagggcgttggacagcaacttggcgatggagcgcagggtttggtttttgtcgcgatcggcgcgctccttggccgcgatgtttagctgcacgtattcgcgcgcaacgcaccgccattcgggaaagacggtggtgcgctcgtcgggcaccaggtgcacgcgccaaccgcggttgtgcagggtgacaaggtcaacgctggtggctacctctccgcgtaggcgctcgttggtccagcagaggcggccgcccttgcgcgagcagaatggcggtagggggtctagctgcgtctcgtccggggggtctgcgtccacggtaaagaccccgggcagcaggcgcgcgtcgaagtagtctatcttgcatccttgcaagtctagcgcctgctgccatgcgcgggcggcaagcgcgcgctcgtatgggttgagtgggggaccccatggcatggggtgggtgagcgcggaggcgtacatgccgcaaatgtcgtaaacgtagaggggctctctgagtattccaagatatgtagggtagcatcttccaccgcggatgctggcgcgcacgtaatcgtatagttcgtgcgagggagcgaggaggtcgggaccgaggttgctacgggcgggctgctctgctcggaagactatctgcctgaagatggcatgtgagttggatgatatggttggacgctggaagacgttgaagctggcgtctgtgagacctaccgcgtcacgcacgaaggaggcgtaggagtcgcgcagcttgttgaccagctcggcggtgacctgcacgtctagggcgcagtagtccagggtttccttgatgatgtcatacttatcctgtcccttttttttccacagctcgcggttgaggacaaactcttcgcggtctttccagtactcttggatcggaaacccgtcggcctccgaacggtaagagcctagcatgtagaactggttgacggcctggtaggcgcagcatcccttttctacgggtagcgcgtatgcctgcgcggccttccggcatgaccagcatgaagggcacgagctgcttcccaaaggcccccatccaagtataggtctctacatcgtaggtgacaaagagacgctcggtgcgaggatgcgagccgatcgggaagaactggatctcccgccaccaattggaggagtggctattgatgtggtgaaagtagaagtccctgcgacgggccgaacactcgtgctggcttttgtaaaaacgtgcgcagtactggcagcggtgcacgggctgtacatcctgcacgaggttgacctgacgaccgcgcacaaggaagcagagtgggaatttgagcccctcgcctggcgggtttggctggtggtcttctacttcggctgcttgtccttgaccgtctggctgctcgaggggagttacggtggatcggaccaccacgccgcgcgagcccaaagtccagatgtccgcgcgcggcggtcggagcttgatgacaacatcgcgcagatgggagctgtccatggtctggagctcccgcggcgtcaggtcaggcgggagctcctgcaggtttacctcgcatagacgggtcagggcgcgggctagatccaggtgatacctaatttccaggggctggttggtggcggcgtcgatggcttgcaagaggccgcatccccgcggcgcgactacggtaccgcgcggcgggcggtgggccgcgggggtgtccttggatgatgcatctaaaagcggtgacgcgggcgagcccccggaggtagggggggctccggacccgccgggagagggggcaggggcacgtcggcgccgcgcgcgggcaggagctggtgctgcgcgcgtaggttgctggcgaacgcgacgacgcggcggttgatctcctgaatctggcgcctctgcgtgaagacgacgggcccggtgagcttgaacctgaaagagagttcgacagaatcaatttcggtgtcgttgacggcggcctggcgcaaaatctcctgcacgtctcctgagttgtcttgataggcgatctcggccatgaactgctcgatctcttcctcctggagatctccgcgtccggctcgctccacggtggcggcgaggtcgttggaaatgcgggccatgagctgcgagaaggcgttgaggcctccctcgttccagacgcggctgtagaccacgcccccttcggcatcgcgggcgcgcatgaccacctgcgcgagattgagctccacgtgccgggcgaagacggcgtagtttcgcaggcgctgaaagaggtagttgagggtggtggcggtgtgttctgccacgaagaagtacataacccagcgtcgcaacgtggattcgttgataattgttgtgtaggtactccgccgccgagggacctgagcgagtccgcatcgaccggatcggaaaacctctcgagaaaggcgtctaaccagtcacagtcgcaaggtaggctgagcaccgtggcgggcggcagcgggcggcggtcggggttgtttctggcggaggtgctgctgatgatgtaattaaagtaggcggtcttgagacggcggatggtcgacagaagcaccatgtccttgggtccggcctgctgaatgcgcaggcggtcggccatgccccaggcttcgttttgacatcggcgcaggtctttgtagtagtcttgcatgagcctttctaccggcacttcttcttctccttcctcttgtcctgcatctcttgcatctatcgctgcggcggcggcggagtttggccgtaggtggcgccctcttcctcccatgcgtgtgaccccgaagcccctcatcggctgaagcagggctaggtcggcgacaacgcgctcggctaatatggcctgctgcacctgcgtgagggtagactggaagtcatccatgtccacaaagcggtggtatgcgcccgtgttgatggtgtaagtgcagttggccataacggaccagttaacggtctggtgacccggctgcgagagctcggtgtacctgagacgcgagtaagccctcgagtcaaatacgtagtcgttgcaagtccgcaccaggtactggtatcccaccaaaaagtgcggcggcggctggcggtagaggggccagcgtagggtggccggggctccgggggcgagatcttccaacataaggcgatgatatccgtagatgtacctggacatccaggtgatgccggcggcggtggtggaggcgcgcggaaagtcgcggacgcggttccagatgttgcgcagcggcaaaaagtgctccatggtcgggacgctctggccggtcaggcgcgcgcaatcgttgacgctctagcgtgcaaaaggagagcctgtaagcgggcactcttccgtggtctggtggataaattcgcaagggtatcatggcggacgaccggggttcgagccccgtatccggccgtccgccgtgatccatgcggttaccgcccgcgtgtcgaacccaggtgtgcgacgtcagacaacgggggagtgctccttttggcttccttccaggcgcggcggctgctgcgctagcttttttggccactggccgcgcgcagcgtaagcggttaggctggaaagcgaaagcattaagtggctcgctccctgtagccggagggttattttccaagggttgagtcgcgggacccccggttcgagtctcggaccggccggactgcggcgaacgggggtttgcctccccgtcatgcaagaccccgcttgcaaattcctccggaaacagggacgagccccttttttgcttttcccagatgcatccggtgctgcggcagatgcgcccccctcctcagcagcggcaagagcaagagcagcggcagacatgcagggcaccctcccctcctcctaccgcgtcaggaggggcgacatccgcggttgacgcggcagcagatggtgattacgaacccccgcggcgccgggcccggcactacctggacttggaggagggcgagggcctggcgcggctaggagcgccctctcctgagcggcacccaagggtgcagctgaagcgtgatacgcgtgaggcgtacgtgccgcggcagaacctgtttcgcgaccgcgagggagaggagcccgaggagatgcgggatcgaaagttccacgcagggcgcgagctgcggcatggcctgaatcgcgagcggttgctgcgcgaggaggactttgagcccgacgcgcgaaccgggattagtcccgcgcgcgcacacgtggcggccgccgacctggtaaccgcatacgagcagacggtgaaccaggagattaactttcaaaaaagctttaacaaccacgtgcgtacgcttgtggcgcgcgaggaggtggctataggactgatgcatctgtgggactttgtaagcgcgctggagcaaaacccaaatagcaagccgctcatggcgcagctgttccttatagtgcagcacagcagggacaacgaggcattcagggatgcgctgctaaacatagtagagcccgagggccgctggctgctcgatttgataaacatcctgcagagcatagtggtgcaggagcgcagcttgagcctggctgacaaggtggccgccatcaactattccatgcttagcctgggcaagttttacgcccgcaagatataccataccccttacgttcccatagacaaggaggtaaagatcgaggggttctacatgcgcatggcgctgaaggtgcttaccttgagcgacgacctgggcgtttatcgcaacgagcgcatccacaaggccgtgagcgtgagccggcggcgcgagctcagcgaccgcgagctgatgcacagcctgcaaagggccctggctggcacgggcagcggcgatagagaggccgagtcctactttgacgcgggcgctgacctgcgctgggccccaagccgacgcgccctggaggcagctggggccggacctgggctggcggtggcacccgcgcgcgctggcaacgtcggcggcgtggaggaatatgacgaggacgatgagtacgagccagaggacggcgagtactaagcggtgatgtttctgatcagatgatgcaagacgcaacggacccggcggtgcgggcggcgctgcagagccagccgtccggccttaactccacggacgactggcgccaggtcatggaccgcatcatgtcgctgactgcgcgcaatcctgacgcgttccggcagcagccgcaggccaaccggctctccgcaattctggaagcggtggtcccggcgcgcgcaaaccccacgcacgagaaggtgctggcgatcgtaaacgcgctggccgaaaacagggccatccggcccgacgaggccggcctggtctacgacgcgctgcttcagcgcgtggctcgttacaacagcggcaacgtgcagaccaacctggaccggctggtgggggatgtgcgcgaggccgtggcgcagcgtgagcgcgcgcagcagcagggcaacctgggctccatggttgcactaaacgccttcctgagtacacagcccgccaacgtgccgcggggacaggaggactacaccaactttgtgagcgcactgcggctaatggtgactgagacaccgcaaagtgaggtgtaccagtctgggccagactattttttccagaccagtagacaaggcctgcagaccgtaaacctgagccaggctttcaaaaacttgcaggggctgtggggggtgcgggctcccacaggcgaccgcgcgaccgtgtctagcttgctgacgcccaactcgcgcctgttgctgctgctaatagcgcccttcacggacagtggcagcgtgtcccgggacacatacctaggtcacttgctgacactgtaccgcgaggccataggtcaggcgcatgtggacgagcatactttccaggagattacaagtgtcagccgcgcgctggggcaggaggacacgggcagcctggaggcaaccctaaactacctgctgaccaaccggcggcagaagatcccctcgttgcacagtttaaacagcgaggaggagcgcattttgcgctacgtgcagcagagcgtgagccttaacctgatgcgcgacggggtaacgcccagcgtggcgctggacatgaccgcgcgcaacatggaaccgggcatgtatgcctcaaaccggccgtttatcaaccgcctaatggactacttgcatcgcgcggccgccgtgaaccccgagtatttcaccaatgccatcttgaacccgcactggctaccgccccctggtttctacaccgggggattcgaggtgcccgagggtaacgatggattcctctgggacgacatagacgacagcgtgttttccccgcaaccgcagaccctgctagagttgcaacagcgcgagcaggcagaggcggcgctgcgaaaggaaagcttccgcaggccaagcagcttgtccgatctaggcgctgcggccccgcggtcagatgctagtagcccatttccaagcttgatagggtctcttaccagcactcgcaccacccgcccgcgcctgctgggcgaggaggagtacctaaacaactcgctgctgcagccgcagcgcgaaaaaaacctgcctccggcatttcccaacaacgggatagagagcctagtggacaagatgagtagatggaagacgtacgcgcaggagcacagggacgtgccaggcccgcgcccgcccacccgtcgtcaaaggcacgaccgtcagcggggtctggtgtgggaggacgatgactcggcagacgacagcagcgtcctggatttgggagggagtggcaacccgtttgcgcaccttcgccccaggctggggagaatgttttaaaaaaaaaaaagcatgatgcaaaataaaaaactcaccaaggccatggcaccgagcgttggttttcttgtattccccttagtatgcggcgcgcggcgatgtatgaggaaggtcctcctccctcctacgagagtgtggtgagcgcggcgccagtggcggcggcgctgggttctcccttcgatgctcccctggacccgccgtttgtgcctccgcggtacctgcggcctaccggggggagaaacagcatccgttactctgagttggcacccctattcgacaccacccgtgtgtacctggtggacaacaagtcaacggatgtggcatccctgaactaccagaacgaccacagcaactttctgaccacggtcattcaaaacaatgactacagcccgggggaggcaagcacacagaccatcaatcttgacgaccggtcgcactggggcggcgacctgaaaaccatcctgcataccaacatgccaaatgtgaacgagttcatgtttaccaataagtttaaggcgcgggtgatggtgtcgcgcttgcctactaaggacaatcaggtggagctgaaatacgagtgggtggagttcacgctgcccgagggcaactactccgagaccatgaccatagaccttatgaacaacgcgatcgtggagcactacttgaaagtgggcagacagaacggggttctggaaagcgacatcggggtaaagtttgacacccgcaacttcagactggggtttgaccccgtcactggtcttgtcatgcctggggtatatacaaacgaagccttccatccagacatcattttgctgccaggatgcggggtggacttcacccacagccgcctgagcaacttgttgggcatccgcaagcggcaacccttccaggagggctttaggatcacctacgatgatctggagggtggtaacattcccgcactgttggatgtggacgcctaccaggcgagcttgaaagatgacaccgaacagggcgggggtggcgcaggcggcagcaacagcagtggcagcggcgcggaagagaactccaacgcggcagccgcggcaatgcagccggtggaggacatgaacgatcatgccattcgcggcgacacctttgccacacgggctgaggagaagcgcgctgaggccgaagcagcggccgaagctgccgcccccgctgcgcaacccgaggtcgagaagcctcagaagaaaccggtgatcaaacccctgacagaggacagcaagaaacgcagttacaacctaataagcaatgacagcaccttcacccagtaccgcagctggtaccttgcatacaactacggcgaccctcagaccggaatccgctcatggaccctgctttgcactcctgacgtaacctgcggctcggagcaggtctactggtcgttgccagacatgatgcaagaccccgtgaccttccgctccacgcgccagatcagcaactttccggtggtgggcgccgagctgttgcccgtgcactccaagagcttctacaacgaccaggccgtctactcccaactcatccgccagtttacctctctgacccacgtgttcaatcgctttcccgagaaccagattttggcgcgcccgccagcccccaccatcaccaccgtcagtgaaaacgttcctgctctcacagatcacgggacgctaccgctgcgcaacagcatcggaggagtccagcgagtgaccattactgacgccagacgccgcacctgcccctacgtttacaaggccctgggcatagtctcgccgcgcgtcctatcgagccgcactttttgagcaagcatgtccatccttatatcgcccagcaataacacaggctggggcctgcgcttcccaagcaagatgtttggcggggccaagaagcgctccgaccaacacccagtgcgcgtgcgcgggcactaccgcgcgccctggggcgcgcacaaacgcggccgcactgggcgcaccaccgtcgatgacgccatcgacgcggtggtggaggaggcgcgcaactacacgcccacgccgccaccagtgtccacagtggacgcggccattcagaccgtggtgcgcggagcccggcgctatgctaaaatgaagagacggcggaggcgcgtagcacgtcgccaccgccgccgacccggcactgccgcccaacgcgcggcggcggccctgcttaaccgcgcacgtcgcaccggccgacgggcggccatgcgggccgctcgaaggctggccgcgggtattgtcactgtgccccccaggtccaggcgacgagcggccgccgcagcagccgcggccattagtgctatgactcagggtcgcaggggcaacgtgtattgggtgcgcgactcggttagcggcctgcgcgtgcccgtgcgcacccgccccccgcgcaactagattgcaagaaaaaactacttagactcgtactgttgtatgtatccagcggcggcggcgcgcaacgaagctatgtccaagcgcaaaatcaaagaagagatgctccaggtcatcgcgccggagatctatggccccccgaagaaggaagagcaggattacaagccccgaaagctaaagcgggtcaaaaagaaaaagaaagatgatgatgatgaacttgacgacgaggtggaactgctgcacgctaccgcgcccaggcgacgggtacagtggaaaggtcgacgcgtaaaacgtgttttgcgacccggcaccaccgtagtctttacgcccggtgagcgctccacccgcacctacaagcgcgtgtatgatgaggtgtacggcgacgaggacctgcttgagcaggccaacgagcgcctcggggagtttgcctacggaaagcggcataaggacatgctggcgttgccgctggacgagggcaacccaacacctagcctaaagcccgtaacactgcagcaggtgctgcccgcgcttgcaccgtccgaagaaaagcgcggcctaaagcgcgagtctggtgacttggcacccaccgtgcagctgatggtacccaagcgccagcgactggaagatgtcttggaaaaaatgaccgtggaacctgggctggagcccgaggtccgcgtgcggccaatcaagcaggtggcgccgggactgggcgtgcagaccgtggacgttcagatacccactaccagtagcaccagtattgccaccgccacagagggcatggagacacaaacgtccccggttgcctcagcggtggcggatgccgcggtgcaggcggtcgctgcggccgcgtccaagacctctacggaggtgcaaacggacccgtggatgtttcgcgtttcagccccccggcgcccgcgccgttcgaggaagtacggcgccgccagcgcgctactgcccgaatatgccctacatccttccattgcgcctacccccggctatcgtggctacacctaccgccccagaagacgagcaactacccgacgccgaaccaccactggaacccgccgccgccgtcgccgtcgccagcccgtgctggccccgatttccgtgcgcagggtggctcgcgaaggaggcaggaccctggtgctgccaacagcgcgctaccaccccagcatcgtttaaaagccggtctttgtggttcttgcagatatggccctcacctgccgcctccgtttcccggtgccgggattccgaggaagaatgcaccgtaggaggggcatggccggccacggcctgacgggcggcatgcgtcgtgcgcaccaccggcggcggcgcgcgtcgcaccgtcgcatgcgcggcggtatcctgcccctccttattccactgatcgccgcggcgattggcgccgtgcccggaattgcatccgtggccttgcaggcgcagagacactgattaaaaacaagttgcatgtggaaaaatcaaaataaaaagtctggactctcacgctcgcttggtcctgtaactattttgtagaatggaagacatcaactttgcgtctctggccccgcgacacggctcgcgcccgttcatgggaaactggcaagatatcggcaccagcaatatgagcggtggcgccttcagctggggctcgctgtggagcggcattaaaaatttcggttccaccgttaagaactatggcagcaaggcctggaacagcagcacaggccagatgctgagggataagttgaaagagcaaaatttccaacaaaaggtggtagatggcctggcctctggcattagcggggtggtggacctggccaaccaggcagtgcaaaataagattaacagtaagcttgatccccgccctcccgtagaggagcctccaccggccgtggagacagtgtctccagaggggcgtggcgaaaagcgtccgcgccccgacagggaagaaactctggtgacgcaaatagacgagcctccctcgtacgaggaggcactaaagcaaggcctgcccaccacccgtcccatcgcgcccatggctaccggagtgctgggccagcacacacccgtaacgctggacctgcctccccccgccgacacccagcagaaacctgtgctgccaggcccgaccgccgttgttgtaacccgtcctagccgcgcgtccctgcgccgcgccgccagcggtccgcgatcgttgcggcccgtagccagtggcaactggcaaagcacactgaacagcatcgtgggtctgggggtgcaatccctgaagcgccgacgatgcttctgatagctaacgtgtcgtatgtgtgtcatgtatgcgtccatgtcgccgccagaggagctgctgagccgccgcgcgcccgctttccaagatggctaccccttcgatgatgccgcagtggtcttacatgcacatctcgggccaggacgcctcggagtacctgagccccgggctggtgcagtttgcccgcgccaccgagacgtacttcagcctgaataacaagtttagaaaccccacggtggcgcctacgcacgacgtgaccacagaccggtcccagcgtttgacgctgcggttcatccctgtggaccgtgaggatactgcgtactcgtacaaggcgcggttcaccctagctgtgggtgataaccgtgtgctggacatggcttccacgtactttgacatccgcggcgtgctggacaggggccctacttttaagccctactctggcactgcctacaacgccctggctcccaagggtgccccaaatccttgcgaatgggatgaagctgctactgctcttgaaataaacctagaagaagaggacgatgacaacgaagacgaagtagacgagcaagctgagcagcaaaaaactcacgtatttgggcaggcgccttattctggtataaatattacaaaggagggtattcaaataggtgtcgaaggtcaaacacctaaatatgccgataaaacatttcaacctgaacctcaaataggagaatctcagtggtacgaaacagaaattaatcatgcagctgggagagtcctaaaaaagactaccccaatgaaaccatgttacggttcatatgcaaaacccacaaatgaaaatggagggcaaggcattcttgtaaagcaacaaaatggaaagctagaaagtcaagtggaaatgcaatttttctcaactactgaggcagccgcaggcaatggtgataacttgactcctaaagtggtattgtacagtgaagatgtagatatagaaaccccagacactcatatttcttacatgcccactattaaggaaggtaactcacgagaactaatgggccaacaatctatgcccaacaggcctaattacattgcttttagggacaattttattggtctaatgtattacaacagcacgggtaatatgggtgttctggcgggccaagcatcgcagttgaatgctgttgtagatttgcaagacagaaacacagagctttcataccagcttttgcttgattccattggtgatagaaccaggtacttttctatgtggaatcaggctgttgacagctatgatccagatgttagaattattgaaaatcatggaactgaagatgaacttccaaattactgctttccactgggaggtgtgattaatacagagactcttaccaaggtaaaacctaaaacaggtcaggaaaatggatgggaaaaagatgctacagaattttcagataaaaatgaaataagagttggaaataattttgccatggaaatcaatctaaatgccaacctgtggagaaatttcctgtactccaacatagcgctgtatttgcccgacaagctaaagtacagtccttccaacgtaaaaatttctgataacccaaacacctacgactacatgaacaagcgagtggtggctcccgggctagtggactgctacattaaccttggagcacgctggtcccttgactatatggacaacgtcaacccatttaaccaccaccgcaatgctggcctgcgctaccgctcaatgttgctgggcaatggtcgctatgtgcccttccacatccaggtgcctcagaagttctttgccattaaaaacctccttctcctgccgggctcatacacctacgagtggaacttcaggaaggatgttaacatggttctgcagagctccctaggaaatgacctaagggttgacggagccagcattaagtttgatagcatttgcctttacgccaccttcttccccatggcccacaacaccgcctccacgcttgaggccatgcttagaaacgacaccaacgaccagtcctttaacgactatctctccgccgccaacatgctctaccctatacccgccaacgctaccaacgtgcccatatccatcccctcccgcaactgggcggctttccgcggctgggccttcacgcgccttaagactaaggaaaccccatcactgggctcgggctacgacccttattacacctactctggctctataccctacctagatggaaccttttacctcaaccacacctttaagaaggtggccattacctttgactcttctgtcagctggcctggcaatgaccgcctgcttacccccaacgagtttgaaattaagcgctcagttgacggggagggttacaacgttgcccagtgtaacatgaccaaagactggttcctggtacaaatgctagctaactataacattggctaccagggcttctatatcccagagagctacaaggaccgcatgtactccttctttagaaacttccagcccatgagccgtcaggtggtggatgatactaaatacaaggactaccaacaggtgggcatcctacaccaacacaacaactctggatttgttggctaccttgcccccaccatgcgcgaaggacaggcctaccctgctaacttcccctatccgcttataggcaagaccgcagttgacagcattacccagaaaaagtttctttgcgatcgcaccctttggcgcatcccattctccagtaactttatgtccatgggcgcactcacagacctgggccaaaaccttctctacgccaactccgcccacgcgctagacatgacttttgaggtggatcccatggacgagcccacccttctttatgttttgtttgaagtctttgacgtggtccgtgtgcaccagccgcaccgcggcgtcatcgaaaccgtgtacctgcgcacgcccttctcggccggcaacgccacaacataaagaagcaagcaacatcaacaacagctgccgccatgggctccagtgagcaggaactgaaagccattgtcaaagatcttggttgtgggccatattttttgggcacctatgacaagcgctttccaggctttgtttctccacacaagctcgcctgcgccatagtcaatacggccggtcgcgagactgggggcgtacactggatggcctttgcctggaacccgcactcaaaaacatgctacctctttgagccctttggcttttctgaccagcgactcaagcaggtttaccagtttgagtacgagtcactcctgcgccgtagcgccattgcttcttcccccgaccgctgtataacgctggaaaagtccacccaaagcgtacaggggcccaactcggccgcctgtggactattctgctgcatgtttctccacgcctttgccaactggccccaaactcccatggatcacaaccccaccatgaaccttattaccggggtacccaactccatgctcaacagtccccaggtacagcccaccctgcgtcgcaaccaggaacagctctacagcttcctggagcgccactcgccctacttccgcagccacagtgcgcagattaggagcgccacttctttttgtcacttgaaaaacatgtaaaaataatgtactagagacactttcaataaaggcaaatgcttttatttgtacactctcgggtgattatttacccccacccttgccgtctgcgccgtttaaaaatcaaaggggttctgccgcgcatcgctatgcgccactggcagggacacgttgcgatactggtgtttagtgctccacttaaactcaggcacaaccatccgcggcagctcggtgaagttttcactccacaggctgcgcaccatcaccaacgcgtttagcaggtcgggcgccgatatcttgaagtcgcagttggggcctccgccctgcgcgcgcgagttgcgatacacagggttgcagcactggaacactatcagcgccgggtggtgcacgctggccagcacgctcttgtcggagatcagatccgcgtccaggtcctccgcgttgctcagggcgaacggagtcaactttggtagctgccttcccaaaaagggcgcgtgcccaggctttgagttgcactcgcaccgtagtggcatcaaaaggtgaccgtgcccggtctgggcgttaggatacagcgcctgcataaaagccttgatctgcttaaaagccacctgagcctttgcgccttcagagaagaacatgccgcaagacttgccggaaaactgattggccggacaggccgcgtcgtgcacgcagcaccttgcgtcggtgttggagatctgcaccacatttcggccccaccggttcttcacgatcttggccttgctagactgctccttcagcgcgcgctgcccgttttcgctcgtcacatccatttcaatcacgtgctccttatttatcataatgcttccgtgtagacacttaagctcgccttcgatctcagcgcagcggtgcagccacaacgcgcagcccgtgggctcgtgatgcttgtaggtcacctctgcaaacgactgcaggtacgcctgcaggaatcgccccatcatcgtcacaaaggtcttgttgctggtgaaggtcagctgcaacccgcggtgctcctcgttcagccaggtcttgcatacggccgccagagcttccacttggtcaggcagtagtttgaagttcgcctttagatcgttatccacgtggtacttgtccatcagcgcgcgcgcagcctccatgcccttctcccacgcagacacgatcggcacactcagcgggttcatcaccgtaatttcactttccgcttcgctgggctcttcctcttcctcttgcgtccgcataccacgcgccactgggtcgtcttcattcagccgccgcactgtgcgcttacctcctttgccatgcttgattagcaccggtgggttgctgaaacccaccatttgtagcgccacatcttctctttcttcctcgctgtccacgattacctctggtgatggcgggcgctcgggcttgggagaagggcgcttctttttcttcttgggcgcaatggccaaatccgccgccgaggtcgatggccgcgggctgggtgtgcgcggcaccagcgcgtcttgtgatgagtcttcctcgtcctcggactcgatacgccgcctcatccgcttttttgggggcgcccggggaggcggcggcgacggggacggggacgacacgtcctccatggttgggggacgtcgcgccgcaccgcgtccgcgctcgggggtggtttcgcgctgctcctcttcccgactggccatttccttctcctataggcagaaaaagatcatggagtcagtcgagaagaaggacagcctaaccgccccctctgagttcgccaccaccgcctccaccgatgccgccaacgcgcctaccaccttccccgtcgaggcacccccgcttgaggaggaggaagtgattatcgagcaggacccaggttttgtaagcgaagacgacgaggaccgctcagtaccaacagaggataaaaagcaagaccaggacaacgcagaggcaaacgaggaacaagtcgggcggggggacgaaaggcatggcgactacctagatgtgggagacgacgtgctgttgaagcatctgcagcgccagtgcgccattatctgcgacgcgttgcaagagcgcagcgatgtgcccctcgccatagcggatgtcagccttgcctacgaacgccacctattctcaccgcgcgtaccccccaaacgccaagaaaacggcacatgcgagcccaacccgcgcctcaacttctaccccgtatttgccgtgccagaggtgcttgccacctatcacatctttttccaaaactgcaagatacccctatcctgccgtgccaaccgcagccgagcggacaagcagctggccttgcggcagggcgctgtcatacctgatatcgcctcgctcaacgaagtgccaaaaatctttgagggtcttggacgcgacgagaagcgcgcggcaaacgctctgcaacaggaaaacagcgaaaatgaaagtcactctggagtgttggtggaactcgagggtgacaacgcgcgcctagccgtactaaaacgcagcatcgaggtcacccactttgcctacccggcacttaacctaccccccaaggtcatgagcacagtcatgagtgagctgatcgtgcgccgtgcgcagcccctggagagggatgcaaatttgcaagaacaaacagaggagggcctacccgcagttggcgacgagcagctagcgcgctggcttcaaacgcgcgagcctgccgacttggaggagcgacgcaaactaatgatggccgcagtgctcgttaccgtggagcttgagtgcatgcagcggttctttgctgacccggagatgcagcgcaagctagaggaaacattgcactacacctttcgacagggctacgtacgccaggcctgcaagatctccaacgtggagctctgcaacctggtctcctaccttggaattttgcacgaaaaccgccttgggcaaaacgtgcttcattccacgctcaagggcgaggcgcgccgcgactacgtccgcgactgcgtttacttatttctatgctacacctggcagacggccatgggcgtttggcagcagtgcttggaggagtgcaacctcaaggagctgcagaaactgctaaagcaaaacttgaaggacctatggacggccttcaacgagcgctccgtggccgcgcacctggcggacatcattttccccgaacgcctgcttaaaaccctgcaacagggtctgccagacttcaccagtcaaagcatgttgcagaactttaggaactttatcctagagcgctcaggaatcttgcccgccacctgctgtgcacttcctagcgactttgtgcccattaagtaccgcgaatgccctccgccgctttggggccactgctaccttctgcagctagccaactaccttgcctaccactctgacataatggaagacgtgagcggtgacggtctactggagtgtcactgtcgctgcaacctatgcaccccgcaccgctccctggtttgcaattcgcagctgcttaacgaaagtcaaattatcggtacctttgagctgcagggtccctcgcctgacgaaaagtccgcggctccggggttgaaactcactccggggctgtggacgtcggcttaccttcgcaaatttgtacctgaggactaccacgcccacgagattaggttctacgaagaccaatcccgcccgcctaatgcggagcttaccgcctgcgtcattacccagggccacattcttggccaattgcaagccatcaacaaagcccgccaagagtttctgctacgaaagggacggggggtttacttggacccccagtccggcgaggagctcaacccaatccccccgccgccgcagccctatcagcagcagccgcgggcccttgcttcccaggatggcacccaaaaagaagctgcagctgccgccgccacccacggacgaggaggaatactgggacagtcaggcagaggaggttttggacgaggaggaggaggacatgatggaagactgggagagcctagacgaggaagcttccgaggtcgaagaggtgtcagacgaaacaccgtcaccctcggtcgcattcccctcgccggcgccccagaaatcggcaaccggttccagcatggctacaacctccgctcctcaggcgccgccggcactgcccgttcgccgacccaaccgtagatgggacaccactggaaccagggccggtaagtccaagcagccgccgccgttagcccaagagcaacaacagcgccaaggctaccgctcatggcgcgggcacaagaacgccatagttgcttgcttgcaagactgtgggggcaacatctccttcgcccgccgctttcttctctaccatcacggcgtggccttcccccgtaacatcctgcattactaccgtcatctctacagcccatactgcaccggcggcagcggcagcaacagcagcggccacacagaagcaaaggcgaccggatagcaagactctgacaaagcccaagaaatccacagcggcggcagcagcaggaggaggagcgctgcgtctggcgcccaacgaacccgtatcgacccgcgagcttagaaacaggatttttcccactctgtatgctatatttcaacagagcaggggccaagaacaagagctgaaaataaaaaacaggtctctgcgatccctcacccgcagctgcctgtatcacaaaagcgaagatcagcttcggcgcacgctggaagacgcggaggctctcttcagtaaatactgcgcgctgactcttaaggactagtttcgcgccctttctcaaatttaagcgcgaaaactacgtcatctccagcggccacacccggcgccagcacctgttgtcagcgccattatgagcaaggaaattcccacgccctacatgtggagttaccagccacaaatgggacttgcggctggagctgcccaagactactcaacccgaataaactacatgagcgcgggaccccacatgatatcccgggtcaacggaatacgcgcccaccgaaaccgaattctcctggaacaggcggctattaccaccacacctcgtaataaccttaatccccgtagttggcccgctgccctggtgtaccaggaaagtcccgctcccaccactgtggtacttcccagagacgcccaggccgaagttcagatgactaactcaggggcgcagcttgcgggcggctttcgtcacagggtgcggtcgcccgggcagggtataactcacctgacaatcagagggcgaggtattcagctcaacgacgagtcggtgagctcctcgcttggtctccgtccggacgggacatttcagatcggcggcgccggccgctcttcattcacgcctcgtcaggcaatcctaactctgcagacctcgtcctctgagccgcgctctggaggcattggaactctgcaatttattgaggagtttgtgccatcggtctactttaaccccttctcgggacctcccggccactatccggatcaatttattcctaactttgacgcggtaaaggactcggcggacggctacgactgaatgttaagtggagaggcagagcaactgcgcctgaaacacctggtccactgtcgccgccacaagtgctttgcccgcgactccggtgagttttgctactttgaattgcccgaggatcatatcgagggcccggcgcacggcgtccggcttaccgcccagggagagcttgcccgtagcctgattcgggagtttacccagcgccccctgctagttgagcgggacaggggaccctgtgttctcactgtgatttgcaactgtcctaaccctggattacatcaagatcctctagttaatgtcaggtcgcctaagtcgattaactagagtacccggggatcttattccctttaactaataaaaaaaaataataaagcatcacttacttaaaatcagttagcaaatttctgtccagtttattcagcagcacctccttgccctcctcccagctctggtattgcagcttcctcctggctgcaaactttctccacaatctaaatggaatgtcagtttcctcctgttcctgtccatccgcacccactatcttcatgttgttgcagatgaagcgcgcaagaccgtctgaagataccttcaaccccgtgtatccatatgacacggaaaccggtcctccaactgtgccttttcttactcctccctttgtatcccccaatgggtttcaagagagtccccctggggtactctctttgcgcctatccgaacctctagttacctccaatggcatgcttgcgctcaaaatgggcaacggcctctctctggacgaggccggcaaccttacctcccaaaatgtaaccactgtgagcccacctctcaaaaaaaccaagtcaaacataaacctggaaatatctgcacccctcacagttacctcagaagccctaactgtggctgccgccgcacctctaatggtcgcgggcaacacactcaccatgcaatcacaggccccgctaaccgtgcacgactccaaacttagcattgccacccaaggacccctcacagtgtcagaaggaaagctagccctgcaaacatcaggccccctcaccaccaccgatagcagtacccttactatcactgcctcaccccctctaactactgccactggtagcttgggcattgacttgaaagagcccatttatacacaaaatggaaaactaggactaaagtacggggctcctttgcatgtaacagacgacctaaacactttgaccgtagcaactggtccaggtgtgactattaataatacttccttgcaaactaaagttactggagccttgggttttgattcacaaggcaatatgcaacttaatgtagcaggaggactaaggattgattctcaaaacagacgccttatacttgatgttagttatccgtttgatgctcaaaaccaactaaatctaagactaggacagggccctctttttataaactcagcccacaacttggatattaactacaacaaaggcctttacttgtttacagcttcaaacaattccaaaaagcttgaggttaacctaagcactgccaaggggttgatgtttgacgctacagccatagccattaatgcaggagatgggcttgaatttggttcacctaatgcaccaaacacaaatcccctcaaaacaaaaattggccatggcctagaatttgattcaaacaaggctatggttcctaaactaggaactggccttagttttgacagcacaggtgccattacagtaggaaacaaaaataatgataagctaactttgtggaccacaccagctccatctcctaactgtagactaaatgcagagaaagatgctaaactcactttggtcttaacaaaatgtggcagtcaaatacttgctacagtttcagttttggctgttaaaggcagtttggctccaatatctggaacagttcaaagtgctcatcttattataagatttgacgaaaatggagtgctactaaacaattccttcctggacccagaatattggaactttagaaatggagatcttactgaaggcacagcctatacaaacgctgttggatttatgcctaacctatcagcttatccaaaatctcacggtaaaactgccaaaagtaacattgtcagtcaagtttacttaaacggagacaaaactaaacctgtaacactaaccattacactaaacggtacacaggaaacaggagacacaactccaagtgcatactctatgtcattttcatgggactggtctggccacaactacattaatgaaatatttgccacatcctcttacactttttcatacattgcccaagaataaagaatcgtttgtgttatgtttcaacgtgtttatttttcaattgcagaaaatttcaagtcatttttcattcagtagtatagccccaccaccacatagcttatacagatcaccgtaccttaatcaaactcacagaaccctagtattcaacctgccacctccctcccaacacacagagtacacagtcctttctccccggctggccttaaaaagcatcatatcatgggtaacagacatattcttaggtgttatattccacacggtttcctgtcgagccaaacgctcatcagtgatattaataaactccccgggcagctcacttaagttcatgtcgctgtccagctgctgagccacaggctgctgtccaacttgcggttgcttaacgggcggcgaaggagaagtccacgcctacatgggggtagagtcataatcgtgcatcaggatagggcggtggtgctgcagcagcgcgcgaataaactgctgccgccgccgctccgtcctgcaggaatacaacatggcagtggtctcctcagcgatgattcgcaccgcccgcagcataaggcgccttgtcctccgggcacagcagcgcaccctgatctcacttaaatcagcacagtaactgcagcacagcaccacaatattgttcaaaatcccacagtgcaaggcgctgtatccaaagctcatggcggggaccacagaacccacgtggccatcataccacaagcgcaggtagattaagtggcgacccctcataaacacgctggacataaacattacctcttttggcatgttgtaattcaccacctcccggtaccatataaacctctgattaaacatggcgccatccaccaccatcctaaaccagctggccaaaacctgcccgccggctatacactgcagggaaccgggactggaacaatgacagtggagagcccaggactcgtaaccatggatcatcatgctcgtcatgatatcaatgttggcacaacacaggcacacgtgcatacacttcctcaggattacaagctcctcccgcgttagaaccatatcccagggaacaacccattcctgaatcagcgtaaatcccacactgcagggaagacctcgcacgtaactcacgttgtgcattgtcaaagtgttacattcgggcagcagcggatgatcctccagtatggtagcgcgggtttctgtctcaaaaggaggtagacgatccctactgtacggagtgcgccgagacaaccgagatcgtgttggtcgtagtgtcatgccaaatggaacgccggacgtagtcatatttcctgaagcaaaaccaggtgcgggcgtgacaaacagatctgcgtctccggtctcgccgcttagatcgctctgtgtagtagttgtagtatatccactctctcaaagcatccaggcgccccctggcttcgggttctatgtaaactccttcatgcgccgctgccctgataacatccaccaccgcagaataagccacacccagccaacctacacattcgttctgcgagtcacacacgggaggagcgggaagagctggaagaaccatgtttttttttttattccaaaagattatccaaaacctcaaaatgaagatctattaagtgaacgcgctcccctccggtggcgtggtcaaactctacagccaaagaacagataatggcatttgtaagatgttgcacaatggcttccaaaaggcaaacggccctcacgtccaagtggacgtaaaggctaaacccttcagggtgaatctcctctataaacattccagcaccttcaaccatgcccaaataattctcatctcgccaccttctcaatatatctctaagcaaatcccgaatattaagtccggccattgtaaaaatctgctccagagcgccctccaccttcagcctcaagcagcgaatcatgattgcaaaaattcaggttcctcacagacctgtataagattcaaaagcggaacattaacaaaaataccgcgatcccgtaggtcccttcgcagggccagctgaacataatcgtgcaggtctgcacggaccagcgcggccacttccccgccaggaaccatgacaaaagaacccacactgattatgacacgcatactcggagctatgctaaccagcgtagccccgatgtaagcttgttgcatgggcggcgatataaaatgcaaggtgctgctcaaaaaatcaggcaaagcctcgcgcaaaaaagaaagcacatcgtagtcatgctcatgcagataaaggcaggtaagctccggaaccaccacagaaaaagacaccatttttctctcaaacatgtctgcgggtttctgcataaacacaaaataaaataacaaaaaaacatttaaacattagaagcctgtcttacaacaggaaaaacaacccttataagcataagacggactacggccatgccggcgtgaccgtaaaaaaactggtcaccgtgattaaaaagcaccaccgacagctcctcggtcatgtccggagtcataatgtaagactcggtaaacacatcaggttgattcacatcggtcagtgctaaaaagcgaccgaaatagcccgggggaatacatacccgcaggcgtagagacaacattacagcccccataggaggtataacaaaattaataggagagaaaaacacataaacacctgaaaaaccctcctgcctaggcaaaatagcaccctcccgctccagaacaacatacagcgcttccacagcggcagccataacagtcagccttaccagtaaaaaagaaaacctattaaaaaaacaccactcgacacggcaccagctcaatcagtcacagtgtaaaaaagggccaagtgcagagcgagtatatataggactaaaaaatgacgtaacggttaaagtccacaaaaaacacccagaaaaccgcacgcgaacctacgcccagaaacgaaagccaaaaaacccacaacttcctcaaatcgtcacttccgttttcccacgttacgtcacttcccattttaagaaaactacaattcccaacacatacaagttactccgccctaaaacctacgtcacccgccccgttcccacgccccgcgccacgtcacaaactccaccccctcattatcatattggcttcaatccaaaataaggta

SEQ ID NO: 223 - DNA, 9701 bp, synthetic construct
  misc_feature 1..9701: note = vector for IgG1 against T27Y H34A R273L ACE2 mutant
  misc_feature 2929..2930: note = n is a, c, g, or t
  misc_feature 2934: note = n is a, c, g, or t
  source 1..9701: mol_type = other DNA
ggcgtaatctgctgcttgcaaacaaaaaaaccaccgctaccagcggtggtttgtttgccggatcaagagctaccaactctttttccgaaggtaactggcttcagcagagcgcagataccaaatactgtccttctagtgtagccgtagttaggccaccacttcaagaactctgtagcaccgcctacatacctcgctctgctgaagccagttaccagtggctgctgccagtggcgataagtcgtgtcttaccgggttggactcaagagatagttaccggataaggcgcagcggtcgggctgaacggggggttcgtgcacacagcccagcttggagcgaacgacctacaccgaactgagatacctacagcgtgagctatgagaaagcgccacgcttcccgaagggagaaaggcggacaggtatccggtaagcggcagggtcggaacaggagagcgcacgagggagcttccagggggaaacgcctggtatctttatagtcctgtcgggtttcgccacctctgacttgagcgtcgatttttgtgatgctcgtcaggggggcggagcctatggaaaaacgccagcaacgcaagctagagtttaaacttgacagatgagacaataaccctgataaatgcttcaataatattgaaaaaggaaaagtatgagtattcaacatttccgtgtcgcccttattcccttttttgcggcattttgccttcctgtttttgctcacccagaaacgctggtgaaagtaaaagatgcagaagatcacttgggtgcgcgagtgggttacatcgaactggatctcaacagcggtaagatccttgagagttttcgccccgaagaacgtttcccaatgatgagcacttttaaagttctgctatgtggcgcggtattatcccgtattgatgccgggcaagagcaactcggtcgccgcatacactattctcagaatgacttggttgaatactcaccagtcacagaaaagcatcttacggatggcatgacagtaagagaattatgcagtgctgccataaccatgagtgataacactgcggccaacttacttctgacaactatcggaggaccgaaggagctaaccgcttttttgcacaacatgggggatcatgtaactcgccttgatcgttgggaaccggagctgaatgaagccataccaaacgacgagcgtgacaccacgatgcctgtagcaatggcaacaacgttgcgaaaactattaactggcgaactacttactctagcttcccggcaacaactaatagactggatggaggcggataaagttgcaggaccacttctgcgctcggcacttccggctggctggtttattgctgataaatcaggagccggtgagcgtgggtcacgcggtatcattgcagcactggggccggatggtaagccctcccgtatcgtagttatctacactacggggagtcaggcaactatggatgaacgaaatagacagatcgctgagataggtgcctcactgattaagcattggtaaggataaatttctggtaaggaggacacgtatggaagtgggcaagttggggaagccgtatccgttgctgaatctggcatatgtgggagtataagacgcgcagcgtcgcatcaggcatttttttctgcgccaatgcaaaaaggccatccgtcaggatggcctttcggcataactagggccgccgatatttgaaaatatggcatattgaaaatgtcgccgatgtgagtttctgtgtaactgatatcgccatttttccaaaagtgatttttgggcatacgcgatatctggcgatagcgcttatatcgtttacgggggatggcgatagacgactttggtgacttgggcgattctgtgtgtcgcaaatatcgcagtttcgatataggtgacagacgatatgaggctatatcgccgatagaggcgacatcaagctggcacatggccaatgcatatcgatctatacattgaatcaatattggccattagccatattattcattggttatatagcataaatcaatattggctattggccattgcatacgttgtatccatatcataatatgtacatttatattggctcatgtccaacattaccgccatgttgacattgattattgactagttattaatagtaatcaattacggggtcattagttcatagcccatatatggagttccgcgttacataacttacggtaaatggcccgcctggctgaccgcccaacgacccccgcccattgacgtcaataatgacgtatgttcccatagtaacgccaatagggactttccattgacgtcaatgggtggagtatttacggtaaactgcccacttggcagtacatcaagtgtatcatatgccaagtacgccccctattgacgtcaatgacggtaaatggcccgcctggcattatgcccagtacatgaccttatgggactttcctacttggcagtacatctacgtattagtcatcgctattaccatggtgatgcggttttggcagtacatcaatgggcgtggatagcggtttgactcacggggatttccaagtctccaccccattgacgtcaatgggagtttgttttggcaccaaaatcaacgggactttccaaaatgtcgtaacaactccgccccattgacgcaaatgggcggtaggcgtgtacggtgggaggtctatataagcagagctcgtttagtgaaccgtcagatcgcctggagacgccatccacgctgttttgacctccatagaagacaccgggaccgatccagcctccgcggccgggaacggtgcattggaacgcggattccccgtgccaagagtgacgtaagtaccgcctatagagtctataggcccacccccttggcttcttatgcatgctatactgtttttggcttggggtctatacaccccccgnnttcntcatgttataggtgatggtatagcttagcctataggtgtgggttattgaccattattgaccactccccctattggtgacgatactttccattactaatccataacatggctctttgccacaactctctttattggctatatgccaatacactgtccttcagagactgacacggactctgtatttttacaggatggggtctcatttattatttacaaattcacatatacaacaccaccgtccccagtgcccgcagtttttattaaacataacgtgggatctccacgcgaatctcgggtacgtgttccggacatgggctcttctccggtagcggcggagcttctacatccgagccctgctcccatgcctccagcgactcatggtcgctcggcagctccttgctcctaacagtggaggccagacttaggcacagcacgatgcccaccaccaccagtgtgccgcacaaggccgtggcggtagggtatgtgtctgaaaatgagctcggggagcgggcttgcaccgctgacgcatttggaagacttaaggcagcggcagaagaagatgcaggcagctgagttgttgtgttctgataagagtcagaggtaactcccgttgcggtgctgttaacggtggagggcagtgtagtctgagcagtactcgttgctgccgcgcgcgccaccagacataatagctgacagactaacagactgttcctttccatgggtcttttctgcagtcaccgtccttgacacgaagctgctagcgccaccatgagcagcagtagttggcttctcttgagtttggtggcagtgacagcagcccagagtactatcgaggagcaggctaaatactttctggataagtttaacgccgaggccgaagacttgttctatcaatcttctctcgcttcatggaattacaatactaacatcactgaggagaacgtccagaatatgaacaatgctggcgacaaatggagcgccttcttgaaggagcagtctacccttgcacaaatgtatccactgcaggagatacagaaccttacagtaaagttgcagctccaggctctccagcagaacggatctagcgtgctttcagaggataaaagcaaaaggctgaacaccatacttaataccatgtccacaatttactctactggtaaagtatgtaaccccgacaaccctcaagaatgcctccttcttgagccaggcctcaatgagatcatggctaatagtctggactataatgaaagactgtgggcatgggagtcctggagatctgaagtagggaagcaactgaggcccctttatgaagagtacgtcgtacttaagaatgaaatggcccgcgctaaccactacgaggattacggcgattactggcgtggggactatgaagtaaatggtgtagatggatacgactatagtcgtgggcaattgattgaggatgtggagcacacttttgaggagataaaaccactctatgagcatcttcacgcatatgtgagagctaaactgatgaacgcctacccaagttacatcagtccaatcggatgtctcccagctcacctccttggcgacatgtggggactgttctggaccaatctgtattccctcacagtccctttcgggcaaaagcctaatatagacgtgacagacgcaatggttgatcaggcttgggatgctcaaaggatttttaaggaagctgagaagttttttgtgtcagtcggtttgccaaatatgacacaaggcttctgggaaaatagcatgttgactgatcccggtaatgttcaaaaggctgtgtgtcaccctaccgcttgggaccttgggaaaggtgactttcgaatcttgatgtgtaccaaggtgacaatggatgactttcttacagcccatcatgaaatgggtcacatccagtatgatatggcttatgcagctcaacctttcctcttgagaaatggtgcaaatgaaggttttcatgaagctgtaggggaaataatgtccctgagtgctgcaaccccaaagcatctcaagagtatcggattgttgagcccagattttcaagaagataacgagaccgaaatcaacttccttctgaaacaagccctcacaatagttggtactcttccattcacatacatgctggagaaatggcgttggatggtttttaagggggagatacctaaagatcagtggatgaaaaagtggtgggagatgaagcgtgagatcgtaggggtcgtggagccagtgcctcatgatgagacttactgtgacccagcatcactcttccacgttagcaatgactattcatttatacgttattacactcgcactctttaccagtttcaatttcaggaggctctgtgtcaggctgccaagcatgagggaccccttcacaagtgtgatattagtaacagtactgaggcaggccaaaaactgttcaatatgttgaggcttggcaaaagcgagccatggactctcgccttggaaaatgttgtcggggctaaaaacatgaatgtacgccctctgcttaactattttgagcccctttttacatggctcaaggaccagaataagaactcctttgtcggctggtcaacagactggtctccctatgcagacaaaacacatacttgcccaccttgtcctgcaccagagctgctgggaggtccaagcgtgttcctgtttccacccaagcccaaagacacactgatgatttctcgaactccagaagtgacctgcgtggtcgtggacgtgagccacgaggatcccgaagtgaagttcaactggtacgtggatggcgtggaggtccataatgctaagactaaaccccgggaggaacagtacaacagcacttatagggtcgtgtccgtgctgaccgtcctgcatcaggattggctgaacgggaaggaatataagtgcaaagtgtctaataaggcactgcccgcccctatcgagaaaacaattagcaaggctaagggtcagcctagagaaccacaggtgtacactctgcctccaagtcgcgacgagctgaccaagaaccaggtgtcactgacatgtctggtcaaaggcttttatccctcagatatcgcagtggagtgggaaagcaatggacagcctgagaacaattacaagaccacaccccctgtgctggacagtgatggctcattctttctgtattctaagctgacagtggacaaaagtaggtggcagcagggaaacgtgttctcctgctctgtcatgcacgaagcactgcacaatcattatacccagaagagtctgtcactgagccctggcaaatgagcgataccgattctagaactagatcataatcagccataccacatttgtagaggttttacttgctttaaaaaacctcccacacctccccctgaacctgaaacataaaatgaatgcaattgttgttgttaacttgtttattgcagcttataatggttacaaataaagcaatagcatcacaaatttcacaaataaagcatttttttcactgcattctagttgtggtttgtccaaactcatcaatgtatcttaaggccgcaggtaagccagcccaggcctcgccctccagctcaaggcgggacaggtgccctagagtagcctgcatccagggacaggccccagccgggtgctgacacgtccacctccatctcttcctcaggtctgcccgggtggcatccctgtgacccctccccagtgcctctcctggtcgtggaaggtgctactccagtgcccaccagccttgtcctaataaaattaagttgcatcattttgtttgactaggtgtccttgtataatattatggggtggaggcgggtggtatggagcaaggggcccaagttaacttgtttattgcagcttataatggttacaaataaagcaatagcatcacaaatttcacaaataaagcatttttttcactgcattctagttgtggtttgtccaaactcatcaatgtatcttatcatgtctggatccgcttcaggcaccgggcttgcgggtcatgcaccaggtgcgcggtccttcgggcacctcgacgtcggcggtgacggtgaagccgagccgctcgtagaaggggaggttgcggggcgcggaggtctccaggaaggcgggcaccccggcgcgctcggccgcctccactccggggagcacgacggcgctgcccagacccttgccctggtggtcgggcgagacgccgacggtggccaggaaccacgcgggctccttgggccggtgcggcgccaggaggccttccatctgttgctgcgcggccagcctggaaccgctcaactcggccatgcgcgggccgatctcggcgaacaccgcccccgcttcgacgctctccggcgtggtccagaccgccaccgcggcgccgtcgtccgcgacccacaccttgccgatgtcgagcccgacgcgcgtgaggaagagttcttgcagctcggtgacccgctcgatgtggcggtccgggtcgacggtgtggcgcgtggcggggtagtcggcgaacgcggcggcgagggtgcgtacggcccgggggacgtcgtcgcgggtggcgaggcgcaccgtgggcttgtactcggtcatggtggcctgcagagtcgctctgtgttcgaggccacacgcgtcaccttaatatgcgaagtggacctgggaccgcgccgccccgactgcatctgcgtgttttcgccaatgacaagacgctgggcggggtttgtgtcatcatagaactaaagacatgcaaatatatttcttccggggacaccgccagcaaacgcgagcaacgggccacggggatgaagcagctgcgccactccctgaagatccatcgtctcctaacaagttacatcactcctgcccttcctcaccctcatctccatcacctccttcatctccgtcatctccgtcatcaccctccgcggcagccccttccaccataggtggaaaccagggaggcaaatctactccatcgtcaaagctgcacacagtcaccctgatattgcaggtaggagcgggctttgtcataacaaggtccttaatcgcatccttcaaaacctcagcaaatatatgagtttgtaaaaagaccatgaaataacagacaatggactcccttagcgggccaggttgtgggccgggtccaggggccattccaaaggggagacgactcaatggtgtaagacgacattgtggaatagcaagggcagttcctcgccttaggttgtaaagggaggtcttactacctccatatacgaacacaccggcgacccaagttccttcgtcggtagtcctttctacgtgactcctagccaggagagctcttaaaccttctgcaatgttctcaaatttcgggttggaacctccttgaccacgatgctttccaaaccaccctccttttttgcgcctgcctccatcaccctgacccccgctgcgcgggggcacgtcaggctcaccatctgggccgccttcttggtggtattcaaaataatcggcttcccctacagggtggaaaaatggccttctacctggagggggcctgcgcggtggagacccggatgatgatgactgactactgggactcctgggcctcttttctccacgtccacgacctctccccctggctctttcacgacttccccccctggctctttcacgtcctctaccccggcggcctccactacctcctcgaccccggcctccactacctcctcgaccccggcctccactgcctcctcgaccccggcctccacctcctgctcctgcccctcccgctcctgctcctgctcctgttccaccgtgggtccctttgcagccaatgcaacttggacgtttttggggtctccggacaccatctctatgtcttggccctgatcctgagccgcccggggctcctggtcttccgcctcctcgtcctcgtcctcttccccgtcctcgtccatgtgccatgatggcggcctgcagctgtgttcgaggccgcgcgtgtcaccttaatatgcgaagtggacctgggaccgcgccgccccgactgcatctgcgtgttcgagttcgccaatgacaagacgctgggcggggagatcccccttattaaccctaaacgggtagcatatgcttcccgggtagtagtatatactatccagactaaccctaattcaatagcatatgttacccaacgggaagcatatgctatcgaattagggttagtaaaagggtcctaaggaacagcgatctggatagcatatgctatcctaatctatatctgggtagcatatgctatcctaatctatatctgggtagcataggctatcctaatctatatctgggtagcatatgctatcctaatctatatctgggtagtatatgctatcctaatttatatctgggtagcataggctatcctaatctatatctgggtagcatatgctatcctaatctatatctgggtagtatatgctatcctaatctgtatccgggtagcatatgctatcctcatgcatatacagtcagcatatgatacccagtagtagagtgggagtgctatcctttgcatatgccgccacctcccaaggagatctgtcgacatcgatgggcgcgggtgtacactccgcccatcccgcccctaactccgcccagttccgcccattctccgcctcatggctgactaattttttttatttatgcagaggccgaggccgcctcggcctctgagctattccagaagtagtgaggaggcttttttggaggcctaggcttttgcaaaaagctaattc

SEQ ID NO: 224 - DNA, 38496 bp, synthetic construct
  misc_feature 1..38496: note = vector for IgA against T27Y H34A H505L ACE2 mutant
  source 1..38496: mol_type = other DNA
tattattgatgatgttaattaacatgcatggatcctacgtctcgaccgatgcccttgagagccttcaacccagtcagctccttccggtgggcgcggggcatgactatcgtcgccgcacttatgactgtcttctttatcatgcaactcgtaggacaggtgccggcagcgctctgggtcattttcggcgaggaccgctttcgctggagcgcgacgatgatcggcctgtcgcttgcggtattcggaatcttgcacgccctcgctcaagccttcgtcactggtcccgccaccaaacgtttcggcgagaagcaggccattatcgccggcatggcggccgacgcgctgggctacgtcttgctggcgttcgcgacgcgaggctggatggccttccccattatgattcttctcgcttccggcggcatcgggatgcccgcgttgcaggccatgctgtccaggcaggtagatgacgaccatcagggacagcttcaaggatcgctcgcggctcttaccagcctaacttcgatcattggaccgctgatcgtcacggcgatttatgccgcctcggcgagcacatggaacgggttggcatggattgtaggcgccgccctataccttgtctgcctccccgcgttgcgtcgcggtgcatggagccgggccacctcgacctgaatggaagccggcggcacctcgctaacggattcaccactccaagaattggagccaatcaattcttgcggagaactgtgaatgcgcaaaccaacccttggcagaacatatccatcgcgtccgccatctccagcagccgcacgcggcgcatctcgggcagcgttgggtcctggccacgggtgcgcatgatcgtgctcctgtcgttgaggacccggctaggctggcggggttgccttactggttagcagaatgaatcaccgatacgcgagcgaacgtgaagcgactgctgctgcaaaacgtctgcgacctgagcaacaacatgaatggtcttcggtttccgtgtttcgtaaagtctggaaacgcggaagtcagcgccctgcaccattatgttccggatctgcatcgcaggatgctgctggctaccctgtggaacacctacatctgtattaacgaagcgctggcattgaccctgagtgatttttctctggtcccgccgcatccataccgccagttgtttaccctcacaacgttccagtaaccgggcatgttcatcatcagtaacccgtatcgtgagcatcctctctcgtttcatcggtatcattacccccatgaacagaaatcccccttacacggaggcatcagtgaccaaacaggaaaaaaccgcccttaacatggcccgctttatcagaagccagacattaacgcttctggagaaactcaacgagctggacgcggatgaacaggcagacatctgtgaatcgcttcacgaccacgctgatgagctttaccgcagctgcctcgcgcgtttcggtgatgacggtgaaaacctctgacacatgcagctcccggagacggtcacagcttgtctgtaagcggatgccgggagcagacaagcccgtcagggcgcgtcagcgggtgttggcgggtgtcggggcgcagccatgacccagtcacgtagcgatagcggagtgtatactggcttaactatgcggcatcagagcagattgtactgagagtgcaccatatgcggtgtgaaataccgcacagatgcgtaaggagaaaataccgcatcaggcgctcttccgcttcctcgctcactgactcgctgcgctcggtcgttcggctgcggcgagcggtatcagctcactcaaaggcggtaatacggttatccacagaatcaggggataacgcaggaaagaacatgtgagcaaaaggccagcaaaaggccaggaaccgtaaaaaggccgcgttgctggcgtttttccataggctccgcccccctgacgagcatcacaaaaatcgacgctcaagtcagaggtggcgaaacccgacaggactataaagataccaggcgtttccccctggaagctccctcgtgcgctctcctgttccgaccctgccgcttaccggatacctgtccgcctttctcccttcgggaagcgtggcgctttctcatagctcacgctgtaggtatctcagttcggtgtaggtcgttcgctccaagctgggctgtgtgcacgaaccccccgttcagcccgaccgctgcgccttatccggtaactatcgtcttgagtccaacccggtaagacacgacttatcgccactggcagcagccactggtaacaggattagcagagcgaggtatgtaggcggtgctacagagttcttgaagtggtggcctaactacggctacactagaaggacagtatttggtatctgcgctctgctgaagccagttaccttcggaaaaagagttggtagctcttgatccggcaaacaaaccaccgctggtagcggtggtttttttgtttgcaagcagcagattacgcgcagaaaaaaaggatctcaagaagatcctttgatcttttctacggggtctgacgctcagtggaacgaaaactcacgttaagggattttggtcatgagattatcaaaaaggatcttcacctagatccttttaaattaaaaatgaagttttaaatcaatctaaagtatatatgagtaaacttggtctgacagttaccaatgcttaatcagtgaggcacctatctcagcgatctgtctatttcgttcatccatagttgcctgactccccgtcgtgtagataactacgatacgggagggcttaccatctggccccagtgctgcaatgataccgcgagacccacgctcaccggctccagatttatcagcaataaaccagccagccggaagggccgagcgcagaagtggtcctgcaactttatccgcctccatccagtctattaattgttgccgggaagctagagtaagtagttcgccagttaatagtttgcgcaacgttgttgccattgctgcagccatgagattatcaaaaaggatcttcacctagatccttttcacgtagaaagccagtccgcagaaacggtgctgaccccggatgaatgtcagctactgggctatctggacaagggaaaacgcaagcgcaaagagaaagcaggtagcttgcagtgggcttacatggcgatagctagactgggcggttttatggacagcaagcgaaccggaattgccagctggggcgccctctggtaaggttgggaagccctgcaaagtaaactggatggctttcttgccgccaaggatctgatggcgcaggggatcaagctctgatcaagagacaggatgaggatcgtttcgcatgattgaacaagatggattgcacgcaggttctccggccgcttgggtggagaggctattcggctatgactgggcacaacagacaatcggctgctctgatgccgccgtgttccggctgtcagcgcaggggcgcccggttctttttgtcaagaccgacctgtccggtgccctgaatgaactgcaagacgaggcagcgcggctatcgtggctggccacgacgggcgttccttgcgcagctgtgctcgacgttgtcactgaagcgggaagggactggctgctattgggcgaagtgccggggcaggatctcctgtcatctcaccttgctcctgccgagaaagtatccatcatggctgatgcaatgcggcggctgcatacgcttgatccggctacctgcccattcgaccaccaagcgaaacatcgcatcgagcgagcacgtactcggatggaagccggtcttgtcgatcaggatgatctggacgaagagcatcaggggctcgcgccagccgaactgttcgccaggctcaaggcgagcatgcccgacggcgaggatctcgtcgtgacccatggcgatgcctgcttgccgaatatcatggtggaaaatggccgcttttctggattcatcgactgtggccggctgggtgtggcggaccgctatcaggacatagcgttggctacccgtgatattgctgaagagcttggcggcgaatgggctgaccgcttcctcgtgctttacggtatcgccgctcccgattcgcagcgcatcgccttctatcgccttcttgacgagttcttctgaattttgttaaaatttttgttaaatcagctcattttttaaccaataggccgaaatcggcaaaatcccttataaatcaaaagaatagaccgagatagggttgagtgttgttccagtttggaacaagagtccactattaaagaacgtggactccaacgtcaaagggcgaaaaaccgtctatcagggcgatggcccactacgtgaaccatcaccctaatcaagttttttggggtcgaggtgccgtaaagcactaaatcggaaccctaaagggagcccccgatttagagcttgacggggaaagccggcgaacgtggcgagaaaggaagggaagaaagcgaaaggagcgggcgctagggcgctggcaagtgtagcggtcacgctgcgcgtaaccaccacacccgccgcgcttaatgcgccgctacagggcgcgtccattcgccattcaggatcgaattaattcttaattaacatcatcaataatataccttattttggattgaagccaatatgataatgagggggtggagtttgtgacgtggcgcggggcgtgggaacggggcgggtgacgtagtagtgtggcggaagtgtgatgttgcaagtgtggcggaacacatgtaagcgacggatgtggcaaaagtgacgtttttggtgtgcgccggtgtacacaggaagtgacaattttcgcgcggttttaggcggatgttgtagtaaatttgggcgtaaccgagtaagatttggccattttcgcgggaaaactgaataagaggaagtgaaatctgaataattttgtgttactcatagcgcgtaatactgtaatagtaatcaattacggggtcattagttcatagcccatatatggagttccgcgttacataacttacggtaaatggcccgcctggctgaccgcccaacgacccccgcccattgacgtcaataatgacgtatgttcccatagtaacgccaatagggactttccattgacgtcaatgggtggagtatttacggtaaactgcccacttggcagtacatcaagtgtatcatatgccaagtacgccccctattgacgtcaatgacggtaaatggcccgcctggcattatgcccagtacatgaccttatgggactttcctacttggcagtacatctacgtattagtcatcgctattaccatggtgatgcggttttggcagtacatcaatgggcgtggatagcggtttgactcacggggatttccaagtctccaccccattgacgtcaatgggagtttgttttggcaccaaaatcaacgggactttccaaaatgtcgtaacaactccgccccattgacgcaaatgggcggtaggcgtgtacggtgggaggtctatataagcagagctggtttagtgaaccgtcagatccgctagagatctggtaccgtcgacgcggccgctcgagcctaagcttatgagcagcagtagttggcttctcttgagtttggtggcagtgacagcagcccagagtactatcgaggagcaggctaaatactttctggataagtttaacgccgaggccgaagacttgttctatcaatcttctctcgcttcatggaattacaatactaacatcactgaggagaacgtccagaatatgaacaatgctggcgacaaatggagcgccttcttgaaggagcagtctacccttgcacaaatgtatccactgcaggagatacagaaccttacagtaaagttgcagctccaggctctccagcagaacggatctagcgtgctttcagaggataaaagcaaaaggctgaacaccatacttaataccatgtccacaatttactctactggtaaagtatgtaaccccgacaaccctcaagaatgcctccttcttgagccaggcctcaatgagatcatggctaatagtctggactataatgaaagactgtgggcatgggagtcctggagatctgaagtagggaagcaactgaggcccctttatgaagagtacgtcgtacttaagaatgaaatggcccgcgctaaccactacgaggattacggcgattactggcgtggggactatgaagtaaatggtgtagatggatacgactatagtcgtgggcaattgattgaggatgtggagcacacttttgaggagataaaaccactctatgagcatcttcacgcatatgtgagagctaaactgatgaacgcctacccaagttacatcagtccaatcggatgtctcccagctcacctccttggcgacatgtggggacgtttctggaccaatctgtattccctcacagtccctttcgggcaaaagcctaatatagacgtgacagacgcaatggttgatcaggcttgggatgctcaaaggatttttaaggaagctgagaagttttttgtgtcagtcggtttgccaaatatgacacaaggcttctgggaaaatagcatgttgactgatcccggtaatgttcaaaaggctgtgtgtcaccctaccgcttgggaccttgggaaaggtgactttcgaatcttgatgtgtaccaaggtgacaatggatgactttcttacagcccatcatgaaatgggtcacatccagtatgatatggcttatgcagctcaacctttcctcttgagaaatggtgcaaatgaaggttttcatgaagctgtaggggaaataatgtccctgagtgctgcaaccccaaagcatctcaagagtatcggattgttgagcccagattttcaagaagataacgagaccgaaatcaacttccttctgaaacaagccctcacaatagttggtactcttccattcacatacatgctggagaaatggcgttggatggtttttaagggggagatacctaaagatcagtggatgaaaaagtggtgggagatgaagcgtgagatcgtaggggtcgtggagccagtgcctcatgatgagacttactgtgacccagcatcactcttcctggttagcaatgactattcatttatacgttattacactcgcactctttaccagtttcaatttcaggaggctctgtgtcaggctgccaagcatgagggaccccttcacaagtgtgatattagtaacagtactgaggcaggccaaaaactgttcaatatgttgaggcttggcaaaagcgagccatggactctcgccttggaaaatgttgtcggggctaaaaacatgaatgtacgccctctgcttaactattttgagcccctttttacatggctcaaggaccagaataagaactcctttgtcggctggtcaacagactggtctccctatgcagaccctagtactcctcctactccttctccatcaaccccaccaactccatcccctagctgctgtcacccaaggctgtctctgcaccgacctgcactcgaagaccttctgttgggctctgaagctaacctgacctgtactcttactggcttgcgcgatgctagcggcgtgactttcacctggacacctagtagcggtaaaagtgctgtacaaggacctcctgaacgcgacctgtgtggttgctactctgtgtcttctgtacttcccggctgtgccgagccctggaatcacgggaaaacctttacctgcaccgccgcttaccctgagtcaaaaactcccctcactgccacattgagtaagtcagggaatacattcaggccagaggttcatttgttgcctcctccatctgaagaacttgctttgaacgagctggtcactctgacctgcttggctaggggtttctcccccaaagatgtacttgtacggtggttgcagggcagccaagagttgccccgcgaaaagtatttgacctgggcctcaagacaagaacccagccaggggactaccacatttgccgtgaccagtattctgcgtgtagccgctgaagattggaagaaaggggatacattttcttgcatggtagggcatgaggcccttcccctcgctttcactcagaagacaatagacagactcgccggaaagcctactcacgtgaatgttagcgtagtcatggctgaggttgacggaacttgctactgagatatccgatccaccggatctagataactgatcataatcagccataccacatttgtagaggttttacttgctttaaaaaacctcccacacctccccctgaacctgaaacataaaatgaatgcaattgttgttgttaacttgtttattgcagcttataatggttacaaataaagcaatagcatcacaaatttcacaaataaagcatttttttcactgcattctagttgtggtttgtccaaactcatcaatgtatcttaggtttagtgaaccgtcagatccgctagcgttacataacttacggtaaatggcccgcctggctgaccgcccaacgacccccgcccattgacgtcaataatgacgtatgttcccatagtaacgccaatagggactttccattgacgtcaatgggtggagtatttacggtaaactgcccacttggcagtacatcaagtgtatcatatgccaagtacgccccctattgacgtcaatgacggtaaatggcccgcctggcattatgcccagtacatgaccttatgggactttcctacttggcagtacatctacgtattagtcatcgctattaccatggtgatgcggttttggcagtacatcaatgggcgtggatagcggtttgactcacggggatttccaagtctccaccccattgacgtcaatgggagtttgttttggcaccaaaatcaacgggactttccaaaatgtcgtaacaactccgccccattgacgcaaatgggcggtaggcgtgtacggtgggaggtctatataagcagagctggtttagtgaaccgtcagatccgctagagatctggtaccgtcgacgcggccgctcgagcctaagcttatgaagaaccatctgcttttctggggagtacttgccgttttcataaaagccgtacatgttaaagcacaagaggacgaacgcattgtgttggttgataataaatgcaaatgtgctcggataacatctcggatcattcgtagctcagaggaccccaatgaggatatagtagagcgaaacatcagaattatagtacccctgaacaacagagagaacataagtgatcccacaagtccattgcggacacgctttgtttaccatttgtctgatctgtgtaaaaaatgtgatccaacagaggtggaactcgacaatcagatcgtcaccgccacccagtctaacatctgcgatgaagattcagctacagagacatgctacacatacgaccggaacaagtgctatactgccgttgtgccactcgtttacggtggagaaacaaagatggttgaaactgcacttacaccagatgcctgctatccagattgagatatccgatccaccggatctagataactgatcataatcagccataccacatttgtagaggttttacttgctttaaaaaacctcccacacctccccctgaacctgaaacataaaatgaatgcaattgttgttgttaacttgtttattgcagcttataatggttacaaataaagcaatagcatcacaaatttcacaaataaagcatttttttcactgcattctagttgtggtttgtccaaactcatcaatgtatcttaacgcggatctgggcgtggttaagggtgggaaagaatatataaggtgggggtcttatgtagttttgtatctgttttgcagcagccgccgccgccatgagcaccaactcgtttgatggaagcattgtgagctcatatttgacaacgcgcatgcccccatgggccggggtgcgtcagaatgtgatgggctccagcattgatggtcgccccgtcctgcccgcaaactctactaccttgacctacgagaccgtgtctggaacgccgttggagactgcagcctccgccgccgcttcagccgctgcagccaccgcccgcgggattgtgactgactttgctttcctgagcccgcttgcaagcagtgcagcttcccgttcatccgcccgcgatgacaagttgacggctcttttggcacaattggattctttgacccgggaacttaatgtcgtttctcagcagctgttggatctgcgccagcaggtttctgccctgaaggcttcctcccctcccaatgcggtttaaaacataaataaaaaaccagactctgtttggatttggatcaagcaagtgtcttgctgtctttatttaggggttttgcgcgcgcggtaggcccgggaccagcggtctcggtcgttgagggtcctgtgtattttttccaggacgtggtaaaggtgactctggatgttcagatacatgggcataagcccgtctctggggtggaggtagcaccactgcagagcttcatgctgcggggtggtgttgtagatgatccagtcgtagcaggagcgctgggcgtggtgcctaaaaatgtctttcagtagcaagctgattgccaggggcaggcccttggtgtaagtgtttacaaagcggttaagctgggatgggtgcatacgtggggatatgagatgcatcttggactgtatttttaggttggctatgttcccagccatatccctccggggattcatgttgtgcagaaccaccagcacagtgtatccggtgcacttgggaaatttgtcatgtagcttagaaggaaatgcgtggaagaacttggagacgcccttgtgacctccaagattttccatgcattcgtccataatgatggcaatgggcccacgggcggcggcctgggcgaagatatttctgggatcactaacgtcatagttgtgttccaggatgagatcgtcataggccatttttacaaagcgcgggcggagggtgccagactgcggtataatggttccatccggcccaggggcgtagttaccctcacagatttgcatttcccacgctttgagttcagatggggggatcatgtctacctgcggggcgatgaagaaaacggtttccggggtaggggagatcagctgggaagaaagcaggttcctgagcagctgcgacttaccgcagccggtgggcccgtaaatcacacctattaccggctgcaactggtagttaagagagctgcagctgccgtcatccctgagcaggggggccacttcgttaagcatgtccctgactcgcatgttttccctgaccaaatccgccagaaggcgctcgccgcccagcgatagcagttcttgcaaggaagcaaagtttttcaacggtttgagaccgtccgccgtaggcatgcttttgagcgtttgaccaagcagttccaggcggtcccacagctcggtcacctgctctacggcatctcgatccagcatatctcctcgtttcgcgggttggggcggctttcgctgtacggcagtagtcggtgctcgtccagacgggccagggtcatgtctttccacgggcgcagggtcctcgtcagcgtagtctgggtcacggtgaaggggtgcgctccgggctgcgcgctggccagggtgcgcttgaggctggtcctgctggtgctgaagcgctgccggtcttcgccctgcgcgtcggccaggtagcatttgaccatggtgtcatagtccagcccctccgcggcgtggcccttggcgcgcagcttgcccttggaggaggcgccgcacgaggggcagtgcagacttttgagggcgtagagcttgggcgcgagaaataccgattccggggagtaggcatccgcgccgcaggccccgcagacggtctcgcattccacgagccaggtgagctctggccgttcggggtcaaaaaccaggtttcccccatgctttttgatgcgtttcttacctctggtttccatgagccggtgtccacgctcggtgacgaaaaggctgtccgtgtccccgtatacagacttgagaggcctgtcctcgagcggtgttccgcggtcctcctcgtatagaaactcggaccactctgagacaaaggctcgcgtccaggccagcacgaaggaggctaagtgggaggggtagcggtcgttgtccactagggggtccactcgctccagggtgtgaagacacatgtcgccctcttcggcatcaaggaaggtgattggtttgtaggtgtaggccacgtgaccgggtgttcctgaaggggggctataaaagggggtgggggcgcgttcgtcctcactctcttccgcatcgctgtctgcgagggccagctgttggggtgagtactccctctgaaaagcgggcatgacttctgcgctaagattgtcagtttccaaaaacgaggaggatttgatattcacctggcccgcggtgatgcctttgagggtggccgcatccatctggtcagaaaagacaatctttttgttgtcaagcttggtggcaaacgacccgtagagggcgttggacagcaacttggcgatggagcgcagggtttggtttttgtcgcgatcggcgcgctccttggccgcgatgtttagctgcacgtattcgcgcgcaacgcaccgccattcgggaaagacggtggtgcgctcgtcgggcaccaggtgcacgcgccaaccgcggttgtgcagggtgacaaggtcaacgctggtggctacctctccgcgtaggcgctcgttggtccagcagaggcggccgcccttgcgcgagcagaatggcggtagggggtctagctgcgtctcgtccggggggtctgcgtccacggtaaagaccccgggcagcaggcgcgcgtcgaagtagtctatcttgcatccttgcaagtctagcgcctgctgccatgcgcgggcggcaagcgcgcgctcgtatgggttgagtgggggaccccatggcatggggtgggtgagcgcggaggcgtacatgccgcaaatgtcgtaaacgtagaggggctctctgagtattccaagatatgtagggtagcatcttccaccgcggatgctggcgcgcacgtaatcgtatagttcgtgcgagggagcgaggaggtcgggaccgaggttgctacgggcgggctgctctgctcggaagactatctgcctgaagatggcatgtgagttggatgatatggttggacgctggaagacgttgaagctggcgtctgtgagacctaccgcgtcacgcacgaaggaggcgtaggagtcgcgcagcttgttgaccagctcggcggtgacctgcacgtctagggcgcagtagtccagggtttccttgatgatgtcatacttatcctgtcccttttttttccacagctcgcggttgaggacaaactcttcgcggtctttccagtactcttggatcggaaacccgtcggcctccgaacggtaagagcctagcatgtagaactggttgacggcctggtaggcgcagcatcccttttctacgggtagcgcgtatgcctgcgcggccttccggcatgaccagcatgaagggcacgagctgcttcccaaaggcccccatccaagtataggtctctacatcgtaggtgacaaagagacgctcggtgcgaggatgcgagccgatcgggaagaactggatctcccgccaccaattggaggagtggctattgatgtggtgaaagtagaagtccctgcgacgggccgaacactcgtgctggcttttgtaaaaacgtgcgcagtactggcagcggtgcacgggctgtacatcctgcacgaggttgacctgacgaccgcgcacaaggaagcagagtgggaatttgagcccctcgcctggcgggtttggctggtggtcttctacttcggctgcttgtccttgaccgtctggctgctcgaggggagttacggtggatcggaccaccacgccgcgcgagcccaaagtccagatgtccgcgcgcggcggtcggagcttgatgacaacatcgcgcagatgggagctgtccatggtctggagctcccgcggcgtcaggtcaggcgggagctcctgcaggtttacctcgcatagacgggtcagggcgcgggctagatccaggtgatacctaatttccaggggctggttggtggcggcgtcgatggcttgcaagaggccgcatccccgcggcgcgactacggtaccgcgcggcgggcggtgggccgcgggggtgtccttggatgatgcatctaaaagcggtgacgcgggcgagcccccggaggtagggggggctccggacccgccgggagagggggcaggggcacgtcggcgccgcgcgcgggcaggagctggtgctgcgcgcgtaggttgctggcgaacgcgacgacgcggcggttgatctcctgaatctggcgcctctgcgtgaagacgacgggcccggtgagcttgaacctgaaagagagttcgacagaatcaatttcggtgtcgttgacggcggcctggcgcaaaatctcctgcacgtctcctgagttgtcttgataggcgatctcggccatgaactgctcgatctcttcctcctggagatctccgcgtccggctcgctccacggtggcggcgaggtcgttggaaatgcgggccatgagctgcgagaaggcgttgaggcctccctcgttccagacgcggctgtagaccacgcccccttcggcatcgcgggcgcgcatgaccacctgcgcgagattgagctccacgtgccgggcgaagacggcgtagtttcgcaggcgctgaaagaggtagttgagggtggtggcggtgtgttctgccacgaagaagtacataacccagcgtcgcaacgtggattcgttgataattgttgtgtaggtactccgccgccgagggacctgagcgagtccgcatcgaccggatcggaaaacctctcgagaaaggcgtctaaccagtcacagtcgcaaggtaggctgagcaccgtggcgggcggcagcgggcggcggtcggggttgtttctggcggaggtgctgctgatgatgtaattaaagtaggcggtcttgagacggcggatggtcgacagaagcaccatgtccttgggtccggcctgctgaatgcgcaggcggtcggccatgccccaggcttcgttttgacatcggcgcaggtctttgtagtagtcttgcatgagcctttctaccggcacttcttcttctccttcctcttgtcctgcatctcttgcatctatcgctgcggcggcggcggagtttggccgtaggtggcgccctcttcctcccatgcgtgtgaccccgaagcccctcatcggctgaagcagggctaggtcggcgacaacgcgctcggctaatatggcctgctgcacctgcgtgagggtagactggaagtcatccatgtccacaaagcggtggtatgcgcccgtgttgatggtgtaagtgcagttggccataacggaccagttaacggtctggtgacccggctgcgagagctcggtgtacctgagacgcgagtaagccctcgagtcaaatacgtagtcgttgcaagtccgcaccaggtactggtatcccaccaaaaagtgcggcggcggctggcggtagaggggccagcgtagggtggccggggctccgggggcgagatcttccaacataaggcgatgatatccgtagatgtacctggacatccaggtgatgccggcggcggtggtggaggcgcgcggaaagtcgcggacgcggttccagatgttgcgcagcggcaaaaagtgctccatggtcgggacgctctggccggtcaggcgcgcgcaatcgttgacgctctagcgtgcaaaaggagagcctgtaagcgggcactcttccgtggtctggtggataaattcgcaagggtatcatggcggacgaccggggttcgagccccgtatccggccgtccgccgtgatccatgcggttaccgcccgcgtgtcgaacccaggtgtgcgacgtcagacaacgggggagtgctccttttggcttccttccaggcgcggcggctgctgcgctagcttttttggccactggccgcgcgcagcgtaagcggttaggctggaaagcgaaagcattaagtggctcgctccctgtagccggagggttattttccaagggttgagtcgcgggacccccggttcgagtctcggaccggccggactgcggcgaacgggggtttgcctccccgtcatgcaagaccccgcttgcaaattcctccggaaacagggacgagccccttttttgcttttcccagatgcatccggtgctgcggcagatgcgcccccctcctcagcagcggcaagagcaagagcagcggcagacatgcagggcaccctcccctcctcctaccgcgtcaggaggggcgacatccgcggttgacgcggcagcagatggtgattacgaacccccgcggcgccgggcccggcactacctggacttggaggagggcgagggcctggcgcggctaggagcgccctctcctgagcggcacccaagggtgcagctgaagcgtgatacgcgtgaggcgtacgtgccgcggcagaacctgtttcgcgaccgcgagggagaggagcccgaggagatgcgggatcgaaagttccacgcagggcgcgagctgcggcatggcctgaatcgcgagcggttgctgcgcgaggaggactttgagcccgacgcgcgaaccgggattagtcccgcgcgcgcacacgtggcggccgccgacctggtaaccgcatacgagcagacggtgaaccaggagattaactttcaaaaaagctttaacaaccacgtgcgtacgcttgtggcgcgcgaggaggtggctataggactgatgcatctgtgggactttgtaagcgcgctggagcaaaacccaaatagcaagccgctcatggcgcagctgttccttatagtgcagcacagcagggacaacgaggcattcagggatgcgctgctaaacatagtagagcccgagggccgctggctgctcgatttgataaacatcctgcagagcatagtggtgcaggagcgcagcttgagcctggctgacaaggtggccgccatcaactattccatgcttagcctgggcaagttttacgcccgcaagatataccataccccttacgttcccatagacaaggaggtaaagatcgaggggttctacatgcgcatggcgctgaaggtgcttaccttgagcgacgacctgggcgtttatcgcaacgagcgcatccacaaggccgtgagcgtgagccggcggcgcgagctcagcgaccgcgagctgatgcacagcctgcaaagggccctggctggcacgggcagcggcgatagagaggccgagtcctactttgacgcgggcgctgacctgcgctgggccccaagccgacgcgccctggaggcagctggggccggacctgggctggcggtggcacccgcgcgcgctggcaacgtcggcggcgtggaggaatatgacgaggacgatgagtacgagccagaggacggcgagtactaagcggtgatgtttctgatcagatgatgcaagacgcaacggacccggcggtgcgggcggcgctgcagagccagccgtccggccttaactccacggacgactggcgccaggtcatggaccgcatcatgtcgctgactgcgcgcaatcctgacgcgttccggcagcagccgcaggccaaccggctctccgcaattctggaagcggtggtcccggcgcgcgcaaaccccacgcacgagaaggtgctggcgatcgtaaacgcgctggccgaaaacagggccatccggcccgacgaggccggcctggtctacgacgcgctgcttcagcgcgtggctcgttacaacagcggcaacgtgcagaccaacctggaccggctggtgggggatgtgcgcgaggccgtggcgcagcgtgagcgcgcgcagcagcagggcaacctgggctccatggttgcactaaacgccttcctgagtacacagcccgccaacgtgccgcggggacaggaggactacaccaactttgtgagcgcactgcggctaatggtgactgagacaccgcaaagtgaggtgtaccagtctgggccagactattttttccagaccagtagacaaggcctgcagaccgtaaacctgagccaggctttcaaaaacttgcaggggctgtggggggtgcgggctcccacaggcgaccgcgcgaccgtgtctagcttgctgacgcccaactcgcgcctgttgctgctgctaatagcgcccttcacggacagtggcagcgtgtcccgggacacatacctaggtcacttgctgacactgtaccgcgaggccataggtcaggcgcatgtggacgagcatactttccaggagattacaagtgtcagccgcgcgctggggcaggaggacacgggcagcctggaggcaaccctaaactacctgctgaccaaccggcggcagaagatcccctcgttgcacagtttaaacagcgaggaggagcgcattttgcgctacgtgcagcagagcgtgagccttaacctgatgcgcgacggggtaacgcccagcgtggcgctggacatgaccgcgcgcaacatggaaccgggcatgtatgcctcaaaccggccgtttatcaaccgcctaatggactacttgcatcgcgcggccgccgtgaaccccgagtatttcaccaatgccatcttgaacccgcactggctaccgccccctggtttctacaccgggggattcgaggtgcccgagggtaacgatggattcctctgggacgacatagacgacagcgtgttttccccgcaaccgcagaccctgctagagttgcaacagcgcgagcaggcagaggcggcgctgcgaaaggaaagcttccgcaggccaagcagcttgtccgatctaggcgctgcggccccgcggtcagatgctagtagcccatttccaagcttgatagggtctcttaccagcactcgcaccacccgcccgcgcctgctgggcgaggaggagtacctaaacaactcgctgctgcagccgcagcgcgaaaaaaacctgcctccggcatttcccaacaacgggatagagagcctagtggacaagatgagtagatggaagacgtacgcgcaggagcacagggacgtgccaggcccgcgcccgcccacccgtcgtcaaaggcacgaccgtcagcggggtctggtgtgggaggacgatgactcggcagacgacagcagcgtcctggatttgggagggagtggcaacccgtttgcgcaccttcgccccaggctggggagaatgttttaaaaaaaaaaaagcatgatgcaaaataaaaaactcaccaaggccatggcaccgagcgttggttttcttgtattccccttagtatgcggcgcgcggcgatgtatgaggaaggtcctcctccctcctacgagagtgtggtgagcgcggcgccagtggcggcggcgctgggttctcccttcgatgctcccctggacccgccgtttgtgcctccgcggtacctgcggcctaccggggggagaaacagcatccgttactctgagttggcacccctattcgacaccacccgtgtgtacctggtggacaacaagtcaacggatgtggcatccctgaactaccagaacgaccacagcaactttctgaccacggtcattcaaaacaatgactacagcccgggggaggcaagcacacagaccatcaatcttgacgaccggtcgcactggggcggcgacctgaaaaccatcctgcataccaacatgccaaatgtgaacgagttcatgtttaccaataagtttaaggcgcgggtgatggtgtcgcgcttgcctactaaggacaatcaggtggagctgaaatacgagtgggtggagttcacgctgcccgagggcaactactccgagaccatgaccatagaccttatgaacaacgcgatcgtggagcactacttgaaagtgggcagacagaacggggttctggaaagcgacatcggggtaaagtttgacacccgcaacttcagactggggtttgaccccgtcactggtcttgtcatgcctggggtatatacaaacgaagccttccatccagacatcattttgctgccaggatgcggggtggacttcacccacagccgcctgagcaacttgttgggcatccgcaagcggcaacccttccaggagggctttaggatcacctacgatgatctggagggtggtaacattcccgcactgttggatgtggacgcctaccaggcgagcttgaaagatgacaccgaacagggcgggggtggcgcaggcggcagcaacagcagtggcagcggcgcggaagagaactccaacgcggcagccgcggcaatgcagccggtggaggacatgaacgatcatgccattcgcggcgacacctttgccacacgggctgaggagaagcgcgctgaggccgaagcagcggccgaagctgccgcccccgctgcgcaacccgaggtcgagaagcctcagaagaaaccggtgatcaaacccctgacagaggacagcaagaaacgcagttacaacctaataagcaatgacagcaccttcacccagtaccgcagctggtaccttgcatacaactacggcgaccctcagaccggaatccgctcatggaccctgctttgcactcctgacgtaacctgcggctcggagcaggtctactggtcgttgccagacatgatgcaagaccccgtgaccttccgctccacgcgccagatcagcaactttccggtggtgggcgccgagctgttgcccgtgcactccaagagcttctacaacgaccaggccgtctactcccaactcatccgccagtttacctctctgacccacgtgttcaatcgctttcccgagaaccagattttggcgcgcccgccagcccccaccatcaccaccgtcagtgaaaacgttcctgctctcacagatcacgggacgctaccgctgcgcaacagcatcggaggagtccagcgagtgaccattactgacgccagacgccgcacctgcccctacgtttacaaggccctgggcatagtctcgccgcgcgtcctatcgagccgcactttttgagcaagcatgtccatccttatatcgcccagcaataacacaggctggggcctgcgcttcccaagcaagatgtttggcggggccaagaagcgctccgaccaacacccagtgcgcgtgcgcgggcactaccgcgcgccctggggcgcgcacaaacgcggccgcactgggcgcaccaccgtcgatgacgccatcgacgcggtggtggaggaggcgcgcaactacacgcccacgccgccaccagtgtccacagtggacgcggccattcagaccgtggtgcgcggagcccggcgctatgctaaaatgaagagacggcggaggcgcgtagcacgtcgccaccgccgccgacccggcactgccgcccaacgcgcggcggcggccctgcttaaccgcgcacgtcgcaccggccgacgggcggccatgcgggccgctcgaaggctggccgcgggtattgtcactgtgccccccaggtccaggcgacgagcggccgccgcagcagccgcggccattagtgctatgactcagggtcgcaggggcaacgtgtattgggtgcgcgactcggttagcggcctgcgcgtgcccgtgcgcacccgccccccgcgcaactagattgcaagaaaaaactacttagactcgtactgttgtatgtatccagcggcggcggcgcgcaacgaagctatgtccaagcgcaaaatcaaagaagagatgctccaggtcatcgcgccggagatctatggccccccgaagaaggaagagcaggattacaagccccgaaagctaaagcgggtcaaaaagaaaaagaaagatgatgatgatgaacttgacgacgaggtggaactgctgcacgctaccgcgcccaggcgacgggtacagtggaaaggtcgacgcgtaaaacgtgttttgcgacccggcaccaccgtagtctttacgcccggtgagcgctccacccgcacctacaagcgcgtgtatgatgaggtgtacggcgacgaggacctgcttgagcaggccaacgagcgcctcggggagtttgcctacggaaagcggcataaggacatgctggcgttgccgctggacgagggcaacccaacacctagcctaaagcccgtaacactgcagcaggtgctgcccgcgcttgcaccgtccgaagaaaagcgcggcctaaagcgcgagtctggtgacttggcacccaccgtgcagctgatggtacccaagcgccagcgactggaagatgtcttggaaaaaatgaccgtggaacctgggctggagcccgaggtccgcgtgcggccaatcaagcaggtggcgccgggactgggcgtgcagaccgtggacgttcagatacccactaccagtagcaccagtattgccaccgccacagagggcatggagacacaaacgtccccggttgcctcagcggtggcggatgccgcggtgcaggcggtcgctgcggccgcgtccaagacctctacggaggtgcaaacggacccgtggatgtttcgcgtttcagccccccggcgcccgcgccgttcgaggaagtacggcgccgccagcgcgctactgcccgaatatgccctacatccttccattgcgcctacccccggctatcgtggctacacctaccgccccagaagacgagcaactacccgacgccgaaccaccactggaacccgccgccgccgtcgccgtcgccagcccgtgctggccccgatttccgtgcgcagggtggctcgcgaaggaggcaggaccctggtgctgccaacagcgcgctaccaccccagcatcgtttaaaagccggtctttgtggttcttgcagatatggccctcacctgccgcctccgtttcccggtgccgggattccgaggaagaatgcaccgtaggaggggcatggccggccacggcctgacgggcggcatgcgtcgtgcgcaccaccggcggcggcgcgcgtcgcaccgtcgcatgcgcggcggtatcctgcccctccttattccactgatcgccgcggcgattggcgccgtgcccggaattgcatccgtggccttgcaggcgcagagacactgattaaaaacaagttgcatgtggaaaaatcaaaataaaaagtctggactctcacgctcgcttggtcctgtaactattttgtagaatggaagacatcaactttgcgtctctggccccgcgacacggctcgcgcccgttcatgggaaactggcaagatatcggcaccagcaatatgagcggtggcgccttcagctggggctcgctgtggagcggcattaaaaatttcggttccaccgttaagaactatggcagcaaggcctggaacagcagcacaggccagatgctgagggataagttgaaagagcaaaatttccaacaaaaggtggtagatggcctggcctctggcattagcggggtggtggacctggccaaccaggcagtgcaaaataagattaacagtaagcttgatccccgccctcccgtagaggagcctccaccggccgtggagacagtgtctccagaggggcgtggcgaaaagcgtccgcgccccgacagggaagaaactctggtgacgcaaatagacgagcctccctcgtacgaggaggcactaaagcaaggcctgcccaccacccgtcccatcgcgcccatggctaccggagtgctgggccagcacacacccgtaacgctggacctgcctccccccgccgacacccagcagaaacctgtgctgccaggcccgaccgccgttgttgtaacccgtcctagccgcgcgtccctgcgccgcgccgccagcggtccgcgatcgttgcggcccgtagccagtggcaactggcaaagcacactgaacagcatcgtgggtctgggggtgcaatccctgaagcgccgacgatgcttctgatagctaacgtgtcgtatgtgtgtcatgtatgcgtccatgtcgccgccagaggagctgctgagccgccgcgcgcccgctttccaagatggctaccccttcgatgatgccgcagtggtcttacatgcacatctcgggccaggacgcctcggagtacctgagccccgggctggtgcagtttgcccgcgccaccgagacgtacttcagcctgaataacaagtttagaaaccccacggtggcgcctacgcacgacgtgaccacagaccggtcccagcgtttgacgctgcggttcatccctgtggaccgtgaggatactgcgtactcgtacaaggcgcggttcaccctagctgtgggtgataaccgtgtgctggacatggcttccacgtactttgacatccgcggcgtgctggacaggggccctacttttaagccctactctggcactgcctacaacgccctggctcccaagggtgccccaaatccttgcgaatgggatgaagctgctactgctcttgaaataaacctagaagaagaggacgatgacaacgaagacgaagtagacgagcaagctgagcagcaaaaaactcacgtatttgggcaggcgccttattctggtataaatattacaaaggagggtattcaaataggtgtcgaaggtcaaacacctaaatatgccgataaaacatttcaacctgaacctcaaataggagaatctcagtggtacgaaacagaaattaatcatgcagctgggagagtcctaaaaaagactaccccaatgaaaccatgttacggttcatatgcaaaacccacaaatgaaaatggagggcaaggcattcttgtaaagcaacaaaatggaaagctagaaagtcaagtggaaatgcaatttttctcaactactgaggcagccgcaggcaatggtgataacttgactcctaaagtggtattgtacagtgaagatgtagatatagaaaccccagacactcatatttcttacatgcccactattaaggaaggtaactcacgagaactaatgggccaacaatctatgcccaacaggcctaattacattgcttttagggacaattttattggtctaatgtattacaacagcacgggtaatatgggtgttctggcgggccaagcatcgcagttgaatgctgttgtagatttgcaagacagaaacacagagctttcataccagcttttgcttgattccattggtgatagaaccaggtacttttctatgtggaatcaggctgttgacagctatgatccagatgttagaattattgaaaatcatggaactgaagatgaacttccaaattactgctttccactgggaggtgtgattaatacagagactcttaccaaggtaaaacctaaaacaggtcaggaaaatggatgggaaaaagatgctacagaattttcagataaaaatgaaataagagttggaaataattttgccatggaaatcaatctaaatgccaacctgtggagaaatttcctgtactccaacatagcgctgtatttgcccgacaagctaaagtacagtccttccaacgtaaaaatttctgataacccaaacacctacgactacatgaacaagcgagtggtggctcccgggctagtggactgctacattaaccttggagcacgctggtcccttgactatatggacaacgtcaacccatttaaccaccaccgcaatgctggcctgcgctaccgctcaatgttgctgggcaatggtcgctatgtgcccttccacatccaggtgcctcagaagttctttgccattaaaaacctccttctcctgccgggctcatacacctacgagtggaacttcaggaaggatgttaacatggttctgcagagctccctaggaaatgacctaagggttgacggagccagcattaagtttgatagcatttgcctttacgccaccttcttccccatggcccacaacaccgcctccacgcttgaggccatgcttagaaacgacaccaacgaccagtcctttaacgactatctctccgccgccaacatgctctaccctatacccgccaacgctaccaacgtgcccatatccatcccctcccgcaactgggcggctttccgcggctgggccttcacgcgccttaagactaaggaaaccccatcactgggctcgggctacgacccttattacacctactctggctctataccctacctagatggaaccttttacctcaaccacacctttaagaaggtggccattacctttgactcttctgtcagctggcctggcaatgaccgcctgcttacccccaacgagtttgaaattaagcgctcagttgacggggagggttacaacgttgcccagtgtaacatgaccaaagactggttcctggtacaaatgctagctaactataacattggctaccagggcttctatatcccagagagctacaaggaccgcatgtactccttctttagaaacttccagcccatgagccgtcaggtggtggatgatactaaatacaaggactaccaacaggtgggcatcctacaccaacacaacaactctggatttgttggctaccttgcccccaccatgcgcgaaggacaggcctaccctgctaacttcccctatccgcttataggcaagaccgcagttgacagcattacccagaaaaagtttctttgcgatcgcaccctttggcgcatcccattctccagtaactttatgtccatgggcgcactcacagacctgggccaaaaccttctctacgccaactccgcccacgcgctagacatgacttttgaggtggatcccatggacgagcccacccttctttatgttttgtttgaagtctttgacgtggtccgtgtgcaccagccgcaccgcggcgtcatcgaaaccgtgtacctgcgcacgcccttctcggccggcaacgccacaacataaagaagcaagcaacatcaacaacagctgccgccatgggctccagtgagcaggaactgaaagccattgtcaaagatcttggttgtgggccatattttttgggcacctatgacaagcgctttccaggctttgtttctccacacaagctcgcctgcgccatagtcaatacggccggtcgcgagactgggggcgtacactggatggcctttgcctggaacccgcactcaaaaacatgctacctctttgagccctttggcttttctgaccagcgactcaagcaggtttaccagtttgagtacgagtcactcctgcgccgtagcgccattgcttcttcccccgaccgctgtataacgctggaaaagtccacccaaagcgtacaggggcccaactcggccgcctgtggactattctgctgcatgtttctccacgcctttgccaactggccccaaactcccatggatcacaaccccaccatgaaccttattaccggggtacccaactccatgctcaacagtccccaggtacagcccaccctgcgtcgcaaccaggaacagctctacagcttcctggagcgccactcgccctacttccgcagccacagtgcgcagattaggagcgccacttctttttgtcacttgaaaaacatgtaaaaataatgtactagagacactttcaataaaggcaaatgcttttatttgtacactctcgggtgattatttacccccacccttgccgtctgcgccgtttaaaaatcaaaggggttctgccgcgcatcgctatgcgccactggcagggacacgttgcgatactggtgtttagtgctccacttaaactcaggcacaaccatccgcggcagctcggtgaagttttcactccacaggctgcgcaccatcaccaacgcgtttagcaggtcgggcgccgatatcttgaagtcgcagttggggcctccgccctgcgcgcgcgagttgcgatacacagggttgcagcactggaacactatcagcgccgggtggtgcacgctggccagcacgctcttgtcggagatcagatccgcgtccaggtcctccgcgttgctcagggcgaacggagtcaactttggtagctgccttcccaaaaagggcgcgtgcccaggctttgagttgcactcgcaccgtagtggcatcaaaaggtgaccgtgcccggtctgggcgttaggatacagcgcctgcataaaagccttgatctgcttaaaagccacctgagcctttgcgccttcagagaagaacatgccgcaagacttgccggaaaactgattggccggacaggccgcgtcgtgcacgcagcaccttgcgtcggtgttggagatctgcaccacatttcggccccaccggttcttcacgatcttggccttgctagactgctccttcagcgcgcgctgcccgttttcgctcgtcacatccatttcaatcacgtgctccttatttatcataatgcttccgtgtagacacttaagctcgccttcgatctcagcgcagcggtgcagccacaacgcgcagcccgtgggctcgtgatgcttgtaggtcacctctgcaaacgactgcaggtacgcctgcaggaatcgccccatcatcgtcacaaaggtcttgttgctggtgaaggtcagctgcaacccgcggtgctcctcgttcagccaggtcttgcatacggccgccagagcttccacttggtcaggcagtagtttgaagttcgcctttagatcgttatccacgtggtacttgtccatcagcgcgcgcgcagcctccatgcccttctcccacgcagacacgatcggcacactcagcgggttcatcaccgtaatttcactttccgcttcgctgggctcttcctcttcctcttgcgtccgcataccacgcgccactgggtcgtcttcattcagccgccgcactgtgcgcttacctcctttgccatgcttgattagcaccggtgggttgctgaaacccaccatttgtagcgccacatcttctctttcttcctcgctgtccacgattacctctggtgatggcgggcgctcgggcttgggagaagggcgcttctttttcttcttgggcgcaatggccaaatccgccgccgaggtcgatggccgcgggctgggtgtgcgcggcaccagcgcgtcttgtgatgagtcttcctcgtcctcggactcgatacgccgcctcatccgcttttttgggggcgcccggggaggcggcggcgacggggacggggacgacacgtcctccatggttgggggacgtcgcgccgcaccgcgtccgcgctcgggggtggtttcgcgctgctcctcttcccgactggccatttccttctcctataggcagaaaaagatcatggagtcagtcgagaagaaggacagcctaaccgccccctctgagttcgccaccaccgcctccaccgatgccgccaacgcgcctaccaccttccccgtcgaggcacccccgcttgaggaggaggaagtgattatcgagcaggacccaggttttgtaagcgaagacgacgaggaccgctcagtaccaacagaggataaaaagcaagaccaggacaacgcagaggcaaacgaggaacaagtcgggcggggggacgaaaggcatggcgactacctagatgtgggagacgacgtgctgttgaagcatctgcagcgccagtgcgccattatctgcgacgcgttgcaagagcgcagcgatgtgcccctcgccatagcggatgtcagccttgcctacgaacgccacctattctcaccgcgcgtaccccccaaacgccaagaaaacggcacatgcgagcccaacccgcgcctcaacttctaccccgtatttgccgtgccagaggtgcttgccacctatcacatctttttccaaaactgcaagatacccctatcctgccgtgccaaccgcagccgagcggacaagcagctggccttgcggcagggcgctgtcatacctgatatcgcctcgctcaacgaagtgccaaaaatctttgagggtcttggacgcgacgagaagcgcgcggcaaacgctctgcaacaggaaaacagcgaaaatgaaagtcactctggagtgttggtggaactcgagggtgacaacgcgcgcctagccgtactaaaacgcagcatcgaggtcacccactttgcctacccggcacttaacctaccccccaaggtcatgagcacagtcatgagtgagctgatcgtgcgccgtgcgcagcccctggagagggatgcaaatttgcaagaacaaacagaggagggcctacccgcagttggcgacgagcagctagcgcgctggcttcaaacgcgcgagcctgccgacttggaggagcgacgcaaactaatgatggccgcagtgctcgttaccgtggagcttgagtgcatgcagcggttctttgctgacccggagatgcagcgcaagctagaggaaacattgcactacacctttcgacagggctacgtacgccaggcctgcaagatctccaacgtggagctctgcaacctggtctcctaccttggaattttgcacgaaaaccgccttgggcaaaacgtgcttcattccacgctcaagggcgaggcgcgccgcgactacgtccgcgactgcgtttacttatttctatgctacacctggcagacggccatgggcgtttggcagcagtgcttggaggagtgcaacctcaaggagctgcagaaactgctaaagcaaaacttgaaggacctatggacggccttcaacgagcgctccgtggccgcgcacctggcggacatcattttccccgaacgcctgcttaaaaccctgcaacagggtctgccagacttcaccagtcaaagcatgttgcagaactttaggaactttatcctagagcgctcaggaatcttgcccgccacctgctgtgcacttcctagcgactttgtgcccattaagtaccgcgaatgccctccgccgctttggggccactgctaccttctgcagctagccaactaccttgcctaccactctgacataatggaagacgtgagcggtgacggtctactggagtgtcactgtcgctgcaacctatgcaccccgcaccgctccctggtttgcaattcgcagctgcttaacgaaagtcaaattatcggtacctttgagctgcagggtccctcgcctgacgaaaagtccgcggctccggggttgaaactcactccggggctgtggacgtcggcttaccttcgcaaatttgtacctgaggactaccacgcccacgagattaggttctacgaagaccaatcccgcccgcctaatgcggagcttaccgcctgcgtcattacccagggccacattcttggccaattgcaagccatcaacaaagcccgccaagagtttctgctacgaaagggacggggggtttacttggacccccagtccggcgaggagctcaacccaatccccccgccgccgcagccctatcagcagcagccgcgggcccttgcttcccaggatggcacccaaaaagaagctgcagctgccgccgccacccacggacgaggaggaatactgggacagtcaggcagaggaggttttggacgaggaggaggaggacatgatggaagactgggagagcctagacgaggaagcttccgaggtcgaagaggtgtcagacgaaacaccgtcaccctcggtcgcattcccctcgccggcgccccagaaatcggcaaccggttccagcatggctacaacctccgctcctcaggcgccgccggcactgcccgttcgccgacccaaccgtagatgggacaccactggaaccagggccggtaagtccaagcagccgccgccgttagcccaagagcaacaacagcgccaaggctaccgctcatggcgcgggcacaagaacgccatagttgcttgcttgcaagactgtgggggcaacatctccttcgcccgccgctttcttctctaccatcacggcgtggccttcccccgtaacatcctgcattactaccgtcatctctacagcccatactgcaccggcggcagcggcagcaacagcagcggccacacagaagcaaaggcgaccggatagcaagactctgacaaagcccaagaaatccacagcggcggcagcagcaggaggaggagcgctgcgtctggcgcccaacgaacccgtatcgacccgcgagcttagaaacaggatttttcccactctgtatgctatatttcaacagagcaggggccaagaacaagagctgaaaataaaaaacaggtctctgcgatccctcacccgcagctgcctgtatcacaaaagcgaagatcagcttcggcgcacgctggaagacgcggaggctctcttcagtaaatactgcgcgctgactcttaaggactagtttcgcgccctttctcaaatttaagcgcgaaaactacgtcatctccagcggccacacccggcgccagcacctgttgtcagcgccattatgagcaaggaaattcccacgccctacatgtggagttaccagccacaaatgggacttgcggctggagctgcccaagactactcaacccgaataaactacatgagcgcgggaccccacatgatatcccgggtcaacggaatacgcgcccaccgaaaccgaattctcctggaacaggcggctattaccaccacacctcgtaataaccttaatccccgtagttggcccgctgccctggtgtaccaggaaagtcccgctcccaccactgtggtacttcccagagacgcccaggccgaagttcagatgactaactcaggggcgcagcttgcgggcggctttcgtcacagggtgcggtcgcccgggcagggtataactcacctgacaatcagagggcgaggtattcagctcaacgacgagtcggtgagctcctcgcttggtctccgtccggacgggacatttcagatcggcggcgccggccgctcttcattcacgcctcgtcaggcaatcctaactctgcagacctcgtcctctgagccgcgctctggaggcattggaactctgcaatttattgaggagtttgtgccatcggtctactttaaccccttctcgggacctcccggccactatccggatcaatttattcctaactttgacgcggtaaaggactcggcggacggctacgactgaatgttaagtggagaggcagagcaactgcgcctgaaacacctggtccactgtcgccgccacaagtgctttgcccgcgactccggtgagttttgctactttgaattgcccgaggatcatatcgagggcccggcgcacggcgtccggcttaccgcccagggagagcttgcccgtagcctgattcgggagtttacccagcgccccctgctagttgagcgggacaggggaccctgtgttctcactgtgatttgcaactgtcctaaccctggattacatcaagatcctctagttaatgtcaggtcgcctaagtcgattaactagagtacccggggatcttattccctttaactaataaaaaaaaataataaagcatcacttacttaaaatcagttagcaaatttctgtccagtttattcagcagcacctccttgccctcctcccagctctggtattgcagcttcctcctggctgcaaactttctccacaatctaaatggaatgtcagtttcctcctgttcctgtccatccgcacccactatcttcatgttgttgcagatgaagcgcgcaagaccgtctgaagataccttcaaccccgtgtatccatatgacacggaaaccggtcctccaactgtgccttttcttactcctccctttgtatcccccaatgggtttcaagagagtccccctggggtactctctttgcgcctatccgaacctctagttacctccaatggcatgcttgcgctcaaaatgggcaacggcctctctctggacgaggccggcaaccttacctcccaaaatgtaaccactgtgagcccacctctcaaaaaaaccaagtcaaacataaacctggaaatatctgcacccctcacagttacctcagaagccctaactgtggctgccgccgcacctctaatggtcgcgggcaacacactcaccatgcaatcacaggccccgctaaccgtgcacgactccaaacttagcattgccacccaaggacccctcacagtgtcagaaggaaagctagccctgcaaacatcaggccccctcaccaccaccgatagcagtacccttactatcactgcctcaccccctctaactactgccactggtagcttgggcattgacttgaaagagcccatttatacacaaaatggaaaactaggactaaagtacggggctcctttgcatgtaacagacgacctaaacactttgaccgtagcaactggtccaggtgtgactattaataatacttccttgcaaactaaagttactggagccttgggttttgattcacaaggcaatatgcaacttaatgtagcaggaggactaaggattgattctcaaaacagacgccttatacttgatgttagttatccgtttgatgctcaaaaccaactaaatctaagactaggacagggccctctttttataaactcagcccacaacttggatattaactacaacaaaggcctttacttgtttacagcttcaaacaattccaaaaagcttgaggttaacctaagcactgccaaggggttgatgtttgacgctacagccatagccattaatgcaggagatgggcttgaatttggttcacctaatgcaccaaacacaaatcccctcaaaacaaaaattggccatggcctagaatttgattcaaacaaggctatggttcctaaactaggaactggccttagttttgacagcacaggtgccattacagtaggaaacaaaaataatgataagctaactttgtggaccacaccagctccatctcctaactgtagactaaatgcagagaaagatgctaaactcactttggtcttaacaaaatgtggcagtcaaatacttgctacagtttcagttttggctgttaaaggcagtttggctccaatatctggaacagttcaaagtgctcatcttattataagatttgacgaaaatggagtgctactaaacaattccttcctggacccagaatattggaactttagaaatggagatcttactgaaggcacagcctatacaaacgctgttggatttatgcctaacctatcagcttatccaaaatctcacggtaaaactgccaaaagtaacattgtcagtcaagtttacttaaacggagacaaaactaaacctgtaacactaaccattacactaaacggtacacaggaaacaggagacacaactccaagtgcatactctatgtcattttcatgggactggtctggccacaactacattaatgaaatatttgccacatcctcttacactttttcatacattgcccaagaataaagaatcgtttgtgttatgtttcaacgtgtttatttttcaattgcagaaaatttcaagtcatttttcattcagtagtatagccccaccaccacatagcttatacagatcaccgtaccttaatcaaactcacagaaccctagtattcaacctgccacctccctcccaacacacagagtacacagtcctttctccccggctggccttaaaaagcatcatatcatgggtaacagacatattcttaggtgttatattccacacggtttcctgtcgagccaaacgctcatcagtgatattaataaactccccgggcagctcacttaagttcatgtcgctgtccagctgctgagccacaggctgctgtccaacttgcggttgcttaacgggcggcgaaggagaagtccacgcctacatgggggtagagtcataatcgtgcatcaggatagggcggtggtgctgcagcagcgcgcgaataaactgctgccgccgccgctccgtcctgcaggaatacaacatggcagtggtctcctcagcgatgattcgcaccgcccgcagcataaggcgccttgtcctccgggcacagcagcgcaccctgatctcacttaaatcagcacagtaactgcagcacagcaccacaatattgttcaaaatcccacagtgcaaggcgctgtatccaaagctcatggcggggaccacagaacccacgtggccatcataccacaagcgcaggtagattaagtggcgacccctcataaacacgctggacataaacattacctcttttggcatgttgtaattcaccacctcccggtaccatataaacctctgattaaacatggcgccatccaccaccatcctaaaccagctggccaaaacctgcccgccggctatacactgcagggaaccgggactggaacaatgacagtggagagcccaggactcgtaaccatggatcatcatgctcgtcatgatatcaatgttggcacaacacaggcacacgtgcatacacttcctcaggattacaagctcctcccgcgttagaaccatatcccagggaacaacccattcctgaatcagcgtaaatcccacactgcagggaagacctcgcacgtaactcacgttgtgcattgtcaaagtgttacattcgggcagcagcggatgatcctccagtatggtagcgcgggtttctgtctcaaaaggaggtagacgatccctactgtacggagtgcgccgagacaaccgagatcgtgttggtcgtagtgtcatgccaaatggaacgccggacgtagtcatatttcctgaagcaaaaccaggtgcgggcgtgacaaacagatctgcgtctccggtctcgccgcttagatcgctctgtgtagtagttgtagtatatccactctctcaaagcatccaggcgccccctggcttcgggttctatgtaaactccttcatgcgccgctgccctgataacatccaccaccgcagaataagccacacccagccaacctacacattcgttctgcgagtcacacacgggaggagcgggaagagctggaagaaccatgtttttttttttattccaaaagattatccaaaacctcaaaatgaagatctattaagtgaacgcgctcccctccggtggcgtggtcaaactctacagccaaagaacagataatggcatttgtaagatgttgcacaatggcttccaaaaggcaaacggccctcacgtccaagtggacgtaaaggctaaacccttcagggtgaatctcctctataaacattccagcaccttcaaccatgcccaaataattctcatctcgccaccttctcaatatatctctaagcaaatcccgaatattaagtccggccattgtaaaaatctgctccagagcgccctccaccttcagcctcaagcagcgaatcatgattgcaaaaattcaggttcctcacagacctgtataagattcaaaagcggaacattaacaaaaataccgcgatcccgtaggtcccttcgcagggccagctgaacataatcgtgcaggtctgcacggaccagcgcggccacttccccgccaggaaccatgacaaaagaacccacactgattatgacacgcatactcggagctatgctaaccagcgtagccccgatgtaagcttgttgcatgggcggcgatataaaatgcaaggtgctgctcaaaaaatcaggcaaagcctcgcgcaaaaaagaaagcacatcgtagtcatgctcatgcagataaaggcaggtaagctccggaaccaccacagaaaaagacaccatttttctctcaaacatgtctgcgggtttctgcataaacacaaaataaaataacaaaaaaacatttaaacattagaagcctgtcttacaacaggaaaaacaacccttataagcataagacggactacggccatgccggcgtgaccgtaaaaaaactggtcaccgtgattaaaaagcaccaccgacagctcctcggtcatgtccggagtcataatgtaagactcggtaaacacatcaggttgattcacatcggtcagtgctaaaaagcgaccgaaatagcccgggggaatacatacccgcaggcgtagagacaacattacagcccccataggaggtataacaaaattaataggagagaaaaacacataaacacctgaaaaaccctcctgcctaggcaaaatagcaccctcccgctccagaacaacatacagcgcttccacagcggcagccataacagtcagccttaccagtaaaaaagaaaacctattaaaaaaacaccactcgacacggcaccagctcaatcagtcacagtgtaaaaaagggccaagtgcagagcgagtatatataggactaaaaaatgacgtaacggttaaagtccacaaaaaacacccagaaaaccgcacgcgaacctacgcccagaaacgaaagccaaaaaacccacaacttcctcaaatcgtcacttccgttttcccacgttacgtcacttcccattttaagaaaactacaattcccaacacatacaagttactccgccctaaaacctacgtcacccgccccgttcccacgccccgcgccacgtcacaaactccaccccctcattatcatattggcttcaatccaaaataaggta

SEQ ID NO: 225 - DNA, 9701 bp, synthetic construct
  misc_feature 1..9701: note = vector for IgG1 against T27Y H34A H505L ACE2 mutant
  misc_feature 2929..2930: note = n is a, c, g, or t
  misc_feature 2934: note = n is a, c, g, or t
  source 1..9701: mol_type = other DNA
ggcgtaatctgctgcttgcaaacaaaaaaaccaccgctaccagcggtggtttgtttgccggatcaagagctaccaactctttttccgaaggtaactggcttcagcagagcgcagataccaaatactgtccttctagtgtagccgtagttaggccaccacttcaagaactctgtagcaccgcctacatacctcgctctgctgaagccagttaccagtggctgctgccagtggcgataagtcgtgtcttaccgggttggactcaagagatagttaccggataaggcgcagcggtcgggctgaacggggggttcgtgcacacagcccagcttggagcgaacgacctacaccgaactgagatacctacagcgtgagctatgagaaagcgccacgcttcccgaagggagaaaggcggacaggtatccggtaagcggcagggtcggaacaggagagcgcacgagggagcttccagggggaaacgcctggtatctttatagtcctgtcgggtttcgccacctctgacttgagcgtcgatttttgtgatgctcgtcaggggggcggagcctatggaaaaacgccagcaacgcaagctagagtttaaacttgacagatgagacaataaccctgataaatgcttcaataatattgaaaaaggaaaagtatgagtattcaacatttccgtgtcgcccttattcccttttttgcggcattttgccttcctgtttttgctcacccagaaacgctggtgaaagtaaaagatgcagaagatcacttgggtgcgcgagtgggttacatcgaactggatctcaacagcggtaagatccttgagagttttcgccccgaagaacgtttcccaatgatgagcacttttaaagttctgctatgtggcgcggtattatcccgtattgatgccgggcaagagcaactcggtcgccgcatacactattctcagaatgacttggttgaatactcaccagtcacagaaaagcatcttacggatggcatgacagtaagagaattatgcagtgctgccataaccatgagtgataacactgcggccaacttacttctgacaactatcggaggaccgaaggagctaaccgcttttttgcacaacatgggggatcatgtaactcgccttgatcgttgggaaccggagctgaatgaagccataccaaacgacgagcgtgacaccacgatgcctgtagcaatggcaacaacgttgcgaaaactattaactggcgaactacttactctagcttcccggcaacaactaatagactggatggaggcggataaagttgcaggaccacttctgcgctcggcacttccggctggctggtttattgctgataaatcaggagccggtgagcgtgggtcacgcggtatcattgcagcactggggccggatggtaagccctcccgtatcgtagttatctacactacggggagtcaggcaactatggatgaacgaaatagacagatcgctgagataggtgcctcactgattaagcattggtaaggataaatttctggtaaggaggacacgtatggaagtgggcaagttggggaagccgtatccgttgctgaatctggcatatgtgggagtataagacgcgcagcgtcgcatcaggcatttttttctgcgccaatgcaaaaaggccatccgtcaggatggcctttcggcataactagggccgccgatatttgaaaatatggcatattgaaaatgtcgccgatgtgagtttctgtgtaactgatatcgccatttttccaaaagtgatttttgggcatacgcgatatctggcgatagcgcttatatcgtttacgggggatggcgatagacgactttggtgacttgggcgattctgtgtgtcgcaaatatcgcagtttcgatataggtgacagacgatatgaggctatatcgccgatagaggcgacatcaagctggcacatggccaatgcatatcgatctatacattgaatcaatattggccattagccatattattcattggttatatagcataaatcaatattggctattggccattgcatacgttgtatccatatcataatatgtacatttatattggctcatgtccaacattaccgccatgttgacattgattattgactagttattaatagtaatcaattacggggtcattagttcatagcccatatatggagttccgcgttacataacttacggtaaatggcccgcctggctgaccgcccaacgacccccgcccattgacgtcaataatgacgtatgttcccatagtaacgccaatagggactttccattgacgtcaatgggtggagtatttacggtaaactgcccacttggcagtacatcaagtgtatcatatgccaagtacgccccctattgacgtcaatgacggtaaatggcccgcctggcattatgcccagtacatgaccttatgggactttcctacttggcagtacatctacgtattagtcatcgctattaccatggtgatgcggttttggcagtacatcaatgggcgtggatagcggtttgactcacggggatttccaagtctccaccccattgacgtcaatgggagtttgttttggcaccaaaatcaacgggactttccaaaatgtcgtaacaactccgccccattgacgcaaatgggcggtaggcgtgtacggtgggaggtctatataagcagagctcgtttagtgaaccgtcagatcgcctggagacgccatccacgctgttttgacctccatagaagacaccgggaccgatccagcctccgcggccgggaacggtgcattggaacgcggattccccgtgccaagagtgacgtaagtaccgcctatagagtctataggcccacccccttggcttcttatgcatgctatactgtttttggcttggggtctatacaccccccgnnttcntcatgttataggtgatggtatagcttagcctataggtgtgggttattgaccattattgaccactccccctattggtgacgatactttccattactaatccataacatggctctttgccacaactctctttattggctatatgccaatacactgtccttcagagactgacacggactctgtatttttacaggatggggtctcatttattatttacaaattcacatatacaacaccaccgtccccagtgcccgcagtttttattaaacataacgtgggatctccacgcgaatctcgggtacgtgttccggacatgggctcttctccggtagcggcggagcttctacatccgagccctgctcccatgcctccagcgactcatggtcgctcggcagctccttgctcctaacagtggaggccagacttaggcacagcacgatgcccaccaccaccagtgtgccgcacaaggccgtggcggtagggtatgtgtctgaaaatgagctcggggagcgggcttgcaccgctgacgcatttggaagacttaaggcagcggcagaagaagatgcaggcagctgagttgttgtgttctgataagagtcagaggtaactcccgttgcggtgctgttaacggtggagggcagtgtagtctgagcagtactcgttgctgccgcgcgcgccaccagacataatagctgacagactaacagactgttcctttccatgggtcttttctgcagtcaccgtccttgacacgaagctgctagcgccaccatgagcagcagtagttggcttctcttgagtttggtggcagtgacagcagcccagagtactatcgaggagcaggctaaatactttctggataagtttaacgccgaggccgaagacttgttctatcaatcttctctcgcttcatggaattacaatactaacatcactgaggagaacgtccagaatatgaacaatgctggcgacaaatggagcgccttcttgaaggagcagtctacccttgcacaaatgtatccactgcaggagatacagaaccttacagtaaagttgcagctccaggctctccagcagaacggatctagcgtgctttcagaggataaaagcaaaaggctgaacaccatacttaataccatgtccacaatttactctactggtaaagtatgtaaccccgacaaccctcaagaatgcctccttcttgagccaggcctcaatgagatcatggctaatagtctggactataatgaaagactgtgggcatgggagtcctggagatctgaagtagggaagcaactgaggcccctttatgaagagtacgtcgtacttaagaatgaaatggcccgcgctaaccactacgaggattacggcgattactggcgtggggactatgaagtaaatggtgtagatggatacgactatagtcgtgggcaattgattgaggatgtggagcacacttttgaggagataaaaccactctatgagcatcttcacgcatatgtgagagctaaactgatgaacgcctacccaagttacatcagtccaatcggatgtctcccagctcacctccttggcgacatgtggggacgtttctggaccaatctgtattccctcacagtccctttcgggcaaaagcctaatatagacgtgacagacgcaatggttgatcaggcttgggatgctcaaaggatttttaaggaagctgagaagttttttgtgtcagtcggtttgccaaatatgacacaaggcttctgggaaaatagcatgttgactgatcccggtaatgttcaaaaggctgtgtgtcaccctaccgcttgggaccttgggaaaggtgactttcgaatcttgatgtgtaccaaggtgacaatggatgactttcttacagcccatcatgaaatgggtcacatccagtatgatatggcttatgcagctcaacctttcctcttgagaaatggtgcaaatgaaggttttcatgaagctgtaggggaaataatgtccctgagtgctgcaaccccaaagcatctcaagagtatcggattgttgagcccagattttcaagaagataacgagaccgaaatcaacttccttctgaaacaagccctcacaatagttggtactcttccattcacatacatgctggagaaatggcgttggatggtttttaagggggagatacctaaagatcagtggatgaaaaagtggtgggagatgaagcgtgagatcgtaggggtcgtggagccagtgcctcatgatgagacttactgtgacccagcatcactcttcctggttagcaatgactattcatttatacgttattacactcgcactctttaccagtttcaatttcaggaggctctgtgtcaggctgccaagcatgagggaccccttcacaagtgtgatattagtaacagtactgaggcaggccaaaaactgttcaatatgttgaggcttggcaaaagcgagccatggactctcgccttggaaaatgttgtcggggctaaaaacatgaatgtacgccctctgcttaactattttgagcccctttttacatggctcaaggaccagaataagaactcctttgtcggctggtcaacagactggtctccctatgcagacaaaacacatacttgcccaccttgtcctgcaccagagctgctgggaggtccaagcgtgttcctgtttccacccaagcccaaagacacactgatgatttctcgaactccagaagtgacctgcgtggtcgtggacgtgagccacgaggatcccgaagtgaagttcaactggtacgtggatggcgtggaggtccataatgctaagactaaaccccgggaggaacagtacaacagcacttatagggtcgtgtccgtgctgaccgtcctgcatcaggattggctgaacgggaaggaatataagtgcaaagtgtctaataaggcactgcccgcccctatcgagaaaacaattagcaaggctaagggtcagcctagagaaccacaggtgtacactctgcctccaagtcgcgacgagctgaccaagaaccaggtgtcactgacatgtctggtcaaaggcttttatccctcagatatcgcagtggagtgggaaagcaatggacagcctgagaacaattacaagaccacaccccctgtgctggacagtgatggctcattctttctgtattctaagctgacagtggacaaaagtaggtggcagcagggaaacgtgttctcctgctctgtcatgcacgaagcactgcacaatcattatacccagaagagtctgtcactgagccctggcaaatgagcgataccgattctagaactagatcataatcagccataccacatttgtagaggttttacttgctttaaaaaacctcccacacctccccctgaacctgaaacataaaatgaatgcaattgttgttgttaacttgtttattgcagcttataatggttacaaataaagcaatagcatcacaaatttcacaaataaagcatttttttcactgcattctagttgtggtttgtccaaactcatcaatgtatcttaaggccgcaggtaagccagcccaggcctcgccctccagctcaaggcgggacaggtgccctagagtagcctgcatccagggacaggccccagccgggtgctgacacgtccacctccatctcttcctcaggtctgcccgggtggcatccctgtgacccctccccagtgcctctcctggtcgtggaaggtgctactccagtgcccaccagccttgtcctaataaaattaagttgcatcattttgtttgactaggtgtccttgtataatattatggggtggaggcgggtggtatggagcaaggggcccaagttaacttgtttattgcagcttataatggttacaaataaagcaatagcatcacaaatttcacaaataaagcatttttttcactgcattctagttgtggtttgtccaaactcatcaatgtatcttatcatgtctggatccgcttcaggcaccgggcttgcgggtcatgcaccaggtgcgcggtccttcgggcacctcgacgtcggcggtgacggtgaagccgagccgctcgtagaaggggaggttgcggggcgcggaggtctccaggaaggcgggcaccccggcgcgctcggccgcctccactccggggagcacgacggcgctgcccagacccttgccctggtggtcgggcgagacgccgacggtggccaggaaccacgcgggctccttgggccggtgcggcgccaggaggccttccatctgttgctgcgcggccagcctggaaccgctcaactcggccatgcgcgggccgatctcggcgaacaccgcccccgcttcgacgctctccggcgtggtccagaccgccaccgcggcgccgtcgtccgcgacccacaccttgccgatgtcgagcccgacgcgcgtgaggaagagttcttgcagctcggtgacccgctcgatgtggcggtccgggtcgacggtgtggcgcgtggcggggtagtcggcgaacgcggcggcgagggtgcgtacggcccgggggacgtcgtcgcgggtggcgaggcgcaccgtgggcttgtactcggtcatggtggcctgcagagtcgctctgtgttcgaggccacacgcgtcaccttaatatgcgaagtggacctgggaccgcgccgccccgactgcatctgcgtgttttcgccaatgacaagacgctgggcggggtttgtgtcatcatagaactaaagacatgcaaatatatttcttccggggacaccgccagcaaacgcgagcaacgggccacggggatgaagcagctgcgccactccctgaagatccatcgtctcctaacaagttacatcactcctgcccttcctcaccctcatctccatcacctccttcatctccgtcatctccgtcatcaccctccgcggcagccccttccaccataggtggaaaccagggaggcaaatctactccatcgtcaaagctgcacacagtcaccctgatattgcaggtaggagcgggctttgtcataacaaggtccttaatcgcatccttcaaaacctcagcaaatatatgagtttgtaaaaagaccatgaaataacagacaatggactcccttagcgggccaggttgtgggccgggtccaggggccattccaaaggggagacgactcaatggtgtaagacgacattgtggaatagcaagggcagttcctcgccttaggttgtaaagggaggtcttactacctccatatacgaacacaccggcgacccaagttccttcgtcggtagtcctttctacgtgactcctagccaggagagctcttaaaccttctgcaatgttctcaaatttcgggttggaacctccttgaccacgatgctttccaaaccaccctccttttttgcgcctgcctccatcaccctgacccccgctgcgcgggggcacgtcaggctcaccatctgggccgccttcttggtggtattcaaaataatcggcttcccctacagggtggaaaaatggccttctacctggagggggcctgcgcggtggagacccggatgatgatgactgactactgggactcctgggcctcttttctccacgtccacgacctctccccctggctctttcacgacttccccccctggctctttcacgtcctctaccccggcggcctccactacctcctcgaccccggcctccactacctcctcgaccccggcctccactgcctcctcgaccccggcctccacctcctgctcctgcccctcccgctcctgctcctgctcctgttccaccgtgggtccctttgcagccaatgcaacttggacgtttttggggtctccggacaccatctctatgtcttggccctgatcctgagccgcccggggctcctggtcttccgcctcctcgtcctcgtcctcttccccgtcctcgtccatgtgccatgatggcggcctgcagctgtgttcgaggccgcgcgtgtcaccttaatatgcgaagtggacctgggaccgcgccgccccgactgcatctgcgtgttcgagttcgccaatgacaagacgctgggcggggagatcccccttattaaccctaaacgggtagcatatgcttcccgggtagtagtatatactatccagactaaccctaattcaatagcatatgttacccaacgggaagcatatgctatcgaattagggttagtaaaagggtcctaaggaacagcgatctggatagcatatgctatcctaatctatatctgggtagcatatgctatcctaatctatatctgggtagcataggctatcctaatctatatctgggtagcatatgctatcctaatctatatctgggtagtatatgctatcctaatttatatctgggtagcataggctatcctaatctatatctgggtagcatatgctatcctaatctatatctgggtagtatatgctatcctaatctgtatccgggtagcatatgctatcctcatgcatatacagtcagcatatgatacccagtagtagagtgggagtgctatcctttgcatatgccgccacctcccaaggagatctgtcgacatcgatgggcgcgggtgtacactccgcccatcccgcccctaactccgcccagttccgcccattctccgcctcatggctgactaattttttttatttatgcagaggccgaggccgcctcggcctctgagctattccagaagtagtgaggaggcttttttggaggcctaggcttttgcaaaaagctaattc

SEQ ID NO: 226 - DNA, 38496 bp, synthetic construct
  misc_feature 1..38496: note = vector for IgA against T27Y H34A H374N ACE2 mutant
  source 1..38496: mol_type = other DNA
tattattgatgatgttaattaacatgcatggatcctacgtctcgaccgatgcccttgagagccttcaacccagtcagctccttccggtgggcgcggggcatgactatcgtcgccgcacttatgactgtcttctttatcatgcaactcgtaggacaggtgccggcagcgctctgggtcattttcggcgaggaccgctttcgctggagcgcgacgatgatcggcctgtcgcttgcggtattcggaatcttgcacgccctcgctcaagccttcgtcactggtcccgccaccaaacgtttcggcgagaagcaggccattatcgccggcatggcggccgacgcgctgggctacgtcttgctggcgttcgcgacgcgaggctggatggccttccccattatgattcttctcgcttccggcggcatcgggatgcccgcgttgcaggccatgctgtccaggcaggtagatgacgaccatcagggacagcttcaaggatcgctcgcggctcttaccagcctaacttcgatcattggaccgctgatcgtcacggcgatttatgccgcctcggcgagcacatggaacgggttggcatggattgtaggcgccgccctataccttgtctgcctccccgcgttgcgtcgcggtgcatggagccgggccacctcgacctgaatggaagccggcggcacctcgctaacggattcaccactccaagaattggagccaatcaattcttgcggagaactgtgaatgcgcaaaccaacccttggcagaacatatccatcgcgtccgccatctccagcagccgcacgcggcgcatctcgggcagcgttgggtcctggccacgggtgcgcatgatcgtgctcctgtcgttgaggacccggctaggctggcggggttgccttactggttagcagaatgaatcaccgatacgcgagcgaacgtgaagcgactgctgctgcaaaacgtctgcgacctgagcaacaacatgaatggtcttcggtttccgtgtttcgtaaagtctggaaacgcggaagtcagcgccctgcaccattatgttccggatctgcatcgcaggatgctgctggctaccctgtggaacacctacatctgtattaacgaagcgctggcattgaccctgagtgatttttctctggtcccgccgcatccataccgccagttgtttaccctcacaacgttccagtaaccgggcatgttcatcatcagtaacccgtatcgtgagcatcctctctcgtttcatcggtatcattacccccatgaacagaaatcccccttacacggaggcatcagtgaccaaacaggaaaaaaccgcccttaacatggcccgctttatcagaagccagacattaacgcttctggagaaactcaacgagctggacgcggatgaacaggcagacatctgtgaatcgcttcacgaccacgctgatgagctttaccgcagctgcctcgcgcgtttcggtgatgacggtgaaaacctctgacacatgcagctcccggagacggtcacagcttgtctgtaagcggatgccgggagcagacaagcccgtcagggcgcgtcagcgggtgttggcgggtgtcggggcgcagccatgacccagtcacgtagcgatagcggagtgtatactggcttaactatgcggcatcagagcagattgtactgagagtgcaccatatgcggtgtgaaataccgcacagatgcgtaaggagaaaataccgcatcaggcgctcttccgcttcctcgctcactgactcgctgcgctcggtcgttcggctgcggcgagcggtatcagctcactcaaaggcggtaatacggttatccacagaatcaggggataacgcaggaaagaacatgtgagcaaaaggccagcaaaaggccaggaaccgtaaaaaggccgcgttgctggcgtttttccataggctccgcccccctgacgagcatcacaaaaatcgacgctcaagtcagaggtggcgaaacccgacaggactataaagataccaggcgtttccccctggaagctccctcgtgcgctctcctgttccgaccctgccgcttaccggatacctgtccgcctttctcccttcgggaagcgtggcgctttctcatagctcacgctgtaggtatctcagttcggtgtaggtcgttcgctccaagctgggctgtgtgcacgaaccccccgttcagcccgaccgctgcgccttatccggtaactatcgtcttgagtccaacccggtaagacacgacttatcgccactggcagcagccactggtaacaggattagcagagcgaggtatgtaggcggtgctacagagttcttgaagtggtggcctaactacggctacactagaaggacagtatttggtatctgcgctctgctgaagccagttaccttcggaaaaagagttggtagctcttgatccggcaaacaaaccaccgctggtagcggtggtttttttgtttgcaagcagcagattacgcgcagaaaaaaaggatctcaagaagatcctttgatcttttctacggggtctgacgctcagtggaacgaaaactcacgttaagggattttggtcatgagattatcaaaaaggatcttcacctagatccttttaaattaaaaatgaagttttaaatcaatctaaagtatatatgagtaaacttggtctgacagttaccaatgcttaatcagtgaggcacctatctcagcgatctgtctatttcgttcatccatagttgcctgactccccgtcgtgtagataactacgatacgggagggcttaccatctggccccagtgctgcaatgataccgcgagacccacgctcaccggctccagatttatcagcaataaaccagccagccggaagggccgagcgcagaagtggtcctgcaactttatccgcctccatccagtctattaattgttgccgggaagctagagtaagtagttcgccagttaatagtttgcgcaacgttgttgccattgctgcagccatgagattatcaaaaaggatcttcacctagatccttttcacgtagaaagccagtccgcagaaacggtgctgaccccggatgaatgtcagctactgggctatctggacaagggaaaacgcaagcgcaaagagaaagcaggtagcttgcagtgggcttacatggcgatagctagactgggcggttttatggacagcaagcgaaccggaattgccagctggggcgccctctggtaaggttgggaagccctgcaaagtaaactggatggctttcttgccgccaaggatctgatggcgcaggggatcaagctctgatcaagagacaggatgaggatcgtttcgcatgattgaacaagatggattgcacgcaggttctccggccgcttgggtggagaggctattcggctatgactgggcacaacagacaatcggctgctctgatgccgccgtgttccggctgtcagcgcaggggcgcccggttctttttgtcaagaccgacctgtccggtgccctgaatgaactgcaagacgaggcagcgcggctatcgtggctggccacgacgggcgttccttgcgcagctgtgctcgacgttgtcactgaagcgggaagggactggctgctattgggcgaagtgccggggcaggatctcctgtcatctcaccttgctcctgccgagaaagtatccatcatggctgatgcaatgcggcggctgcatacgcttgatccggctacctgcccattcgaccaccaagcgaaacatcgcatcgagcgagcacgtactcggatggaagccggtcttgtcgatcaggatgatctggacgaagagcatcaggggctcgcgccagccgaactgttcgccaggctcaaggcgagcatgcccgacggcgaggatctcgtcgtgacccatggcgatgcctgcttgccgaatatcatggtggaaaatggccgcttttctggattcatcgactgtggccggctgggtgtggcggaccgctatcaggacatagcgttggctacccgtgatattgctgaagagcttggcggcgaatgggctgaccgcttcctcgtgctttacggtatcgccgctcccgattcgcagcgcatcgccttctatcgccttcttgacgagttcttctgaattttgttaaaatttttgttaaatcagctcattttttaaccaataggccgaaatcggcaaaatcccttataaatcaaaagaatagaccgagatagggttgagtgttgttccagtttggaacaagagtccactattaaagaacgtggactccaacgtcaaagggcgaaaaaccgtctatcagggcgatggcccactacgtgaaccatcaccctaatcaagttttttggggtcgaggtgccgtaaagcactaaatcggaaccctaaagggagcccccgatttagagcttgacggggaaagccggcgaacgtggcgagaaaggaagggaagaaagcgaaaggagcgggcgctagggcgctggcaagtgtagcggtcacgctgcgcgtaaccaccacacccgccgcgcttaatgcgccgctacagggcgcgtccattcgccattcaggatcgaattaattcttaattaacatcatcaataatataccttattttggattgaagccaatatgataatgagggggtggagtttgtgacgtggcgcggggcgtgggaacggggcgggtgacgtagtagtgtggcggaagtgtgatgttgcaagtgtggcggaacacatgtaagcgacggatgtggcaaaagtgacgtttttggtgtgcgccggtgtacacaggaagtgacaattttcgcgcggttttaggcggatgttgtagtaaatttgggcgtaaccgagtaagatttggccattttcgcgggaaaactgaataagaggaagtgaaatctgaataattttgtgttactcatagcgcgtaatactgtaatagtaatcaattacggggtcattagttcatagcccatatatggagttccgcgttacataacttacggtaaatggcccgcctggctgaccgcccaacgacccccgcccattgacgtcaataatgacgtatgttcccatagtaacgccaatagggactttccattgacgtcaatgggtggagtatttacggtaaactgcccacttggcagtacatcaagtgtatcatatgccaagtacgccccctattgacgtcaatgacggtaaatggcccgcctggcattatgcccagtacatgaccttatgggactttcctacttggcagtacatctacgtattagtcatcgctattaccatggtgatgcggttttggcagtacatcaatgggcgtggatagcggtttgactcacggggatttccaagtctccaccccattgacgtcaatgggagtttgttttggcaccaaaatcaacgggactttccaaaatgtcgtaacaactccgccccattgacgcaaatgggcggtaggcgtgtacggtgggaggtctatataagcagagctggtttagtgaaccgtcagatccgctagagatctggtaccgtcgacgcggccgctcgagcctaagcttatgagcagcagtagttggcttctcttgagtttggtggcagtgacagcagcccagagtactatcgaggagcaggctaaatactttctggataagtttaacgccgaggccgaagacttgttctatcaatcttctctcgcttcatggaattacaatactaacatcactgaggagaacgtccagaatatgaacaatgctggcgacaaatggagcgccttcttgaaggagcagtctacccttgcacaaatgtatccactgcaggagatacagaaccttacagtaaagttgcagctccaggctctccagcagaacggatctagcgtgctttcagaggataaaagcaaaaggctgaacaccatacttaataccatgtccacaatttactctactggtaaagtatgtaaccccgacaaccctcaagaatgcctccttcttgagccaggcctcaatgagatcatggctaatagtctggactataatgaaagactgtgggcatgggagtcctggagatctgaagtagggaagcaactgaggcccctttatgaagagtacgtcgtacttaagaatgaaatggcccgcgctaaccactacgaggattacggcgattactggcgtggggactatgaagtaaatggtgtagatggatacgactatagtcgtgggcaattgattgaggatgtggagcacacttttgaggagataaaaccactctatgagcatcttcacgcatatgtgagagctaaactgatgaacgcctacccaagttacatcagtccaatcggatgtctcccagctcacctccttggcgacatgtggggacgtttctggaccaatctgtattccctcacagtccctttcgggcaaaagcctaatatagacgtgacagacgcaatggttgatcaggcttgggatgctcaaaggatttttaaggaagctgagaagttttttgtgtcagtcggtttgccaaatatgacacaaggcttctgggaaaatagcatgttgactgatcccggtaatgttcaaaaggctgtgtgtcaccctaccgcttgggaccttgggaaaggtgactttcgaatcttgatgtgtaccaaggtgacaatggatgactttcttacagcccataatgaaatgggtcacatccagtatgatatggcttatgcagctcaacctttcctcttgagaaatggtgcaaatgaaggttttcatgaagctgtaggggaaataatgtccctgagtgctgcaaccccaaagcatctcaagagtatcggattgttgagcccagattttcaagaagataacgagaccgaaatcaacttccttctgaaacaagccctcacaatagttggtactcttccattcacatacatgctggagaaatggcgttggatggtttttaagggggagatacctaaagatcagtggatgaaaaagtggtgggagatgaagcgtgagatcgtaggggtcgtggagccagtgcctcatgatgagacttactgtgacccagcatcactcttccacgttagcaatgactattcatttatacgttattacactcgcactctttaccagtttcaatttcaggaggctctgtgtcaggctgccaagcatgagggaccccttcacaagtgtgatattagtaacagtactgaggcaggccaaaaactgttcaatatgttgaggcttggcaaaagcgagccatggactctcgccttggaaaatgttgtcggggctaaaaacatgaatgtacgccctctgcttaactattttgagcccctttttacatggctcaaggaccagaataagaactcctttgtcggctggtcaacagactggtctccctatgcagaccctagtactcctcctactccttctccatcaaccccaccaactccatcccctagctgctgtcacccaaggctgtctctgcaccgacctgcactcgaagaccttctgttgggctctgaagctaacctgacctgtactcttactggcttgcgcgatgctagcggcgtgactttcacctggacacctagtagcggtaaaagtgctgtacaaggacctcctgaacgcgacctgtgtggttgctactctgtgtcttctgtacttcccggctgtgccgagccctggaatcacgggaaaacctttacctgcaccgccgcttaccctgagtcaaaaactcccctcactgccacattgagtaagtcagggaatacattcaggccagaggttcatttgttgcctcctccatctgaagaacttgctttgaacgagctggtcactctgacctgcttggctaggggtttctcccccaaagatgtacttgtacggtggttgcagggcagccaagagttgccccgcgaaaagtatttgacctgggcctcaagacaagaacccagccaggggactaccacatttgccgtgaccagtattctgcgtgtagccgctgaagattggaagaaaggggatacattttcttgcatggtagggcatgaggcccttcccctcgctttcactcagaagacaatagacagactcgccggaaagcctactcacgtgaatgttagcgtagtcatggctgaggttgacggaacttgctactgagatatccgatccaccggatctagataactgatcataatcagccataccacatttgtagaggttttacttgctttaaaaaacctcccacacctccccctgaacctgaaacataaaatgaatgcaattgttgttgttaacttgtttattgcagcttataatggttacaaataaagcaatagcatcacaaatttcacaaataaagcatttttttcactgcattctagttgtggtttgtccaaactcatcaatgtatcttaggtttagtgaaccgtcagatccgctagcgttacataacttacggtaaatggcccgcctggctgaccgcccaacgacccccgcccattgacgtcaataatgacgtatgttcccatagtaacgccaatagggactttccattgacgtcaatgggtggagtatttacggtaaactgcccacttggcagtacatcaagtgtatcatatgccaagtacgccccctattgacgtcaatgacggtaaatggcccgcctggcattatgcccagtacatgaccttatgggactttcctacttggcagtacatctacgtattagtcatcgctattaccatggtgatgcggttttggcagtacatcaatgggcgtggatagcggtttgactcacggggatttccaagtctccaccccattgacgtcaatgggagtttgttttggcaccaaaatcaacgggactttccaaaatgtcgtaacaactccgccccattgacgcaaatgggcggtaggcgtgtacggtgggaggtctatataagcagagctggtttagtgaaccgtcagatccgctagagatctggtaccgtcgacgcggccgctcgagcctaagcttatgaagaaccatctgcttttctggggagtacttgccgttttcataaaagccgtacatgttaaagcacaagaggacgaacgcattgtgttggttgataataaatgcaaatgtgctcggataacatctcggatcattcgtagctcagaggaccccaatgaggatatagtagagcgaaacatcagaattatagtacccctgaacaacagagagaacataagtgatcccacaagtccattgcggacacgctttgtttaccatttgtctgatctgtgtaaaaaatgtgatccaacagaggtggaactcgacaatcagatcgtcaccgccacccagtctaacatctgcgatgaagattcagctacagagacatgctacacatacgaccggaacaagtgctatactgccgttgtgccactcgtttacggtggagaaacaaagatggttgaaactgcacttacaccagatgcctgctatccagattgagatatccgatccaccggatctagataactgatcataatcagccataccacatttgtagaggttttacttgctttaaaaaacctcccacacctccccctgaacctgaaacataaaatgaatgcaattgttgttgttaacttgtttattgcagcttataatggttacaaataaagcaatagcatcacaaatttcacaaataaagcatttttttcactgcattctagttgtggtttgtccaaactcatcaatgtatcttaacgcggatctgggcgtggttaagggtgggaaagaatatataaggtgggggtcttatgtagttttgtatctgttttgcagcagccgccgccgccatgagcaccaactcgtttgatggaagcattgtgagctcatatttgacaacgcgcatgcccccatgggccggggtgcgtcagaatgtgatgggctccagcattgatggtcgccccgtcctgcccgcaaactctactaccttgacctacgagaccgtgtctggaacgccgttggagactgcagcctccgccgccgcttcagccgctgcagccaccgcccgcgggattgtgactgactttgctttcctgagcccgcttgcaagcagtgcagcttcccgttcatccgcccgcgatgacaagttgacggctcttttggcacaattggattctttgacccgggaacttaatgtcgtttctcagcagctgttggatctgcgccagcaggtttctgccctgaaggcttcctcccctcccaatgcggtttaaaacataaataaaaaaccagactctgtttggatttggatcaagcaagtgtcttgctgtctttatttaggggttttgcgcgcgcggtaggcccgggaccagcggtctcggtcgttgagggtcctgtgtattttttccaggacgtggtaaaggtgactctggatgttcagatacatgggcataagcccgtctctggggtggaggtagcaccactgcagagcttcatgctgcggggtggtgttgtagatgatccagtcgtagcaggagcgctgggcgtggtgcctaaaaatgtctttcagtagcaagctgattgccaggggcaggcccttggtgtaagtgtttacaaagcggttaagctgggatgggtgcatacgtggggatatgagatgcatcttggactgtatttttaggttggctatgttcccagccatatccctccggggattcatgttgtgcagaaccaccagcacagtgtatccggtgcacttgggaaatttgtcatgtagcttagaaggaaatgcgtggaagaacttggagacgcccttgtgacctccaagattttccatgcattcgtccataatgatggcaatgggcccacgggcggcggcctgggcgaagatatttctgggatcactaacgtcatagttgtgttccaggatgagatcgtcataggccatttttacaaagcgcgggcggagggtgccagactgcggtataatggttccatccggcccaggggcgtagttaccctcacagatttgcatttcccacgctttgagttcagatggggggatcatgtctacctgcggggcgatgaagaaaacggtttccggggtaggggagatcagctgggaagaaagcaggttcctgagcagctgcgacttaccgcagccggtgggcccgtaaatcacacctattaccggctgcaactggtagttaagagagctgcagctgccgtcatccctgagcaggggggccacttcgttaagcatgtccctgactcgcatgttttccctgaccaaatccgccagaaggcgctcgccgcccagcgatagcagttcttgcaaggaagcaaagtttttcaacggtttgagaccgtccgccgtaggcatgcttttgagcgtttgaccaagcagttccaggcggtcccacagctcggtcacctgctctacggcatctcgatccagcatatctcctcgtttcgcgggttggggcggctttcgctgtacggcagtagtcggtgctcgtccagacgggccagggtcatgtctttccacgggcgcagggtcctcgtcagcgtagtctgggtcacggtgaaggggtgcgctccgggctgcgcgctggccagggtgcgcttgaggctggtcctgctggtgctgaagcgctgccggtcttcgccctgcgcgtcggccaggtagcatttgaccatggtgtcatagtccagcccctccgcggcgtggcccttggcgcgcagcttgcccttggaggaggcgccgcacgaggggcagtgcagacttttgagggcgtagagcttgggcgcgagaaataccgattccggggagtaggcatccgcgccgcaggccccgcagacggtctcgcattccacgagccaggtgagctctggccgttcggggtcaaaaaccaggtttcccccatgctttttgatgcgtttcttacctctggtttccatgagccggtgtccacgctcggtgacgaaaaggctgtccgtgtccccgtatacagacttgagaggcctgtcctcgagcggtgttccgcggtcctcctcgtatagaaactcggaccactctgagacaaaggctcgcgtccaggccagcacgaaggaggctaagtgggaggggtagcggtcgttgtccactagggggtccactcgctccagggtgtgaagacacatgtcgccctcttcggcatcaaggaaggtgattggtttgtaggtgtaggccacgtgaccgggtgttcctgaaggggggctataaaagggggtgggggcgcgttcgtcctcactctcttccgcatcgctgtctgcgagggccagctgttggggtgagtactccctctgaaaagcgggcatgacttctgcgctaagattgtcagtttccaaaaacgaggaggatttgatattcacctggcccgcggtgatgcctttgagggtggccgcatccatctggtcagaaaagacaatctttttgttgtcaagcttggtggcaaacgacccgtagagggcgttggacagcaacttggcgatggagcgcagggtttggtttttgtcgcgatcggcgcgctccttggccgcgatgtttagctgcacgtattcgcgcgcaacgcaccgccattcgggaaagacggtggtgcgctcgtcgggcaccaggtgcacgcgccaaccgcggttgtgcagggtgacaaggtcaacgctggtggctacctctccgcgtaggcgctcgttggtccagcagaggcggccgcccttgcgcgagcagaatggcggtagggggtctagctgcgtctcgtccggggggtctgcgtccacggtaaagaccccgggcagcaggcgcgcgtcgaagtagtctatcttgcatccttgcaagtctagcgcctgctgccatgcgcgggcggcaagcgcgcgctcgtatgggttgagtgggggaccccatggcatggggtgggtgagcgcggaggcgtacatgccgcaaatgtcgtaaacgtagaggggctctctgagtattccaagatatgtagggtagcatcttccaccgcggatgctggcgcgcacgtaatcgtatagttcgtgcgagggagcgaggaggtcgggaccgaggttgctacgggcgggctgctctgctcggaagactatctgcctgaagatggcatgtgagttggatgatatggttggacgctggaagacgttgaagctggcgtctgtgagacctaccgcgtcacgcacgaaggaggcgtaggagtcgcgcagcttgttgaccagctcggcggtgacctgcacgtctagggcgcagtagtccagggtttccttgatgatgtcatacttatcctgtcccttttttttccacagctcgcggttgaggacaaactcttcgcggtctttccagtactcttggatcggaaacccgtcggcctccgaacggtaagagcctagcatgtagaactggttgacggcctggtaggcgcagcatcccttttctacgggtagcgcgtatgcctgcgcggccttccggcatgaccagcatgaagggcacgagctgcttcccaaaggcccccatccaagtataggtctctacatcgtaggtgacaaagagacgctcggtgcgaggatgcgagccgatcgggaagaactggatctcccgccaccaattggaggagtggctattgatgtggtgaaagtagaagtccctgcgacgggccgaacactcgtgctggcttttgtaaaaacgtgcgcagtactggcagcggtgcacgggctgtacatcctgcacgaggttgacctgacgaccgcgcacaaggaagcagagtgggaatttgagcccctcgcctggcgggtttggctggtggtcttctacttcggctgcttgtccttgaccgtctggctgctcgaggggagttacggtggatcggaccaccacgccgcgcgagcccaaagtccagatgtccgcgcgcggcggtcggagcttgatgacaacatcgcgcagatgggagctgtccatggtctggagctcccgcggcgtcaggtcaggcgggagctcctgcaggtttacctcgcatagacgggtcagggcgcgggctagatccaggtgatacctaatttccaggggctggttggtggcggcgtcgatggcttgcaagaggccgcatccccgcggcgcgactacggtaccgcgcggcgggcggtgggccgcgggggtgtccttggatgatgcatctaaaagcggtgacgcgggcgagcccccggaggtagggggggctccggacccgccgggagagggggcaggggcacgtcggcgccgcgcgcgggcaggagctggtgctgcgcgcgtaggttgctggcgaacgcgacgacgcggcggttgatctcctgaatctggcgcctctgcgtgaagacgacgggcccggtgagcttgaacctgaaagagagttcgacagaatcaatttcggtgtcgttgacggcggcctggcgcaaaatctcctgcacgtctcctgagttgtcttgataggcgatctcggccatgaactgctcgatctcttcctcctggagatctccgcgtccggctcgctccacggtggcggcgaggtcgttggaaatgcgggccatgagctgcgagaaggcgttgaggcctccctcgttccagacgcggctgtagaccacgcccccttcggcatcgcgggcgcgcatgaccacctgcgcgagattgagctccacgtgccgggcgaagacggcgtagtttcgcaggcgctgaaagaggtagttgagggtggtggcggtgtgttctgccacgaagaagtacataacccagcgtcgcaacgtggattcgttgataattgttgtgtaggtactccgccgccgagggacctgagcgagtccgcatcgaccggatcggaaaacctctcgagaaaggcgtctaaccagtcacagtcgcaaggtaggctgagcaccgtggcgggcggcagcgggcggcggtcggggttgtttctggcggaggtgctgctgatgatgtaattaaagtaggcggtcttgagacggcggatggtcgacagaagcaccatgtccttgggtccggcctgctgaatgcgcaggcggtcggccatgccccaggcttcgttttgacatcggcgcaggtctttgtagtagtcttgcatgagcctttctaccggcacttcttcttctccttcctcttgtcctgcatctcttgcatctatcgctgcggcggcggcggagtttggccgtaggtggcgccctcttcctcccatgcgtgtgaccccgaagcccctcatcggctgaagcagggctaggtcggcgacaacgcgctcggctaatatggcctgctgcacctgcgtgagggtagactggaagtcatccatgtccacaaagcggtggtatgcgcccgtgttgatggtgtaagtgcagttggccataacggaccagttaacggtctggtgacccggctgcgagagctcggtgtacctgagacgcgagtaagccctcgagtcaaatacgtagtcgttgcaagtccgcaccaggtactggtatcccaccaaaaagtgcggcggcggctggcggtagaggggccagcgtagggtggccggggctccgggggcgagatcttccaacataaggcgatgatatccgtagatgtacctggacatccaggtgatgccggcggcggtggtggaggcgcgcggaaagtcgcggacgcggttccagatgttgcgcagcggcaaaaagtgctccatggtcgggacgctctggccggtcaggcgcgcgcaatcgttgacgctctagcgtgcaaaaggagagcctgtaagcgggcactcttccgtggtctggtggataaattcgcaagggtatcatggcggacgaccggggttcgagccccgtatccggccgtccgccgtgatccatgcggttaccgcccgcgtgtcgaacccaggtgtgcgacgtcagacaacgggggagtgctccttttggcttccttccaggcgcggcggctgctgcgctagcttttttggccactggccgcgcgcagcgtaagcggttaggctggaaagcgaaagcattaagtggctcgctccctgtagccggagggttattttccaagggttgagtcgcgggacccccggttcgagtctcggaccggccggactgcggcgaacgggggtttgcctccccgtcatgcaagaccccgcttgcaaattcctccggaaacagggacgagccccttttttgcttttcccagatgcatccggtgctgcggcagatgcgcccccctcctcagcagcggcaagagcaagagcagcggcagacatgcagggcaccctcccctcctcctaccgcgtcaggaggggcgacatccgcggttgacgcggcagcagatggtgattacgaacccccgcggcgccgggcccggcactacctggacttggaggagggcgagggcctggcgcggctaggagcgccctctcctgagcggcacccaagggtgcagctgaagcgtgatacgcgtgaggcgtacgtgccgcggcagaacctgtttcgcgaccgcgagggagaggagcccgaggagatgcgggatcgaaagttccacgcagggcgcgagctgcggcatggcctgaatcgcgagcggttgctgcgcgaggaggactttgagcccgacgcgcgaaccgggattagtcccgcgcgcgcacacgtggcggccgccgacctggtaaccgcatacgagcagacggtgaaccaggagattaactttcaaaaaagctttaacaaccacgtgcgtacgcttgtggcgcgcgaggaggtggctataggactgatgcatctgtgggactttgtaagcgcgctggagcaaaacccaaatagcaagccgctcatggcgcagctgttccttatagtgcagcacagcagggacaacgaggcattcagggatgcgctgctaaacatagtagagcccgagggccgctggctgctcgatttgataaacatcctgcagagcatagtggtgcaggagcgcagcttgagcctggctgacaaggtggccgccatcaactattccatgcttagcctgggcaagttttacgcccgcaagatataccataccccttacgttcccatagacaaggaggtaaagatcgaggggttctacatgcgcatggcgctgaaggtgcttaccttgagcgacgacctgggcgtttatcgcaacgagcgcatccacaaggccgtgagcgtgagccggcggcgcgagctcagcgaccgcgagctgatgcacagcctgcaaagggccctggctggcacgggcagcggcgatagagaggccgagtcctactttgacgcgggcgctgacctgcgctgggccccaagccgacgcgccctggaggcagctggggccggacctgggctggcggtggcacccgcgcgcgctggcaacgtcggcggcgtggaggaatatgacgaggacgatgagtacgagccagaggacggcgagtactaagcggtgatgtttctgatcagatgatgcaagacgcaacggacccggcggtgcgggcggcgctgcagagccagccgtccggccttaactccacggacgactggcgccaggtcatggaccgcatcatgtcgctgactgcgcgcaatcctgacgcgttccggcagcagccgcaggccaaccggctctccgcaattctggaagcggtggtcccggcgcgcgcaaaccccacgcacgagaaggtgctggcgatcgtaaacgcgctggccgaaaacagggccatccggcccgacgaggccggcctggtctacgacgcgctgcttcagcgcgtggctcgttacaacagcggcaacgtgcagaccaacctggaccggctggtgggggatgtgcgcgaggccgtggcgcagcgtgagcgcgcgcagcagcagggcaacctgggctccatggttgcactaaacgccttcctgagtacacagcccgccaacgtgccgcggggacaggaggactacaccaactttgtgagcgcactgcggctaatggtgactgagacaccgcaaagtgaggtgtaccagtctgggccagactattttttccagaccagtagacaaggcctgcagaccgtaaacctgagccaggctttcaaaaacttgcaggggctgtggggggtgcgggctcccacaggcgaccgcgcgaccgtgtctagcttgctgacgcccaactcgcgcctgttgctgctgctaatagcgcccttcacggacagtggcagcgtgtcccgggacacatacctaggtcacttgctgacactgtaccgcgaggccataggtcaggcgcatgtggacgagcatactttccaggagattacaagtgtcagccgcgcgctggggcaggaggacacgggcagcctggaggcaaccctaaactacctgctgaccaaccggcggcagaagatcccctcgttgcacagtttaaacagcgaggaggagcgcattttgcgctacgtgcagcagagcgtgagccttaacctgatgcgcgacggggtaacgcccagcgtggcgctggacatgaccgcgcgcaacatggaaccgggcatgtatgcctcaaaccggccgtttatcaaccgcctaatggactacttgcatcgcgcggccgccgtgaaccccgagtatttcaccaatgccatcttgaacccgcactggctaccgccccctggtttctacaccgggggattcgaggtgcccgagggtaacgatggattcctctgggacgacatagacgacagcgtgttttccccgcaaccgcagaccctgctagagttgcaacagcgcgagcaggcagaggcggcgctgcgaaaggaaagcttccgcaggccaagcagcttgtccgatctaggcgctgcggccccgcggtcagatgctagtagcccatttccaagcttgatagggtctcttaccagcactcgcaccacccgcccgcgcctgctgggcgaggaggagtacctaaacaactcgctgctgcagccgcagcgcgaaaaaaacctgcctccggcatttcccaacaacgggatagagagcctagtggacaagatgagtagatggaagacgtacgcgcaggagcacagggacgtgccaggcccgcgcccgcccacccgtcgtcaaaggcacgaccgtcagcggggtctggtgtgggaggacgatgactcggcagacgacagcagcgtcctggatttgggagggagtggcaacccgtttgcgcaccttcgccccaggctggggagaatgttttaaaaaaaaaaaagcatgatgcaaaataaaaaactcaccaaggccatggcaccgagcgttggttttcttgtattccccttagtatgcggcgcgcggcgatgtatgaggaaggtcctcctccctcctacgagagtgtggtgagcgcggcgccagtggcggcggcgctgggttctcccttcgatgctcccctggacccgccgtttgtgcctccgcggtacctgcggcctaccggggggagaaacagcatccgttactctgagttggcacccctattcgacaccacccgtgtgtacctggtggacaacaagtcaacggatgtggcatccctgaactaccagaacgaccacagcaactttctgaccacggtcattcaaaacaatgactacagcccgggggaggcaagcacacagaccatcaatcttgacgaccggtcgcactggggcggcgacctgaaaaccatcctgcataccaacatgccaaatgtgaacgagttcatgtttaccaataagtttaaggcgcgggtgatggtgtcgcgcttgcctactaaggacaatcaggtggagctgaaatacgagtgggtggagttcacgctgcccgagggcaactactccgagaccatgaccatagaccttatgaacaacgcgatcgtggagcactacttgaaagtgggcagacagaacggggttctggaaagcgacatcggggtaaagtttgacacccgcaacttcagactggggtttgaccccgtcactggtcttgtcatgcctggggtatatacaaacgaagccttccatccagacatcattttgctgccaggatgcggggtggacttcacccacagccgcctgagcaacttgttgggcatccgcaagcggcaacccttccaggagggctttaggatcacctacgatgatctggagggtggtaacattcccgcactgttggatgtggacgcctaccaggcgagcttgaaagatgacaccgaacagggcgggggtggcgcaggcggcagcaacagcagtggcagcggcgcggaagagaactccaacgcggcagccgcggcaatgcagccggtggaggacatgaacgatcatgccattcgcggcgacacctttgccacacgggctgaggagaagcgcgctgaggccgaagcagcggccgaagctgccgcccccgctgcgcaacccgaggtcgagaagcctcagaagaaaccggtgatcaaacccctgacagaggacagcaagaaacgcagttacaacctaataagcaatgacagcaccttcacccagtaccgcagctggtaccttgcatacaactacggcgaccctcagaccggaatccgctcatggaccctgctttgcactcctgacgtaacctgcggctcggagcaggtctactggtcgttgccagacatgatgcaagaccccgtgaccttccgctccacgcgccagatcagcaactttccggtggtgggcgccgagctgttgcccgtgcactccaagagcttctacaacgaccaggccgtctactcccaactcatccgccagtttacctctctgacccacgtgttcaatcgctttcccgagaaccagattttggcgcgcccgccagcccccaccatcaccaccgtcagtgaaaacgttcctgctctcacagatcacgggacgctaccgctgcgcaacagcatcggaggagtccagcgagtgaccattactgacgccagacgccgcacctgcccctacgtttacaaggccctgggcatagtctcgccgcgcgtcctatcgagccgcactttttgagcaagcatgtccatccttatatcgcccagcaataacacaggctggggcctgcgcttcccaagcaagatgtttggcggggccaagaagcgctccgaccaacacccagtgcgcgtgcgcgggcactaccgcgcgccctggggcgcgcacaaacgcggccgcactgggcgcaccaccgtcgatgacgccatcgacgcggtggtggaggaggcgcgcaactacacgcccacgccgccaccagtgtccacagtggacgcggccattcagaccgtggtgcgcggagcccggcgctatgctaaaatgaagagacggcggaggcgcgtagcacgtcgccaccgccgccgacccggcactgccgcccaacgcgcggcggcggccctgcttaaccgcgcacgtcgcaccggccgacgggcggccatgcgggccgctcgaaggctggccgcgggtattgtcactgtgccccccaggtccaggcgacgagcggccgccgcagcagccgcggccattagtgctatgactcagggtcgcaggggcaacgtgtattgggtgcgcgactcggttagcggcctgcgcgtgcccgtgcgcacccgccccccgcgcaactagattgcaagaaaaaactacttagactcgtactgttgtatgtatccagcggcggcggcgcgcaacgaagctatgtccaagcgcaaaatcaaagaagagatgctccaggtcatcgcgccggagatctatggccccccgaagaaggaagagcaggattacaagccccgaaagctaaagcgggtcaaaaagaaaaagaaagatgatgatgatgaacttgacgacgaggtggaactgctgcacgctaccgcgcccaggcgacgggtacagtggaaaggtcgacgcgtaaaacgtgttttgcgacccggcaccaccgtagtctttacgcccggtgagcgctccacccgcacctacaagcgcgtgtatgatgaggtgtacggcgacgaggacctgcttgagcaggccaacgagcgcctcggggagtttgcctacggaaagcggcataaggacatgctggcgttgccgctggacgagggcaacccaacacctagcctaaagcccgtaacactgcagcaggtgctgcccgcgcttgcaccgtccgaagaaaagcgcggcctaaagcgcgagtctggtgacttggcacccaccgtgcagctgatggtacccaagcgccagcgactggaagatgtcttggaaaaaatgaccgtggaacctgggctggagcccgaggtccgcgtgcggccaatcaagcaggtggcgccgggactgggcgtgcagaccgtggacgttcagatacccactaccagtagcaccagtattgccaccgccacagagggcatggagacacaaacgtccccggttgcctcagcggtggcggatgccgcggtgcaggcggtcgctgcggccgcgtccaagacctctacggaggtgcaaacggacccgtggatgtttcgcgtttcagccccccggcgcccgcgccgttcgaggaagtacggcgccgccagcgcgctactgcccgaatatgccctacatccttccattgcgcctacccccggctatcgtggctacacctaccgccccagaagacgagcaactacccgacgccgaaccaccactggaacccgccgccgccgtcgccgtcgccagcccgtgctggccccgatttccgtgcgcagggtggctcgcgaaggaggcaggaccctggtgctgccaacagcgcgctaccaccccagcatcgtttaaaagccggtctttgtggttcttgcagatatggccctcacctgccgcctccgtttcccggtgccgggattccgaggaagaatgcaccgtaggaggggcatggccggccacggcctgacgggcggcatgcgtcgtgcgcaccaccggcggcggcgcgcgtcgcaccgtcgcatgcgcggcggtatcctgcccctccttattccactgatcgccgcggcgattggcgccgtgcccggaattgcatccgtggccttgcaggcgcagagacactgattaaaaacaagttgcatgtggaaaaatcaaaataaaaagtctggactctcacgctcgcttggtcctgtaactattttgtagaatggaagacatcaactttgcgtctctggccccgcgacacggctcgcgcccgttcatgggaaactggcaagatatcggcaccagcaatatgagcggtggcgccttcagctggggctcgctgtggagcggcattaaaaatttcggttccaccgttaagaactatggcagcaaggcctggaacagcagcacaggccagatgctgagggataagttgaaagagcaaaatttccaacaaaaggtggtagatggcctggcctctggcattagcggggtggtggacctggccaaccaggcagtgcaaaataagattaacagtaagcttgatccccgccctcccgtagaggagcctccaccggccgtggagacagtgtctccagaggggcgtggcgaaaagcgtccgcgccccgacagggaagaaactctggtgacgcaaatagacgagcctccctcgtacgaggaggcactaaagcaaggcctgcccaccacccgtcccatcgcgcccatggctaccggagtgctgggccagcacacacccgtaacgctggacctgcctccccccgccgacacccagcagaaacctgtgctgccaggcccgaccgccgttgttgtaacccgtcctagccgcgcgtccctgcgccgcgccgccagcggtccgcgatcgttgcggcccgtagccagtggcaactggcaaagcacactgaacagcatcgtgggtctgggggtgcaatccctgaagcgccgacgatgcttctgatagctaacgtgtcgtatgtgtgtcatgtatgcgtccatgtcgccgccagaggagctgctgagccgccgcgcgcccgctttccaagatggctaccccttcgatgatgccgcagtggtcttacatgcacatctcgggccaggacgcctcggagtacctgagccccgggctggtgcagtttgcccgcgccaccgagacgtacttcagcctgaataacaagtttagaaaccccacggtggcgcctacgcacgacgtgaccacagaccggtcccagcgtttgacgctgcggttcatccctgtggaccgtgaggatactgcgtactcgtacaaggcgcggttcaccctagctgtgggtgataaccgtgtgctggacatggcttccacgtactttgacatccgcggcgtgctggacaggggccctacttttaagccctactctggcactgcctacaacgccctggctcccaagggtgccccaaatccttgcgaatgggatgaagctgctactgctcttgaaataaacctagaagaagaggacgatgacaacgaagacgaagtagacgagcaagctgagcagcaaaaaactcacgtatttgggcaggcgccttattctggtataaatattacaaaggagggtattcaaataggtgtcgaaggtcaaacacctaaatatgccgataaaacatttcaacctgaacctcaaataggagaatctcagtggtacgaaacagaaattaatcatgcagctgggagagtcctaaaaaagactaccccaatgaaaccatgttacggttcatatgcaaaacccacaaatgaaaatggagggcaaggcattcttgtaaagcaacaaaatggaaagctagaaagtcaagtggaaatgcaatttttctcaactactgaggcagccgcaggcaatggtgataacttgactcctaaagtggtattgtacagtgaagatgtagatatagaaaccccagacactcatatttcttacatgcccactattaaggaaggtaactcacgagaactaatgggccaacaatctatgcccaacaggcctaattacattgcttttagggacaattttattggtctaatgtattacaacagcacgggtaatatgggtgttctggcgggccaagcatcgcagttgaatgctgttgtagatttgcaagacagaaacacagagctttcataccagcttttgcttgattccattggtgatagaaccaggtacttttctatgtggaatcaggctgttgacagctatgatccagatgttagaattattgaaaatcatggaactgaagatgaacttccaaattactgctttccactgggaggtgtgattaatacagagactcttaccaaggtaaaacctaaaacaggtcaggaaaatggatgggaaaaagatgctacagaattttcagataaaaatgaaataagagttggaaataattttgccatggaaatcaatctaaatgccaacctgtggagaaatttcctgtactccaacatagcgctgtatttgcccgacaagctaaagtacagtccttccaacgtaaaaatttctgataacccaaacacctacgactacatgaacaagcgagtggtggctcccgggctagtggactgctacattaaccttggagcacgctggtcccttgactatatggacaacgtcaacccatttaaccaccaccgcaatgctggcctgcgctaccgctcaatgttgctgggcaatggtcgctatgtgcccttccacatccaggtgcctcagaagttctttgccattaaaaacctccttctcctgccgggctcatacacctacgagtggaacttcaggaaggatgttaacatggttctgcagagctccctaggaaatgacctaagggttgacggagccagcattaagtttgatagcatttgcctttacgccaccttcttccccatggcccacaacaccgcctccacgcttgaggccatgcttagaaacgacaccaacgaccagtcctttaacgactatctctccgccgccaacatgctctaccctatacccgccaacgctaccaacgtgcccatatccatcccctcccgcaactgggcggctttccgcggctgggccttcacgcgccttaagactaaggaaaccccatcactgggctcgggctacgacccttattacacctactctggctctataccctacctagatggaaccttttacctcaaccacacctttaagaaggtggccattacctttgactcttctgtcagctggcctggcaatgaccgcctgcttacccccaacgagtttgaaattaagcgctcagttgacggggagggttacaacgttgcccagtgtaacatgaccaaagactggttcctggtacaaatgctagctaactataacattggctaccagggcttctatatcccagagagctacaaggaccgcatgtactccttctttagaaacttccagcccatgagccgtcaggtggtggatgatactaaatacaaggactaccaacaggtgggcatcctacaccaacacaacaactctggatttgttggctaccttgcccccaccatgcgcgaaggacaggcctaccctgctaacttcccctatccgcttataggcaagaccgcagttgacagcattacccagaaaaagtttctttgcgatcgcaccctttggcgcatcccattctccagtaactttatgtccatgggcgcactcacagacctgggccaaaaccttctctacgccaactccgcccacgcgctagacatgacttttgaggtggatcccatggacgagcccacccttctttatgttttgtttgaagtctttgacgtggtccgtgtgcaccagccgcaccgcggcgtcatcgaaaccgtgtacctgcgcacgcccttctcggccggcaacgccacaacataaagaagcaagcaacatcaacaacagctgccgccatgggctccagtgagcaggaactgaaagccattgtcaaagatcttggttgtgggccatattttttgggcacctatgacaagcgctttccaggctttgtttctccacacaagctcgcctgcgccatagtcaatacggccggtcgcgagactgggggcgtacactggatggcctttgcctggaacccgcactcaaaaacatgctacctctttgagccctttggcttttctgaccagcgactcaagcaggtttaccagtttgagtacgagtcactcctgcgccgtagcgccattgcttcttcccccgaccgctgtataacgctggaaaagtccacccaaagcgtacaggggcccaactcggccgcctgtggactattctgctgcatgtttctccacgcctttgccaactggccccaaactcccatggatcacaaccccaccatgaaccttattaccggggtacccaactccatgctcaacagtccccaggtacagcccaccctgcgtcgcaaccaggaacagctctacagcttcctggagcgccactcgccctacttccgcagccacagtgcgcagattaggagcgccacttctttttgtcacttgaaaaacatgtaaaaataatgtactagagacactttcaataaaggcaaatgcttttatttgtacactctcgggtgattatttacccccacccttgccgtctgcgccgtttaaaaatcaaaggggttctgccgcgcatcgctatgcgccactggcagggacacgttgcgatactggtgtttagtgctccacttaaactcaggcacaaccatccgcggcagctcggtgaagttttcactccacaggctgcgcaccatcaccaacgcgtttagcaggtcgggcgccgatatcttgaagtcgcagttggggcctccgccctgcgcgcgcgagttgcgatacacagggttgcagcactggaacactatcagcgccgggtggtgcacgctggccagcacgctcttgtcggagatcagatccgcgtccaggtcctccgcgttgctcagggcgaacggagtcaactttggtagctgccttcccaaaaagggcgcgtgcccaggctttgagttgcactcgcaccgtagtggcatcaaaaggtgaccgtgcccggtctgggcgttaggatacagcgcctgcataaaagccttgatctgcttaaaagccacctgagcctttgcgccttcagagaagaacatgccgcaagacttgccggaaaactgattggccggacaggccgcgtcgtgcacgcagcaccttgcgtcggtgttggagatctgcaccacatttcggccccaccggttcttcacgatcttggccttgctagactgctccttcagcgcgcgctgcccgttttcgctcgtcacatccatttcaatcacgtgctccttatttatcataatgcttccgtgtagacacttaagctcgccttcgatctcagcgcagcggtgcagccacaacgcgcagcccgtgggctcgtgatgcttgtaggtcacctctgcaaacgactgcaggtacgcctgcaggaatcgccccatcatcgtcacaaaggtcttgttgctggtgaaggtcagctgcaacccgcggtgctcctcgttcagccaggtcttgcatacggccgccagagcttccacttggtcaggcagtagtttgaagttcgcctttagatcgttatccacgtggtacttgtccatcagcgcgcgcgcagcctccatgcccttctcccacgcagacacgatcggcacactcagcgggttcatcaccgtaatttcactttccgcttcgctgggctcttcctcttcctcttgcgtccgcataccacgcgccactgggtcgtcttcattcagccgccgcactgtgcgcttacctcctttgccatgcttgattagcaccggtgggttgctgaaacccaccatttgtagcgccacatcttctctttcttcctcgctgtccacgattacctctggtgatggcgggcgctcgggcttgggagaagggcgcttctttttcttcttgggcgcaatggccaaatccgccgccgaggtcgatggccgcgggctgggtgtgcgcggcaccagcgcgtcttgtgatgagtcttcctcgtcctcggactcgatacgccgcctcatccgcttttttgggggcgcccggggaggcggcggcgacggggacggggacgacacgtcctccatggttgggggacgtcgcgccgcaccgcgtccgcgctcgggggtggtttcgcgctgctcctcttcccgactggccatttccttctcctataggcagaaaaagatcatggagtcagtcgagaagaaggacagcctaaccgccccctctgagttcgccaccaccgcctccaccgatgccgccaacgcgcctaccaccttccccgtcgaggcacccccgcttgaggaggaggaagtgattatcgagcaggacccaggttttgtaagcgaagacgacgaggaccgctcagtaccaacagaggataaaaagcaagaccaggacaacgcagaggcaaacgaggaacaagtcgggcggggggacgaaaggcatggcgactacctagatgtgggagacgacgtgctgttgaagcatctgcagcgccagtgcgccattatctgcgacgcgttgcaagagcgcagcgatgtgcccctcgccatagcggatgtcagccttgcctacgaacgccacctattctcaccgcgcgtaccccccaaacgccaagaaaacggcacatgcgagcccaacccgcgcctcaacttctaccccgtatttgccgtgccagaggtgcttgccacctatcacatctttttccaaaactgcaagatacccctatcctgccgtgccaaccgcagccgagcggacaagcagctggccttgcggcagggcgctgtcatacctgatatcgcctcgctcaacgaagtgccaaaaatctttgagggtcttggacgcgacgagaagcgcgcggcaaacgctctgcaacaggaaaacagcgaaaatgaaagtcactctggagtgttggtggaactcgagggtgacaacgcgcgcctagccgtactaaaacgcagcatcgaggtcacccactttgcctacccggcacttaacctaccccccaaggtcatgagcacagtcatgagtgagctgatcgtgcgccgtgcgcagcccctggagagggatgcaaatttgcaagaacaaacagaggagggcctacccgcagttggcgacgagcagctagcgcgctggcttcaaacgcgcgagcctgccgacttggaggagcgacgcaaactaatgatggccgcagtgctcgttaccgtggagcttgagtgcatgcagcggttctttgctgacccggagatgcagcgcaagctagaggaaacattgcactacacctttcgacagggctacgtacgccaggcctgcaagatctccaacgtggagctctgcaacctggtctcctaccttggaattttgcacgaaaaccgccttgggcaaaacgtgcttcattccacgctcaagggcgaggcgcgccgcgactacgtccgcgactgcgtttacttatttctatgctacacctggcagacggccatgggcgtttggcagcagtgcttggaggagtgcaacctcaaggagctgcagaaactgctaaagcaaaacttgaaggacctatggacggccttcaacgagcgctccgtggccgcgcacctggcggacatcattttccccgaacgcctgcttaaaaccctgcaacagggtctgccagacttcaccagtcaaagcatgttgcagaactttaggaactttatcctagagcgctcaggaatcttgcccgccacctgctgtgcacttcctagcgactttgtgcccattaagtaccgcgaatgccctccgccgctttggggccactgctaccttctgcagctagccaactaccttgcctaccactctgacataatggaagacgtgagcggtgacggtctactggagtgtcactgtcgctgcaacctatgcaccccgcaccgctccctggtttgcaattcgcagctgcttaacgaaagtcaaattatcggtacctttgagctgcagggtccctcgcctgacgaaaagtccgcggctccggggttgaaactcactccggggctgtggacgtcggcttaccttcgcaaatttgtacctgaggactaccacgcccacgagattaggttctacgaagaccaatcccgcccgcctaatgcggagcttaccgcctgcgtcattacccagggccacattcttggccaattgcaagccatcaacaaagcccgccaagagtttctgctacgaaagggacggggggtttacttggacccccagtccggcgaggagctcaacccaatccccccgccgccgcagccctatcagcagcagccgcgggcccttgcttcccaggatggcacccaaaaagaagctgcagctgccgccgccacccacggacgaggaggaatactgggacagtcaggcagaggaggttttggacgaggaggaggaggacatgatggaagactgggagagcctagacgaggaagcttccgaggtcgaagaggtgtcagacgaaacaccgtcaccctcggtcgcattcccctcgccggcgccccagaaatcggcaaccggttccagcatggctacaacctccgctcctcaggcgccgccggcactgcccgttcgccgacccaaccgtagatgggacaccactggaaccagggccggtaagtccaagcagccgccgccgttagcccaagagcaacaacagcgccaaggctaccgctcatggcgcgggcacaagaacgccatagttgcttgcttgcaagactgtgggggcaacatctccttcgcccgccgctttcttctctaccatcacggcgtggccttcccccgtaacatcctgcattactaccgtcatctctacagcccatactgcaccggcggcagcggcagcaacagcagcggccacacagaagcaaaggcgaccggatagcaagactctgacaaagcccaagaaatccacagcggcggcagcagcaggaggaggagcgctgcgtctggcgcccaacgaacccgtatcgacccgcgagcttagaaacaggatttttcccactctgtatgctatatttcaacagagcaggggccaagaacaagagctgaaaataaaaaacaggtctctgcgatccctcacccgcagctgcctgtatcacaaaagcgaagatcagcttcggcgcacgctggaagacgcggaggctctcttcagtaaatactgcgcgctgactcttaaggactagtttcgcgccctttctcaaatttaagcgcgaaaactacgtcatctccagcggccacacccggcgccagcacctgttgtcagcgccattatgagcaaggaaattcccacgccctacatgtggagttaccagccacaaatgggacttgcggctggagctgcccaagactactcaacccgaataaactacatgagcgcgggaccccacatgatatcccgggtcaacggaatacgcgcccaccgaaaccgaattctcctggaacaggcggctattaccaccacacctcgtaataaccttaatccccgtagttggcccgctgccctggtgtaccaggaaagtcccgctcccaccactgtggtacttcccagagacgcccaggccgaagttcagatgactaactcaggggcgcagcttgcgggcggctttcgtcacagggtgcggtcgcccgggcagggtataactcacctgacaatcagagggcgaggtattcagctcaacgacgagtcggtgagctcctcgcttggtctccgtccggacgggacatttcagatcggcggcgccggccgctcttcattcacgcctcgtcaggcaatcctaactctgcagacctcgtcctctgagccgcgctctggaggcattggaactctgcaatttattgaggagtttgtgccatcggtctactttaaccccttctcgggacctcccggccactatccggatcaatttattcctaactttgacgcggtaaaggactcggcggacggctacgactgaatgttaagtggagaggcagagcaactgcgcctgaaacacctggtccactgtcgccgccacaagtgctttgcccgcgactccggtgagttttgctactttgaattgcccgaggatcatatcgagggcccggcgcacggcgtccggcttaccgcccagggagagcttgcccgtagcctgattcgggagtttacccagcgccccctgctagttgagcgggacaggggaccctgtgttctcactgtgatttgcaactgtcctaaccctggattacatcaagatcctctagttaatgtcaggtcgcctaagtcgattaactagagtacccggggatcttattccctttaactaataaaaaaaaataataaagcatcacttacttaaaatcagttagcaaatttctgtccagtttattcagcagcacctccttgccctcctcccagctctggtattgcagcttcctcctggctgcaaactttctccacaatctaaatggaatgtcagtttcctcctgttcctgtccatccgcacccactatcttcatgttgttgcagatgaagcgcgcaagaccgtctgaagataccttcaaccccgtgtatccatatgacacggaaaccggtcctccaactgtgccttttcttactcctccctttgtatcccccaatgggtttcaagagagtccccctggggtactctctttgcgcctatccgaacctctagttacctccaatggcatgcttgcgctcaaaatgggcaacggcctctctctggacgaggccggcaaccttacctcccaaaatgtaaccactgtgagcccacctctcaaaaaaaccaagtcaaacataaacctggaaatatctgcacccctcacagttacctcagaagccctaactgtggctgccgccgcacctctaatggtcgcgggcaacacactcaccatgcaatcacaggccccgctaaccgtgcacgactccaaacttagcattgccacccaaggacccctcacagtgtcagaaggaaagctagccctgcaaacatcaggccccctcaccaccaccgatagcagtacccttactatcactgcctcaccccctctaactactgccactggtagcttgggcattgacttgaaagagcccatttatacacaaaatggaaaactaggactaaagtacggggctcctttgcatgtaacagacgacctaaacactttgaccgtagcaactggtccaggtgtgactattaataatacttccttgcaaactaaagttactggagccttgggttttgattcacaaggcaatatgcaacttaatgtagcaggaggactaaggattgattctcaaaacagacgccttatacttgatgttagttatccgtttgatgctcaaaaccaactaaatctaagactaggacagggccctctttttataaactcagcccacaacttggatattaactacaacaaaggcctttacttgtttacagcttcaaacaattccaaaaagcttgaggttaacctaagcactgccaaggggttgatgtttgacgctacagccatagccattaatgcaggagatgggcttgaatttggttcacctaatgcaccaaacacaaatcccctcaaaacaaaaattggccatggcctagaatttgattcaaacaaggctatggttcctaaactaggaactggccttagttttgacagcacaggtgccattacagtaggaaacaaaaataatgataagctaactttgtggaccacaccagctccatctcctaactgtagactaaatgcagagaaagatgctaaactcactttggtcttaacaaaatgtggcagtcaaatacttgctacagtttcagttttggctgttaaaggcagtttggctccaatatctggaacagttcaaagtgctcatcttattataagatttgacgaaaatggagtgctactaaacaattccttcctggacccagaatattggaactttagaaatggagatcttactgaaggcacagcctatacaaacgctgttggatttatgcctaacctatcagcttatccaaaatctcacggtaaaactgccaaaagtaacattgtcagtcaagtttacttaaacggagacaaaactaaacctgtaacactaaccattacactaaacggtacacaggaaacaggagacacaactccaagtgcatactctatgtcattttcatgggactggtctggccacaactacattaatgaaatatttgccacatcctcttacactttttcatacattgcccaagaataaagaatcgtttgtgttatgtttcaacgtgtttatttttcaattgcagaaaatttcaagtcatttttcattcagtagtatagccccaccaccacatagcttatacagatcaccgtaccttaatcaaactcacagaaccctagtattcaacctgccacctccctcccaacacacagagtacacagtcctttctccccggctggccttaaaaagcatcatatcatgggtaacagacatattcttaggtgttatattccacacggtttcctgtcgagccaaacgctcatcagtgatattaataaactccccgggcagctcacttaagttcatgtcgctgtccagctgctgagccacaggctgctgtccaacttgcggttgcttaacgggcggcgaaggagaagtccacgcctacatgggggtagagtcataatcgtgcatcaggatagggcggtggtgctgcagcagcgcgcgaataaactgctgccgccgccgctccgtcctgcaggaatacaacatggcagtggtctcctcagcgatgattcgcaccgcccgcagcataaggcgccttgtcctccgggcacagcagcgcaccctgatctcacttaaatcagcacagtaactgcagcacagcaccacaatattgttcaaaatcccacagtgcaaggcgctgtatccaaagctcatggcggggaccacagaacccacgtggccatcataccacaagcgcaggtagattaagtggcgacccctcataaacacgctggacataaacattacctcttttggcatgttgtaattcaccacctcccggtaccatataaacctctgattaaacatggcgccatccaccaccatcctaaaccagctggccaaaacctgcccgccggctatacactgcagggaaccgggactggaacaatgacagtggagagcccaggactcgtaaccatggatcatcatgctcgtcatgatatcaatgttggcacaacacaggcacacgtgcatacacttcctcaggattacaagctcctcccgcgttagaaccatatcccagggaacaacccattcctgaatcagcgtaaatcccacactgcagggaagacctcgcacgtaactcacgttgtgcattgtcaaagtgttacattcgggcagcagcggatgatcctccagtatggtagcgcgggtttctgtctcaaaaggaggtagacgatccctactgtacggagtgcgccgagacaaccgagatcgtgttggtcgtagtgtcatgccaaatggaacgccggacgtagtcatatttcctgaagcaaaaccaggtgcgggcgtgacaaacagatctgcgtctccggtctcgccgcttagatcgctctgtgtagtagttgtagtatatccactctctcaaagcatccaggcgccccctggcttcgggttctatgtaaactccttcatgcgccgctgccctgataacatccaccaccgcagaataagccacacccagccaacctacacattcgttctgcgagtcacacacgggaggagcgggaagagctggaagaaccatgtttttttttttattccaaaagattatccaaaacctcaaaatgaagatctattaagtgaacgcgctcccctccggtggcgtggtcaaactctacagccaaagaacagataatggcatttgtaagatgttgcacaatggcttccaaaaggcaaacggccctcacgtccaagtggacgtaaaggctaaacccttcagggtgaatctcctctataaacattccagcaccttcaaccatgcccaaataattctcatctcgccaccttctcaatatatctctaagcaaatcccgaatattaagtccggccattgtaaaaatctgctccagagcgccctccaccttcagcctcaagcagcgaatcatgattgcaaaaattcaggttcctcacagacctgtataagattcaaaagcggaacattaacaaaaataccgcgatcccgtaggtcccttcgcagggccagctgaacataatcgtgcaggtctgcacggaccagcgcggccacttccccgccaggaaccatgacaaaagaacccacactgattatgacacgcatactcggagctatgctaaccagcgtagccccgatgtaagcttgttgcatgggcggcgatataaaatgcaaggtgctgctcaaaaaatcaggcaaagcctcgcgcaaaaaagaaagcacatcgtagtcatgctcatgcagataaaggcaggtaagctccggaaccaccacagaaaaagacaccatttttctctcaaacatgtctgcgggtttctgcataaacacaaaataaaataacaaaaaaacatttaaacattagaagcctgtcttacaacaggaaaaacaacccttataagcataagacggactacggccatgccggcgtgaccgtaaaaaaactggtcaccgtgattaaaaagcaccaccgacagctcctcggtcatgtccggagtcataatgtaagactcggtaaacacatcaggttgattcacatcggtcagtgctaaaaagcgaccgaaatagcccgggggaatacatacccgcaggcgtagagacaacattacagcccccataggaggtataacaaaattaataggagagaaaaacacataaacacctgaaaaaccctcctgcctaggcaaaatagcaccctcccgctccagaacaacatacagcgcttccacagcggcagccataacagtcagccttaccagtaaaaaagaaaacctattaaaaaaacaccactcgacacggcaccagctcaatcagtcacagtgtaaaaaagggccaagtgcagagcgagtatatataggactaaaaaatgacgtaacggttaaagtccacaaaaaacacccagaaaaccgcacgcgaacctacgcccagaaacgaaagccaaaaaacccacaacttcctcaaatcgtcacttccgttttcccacgttacgtcacttcccattttaagaaaactacaattcccaacacatacaagttactccgccctaaaacctacgtcacccgccccgttcccacgccccgcgccacgtcacaaactccaccccctcattatcatattggcttcaatccaaaataaggta

SEQ ID NO: 227 - DNA, 9701 bp, synthetic construct
  misc_feature 1..9701: note = vector for IgG1 against T27Y H34A H374N ACE2 mutant
  misc_feature 2929..2930: note = n is a, c, g, or t
  misc_feature 2934: note = n is a, c, g, or t
  source 1..9701: mol_type = other DNA
ggcgtaatctgctgcttgcaaacaaaaaaaccaccgctaccagcggtggtttgtttgccggatcaagagctaccaactctttttccgaaggtaactggcttcagcagagcgcagataccaaatactgtccttctagtgtagccgtagttaggccaccacttcaagaactctgtagcaccgcctacatacctcgctctgctgaagccagttaccagtggctgctgccagtggcgataagtcgtgtcttaccgggttggactcaagagatagttaccggataaggcgcagcggtcgggctgaacggggggttcgtgcacacagcccagcttggagcgaacgacctacaccgaactgagatacctacagcgtgagctatgagaaagcgccacgcttcccgaagggagaaaggcggacaggtatccggtaagcggcagggtcggaacaggagagcgcacgagggagcttccagggggaaacgcctggtatctttatagtcctgtcgggtttcgccacctctgacttgagcgtcgatttttgtgatgctcgtcaggggggcggagcctatggaaaaacgccagcaacgcaagctagagtttaaacttgacagatgagacaataaccctgataaatgcttcaataatattgaaaaaggaaaagtatgagtattcaacatttccgtgtcgcccttattcccttttttgcggcattttgccttcctgtttttgctcacccagaaacgctggtgaaagtaaaagatgcagaagatcacttgggtgcgcgagtgggttacatcgaactggatctcaacagcggtaagatccttgagagttttcgccccgaagaacgtttcccaatgatgagcacttttaaagttctgctatgtggcgcggtattatcccgtattgatgccgggcaagagcaactcggtcgccgcatacactattctcagaatgacttggttgaatactcaccagtcacagaaaagcatcttacggatggcatgacagtaagagaattatgcagtgctgccataaccatgagtgataacactgcggccaacttacttctgacaactatcggaggaccgaaggagctaaccgcttttttgcacaacatgggggatcatgtaactcgccttgatcgttgggaaccggagctgaatgaagccataccaaacgacgagcgtgacaccacgatgcctgtagcaatggcaacaacgttgcgaaaactattaactggcgaactacttactctagcttcccggcaacaactaatagactggatggaggcggataaagttgcaggaccacttctgcgctcggcacttccggctggctggtttattgctgataaatcaggagccggtgagcgtgggtcacgcggtatcattgcagcactggggccggatggtaagccctcccgtatcgtagttatctacactacggggagtcaggcaactatggatgaacgaaatagacagatcgctgagataggtgcctcactgattaagcattggtaaggataaatttctggtaaggaggacacgtatggaagtgggcaagttggggaagccgtatccgttgctgaatctggcatatgtgggagtataagacgcgcagcgtcgcatcaggcatttttttctgcgccaatgcaaaaaggccatccgtcaggatggcctttcggcataactagggccgccgatatttgaaaatatggcatattgaaaatgtcgccgatgtgagtttctgtgtaactgatatcgccatttttccaaaagtgatttttgggcatacgcgatatctggcgatagcgcttatatcgtttacgggggatggcgatagacgactttggtgacttgggcgattctgtgtgtcgcaaatatcgcagtttcgatataggtgacagacgatatgaggctatatcgccgatagaggcgacatcaagctggcacatggccaatgcatatcgatctatacattgaatcaatattggccattagccatattattcattggttatatagcataaatcaatattggctattggccattgcatacgttgtatccatatcataatatgtacatttatattggctcatgtccaacattaccgccatgttgacattgattattgactagttattaatagtaatcaattacggggtcattagttcatagcccatatatggagttccgcgttacataacttacggtaaatggcccgcctggctgaccgcccaacgacccccgcccattgacgtcaataatgacgtatgttcccatagtaacgccaatagggactttccattgacgtcaatgggtggagtatttacggtaaactgcccacttggcagtacatcaagtgtatcatatgccaagtacgccccctattgacgtcaatgacggtaaatggcccgcctggcattatgcccagtacatgaccttatgggactttcctacttggcagtacatctacgtattagtcatcgctattaccatggtgatgcggttttggcagtacatcaatgggcgtggatagcggtttgactcacggggatttccaagtctccaccccattgacgtcaatgggagtttgttttggcaccaaaatcaacgggactttccaaaatgtcgtaacaactccgccccattgacgcaaatgggcggtaggcgtgtacggtgggaggtctatataagcagagctcgtttagtgaaccgtcagatcgcctggagacgccatccacgctgttttgacctccatagaagacaccgggaccgatccagcctccgcggccgggaacggtgcattggaacgcggattccccgtgccaagagtgacgtaagtaccgcctatagagtctataggcccacccccttggcttcttatgcatgctatactgtttttggcttggggtctatacaccccccgnnttcntcatgttataggtgatggtatagcttagcctataggtgtgggttattgaccattattgaccactccccctattggtgacgatactttccattactaatccataacatggctctttgccacaactctctttattggctatatgccaatacactgtccttcagagactgacacggactctgtatttttacaggatggggtctcatttattatttacaaattcacatatacaacaccaccgtccccagtgcccgcagtttttattaaacataacgtgggatctccacgcgaatctcgggtacgtgttccggacatgggctcttctccggtagcggcggagcttctacatccgagccctgctcccatgcctccagcgactcatggtcgctcggcagctccttgctcctaacagtggaggccagacttaggcacagcacgatgcccaccaccaccagtgtgccgcacaaggccgtggcggtagggtatgtgtctgaaaatgagctcggggagcgggcttgcaccgctgacgcatttggaagacttaaggcagcggcagaagaagatgcaggcagctgagttgttgtgttctgataagagtcagaggtaactcccgttgcggtgctgttaacggtggagggcagtgtagtctgagcagtactcgttgctgccgcgcgcgccaccagacataatagctgacagactaacagactgttcctttccatgggtcttttctgcagtcaccgtccttgacacgaagctgctagcgccaccatgagcagcagtagttggcttctcttgagtttggtggcagtgacagcagcccagagtactatcgaggagcaggctaaatactttctggataagtttaacgccgaggccgaagacttgttctatcaatcttctctcgcttcatggaattacaatactaacatcactgaggagaacgtccagaatatgaacaatgctggcgacaaatggagcgccttcttgaaggagcagtctacccttgcacaaatgtatccactgcaggagatacagaaccttacagtaaagttgcagctccaggctctccagcagaacggatctagcgtgctttcagaggataaaagcaaaaggctgaacaccatacttaataccatgtccacaatttactctactggtaaagtatgtaaccccgacaaccctcaagaatgcctccttcttgagccaggcctcaatgagatcatggctaatagtctggactataatgaaagactgtgggcatgggagtcctggagatctgaagtagggaagcaactgaggcccctttatgaagagtacgtcgtacttaagaatgaaatggcccgcgctaaccactacgaggattacggcgattactggcgtggggactatgaagtaaatggtgtagatggatacgactatagtcgtgggcaattgattgaggatgtggagcacacttttgaggagataaaaccactctatgagcatcttcacgcatatgtgagagctaaactgatgaacgcctacccaagttacatcagtccaatcggatgtctcccagctcacctccttggcgacatgtggggacgtttctggaccaatctgtattccctcacagtccctttcgggcaaaagcctaatatagacgtgacagacgcaatggttgatcaggcttgggatgctcaaaggatttttaaggaagctgagaagttttttgtgtcagtcggtttgccaaatatgacacaaggcttctgggaaaatagcatgttgactgatcccggtaatgttcaaaaggctgtgtgtcaccctaccgcttgggaccttgggaaaggtgactttcgaatcttgatgtgtaccaaggtgacaatggatgactttcttacagcccataatgaaatgggtcacatccagtatgatatggcttatgcagctcaacctttcctcttgagaaatggtgcaaatgaaggttttcatgaagctgtaggggaaataatgtccctgagtgctgcaaccccaaagcatctcaagagtatcggattgttgagcccagattttcaagaagataacgagaccgaaatcaacttccttctgaaacaagccctcacaatagttggtactcttccattcacatacatgctggagaaatggcgttggatggtttttaagggggagatacctaaagatcagtggatgaaaaagtggtgggagatgaagcgtgagatcgtaggggtcgtggagccagtgcctcatgatgagacttactgtgacccagcatcactcttccacgttagcaatgactattcatttatacgttattacactcgcactctttaccagtttcaatttcaggaggctctgtgtcaggctgccaagcatgagggaccccttcacaagtgtgatattagtaacagtactgaggcaggccaaaaactgttcaatatgttgaggcttggcaaaagcgagccatggactctcgccttggaaaatgttgtcggggctaaaaacatgaatgtacgccctctgcttaactattttgagcccctttttacatggctcaaggaccagaataagaactcctttgtcggctggtcaacagactggtctccctatgcagacaaaacacatacttgcccaccttgtcctgcaccagagctgctgggaggtccaagcgtgttcctgtttccacccaagcccaaagacacactgatgatttctcgaactccagaagtgacctgcgtggtcgtggacgtgagccacgaggatcccgaagtgaagttcaactggtacgtggatggcgtggaggtccataatgctaagactaaaccccgggaggaacagtacaacagcacttatagggtcgtgtccgtgctgaccgtcctgcatcaggattggctgaacgggaaggaatataagtgcaaagtgtctaataaggcactgcccgcccctatcgagaaaacaattagcaaggctaagggtcagcctagagaaccacaggtgtacactctgcctccaagtcgcgacgagctgaccaagaaccaggtgtcactgacatgtctggtcaaaggcttttatccctcagatatcgcagtggagtgggaaagcaatggacagcctgagaacaattacaagaccacaccccctgtgctggacagtgatggctcattctttctgtattctaagctgacagtggacaaaagtaggtggcagcagggaaacgtgttctcctgctctgtcatgcacgaagcactgcacaatcattatacccagaagagtctgtcactgagccctggcaaatgagcgataccgattctagaactagatcataatcagccataccacatttgtagaggttttacttgctttaaaaaacctcccacacctccccctgaacctgaaacataaaatgaatgcaattgttgttgttaacttgtttattgcagcttataatggttacaaataaagcaatagcatcacaaatttcacaaataaagcatttttttcactgcattctagttgtggtttgtccaaactcatcaatgtatcttaaggccgcaggtaagccagcccaggcctcgccctccagctcaaggcgggacaggtgccctagagtagcctgcatccagggacaggccccagccgggtgctgacacgtccacctccatctcttcctcaggtctgcccgggtggcatccctgtgacccctccccagtgcctctcctggtcgtggaaggtgctactccagtgcccaccagccttgtcctaataaaattaagttgcatcattttgtttgactaggtgtccttgtataatattatggggtggaggcgggtggtatggagcaaggggcccaagttaacttgtttattgcagcttataatggttacaaataaagcaatagcatcacaaatttcacaaataaagcatttttttcactgcattctagttgtggtttgtccaaactcatcaatgtatcttatcatgtctggatccgcttcaggcaccgggcttgcgggtcatgcaccaggtgcgcggtccttcgggcacctcgacgtcggcggtgacggtgaagccgagccgctcgtagaaggggaggttgcggggcgcggaggtctccaggaaggcgggcaccccggcgcgctcggccgcctccactccggggagcacgacggcgctgcccagacccttgccctggtggtcgggcgagacgccgacggtggccaggaaccacgcgggctccttgggccggtgcggcgccaggaggccttccatctgttgctgcgcggccagcctggaaccgctcaactcggccatgcgcgggccgatctcggcgaacaccgcccccgcttcgacgctctccggcgtggtccagaccgccaccgcggcgccgtcgtccgcgacccacaccttgccgatgtcgagcccgacgcgcgtgaggaagagttcttgcagctcggtgacccgctcgatgtggcggtccgggtcgacggtgtggcgcgtggcggggtagtcggcgaacgcggcggcgagggtgcgtacggcccgggggacgtcgtcgcgggtggcgaggcgcaccgtgggcttgtactcggtcatggtggcctgcagagtcgctctgtgttcgaggccacacgcgtcaccttaatatgcgaagtggacctgggaccgcgccgccccgactgcatctgcgtgttttcgccaatgacaagacgctgggcggggtttgtgtcatcatagaactaaagacatgcaaatatatttcttccggggacaccgccagcaaacgcgagcaacgggccacggggatgaagcagctgcgccactccctgaagatccatcgtctcctaacaagttacatcactcctgcccttcctcaccctcatctccatcacctccttcatctccgtcatctccgtcatcaccctccgcggcagccccttccaccataggtggaaaccagggaggcaaatctactccatcgtcaaagctgcacacagtcaccctgatattgcaggtaggagcgggctttgtcataacaaggtccttaatcgcatccttcaaaacctcagcaaatatatgagtttgtaaaaagaccatgaaataacagacaatggactcccttagcgggccaggttgtgggccgggtccaggggccattccaaaggggagacgactcaatggtgtaagacgacattgtggaatagcaagggcagttcctcgccttaggttgtaaagggaggtcttactacctccatatacgaacacaccggcgacccaagttccttcgtcggtagtcctttctacgtgactcctagccaggagagctcttaaaccttctgcaatgttctcaaatttcgggttggaacctccttgaccacgatgctttccaaaccaccctccttttttgcgcctgcctccatcaccctgacccccgctgcgcgggggcacgtcaggctcaccatctgggccgccttcttggtggtattcaaaataatcggcttcccctacagggtggaaaaatggccttctacctggagggggcctgcgcggtggagacccggatgatgatgactgactactgggactcctgggcctcttttctccacgtccacgacctctccccctggctctttcacgacttccccccctggctctttcacgtcctctaccccggcggcctccactacctcctcgaccccggcctccactacctcctcgaccccggcctccactgcctcctcgaccccggcctccacctcctgctcctgcccctcccgctcctgctcctgctcctgttccaccgtgggtccctttgcagccaatgcaacttggacgtttttggggtctccggacaccatctctatgtcttggccctgatcctgagccgcccggggctcctggtcttccgcctcctcgtcctcgtcctcttccccgtcctcgtccatgtgccatgatggcggcctgcagctgtgttcgaggccgcgcgtgtcaccttaatatgcgaagtggacctgggaccgcgccgccccgactgcatctgcgtgttcgagttcgccaatgacaagacgctgggcggggagatcccccttattaaccctaaacgggtagcatatgcttcccgggtagtagtatatactatccagactaaccctaattcaatagcatatgttacccaacgggaagcatatgctatcgaattagggttagtaaaagggtcctaaggaacagcgatctggatagcatatgctatcctaatctatatctgggtagcatatgctatcctaatctatatctgggtagcataggctatcctaatctatatctgggtagcatatgctatcctaatctatatctgggtagtatatgctatcctaatttatatctgggtagcataggctatcctaatctatatctgggtagcatatgctatcctaatctatatctgggtagtatatgctatcctaatctgtatccgggtagcatatgctatcctcatgcatatacagtcagcatatgatacccagtagtagagtgggagtgctatcctttgcatatgccgccacctcccaaggagatctgtcgacatcgatgggcgcgggtgtacactccgcccatcccgcccctaactccgcccagttccgcccattctccgcctcatggctgactaattttttttatttatgcagaggccgaggccgcctcggcctctgagctattccagaagtagtgaggaggcttttttggaggcctaggcttttgcaaaaagctaattc

SEQ ID NO: 228 - DNA, 38496 bp, synthetic construct
  misc_feature 1..38496: note = vector for IgA against T27Y H34A H378N ACE2 mutant
  source 1..38496: mol_type = other DNA
tattattgatgatgttaattaacatgcatggatcctacgtctcgaccgatgcccttgagagccttcaacccagtcagctccttccggtgggcgcggggcatgactatcgtcgccgcacttatgactgtcttctttatcatgcaactcgtaggacaggtgccggcagcgctctgggtcattttcggcgaggaccgctttcgctggagcgcgacgatgatcggcctgtcgcttgcggtattcggaatcttgcacgccctcgctcaagccttcgtcactggtcccgccaccaaacgtttcggcgagaagcaggccattatcgccggcatggcggccgacgcgctgggctacgtcttgctggcgttcgcgacgcgaggctggatggccttccccattatgattcttctcgcttccggcggcatcgggatgcccgcgttgcaggccatgctgtccaggcaggtagatgacgaccatcagggacagcttcaaggatcgctcgcggctcttaccagcctaacttcgatcattggaccgctgatcgtcacggcgatttatgccgcctcggcgagcacatggaacgggttggcatggattgtaggcgccgccctataccttgtctgcctccccgcgttgcgtcgcggtgcatggagccgggccacctcgacctgaatggaagccggcggcacctcgctaacggattcaccactccaagaattggagccaatcaattcttgcggagaactgtgaatgcgcaaaccaacccttggcagaacatatccatcgcgtccgccatctccagcagccgcacgcggcgcatctcgggcagcgttgggtcctggccacgggtgcgcatgatcgtgctcctgtcgttgaggacccggctaggctggcggggttgccttactggttagcagaatgaatcaccgatacgcgagcgaacgtgaagcgactgctgctgcaaaacgtctgcgacctgagcaacaacatgaatggtcttcggtttccgtgtttcgtaaagtctggaaacgcggaagtcagcgccctgcaccattatgttccggatctgcatcgcaggatgctgctggctaccctgtggaacacctacatctgtattaacgaagcgctggcattgaccctgagtgatttttctctggtcccgccgcatccataccgccagttgtttaccctcacaacgttccagtaaccgggcatgttcatcatcagtaacccgtatcgtgagcatcctctctcgtttcatcggtatcattacccccatgaacagaaatcccccttacacggaggcatcagtgaccaaacaggaaaaaaccgcccttaacatggcccgctttatcagaagccagacattaacgcttctggagaaactcaacgagctggacgcggatgaacaggcagacatctgtgaatcgcttcacgaccacgctgatgagctttaccgcagctgcctcgcgcgtttcggtgatgacggtgaaaacctctgacacatgcagctcccggagacggtcacagcttgtctgtaagcggatgccgggagcagacaagcccgtcagggcgcgtcagcgggtgttggcgggtgtcggggcgcagccatgacccagtcacgtagcgatagcggagtgtatactggcttaactatgcggcatcagagcagattgtactgagagtgcaccatatgcggtgtgaaataccgcacagatgcgtaaggagaaaataccgcatcaggcgctcttccgcttcctcgctcactgactcgctgcgctcggtcgttcggctgcggcgagcggtatcagctcactcaaaggcggtaatacggttatccacagaatcaggggataacgcaggaaagaacatgtgagcaaaaggccagcaaaaggccaggaaccgtaaaaaggccgcgttgctggcgtttttccataggctccgcccccctgacgagcatcacaaaaatcgacgctcaagtcagaggtggcgaaacccgacaggactataaagataccaggcgtttccccctggaagctccctcgtgcgctctcctgttccgaccctgccgcttaccggatacctgtccgcctttctcccttcgggaagcgtggcgctttctcatagctcacgctgtaggtatctcagttcggtgtaggtcgttcgctccaagctgggctgtgtgcacgaaccccccgttcagcccgaccgctgcgccttatccggtaactatcgtcttgagtccaacccggtaagacacgacttatcgccactggcagcagccactggtaacaggattagcagagcgaggtatgtaggcggtgctacagagttcttgaagtggtggcctaactacggctacactagaaggacagtatttggtatctgcgctctgctgaagccagttaccttcggaaaaagagttggtagctcttgatccggcaaacaaaccaccgctggtagcggtggtttttttgtttgcaagcagcagattacgcgcagaaaaaaaggatctcaagaagatcctttgatcttttctacggggtctgacgctcagtggaacgaaaactcacgttaagggattttggtcatgagattatcaaaaaggatcttcacctagatccttttaaattaaaaatgaagttttaaatcaatctaaagtatatatgagtaaacttggtctgacagttaccaatgcttaatcagtgaggcacctatctcagcgatctgtctatttcgttcatccatagttgcctgactccccgtcgtgtagataactacgatacgggagggcttaccatctggccccagtgctgcaatgataccgcgagacccacgctcaccggctccagatttatcagcaataaaccagccagccggaagggccgagcgcagaagtggtcctgcaactttatccgcctccatccagtctattaattgttgccgggaagctagagtaagtagttcgccagttaatagtttgcgcaacgttgttgccattgctgcagccatgagattatcaaaaaggatcttcacctagatccttttcacgtagaaagccagtccgcagaaacggtgctgaccccggatgaatgtcagctactgggctatctggacaagggaaaacgcaagcgcaaagagaaagcaggtagcttgcagtgggcttacatggcgatagctagactgggcggttttatggacagcaagcgaaccggaattgccagctggggcgccctctggtaaggttgggaagccctgcaaagtaaactggatggctttcttgccgccaaggatctgatggcgcaggggatcaagctctgatcaagagacaggatgaggatcgtttcgcatgattgaacaagatggattgcacgcaggttctccggccgcttgggtggagaggctattcggctatgactgggcacaacagacaatcggctgctctgatgccgccgtgttccggctgtcagcgcaggggcgcccggttctttttgtcaagaccgacctgtccggtgccctgaatgaactgcaagacgaggcagcgcggctatcgtggctggccacgacgggcgttccttgcgcagctgtgctcgacgttgtcactgaagcgggaagggactggctgctattgggcgaagtgccggggcaggatctcctgtcatctcaccttgctcctgccgagaaagtatccatcatggctgatgcaatgcggcggctgcatacgcttgatccggctacctgcccattcgaccaccaagcgaaacatcgcatcgagcgagcacgtactcggatggaagccggtcttgtcgatcaggatgatctggacgaagagcatcaggggctcgcgccagccgaactgttcgccaggctcaaggcgagcatgcccgacggcgaggatctcgtcgtgacccatggcgatgcctgcttgccgaatatcatggtggaaaatggccgcttttctggattcatcgactgtggccggctgggtgtggcggaccgctatcaggacatagcgttggctacccgtgatattgctgaagagcttggcggcgaatgggctgaccgcttcctcgtgctttacggtatcgccgctcccgattcgcagcgcatcgccttctatcgccttcttgacgagttcttctgaattttgttaaaatttttgttaaatcagctcattttttaaccaataggccgaaatcggcaaaatcccttataaatcaaaagaatagaccgagatagggttgagtgttgttccagtttggaacaagagtccactattaaagaacgtggactccaacgtcaaagggcgaaaaaccgtctatcagggcgatggcccactacgtgaaccatcaccctaatcaagttttttggggtcgaggtgccgtaaagcactaaatcggaaccctaaagggagcccccgatttagagcttgacggggaaagccggcgaacgtggcgagaaaggaagggaagaaagcgaaaggagcgggcgctagggcgctggcaagtgtagcggtcacgctgcgcgtaaccaccacacccgccgcgcttaatgcgccgctacagggcgcgtccattcgccattcaggatcgaattaattcttaattaacatcatcaataatataccttattttggattgaagccaatatgataatgagggggtggagtttgtgacgtggcgcggggcgtgggaacggggcgggtgacgtagtagtgtggcggaagtgtgatgttgcaagtgtggcggaacacatgtaagcgacggatgtggcaaaagtgacgtttttggtgtgcgccggtgtacacaggaagtgacaattttcgcgcggttttaggcggatgttgtagtaaatttgggcgtaaccgagtaagatttggccattttcgcgggaaaactgaataagaggaagtgaaatctgaataattttgtgttactcatagcgcgtaatactgtaatagtaatcaattacggggtcattagttcatagcccatatatggagttccgcgttacataacttacggtaaatggcccgcctggctgaccgcccaacgacccccgcccattgacgtcaataatgacgtatgttcccatagtaacgccaatagggactttccattgacgtcaatgggtggagtatttacggtaaactgcccacttggcagtacatcaagtgtatcatatgccaagtacgccccctattgacgtcaatgacggtaaatggcccgcctggcattatgcccagtacatgaccttatgggactttcctacttggcagtacatctacgtattagtcatcgctattaccatggtgatgcggttttggcagtacatcaatgggcgtggatagcggtttgactcacggggatttccaagtctccaccccattgacgtcaatgggagtttgttttggcaccaaaatcaacgggactttccaaaatgtcgtaacaactccgccccattgacgcaaatgggcggtaggcgtgtacggtgggaggtctatataagcagagctggtttagtgaaccgtcagatccgctagagatctggtaccgtcgacgcggccgctcgagcctaagcttatgagcagcagtagttggcttctcttgagtttggtggcagtgacagcagcccagagtactatcgaggagcaggctaaatactttctggataagtttaacgccgaggccgaagacttgttctatcaatcttctctcgcttcatggaattacaatactaacatcactgaggagaacgtccagaatatgaacaatgctggcgacaaatggagcgccttcttgaaggagcagtctacccttgcacaaatgtatccactgcaggagatacagaaccttacagtaaagttgcagctccaggctctccagcagaacggatctagcgtgctttcagaggataaaagcaaaaggctgaacaccatacttaataccatgtccacaatttactctactggtaaagtatgtaaccccgacaaccctcaagaatgcctccttcttgagccaggcctcaatgagatcatggctaatagtctggactataatgaaagactgtgggcatgggagtcctggagatctgaagtagggaagcaactgaggcccctttatgaagagtacgtcgtacttaagaatgaaatggcccgcgctaaccactacgaggattacggcgattactggcgtggggactatgaagtaaatggtgtagatggatacgactatagtcgtgggcaattgattgaggatgtggagcacacttttgaggagataaaaccactctatgagcatcttcacgcatatgtgagagctaaactgatgaacgcctacccaagttacatcagtccaatcggatgtctcccagctcacctccttggcgacatgtggggacgtttctggaccaatctgtattccctcacagtccctttcgggcaaaagcctaatatagacgtgacagacgcaatggttgatcaggcttgggatgctcaaaggatttttaaggaagctgagaagttttttgtgtcagtcggtttgccaaatatgacacaaggcttctgggaaaatagcatgttgactgatcccggtaatgttcaaaaggctgtgtgtcaccctaccgcttgggaccttgggaaaggtgactttcgaatcttgatgtgtaccaaggtgacaatggatgactttcttacagcccatcatgaaatgggtaatatccagtatgatatggcttatgcagctcaacctttcctcttgagaaatggtgcaaatgaaggttttcatgaagctgtaggggaaataatgtccctgagtgctgcaaccccaaagcatctcaagagtatcggattgttgagcccagattttcaagaagataacgagaccgaaatcaacttccttctgaaacaagccctcacaatagttggtactcttccattcacatacatgctggagaaatggcgttggatggtttttaagggggagatacctaaagatcagtggatgaaaaagtggtgggagatgaagcgtgagatcgtaggggtcgtggagccagtgcctcatgatgagacttactgtgacccagcatcactcttccacgttagcaatgactattcatttatacgttattacactcgcactctttaccagtttcaatttcaggaggctctgtgtcaggctgccaagcatgagggaccccttcacaagtgtgatattagtaacagtactgaggcaggccaaaaactgttcaatatgttgaggcttggcaaaagcgagccatggactctcgccttggaaaatgttgtcggggctaaaaacatgaatgtacgccctctgcttaactattttgagcccctttttacatggctcaaggaccagaataagaactcctttgtcggctggtcaacagactggtctccctatgcagaccctagtactcctcctactccttctccatcaaccccaccaactccatcccctagctgctgtcacccaaggctgtctctgcaccgacctgcactcgaagaccttctgttgggctctgaagctaacctgacctgtactcttactggcttgcgcgatgctagcggcgtgactttcacctggacacctagtagcggtaaaagtgctgtacaaggacctcctgaacgcgacctgtgtggttgctactctgtgtcttctgtacttcccggctgtgccgagccctggaatcacgggaaaacctttacctgcaccgccgcttaccctgagtcaaaaactcccctcactgccacattgagtaagtcagggaatacattcaggccagaggttcatttgttgcctcctccatctgaagaacttgctttgaacgagctggtcactctgacctgcttggctaggggtttctcccccaaagatgtacttgtacggtggttgcagggcagccaagagttgccccgcgaaaagtatttgacctgggcctcaagacaagaacccagccaggggactaccacatttgccgtgaccagtattctgcgtgtagccgctgaagattggaagaaaggggatacattttcttgcatggtagggcatgaggcccttcccctcgctttcactcagaagacaatagacagactcgccggaaagcctactcacgtgaatgttagcgtagtcatggctgaggttgacggaacttgctactgagatatccgatccaccggatctagataactgatcataatcagccataccacatttgtagaggttttacttgctttaaaaaacctcccacacctccccctgaacctgaaacataaaatgaatgcaattgttgttgttaacttgtttattgcagcttataatggttacaaataaagcaatagcatcacaaatttcacaaataaagcatttttttcactgcattctagttgtggtttgtccaaactcatcaatgtatcttaggtttagtgaaccgtcagatccgctagcgttacataacttacggtaaatggcccgcctggctgaccgcccaacgacccccgcccattgacgtcaataatgacgtatgttcccatagtaacgccaatagggactttccattgacgtcaatgggtggagtatttacggtaaactgcccacttggcagtacatcaagtgtatcatatgccaagtacgccccctattgacgtcaatgacggtaaatggcccgcctggcattatgcccagtacatgaccttatgggactttcctacttggcagtacatctacgtattagtcatcgctattaccatggtgatgcggttttggcagtacatcaatgggcgtggatagcggtttgactcacggggatttccaagtctccaccccattgacgtcaatgggagtttgttttggcaccaaaatcaacgggactttccaaaatgtcgtaacaactccgccccattgacgcaaatgggcggtaggcgtgtacggtgggaggtctatataagcagagctggtttagtgaaccgtcagatccgctagagatctggtaccgtcgacgcggccgctcgagcctaagcttatgaagaaccatctgcttttctggggagtacttgccgttttcataaaagccgtacatgttaaagcacaagaggacgaacgcattgtgttggttgataataaatgcaaatgtgctcggataacatctcggatcattcgtagctcagaggaccccaatgaggatatagtagagcgaaacatcagaattatagtacccctgaacaacagagagaacataagtgatcccacaagtccattgcggacacgctttgtttaccatttgtctgatctgtgtaaaaaatgtgatccaacagaggtggaactcgacaatcagatcgtcaccgccacccagtctaacatctgcgatgaagattcagctacagagacatgctacacatacgaccggaacaagtgctatactgccgttgtgccactcgtttacggtggagaaacaaagatggttgaaactgcacttacaccagatgcctgctatccagattgagatatccgatccaccggatctagataactgatcataatcagccataccacatttgtagaggttttacttgctttaaaaaacctcccacacctccccctgaacctgaaacataaaatgaatgcaattgttgttgttaacttgtttattgcagcttataatggttacaaataaagcaatagcatcacaaatttcacaaataaagcatttttttcactgcattctagttgtggtttgtccaaactcatcaatgtatcttaacgcggatctgggcgtggttaagggtgggaaagaatatataaggtgggggtcttatgtagttttgtatctgttttgcagcagccgccgccgccatgagcaccaactcgtttgatggaagcattgtgagctcatatttgacaacgcgcatgcccccatgggccggggtgcgtcagaatgtgatgggctccagcattgatggtcgccccgtcctgcccgcaaactctactaccttgacctacgagaccgtgtctggaacgccgttggagactgcagcctccgccgccgcttcagccgctgcagccaccgcccgcgggattgtgactgactttgctttcctgagcccgcttgcaagcagtgcagcttcccgttcatccgcccgcgatgacaagttgacggctcttttggcacaattggattctttgacccgggaacttaatgtcgtttctcagcagctgttggatctgcgccagcaggtttctgccctgaaggcttcctcccctcccaatgcggtttaaaacataaataaaaaaccagactctgtttggatttggatcaagcaagtgtcttgctgtctttatttaggggttttgcgcgcgcggtaggcccgggaccagcggtctcggtcgttgagggtcctgtgtattttttccaggacgtggtaaaggtgactctggatgttcagatacatgggcataagcccgtctctggggtggaggtagcaccactgcagagcttcatgctgcggggtggtgttgtagatgatccagtcgtagcaggagcgctgggcgtggtgcctaaaaatgtctttcagtagcaagctgattgccaggggcaggcccttggtgtaagtgtttacaaagcggttaagctgggatgggtgcatacgtggggatatgagatgcatcttggactgtatttttaggttggctatgttcccagccatatccctccggggattcatgttgtgcagaaccaccagcacagtgtatccggtgcacttgggaaatttgtcatgtagcttagaaggaaatgcgtggaagaacttggagacgcccttgtgacctccaagattttccatgcattcgtccataatgatggcaatgggcccacgggcggcggcctgggcgaagatatttctgggatcactaacgtcatagttgtgttccaggatgagatcgtcataggccatttttacaaagcgcgggcggagggtgccagactgcggtataatggttccatccggcccaggggcgtagttaccctcacagatttgcatttcccacgctttgagttcagatggggggatcatgtctacctgcggggcgatgaagaaaacggtttccggggtaggggagatcagctgggaagaaagcaggttcctgagcagctgcgacttaccgcagccggtgggcccgtaaatcacacctattaccggctgcaactggtagttaagagagctgcagctgccgtcatccctgagcaggggggccacttcgttaagcatgtccctgactcgcatgttttccctgaccaaatccgccagaaggcgctcgccgcccagcgatagcagttcttgcaaggaagcaaagtttttcaacggtttgagaccgtccgccgtaggcatgcttttgagcgtttgaccaagcagttccaggcggtcccacagctcggtcacctgctctacggcatctcgatccagcatatctcctcgtttcgcgggttggggcggctttcgctgtacggcagtagtcggtgctcgtccagacgggccagggtcatgtctttccacgggcgcagggtcctcgtcagcgtagtctgggtcacggtgaaggggtgcgctccgggctgcgcgctggccagggtgcgcttgaggctggtcctgctggtgctgaagcgctgccggtcttcgccctgcgcgtcggccaggtagcatttgaccatggtgtcatagtccagcccctccgcggcgtggcccttggcgcgcagcttgcccttggaggaggcgccgcacgaggggcagtgcagacttttgagggcgtagagcttgggcgcgagaaataccgattccggggagtaggcatccgcgccgcaggccccgcagacggtctcgcattccacgagccaggtgagctctggccgttcggggtcaaaaaccaggtttcccccatgctttttgatgcgtttcttacctctggtttccatgagccggtgtccacgctcggtgacgaaaaggctgtccgtgtccccgtatacagacttgagaggcctgtcctcgagcggtgttccgcggtcctcctcgtatagaaactcggaccactctgagacaaaggctcgcgtccaggccagcacgaaggaggctaagtgggaggggtagcggtcgttgtccactagggggtccactcgctccagggtgtgaagacacatgtcgccctcttcggcatcaaggaaggtgattggtttgtaggtgtaggccacgtgaccgggtgttcctgaaggggggctataaaagggggtgggggcgcgttcgtcctcactctcttccgcatcgctgtctgcgagggccagctgttggggtgagtactccctctgaaaagcgggcatgacttctgcgctaagattgtcagtttccaaaaacgaggaggatttgatattcacctggcccgcggtgatgcctttgagggtggccgcatccatctggtcagaaaagacaatctttttgttgtcaagcttggtggcaaacgacccgtagagggcgttggacagcaacttggcgatggagcgcagggtttggtttttgtcgcgatcggcgcgctccttggccgcgatgtttagctgcacgtattcgcgcgcaacgcaccgccattcgggaaagacggtggtgcgctcgtcgggcaccaggtgcacgcgccaaccgcggttgtgcagggtgacaaggtcaacgctggtggctacctctccgcgtaggcgctcgttggtccagcagaggcggccgcccttgcgcgagcagaatggcggtagggggtctagctgcgtctcgtccggggggtctgcgtccacggtaaagaccccgggcagcaggcgcgcgtcgaagtagtctatcttgcatccttgcaagtctagcgcctgctgccatgcgcgggcggcaagcgcgcgctcgtatgggttgagtgggggaccccatggcatggggtgggtgagcgcggaggcgtacatgccgcaaatgtcgtaaacgtagaggggctctctgagtattccaagatatgtagggtagcatcttccaccgcggatgctggcgcgcacgtaatcgtatagttcgtgcgagggagcgaggaggtcgggaccgaggttgctacgggcgggctgctctgctcggaagactatctgcctgaagatggcatgtgagttggatgatatggttggacgctggaagacgttgaagctggcgtctgtgagacctaccgcgtcacgcacgaaggaggcgtaggagtcgcgcagcttgttgaccagctcggcggtgacctgcacgtctagggcgcagtagtccagggtttccttgatgatgtcatacttatcctgtcccttttttttccacagctcgcggttgaggacaaactcttcgcggtctttccagtactcttggatcggaaacccgtcggcctccgaacggtaagagcctagcatgtagaactggttgacggcctggtaggcgcagcatcccttttctacgggtagcgcgtatgcctgcgcggccttccggcatgaccagcatgaagggcacgagctgcttcccaaaggcccccatccaagtataggtctctacatcgtaggtgacaaagagacgctcggtgcgaggatgcgagccgatcgggaagaactggatctcccgccaccaattggaggagtggctattgatgtggtgaaagtagaagtccctgcgacgggccgaacactcgtgctggcttttgtaaaaacgtgcgcagtactggcagcggtgcacgggctgtacatcctgcacgaggttgacctgacgaccgcgcacaaggaagcagagtgggaatttgagcccctcgcctggcgggtttggctggtggtcttctacttcggctgcttgtccttgaccgtctggctgctcgaggggagttacggtggatcggaccaccacgccgcgcgagcccaaagtccagatgtccgcgcgcggcggtcggagcttgatgacaacatcgcgcagatgggagctgtccatggtctggagctcccgcggcgtcaggtcaggcgggagctcctgcaggtttacctcgcatagacgggtcagggcgcgggctagatccaggtgatacctaatttccaggggctggttggtggcggcgtcgatggcttgcaagaggccgcatccccgcggcgcgactacggtaccgcgcggcgggcggtgggccgcgggggtgtccttggatgatgcatctaaaagcggtgacgcgggcgagcccccggaggtagggggggctccggacccgccgggagagggggcaggggcacgtcggcgccgcgcgcgggcaggagctggtgctgcgcgcgtaggttgctggcgaacgcgacgacgcggcggttgatctcctgaatctggcgcctctgcgtgaagacgacgggcccggtgagcttgaacctgaaagagagttcgacagaatcaatttcggtgtcgttgacggcggcctggcgcaaaatctcctgcacgtctcctgagttgtcttgataggcgatctcggccatgaactgctcgatctcttcctcctggagatctccgcgtccggctcgctccacggtggcggcgaggtcgttggaaatgcgggccatgagctgcgagaaggcgttgaggcctccctcgttccagacgcggctgtagaccacgcccccttcggcatcgcgggcgcgcatgaccacctgcgcgagattgagctccacgtgccgggcgaagacggcgtagtttcgcaggcgctgaaagaggtagttgagggtggtggcggtgtgttctgccacgaagaagtacataacccagcgtcgcaacgtggattcgttgataattgttgtgtaggtactccgccgccgagggacctgagcgagtccgcatcgaccggatcggaaaacctctcgagaaaggcgtctaaccagtcacagtcgcaaggtaggctgagcaccgtggcgggcggcagcgggcggcggtcggggttgtttctggcggaggtgctgctgatgatgtaattaaagtaggcggtcttgagacggcggatggtcgacagaagcaccatgtccttgggtccggcctgctgaatgcgcaggcggtcggccatgccccaggcttcgttttgacatcggcgcaggtctttgtagtagtcttgcatgagcctttctaccggcacttcttcttctccttcctcttgtcctgcatctcttgcatctatcgctgcggcggcggcggagtttggccgtaggtggcgccctcttcctcccatgcgtgtgaccccgaagcccctcatcggctgaagcagggctaggtcggcgacaacgcgctcggctaatatggcctgctgcacctgcgtgagggtagactggaagtcatccatgtccacaaagcggtggtatgcgcccgtgttgatggtgtaagtgcagttggccataacggaccagttaacggtctggtgacccggctgcgagagctcggtgtacctgagacgcgagtaagccctcgagtcaaatacgtagtcgttgcaagtccgcaccaggtactggtatcccaccaaaaagtgcggcggcggctggcggtagaggggccagcgtagggtggccggggctccgggggcgagatcttccaacataaggcgatgatatccgtagatgtacctggacatccaggtgatgccggcggcggtggtggaggcgcgcggaaagtcgcggacgcggttccagatgttgcgcagcggcaaaaagtgctccatggtcgggacgctctggccggtcaggcgcgcgcaatcgttgacgctctagcgtgcaaaaggagagcctgtaagcgggcactcttccgtggtctggtggataaattcgcaagggtatcatggcggacgaccggggttcgagccccgtatccggccgtccgccgtgatccatgcggttaccgcccgcgtgtcgaacccaggtgtgcgacgtcagacaacgggggagtgctccttttggcttccttccaggcgcggcggctgctgcgctagcttttttggccactggccgcgcgcagcgtaagcggttaggctggaaagcgaaagcattaagtggctcgctccctgtagccggagggttattttccaagggttgagtcgcgggacccccggttcgagtctcggaccggccggactgcggcgaacgggggtttgcctccccgtcatgcaagaccccgcttgcaaattcctccggaaacagggacgagccccttttttgcttttcccagatgcatccggtgctgcggcagatgcgcccccctcctcagcagcggcaagagcaagagcagcggcagacatgcagggcaccctcccctcctcctaccgcgtcaggaggggcgacatccgcggttgacgcggcagcagatggtgattacgaacccccgcggcgccgggcccggcactacctggacttggaggagggcgagggcctggcgcggctaggagcgccctctcctgagcggcacccaagggtgcagctgaagcgtgatacgcgtgaggcgtacgtgccgcggcagaacctgtttcgcgaccgcgagggagaggagcccgaggagatgcgggatcgaaagttccacgcagggcgcgagctgcggcatggcctgaatcgcgagcggttgctgcgcgaggaggactttgagcccgacgcgcgaaccgggattagtcccgcgcgcgcacacgtggcggccgccgacctggtaaccgcatacgagcagacggtgaaccaggagattaactttcaaaaaagctttaacaaccacgtgcgtacgcttgtggcgcgcgaggaggtggctataggactgatgcatctgtgggactttgtaagcgcgctggagcaaaacccaaatagcaagccgctcatggcgcagctgttccttatagtgcagcacagcagggacaacgaggcattcagggatgcgctgctaaacatagtagagcccgagggccgctggctgctcgatttgataaacatcctgcagagcatagtggtgcaggagcgcagcttgagcctggctgacaaggtggccgccatcaactattccatgcttagcctgggcaagttttacgcccgcaagatataccataccccttacgttcccatagacaaggaggtaaagatcgaggggttctacatgcgcatggcgctgaaggtgcttaccttgagcgacgacctgggcgtttatcgcaacgagcgcatccacaaggccgtgagcgtgagccggcggcgcgagctcagcgaccgcgagctgatgcacagcctgcaaagggccctggctggcacgggcagcggcgatagagaggccgagtcctactttgacgcgggcgctgacctgcgctgggccccaagccgacgcgccctggaggcagctggggccggacctgggctggcggtggcacccgcgcgcgctggcaacgtcggcggcgtggaggaatatgacgaggacgatgagtacgagccagaggacggcgagtactaagcggtgatgtttctgatcagatgatgcaagacgcaacggacccggcggtgcgggcggcgctgcagagccagccgtccggccttaactccacggacgactggcgccaggtcatggaccgcatcatgtcgctgactgcgcgcaatcctgacgcgttccggcagcagccgcaggccaaccggctctccgcaattctggaagcggtggtcccggcgcgcgcaaaccccacgcacgagaaggtgctggcgatcgtaaacgcgctggccgaaaacagggccatccggcccgacgaggccggcctggtctacgacgcgctgcttcagcgcgtggctcgttacaacagcggcaacgtgcagaccaacctggaccggctggtgggggatgtgcgcgaggccgtggcgcagcgtgagcgcgcgcagcagcagggcaacctgggctccatggttgcactaaacgccttcctgagtacacagcccgccaacgtgccgcggggacaggaggactacaccaactttgtgagcgcactgcggctaatggtgactgagacaccgcaaagtgaggtgtaccagtctgggccagactattttttccagaccagtagacaaggcctgcagaccgtaaacctgagccaggctttcaaaaacttgcaggggctgtggggggtgcgggctcccacaggcgaccgcgcgaccgtgtctagcttgctgacgcccaactcgcgcctgttgctgctgctaatagcgcccttcacggacagtggcagcgtgtcccgggacacatacctaggtcacttgctgacactgtaccgcgaggccataggtcaggcgcatgtggacgagcatactttccaggagattacaagtgtcagccgcgcgctggggcaggaggacacgggcagcctggaggcaaccctaaactacctgctgaccaaccggcggcagaagatcccctcgttgcacagtttaaacagcgaggaggagcgcattttgcgctacgtgcagcagagcgtgagccttaacctgatgcgcgacggggtaacgcccagcgtggcgctggacatgaccgcgcgcaacatggaaccgggcatgtatgcctcaaaccggccgtttatcaaccgcctaatggactacttgcatcgcgcggccgccgtgaaccccgagtatttcaccaatgccatcttgaacccgcactggctaccgccccctggtttctacaccgggggattcgaggtgcccgagggtaacgatggattcctctgggacgacatagacgacagcgtgttttccccgcaaccgcagaccctgctagagttgcaacagcgcgagcaggcagaggcggcgctgcgaaaggaaagcttccgcaggccaagcagcttgtccgatctaggcgctgcggccccgcggtcagatgctagtagcccatttccaagcttgatagggtctcttaccagcactcgcaccacccgcccgcgcctgctgggcgaggaggagtacctaaacaactcgctgctgcagccgcagcgcgaaaaaaacctgcctccggcatttcccaacaacgggatagagagcctagtggacaagatgagtagatggaagacgtacgcgcaggagcacagggacgtgccaggcccgcgcccgcccacccgtcgtcaaaggcacgaccgtcagcggggtctggtgtgggaggacgatgactcggcagacgacagcagcgtcctggatttgggagggagtggcaacccgtttgcgcaccttcgccccaggctggggagaatgttttaaaaaaaaaaaagcatgatgcaaaataaaaaactcaccaaggccatggcaccgagcgttggttttcttgtattccccttagtatgcggcgcgcggcgatgtatgaggaaggtcctcctccctcctacgagagtgtggtgagcgcggcgccagtggcggcggcgctgggttctcccttcgatgctcccctggacccgccgtttgtgcctccgcggtacctgcggcctaccggggggagaaacagcatccgttactctgagttggcacccctattcgacaccacccgtgtgtacctggtggacaacaagtcaacggatgtggcatccctgaactaccagaacgaccacagcaactttctgaccacggtcattcaaaacaatgactacagcccgggggaggcaagcacacagaccatcaatcttgacgaccggtcgcactggggcggcgacctgaaaaccatcctgcataccaacatgccaaatgtgaacgagttcatgtttaccaataagtttaaggcgcgggtgatggtgtcgcgcttgcctactaaggacaatcaggtggagctgaaatacgagtgggtggagttcacgctgcccgagggcaactactccgagaccatgaccatagaccttatgaacaacgcgatcgtggagcactacttgaaagtgggcagacagaacggggttctggaaagcgacatcggggtaaagtttgacacccgcaacttcagactggggtttgaccccgtcactggtcttgtcatgcctggggtatatacaaacgaagccttccatccagacatcattttgctgccaggatgcggggtggacttcacccacagccgcctgagcaacttgttgggcatccgcaagcggcaacccttccaggagggctttaggatcacctacgatgatctggagggtggtaacattcccgcactgttggatgtggacgcctaccaggcgagcttgaaagatgacaccgaacagggcgggggtggcgcaggcggcagcaacagcagtggcagcggcgcggaagagaactccaacgcggcagccgcggcaatgcagccggtggaggacatgaacgatcatgccattcgcggcgacacctttgccacacgggctgaggagaagcgcgctgaggccgaagcagcggccgaagctgccgcccccgctgcgcaacccgaggtcgagaagcctcagaagaaaccggtgatcaaacccctgacagaggacagcaagaaacgcagttacaacctaataagcaatgacagcaccttcacccagtaccgcagctggtaccttgcatacaactacggcgaccctcagaccggaatccgctcatggaccctgctttgcactcctgacgtaacctgcggctcggagcaggtctactggtcgttgccagacatgatgcaagaccccgtgaccttccgctccacgcgccagatcagcaactttccggtggtgggcgccgagctgttgcccgtgcactccaagagcttctacaacgaccaggccgtctactcccaactcatccgccagtttacctctctgacccacgtgttcaatcgctttcccgagaaccagattttggcgcgcccgccagcccccaccatcaccaccgtcagtgaaaacgttcctgctctcacagatcacgggacgctaccgctgcgcaacagcatcggaggagtccagcgagtgaccattactgacgccagacgccgcacctgcccctacgtttacaaggccctgggcatagtctcgccgcgcgtcctatcgagccgcactttttgagcaagcatgtccatccttatatcgcccagcaataacacaggctggggcctgcgcttcccaagcaagatgtttggcggggccaagaagcgctccgaccaacacccagtgcgcgtgcgcgggcactaccgcgcgccctggggcgcgcacaaacgcggccgcactgggcgcaccaccgtcgatgacgccatcgacgcggtggtggaggaggcgcgcaactacacgcccacgccgccaccagtgtccacagtggacgcggccattcagaccgtggtgcgcggagcccggcgctatgctaaaatgaagagacggcggaggcgcgtagcacgtcgccaccgccgccgacccggcactgccgcccaacgcgcggcggcggccctgcttaaccgcgcacgtcgcaccggccgacgggcggccatgcgggccgctcgaaggctggccgcgggtattgtcactgtgccccccaggtccaggcgacgagcggccgccgcagcagccgcggccattagtgctatgactcagggtcgcaggggcaacgtgtattgggtgcgcgactcggttagcggcctgcgcgtgcccgtgcgcacccgccccccgcgcaactagattgcaagaaaaaactacttagactcgtactgttgtatgtatccagcggcggcggcgcgcaacgaagctatgtccaagcgcaaaatcaaagaagagatgctccaggtcatcgcgccggagatctatggccccccgaagaaggaagagcaggattacaagccccgaaagctaaagcgggtcaaaaagaaaaagaaagatgatgatgatgaacttgacgacgaggtggaactgctgcacgctaccgcgcccaggcgacgggtacagtggaaaggtcgacgcgtaaaacgtgttttgcgacccggcaccaccgtagtctttacgcccggtgagcgctccacccgcacctacaagcgcgtgtatgatgaggtgtacggcgacgaggacctgcttgagcaggccaacgagcgcctcggggagtttgcctacggaaagcggcataaggacatgctggcgttgccgctggacgagggcaacccaacacctagcctaaagcccgtaacactgcagcaggtgctgcccgcgcttgcaccgtccgaagaaaagcgcggcctaaagcgcgagtctggtgacttggcacccaccgtgcagctgatggtacccaagcgccagcgactggaagatgtcttggaaaaaatgaccgtggaacctgggctggagcccgaggtccgcgtgcggccaatcaagcaggtggcgccgggactgggcgtgcagaccgtggacgttcagatacccactaccagtagcaccagtattgccaccgccacagagggcatggagacacaaacgtccccggttgcctcagcggtggcggatgccgcggtgcaggcggtcgctgcggccgcgtccaagacctctacggaggtgcaaacggacccgtggatgtttcgcgtttcagccccccggcgcccgcgccgttcgaggaagtacggcgccgccagcgcgctactgcccgaatatgccctacatccttccattgcgcctacccccggctatcgtggctacacctaccgccccagaagacgagcaactacccgacgccgaaccaccactggaacccgccgccgccgtcgccgtcgccagcccgtgctggccccgatttccgtgcgcagggtggctcgcgaaggaggcaggaccctggtgctgccaacagcgcgctaccaccccagcatcgtttaaaagccggtctttgtggttcttgcagatatggccctcacctgccgcctccgtttcccggtgccgggattccgaggaagaatgcaccgtaggaggggcatggccggccacggcctgacgggcggcatgcgtcgtgcgcaccaccggcggcggcgcgcgtcgcaccgtcgcatgcgcggcggtatcctgcccctccttattccactgatcgccgcggcgattggcgccgtgcccggaattgcatccgtggccttgcaggcgcagagacactgattaaaaacaagttgcatgtggaaaaatcaaaataaaaagtctggactctcacgctcgcttggtcctgtaactattttgtagaatggaagacatcaactttgcgtctctggccccgcgacacggctcgcgcccgttcatgggaaactggcaagatatcggcaccagcaatatgagcggtggcgccttcagctggggctcgctgtggagcggcattaaaaatttcggttccaccgttaagaactatggcagcaaggcctggaacagcagcacaggccagatgctgagggataagttgaaagagcaaaatttccaacaaaaggtggtagatggcctggcctctggcattagcggggtggtggacctggccaaccaggcagtgcaaaataagattaacagtaagcttgatccccgccctcccgtagaggagcctccaccggccgtggagacagtgtctccagaggggcgtggcgaaaagcgtccgcgccccgacagggaagaaactctggtgacgcaaatagacgagcctccctcgtacgaggaggcactaaagcaaggcctgcccaccacccgtcccatcgcgcccatggctaccggagtgctgggccagcacacacccgtaacgctggacctgcctccccccgccgacacccagcagaaacctgtgctgccaggcccgaccgccgttgttgtaacccgtcctagccgcgcgtccctgcgccgcgccgccagcggtccgcgatcgttgcggcccgtagccagtggcaactggcaaagcacactgaacagcatcgtgggtctgggggtgcaatccctgaagcgccgacgatgcttctgatagctaacgtgtcgtatgtgtgtcatgtatgcgtccatgtcgccgccagaggagctgctgagccgccgcgcgcccgctttccaagatggctaccccttcgatgatgccgcagtggtcttacatgcacatctcgggccaggacgcctcggagtacctgagccccgggctggtgcagtttgcccgcgccaccgagacgtacttcagcctgaataacaagtttagaaaccccacggtggcgcctacgcacgacgtgaccacagaccggtcccagcgtttgacgctgcggttcatccctgtggaccgtgaggatactgcgtactcgtacaaggcgcggttcaccctagctgtgggtgataaccgtgtgctggacatggcttccacgtactttgacatccgcggcgtgctggacaggggccctacttttaagccctactctggcactgcctacaacgccctggctcccaagggtgccccaaatccttgcgaatgggatgaagctgctactgctcttgaaataaacctagaagaagaggacgatgacaacgaagacgaagtagacgagcaagctgagcagcaaaaaactcacgtatttgggcaggcgccttattctggtataaatattacaaaggagggtattcaaataggtgtcgaaggtcaaacacctaaatatgccgataaaacatttcaacctgaacctcaaataggagaatctcagtggtacgaaacagaaattaatcatgcagctgggagagtcctaaaaaagactaccccaatgaaaccatgttacggttcatatgcaaaacccacaaatgaaaatggagggcaaggcattcttgtaaagcaacaaaatggaaagctagaaagtcaagtggaaatgcaatttttctcaactactgaggcagccgcaggcaatggtgataacttgactcctaaagtggtattgtacagtgaagatgtagatatagaaaccccagacactcatatttcttacatgcccactattaaggaaggtaactcacgagaactaatgggccaacaatctatgcccaacaggcctaattacattgcttttagggacaattttattggtctaatgtattacaacagcacgggtaatatgggtgttctggcgggccaagcatcgcagttgaatgctgttgtagatttgcaagacagaaacacagagctttcataccagcttttgcttgattccattggtgatagaaccaggtacttttctatgtggaatcaggctgttgacagctatgatccagatgttagaattattgaaaatcatggaactgaagatgaacttccaaattactgctttccactgggaggtgtgattaatacagagactcttaccaaggtaaaacctaaaacaggtcaggaaaatggatgggaaaaagatgctacagaattttcagataaaaatgaaataagagttggaaataattttgccatggaaatcaatctaaatgccaacctgtggagaaatttcctgtactccaacatagcgctgtatttgcccgacaagctaaagtacagtccttccaacgtaaaaatttctgataacccaaacacctacgactacatgaacaagcgagtggtggctcccgggctagtggactgctacattaaccttggagcacgctggtcccttgactatatggacaacgtcaacccatttaaccaccaccgcaatgctggcctgcgctaccgctcaatgttgctgggcaatggtcgctatgtgcccttccacatccaggtgcctcagaagttctttgccattaaaaacctccttctcctgccgggctcatacacctacgagtggaacttcaggaaggatgttaacatggttctgcagagctccctaggaaatgacctaagggttgacggagccagcattaagtttgatagcatttgcctttacgccaccttcttccccatggcccacaacaccgcctccacgcttgaggccatgcttagaaacgacaccaacgaccagtcctttaacgactatctctccgccgccaacatgctctaccctatacccgccaacgctaccaacgtgcccatatccatcccctcccgcaactgggcggctttccgcggctgggccttcacgcgccttaagactaaggaaaccccatcactgggctcgggctacgacccttattacacctactctggctctataccctacctagatggaaccttttacctcaaccacacctttaagaaggtggccattacctttgactcttctgtcagctggcctggcaatgaccgcctgcttacccccaacgagtttgaaattaagcgctcagttgacggggagggttacaacgttgcccagtgtaacatgaccaaagactggttcctggtacaaatgctagctaactataacattggctaccagggcttctatatcccagagagctacaaggaccgcatgtactccttctttagaaacttccagcccatgagccgtcaggtggtggatgatactaaatacaaggactaccaacaggtgggcatcctacaccaacacaacaactctggatttgttggctaccttgcccccaccatgcgcgaaggacaggcctaccctgctaacttcccctatccgcttataggcaagaccgcagttgacagcattacccagaaaaagtttctttgcgatcgcaccctttggcgcatcccattctccagtaactttatgtccatgggcgcactcacagacctgggccaaaaccttctctacgccaactccgcccacgcgctagacatgacttttgaggtggatcccatggacgagcccacccttctttatgttttgtttgaagtctttgacgtggtccgtgtgcaccagccgcaccgcggcgtcatcgaaaccgtgtacctgcgcacgcccttctcggccggcaacgccacaacataaagaagcaagcaacatcaacaacagctgccgccatgggctccagtgagcaggaactgaaagccattgtcaaagatcttggttgtgggccatattttttgggcacctatgacaagcgctttccaggctttgtttctccacacaagctcgcctgcgccatagtcaatacggccggtcgcgagactgggggcgtacactggatggcctttgcctggaacccgcactcaaaaacatgctacctctttgagccctttggcttttctgaccagcgactcaagcaggtttaccagtttgagtacgagtcactcctgcgccgtagcgccattgcttcttcccccgaccgctgtataacgctggaaaagtccacccaaagcgtacaggggcccaactcggccgcctgtggactattctgctgcatgtttctccacgcctttgccaactggccccaaactcccatggatcacaaccccaccatgaaccttattaccggggtacccaactccatgctcaacagtccccaggtacagcccaccctgcgtcgcaaccaggaacagctctacagcttcctggagcgccactcgccctacttccgcagccacagtgcgcagattaggagcgccacttctttttgtcacttgaaaaacatgtaaaaataatgtactagagacactttcaataaaggcaaatgcttttatttgtacactctcgggtgattatttacccccacccttgccgtctgcgccgtttaaaaatcaaaggggttctgccgcgcatcgctatgcgccactggcagggacacgttgcgatactggtgtttagtgctccacttaaactcaggcacaaccatccgcggcagctcggtgaagttttcactccacaggctgcgcaccatcaccaacgcgtttagcaggtcgggcgccgatatcttgaagtcgcagttggggcctccgccctgcgcgcgcgagttgcgatacacagggttgcagcactggaacactatcagcgccgggtggtgcacgctggccagcacgctcttgtcggagatcagatccgcgtccaggtcctccgcgttgctcagggcgaacggagtcaactttggtagctgccttcccaaaaagggcgcgtgcccaggctttgagttgcactcgcaccgtagtggcatcaaaaggtgaccgtgcccggtctgggcgttaggatacagcgcctgcataaaagccttgatctgcttaaaagccacctgagcctttgcgccttcagagaagaacatgccgcaagacttgccggaaaactgattggccggacaggccgcgtcgtgcacgcagcaccttgcgtcggtgttggagatctgcaccacatttcggccccaccggttcttcacgatcttggccttgctagactgctccttcagcgcgcgctgcccgttttcgctcgtcacatccatttcaatcacgtgctccttatttatcataatgcttccgtgtagacacttaagctcgccttcgatctcagcgcagcggtgcagccacaacgcgcagcccgtgggctcgtgatgcttgtaggtcacctctgcaaacgactgcaggtacgcctgcaggaatcgccccatcatcgtcacaaaggtcttgttgctggtgaaggtcagctgcaacccgcggtgctcctcgttcagccaggtcttgcatacggccgccagagcttccacttggtcaggcagtagtttgaagttcgcctttagatcgttatccacgtggtacttgtccatcagcgcgcgcgcagcctccatgcccttctcccacgcagacacgatcggcacactcagcgggttcatcaccgtaatttcactttccgcttcgctgggctcttcctcttcctcttgcgtccgcataccacgcgccactgggtcgtcttcattcagccgccgcactgtgcgcttacctcctttgccatgcttgattagcaccggtgggttgctgaaacccaccatttgtagcgccacatcttctctttcttcctcgctgtccacgattacctctggtgatggcgggcgctcgggcttgggagaagggcgcttctttttcttcttgggcgcaatggccaaatccgccgccgaggtcgatggccgcgggctgggtgtgcgcggcaccagcgcgtcttgtgatgagtcttcctcgtcctcggactcgatacgccgcctcatccgcttttttgggggcgcccggggaggcggcggcgacggggacggggacgacacgtcctccatggttgggggacgtcgcgccgcaccgcgtccgcgctcgggggtggtttcgcgctgctcctcttcccgactggccatttccttctcctataggcagaaaaagatcatggagtcagtcgagaagaaggacagcctaaccgccccctctgagttcgccaccaccgcctccaccgatgccgccaacgcgcctaccaccttccccgtcgaggcacccccgcttgaggaggaggaagtgattatcgagcaggacccaggttttgtaagcgaagacgacgaggaccgctcagtaccaacagaggataaaaagcaagaccaggacaacgcagaggcaaacgaggaacaagtcgggcggggggacgaaaggcatggcgactacctagatgtgggagacgacgtgctgttgaagcatctgcagcgccagtgcgccattatctgcgacgcgttgcaagagcgcagcgatgtgcccctcgccatagcggatgtcagccttgcctacgaacgccacctattctcaccgcgcgtaccccccaaacgccaagaaaacggcacatgcgagcccaacccgcgcctcaacttctaccccgtatttgccgtgccagaggtgcttgccacctatcacatctttttccaaaactgcaagatacccctatcctgccgtgccaaccgcagccgagcggacaagcagctggccttgcggcagggcgctgtcatacctgatatcgcctcgctcaacgaagtgccaaaaatctttgagggtcttggacgcgacgagaagcgcgcggcaaacgctctgcaacaggaaaacagcgaaaatgaaagtcactctggagtgttggtggaactcgagggtgacaacgcgcgcctagccgtactaaaacgcagcatcgaggtcacccactttgcctacccggcacttaacctaccccccaaggtcatgagcacagtcatgagtgagctgatcgtgcgccgtgcgcagcccctggagagggatgcaaatttgcaagaacaaacagaggagggcctacccgcagttggcgacgagcagctagcgcgctggcttcaaacgcgcgagcctgccgacttggaggagcgacgcaaactaatgatggccgcagtgctcgttaccgtggagcttgagtgcatgcagcggttctttgctgacccggagatgcagcgcaagctagaggaaacattgcactacacctttcgacagggctacgtacgccaggcctgcaagatctccaacgtggagctctgcaacctggtctcctaccttggaattttgcacgaaaaccgccttgggcaaaacgtgcttcattccacgctcaagggcgaggcgcgccgcgactacgtccgcgactgcgtttacttatttctatgctacacctggcagacggccatgggcgtttggcagcagtgcttggaggagtgcaacctcaaggagctgcagaaactgctaaagcaaaacttgaaggacctatggacggccttcaacgagcgctccgtggccgcgcacctggcggacatcattttccccgaacgcctgcttaaaaccctgcaacagggtctgccagacttcaccagtcaaagcatgttgcagaactttaggaactttatcctagagcgctcaggaatcttgcccgccacctgctgtgcacttcctagcgactttgtgcccattaagtaccgcgaatgccctccgccgctttggggccactgctaccttctgcagctagccaactaccttgcctaccactctgacataatggaagacgtgagcggtgacggtctactggagtgtcactgtcgctgcaacctatgcaccccgcaccgctccctggtttgcaattcgcagctgcttaacgaaagtcaaattatcggtacctttgagctgcagggtccctcgcctgacgaaaagtccgcggctccggggttgaaactcactccggggctgtggacgtcggcttaccttcgcaaatttgtacctgaggactaccacgcccacgagattaggttctacgaagaccaatcccgcccgcctaatgcggagcttaccgcctgcgtcattacccagggccacattcttggccaattgcaagccatcaacaaagcccgccaagagtttctgctacgaaagggacggggggtttacttggacccccagtccggcgaggagctcaacccaatccccccgccgccgcagccctatcagcagcagccgcgggcccttgcttcccaggatggcacccaaaaagaagctgcagctgccgccgccacccacggacgaggaggaatactgggacagtcaggcagaggaggttttggacgaggaggaggaggacatgatggaagactgggagagcctagacgaggaagcttccgaggtcgaagaggtgtcagacgaaacaccgtcaccctcggtcgcattcccctcgccggcgccccagaaatcggcaaccggttccagcatggctacaacctccgctcctcaggcgccgccggcactgcccgttcgccgacccaaccgtagatgggacaccactggaaccagggccggtaagtccaagcagccgccgccgttagcccaagagcaacaacagcgccaaggctaccgctcatggcgcgggcacaagaacgccatagttgcttgcttgcaagactgtgggggcaacatctccttcgcccgccgctttcttctctaccatcacggcgtggccttcccccgtaacatcctgcattactaccgtcatctctacagcccatactgcaccggcggcagcggcagcaacagcagcggccacacagaagcaaaggcgaccggatagcaagactctgacaaagcccaagaaatccacagcggcggcagcagcaggaggaggagcgctgcgtctggcgcccaacgaacccgtatcgacccgcgagcttagaaacaggatttttcccactctgtatgctatatttcaacagagcaggggccaagaacaagagctgaaaataaaaaacaggtctctgcgatccctcacccgcagctgcctgtatcacaaaagcgaagatcagcttcggcgcacgctggaagacgcggaggctctcttcagtaaatactgcgcgctgactcttaaggactagtttcgcgccctttctcaaatttaagcgcgaaaactacgtcatctccagcggccacacccggcgccagcacctgttgtcagcgccattatgagcaaggaaattcccacgccctacatgtggagttaccagccacaaatgggacttgcggctggagctgcccaagactactcaacccgaataaactacatgagcgcgggaccccacatgatatcccgggtcaacggaatacgcgcccaccgaaaccgaattctcctggaacaggcggctattaccaccacacctcgtaataaccttaatccccgtagttggcccgctgccctggtgtaccaggaaagtcccgctcccaccactgtggtacttcccagagacgcccaggccgaagttcagatgactaactcaggggcgcagcttgcgggcggctttcgtcacagggtgcggtcgcccgggcagggtataactcacctgacaatcagagggcgaggtattcagctcaacgacgagtcggtgagctcctcgcttggtctccgtccggacgggacatttcagatcggcggcgccggccgctcttcattcacgcctcgtcaggcaatcctaactctgcagacctcgtcctctgagccgcgctctggaggcattggaactctgcaatttattgaggagtttgtgccatcggtctactttaaccccttctcgggacctcccggccactatccggatcaatttattcctaactttgacgcggtaaaggactcggcggacggctacgactgaatgttaagtggagaggcagagcaactgcgcctgaaacacctggtccactgtcgccgccacaagtgctttgcccgcgactccggtgagttttgctactttgaattgcccgaggatcatatcgagggcccggcgcacggcgtccggcttaccgcccagggagagcttgcccgtagcctgattcgggagtttacccagcgccccctgctagttgagcgggacaggggaccctgtgttctcactgtgatttgcaactgtcctaaccctggattacatcaagatcctctagttaatgtcaggtcgcctaagtcgattaactagagtacccggggatcttattccctttaactaataaaaaaaaataataaagcatcacttacttaaaatcagttagcaaatttctgtccagtttattcagcagcacctccttgccctcctcccagctctggtattgcagcttcctcctggctgcaaactttctccacaatctaaatggaatgtcagtttcctcctgttcctgtccatccgcacccactatcttcatgttgttgcagatgaagcgcgcaagaccgtctgaagataccttcaaccccgtgtatccatatgacacggaaaccggtcctccaactgtgccttttcttactcctccctttgtatcccccaatgggtttcaagagagtccccctggggtactctctttgcgcctatccgaacctctagttacctccaatggcatgcttgcgctcaaaatgggcaacggcctctctctggacgaggccggcaaccttacctcccaaaatgtaaccactgtgagcccacctctcaaaaaaaccaagtcaaacataaacctggaaatatctgcacccctcacagttacctcagaagccctaactgtggctgccgccgcacctctaatggtcgcgggcaacacactcaccatgcaatcacaggccccgctaaccgtgcacgactccaaacttagcattgccacccaaggacccctcacagtgtcagaaggaaagctagccctgcaaacatcaggccccctcaccaccaccgatagcagtacccttactatcactgcctcaccccctctaactactgccactggtagcttgggcattgacttgaaagagcccatttatacacaaaatggaaaactaggactaaagtacggggctcctttgcatgtaacagacgacctaaacactttgaccgtagcaactggtccaggtgtgactattaataatacttccttgcaaactaaagttactggagccttgggttttgattcacaaggcaatatgcaacttaatgtagcaggaggactaaggattgattctcaaaacagacgccttatacttgatgttagttatccgtttgatgctcaaaaccaactaaatctaagactaggacagggccctctttttataaactcagcccacaacttggatattaactacaacaaaggcctttacttgtttacagcttcaaacaattccaaaaagcttgaggttaacctaagcactgccaaggggttgatgtttgacgctacagccatagccattaatgcaggagatgggcttgaatttggttcacctaatgcaccaaacacaaatcccctcaaaacaaaaattggccatggcctagaatttgattcaaacaaggctatggttcctaaactaggaactggccttagttttgacagcacaggtgccattacagtaggaaacaaaaataatgataagctaactttgtggaccacaccagctccatctcctaactgtagactaaatgcagagaaagatgctaaactcactttggtcttaacaaaatgtggcagtcaaatacttgctacagtttcagttttggctgttaaaggcagtttggctccaatatctggaacagttcaaagtgctcatcttattataagatttgacgaaaatggagtgctactaaacaattccttcctggacccagaatattggaactttagaaatggagatcttactgaaggcacagcctatacaaacgctgttggatttatgcctaacctatcagcttatccaaaatctcacggtaaaactgccaaaagtaacattgtcagtcaagtttacttaaacggagacaaaactaaacctgtaacactaaccattacactaaacggtacacaggaaacaggagacacaactccaagtgcatactctatgtcattttcatgggactggtctggccacaactacattaatgaaatatttgccacatcctcttacactttttcatacattgcccaagaataaagaatcgtttgtgttatgtttcaacgtgtttatttttcaattgcagaaaatttcaagtcatttttcattcagtagtatagccccaccaccacatagcttatacagatcaccgtaccttaatcaaactcacagaaccctagtattcaacctgccacctccctcccaacacacagagtacacagtcctttctccccggctggccttaaaaagcatcatatcatgggtaacagacatattcttaggtgttatattccacacggtttcctgtcgagccaaacgctcatcagtgatattaataaactccccgggcagctcacttaagttcatgtcgctgtccagctgctgagccacaggctgctgtccaacttgcggttgcttaacgggcggcgaaggagaagtccacgcctacatgggggtagagtcataatcgtgcatcaggatagggcggtggtgctgcagcagcgcgcgaataaactgctgccgccgccgctccgtcctgcaggaatacaacatggcagtggtctcctcagcgatgattcgcaccgcccgcagcataaggcgccttgtcctccgggcacagcagcgcaccctgatctcacttaaatcagcacagtaactgcagcacagcaccacaatattgttcaaaatcccacagtgcaaggcgctgtatccaaagctcatggcggggaccacagaacccacgtggccatcataccacaagcgcaggtagattaagtggcgacccctcataaacacgctggacataaacattacctcttttggcatgttgtaattcaccacctcccggtaccatataaacctctgattaaacatggcgccatccaccaccatcctaaaccagctggccaaaacctgcccgccggctatacactgcagggaaccgggactggaacaatgacagtggagagcccaggactcgtaaccatggatcatcatgctcgtcatgatatcaatgttggcacaacacaggcacacgtgcatacacttcctcaggattacaagctcctcccgcgttagaaccatatcccagggaacaacccattcctgaatcagcgtaaatcccacactgcagggaagacctcgcacgtaactcacgttgtgcattgtcaaagtgttacattcgggcagcagcggatgatcctccagtatggtagcgcgggtttctgtctcaaaaggaggtagacgatccctactgtacggagtgcgccgagacaaccgagatcgtgttggtcgtagtgtcatgccaaatggaacgccggacgtagtcatatttcctgaagcaaaaccaggtgcgggcgtgacaaacagatctgcgtctccggtctcgccgcttagatcgctctgtgtagtagttgtagtatatccactctctcaaagcatccaggcgccccctggcttcgggttctatgtaaactccttcatgcgccgctgccctgataacatccaccaccgcagaataagccacacccagccaacctacacattcgttctgcgagtcacacacgggaggagcgggaagagctggaagaaccatgtttttttttttattccaaaagattatccaaaacctcaaaatgaagatctattaagtgaacgcgctcccctccggtggcgtggtcaaactctacagccaaagaacagataatggcatttgtaagatgttgcacaatggcttccaaaaggcaaacggccctcacgtccaagtggacgtaaaggctaaacccttcagggtgaatctcctctataaacattccagcaccttcaaccatgcccaaataattctcatctcgccaccttctcaatatatctctaagcaaatcccgaatattaagtccggccattgtaaaaatctgctccagagcgccctccaccttcagcctcaagcagcgaatcatgattgcaaaaattcaggttcctcacagacctgtataagattcaaaagcggaacattaacaaaaataccgcgatcccgtaggtcccttcgcagggccagctgaacataatcgtgcaggtctgcacggaccagcgcggccacttccccgccaggaaccatgacaaaagaacccacactgattatgacacgcatactcggagctatgctaaccagcgtagccccgatgtaagcttgttgcatgggcggcgatataaaatgcaaggtgctgctcaaaaaatcaggcaaagcctcgcgcaaaaaagaaagcacatcgtagtcatgctcatgcagataaaggcaggtaagctccggaaccaccacagaaaaagacaccatttttctctcaaacatgtctgcgggtttctgcataaacacaaaataaaataacaaaaaaacatttaaacattagaagcctgtcttacaacaggaaaaacaacccttataagcataagacggactacggccatgccggcgtgaccgtaaaaaaactggtcaccgtgattaaaaagcaccaccgacagctcctcggtcatgtccggagtcataatgtaagactcggtaaacacatcaggttgattcacatcggtcagtgctaaaaagcgaccgaaatagcccgggggaatacatacccgcaggcgtagagacaacattacagcccccataggaggtataacaaaattaataggagagaaaaacacataaacacctgaaaaaccctcctgcctaggcaaaatagcaccctcccgctccagaacaacatacagcgcttccacagcggcagccataacagtcagccttaccagtaaaaaagaaaacctattaaaaaaacaccactcgacacggcaccagctcaatcagtcacagtgtaaaaaagggccaagtgcagagcgagtatatataggactaaaaaatgacgtaacggttaaagtccacaaaaaacacccagaaaaccgcacgcgaacctacgcccagaaacgaaagccaaaaaacccacaacttcctcaaatcgtcacttccgttttcccacgttacgtcacttcccattttaagaaaactacaattcccaacacatacaagttactccgccctaaaacctacgtcacccgccccgttcccacgccccgcgccacgtcacaaactccaccccctcattatcatattggcttcaatccaaaataaggta

SEQ ID NO: 229 - DNA, 9701 bp, synthetic construct
  misc_feature 1..9701: note = vector for IgG1 against T27Y H34A H378N ACE2 mutant
  misc_feature 2929..2930: note = n is a, c, g, or t
  misc_feature 2934: note = n is a, c, g, or t
  source 1..9701: mol_type = other DNA
ggcgtaatctgctgcttgcaaacaaaaaaaccaccgctaccagcggtggtttgtttgccggatcaagagctaccaactctttttccgaaggtaactggcttcagcagagcgcagataccaaatactgtccttctagtgtagccgtagttaggccaccacttcaagaactctgtagcaccgcctacatacctcgctctgctgaagccagttaccagtggctgctgccagtggcgataagtcgtgtcttaccgggttggactcaagagatagttaccggataaggcgcagcggtcgggctgaacggggggttcgtgcacacagcccagcttggagcgaacgacctacaccgaactgagatacctacagcgtgagctatgagaaagcgccacgcttcccgaagggagaaaggcggacaggtatccggtaagcggcagggtcggaacaggagagcgcacgagggagcttccagggggaaacgcctggtatctttatagtcctgtcgggtttcgccacctctgacttgagcgtcgatttttgtgatgctcgtcaggggggcggagcctatggaaaaacgccagcaacgcaagctagagtttaaacttgacagatgagacaataaccctgataaatgcttcaataatattgaaaaaggaaaagtatgagtattcaacatttccgtgtcgcccttattcccttttttgcggcattttgccttcctgtttttgctcacccagaaacgctggtgaaagtaaaagatgcagaagatcacttgggtgcgcgagtgggttacatcgaactggatctcaacagcggtaagatccttgagagttttcgccccgaagaacgtttcccaatgatgagcacttttaaagttctgctatgtggcgcggtattatcccgtattgatgccgggcaagagcaactcggtcgccgcatacactattctcagaatgacttggttgaatactcaccagtcacagaaaagcatcttacggatggcatgacagtaagagaattatgcagtgctgccataaccatgagtgataacactgcggccaacttacttctgacaactatcggaggaccgaaggagctaaccgcttttttgcacaacatgggggatcatgtaactcgccttgatcgttgggaaccggagctgaatgaagccataccaaacgacgagcgtgacaccacgatgcctgtagcaatggcaacaacgttgcgaaaactattaactggcgaactacttactctagcttcccggcaacaactaatagactggatggaggcggataaagttgcaggaccacttctgcgctcggcacttccggctggctggtttattgctgataaatcaggagccggtgagcgtgggtcacgcggtatcattgcagcactggggccggatggtaagccctcccgtatcgtagttatctacactacggggagtcaggcaactatggatgaacgaaatagacagatcgctgagataggtgcctcactgattaagcattggtaaggataaatttctggtaaggaggacacgtatggaagtgggcaagttggggaagccgtatccgttgctgaatctggcatatgtgggagtataagacgcgcagcgtcgcatcaggcatttttttctgcgccaatgcaaaaaggccatccgtcaggatggcctttcggcataactagggccgccgatatttgaaaatatggcatattgaaaatgtcgccgatgtgagtttctgtgtaactgatatcgccatttttccaaaagtgatttttgggcatacgcgatatctggcgatagcgcttatatcgtttacgggggatggcgatagacgactttggtgacttgggcgattctgtgtgtcgcaaatatcgcagtttcgatataggtgacagacgatatgaggctatatcgccgatagaggcgacatcaagctggcacatggccaatgcatatcgatctatacattgaatcaatattggccattagccatattattcattggttatatagcataaatcaatattggctattggccattgcatacgttgtatccatatcataatatgtacatttatattggctcatgtccaacattaccgccatgttgacattgattattgactagttattaatagtaatcaattacggggtcattagttcatagcccatatatggagttccgcgttacataacttacggtaaatggcccgcctggctgaccgcccaacgacccccgcccattgacgtcaataatgacgtatgttcccatagtaacgccaatagggactttccattgacgtcaatgggtggagtatttacggtaaactgcccacttggcagtacatcaagtgtatcatatgccaagtacgccccctattgacgtcaatgacggtaaatggcccgcctggcattatgcccagtacatgaccttatgggactttcctacttggcagtacatctacgtattagtcatcgctattaccatggtgatgcggttttggcagtacatcaatgggcgtggatagcggtttgactcacggggatttccaagtctccaccccattgacgtcaatgggagtttgttttggcaccaaaatcaacgggactttccaaaatgtcgtaacaactccgccccattgacgcaaatgggcggtaggcgtgtacggtgggaggtctatataagcagagctcgtttagtgaaccgtcagatcgcctggagacgccatccacgctgttttgacctccatagaagacaccgggaccgatccagcctccgcggccgggaacggtgcattggaacgcggattccccgtgccaagagtgacgtaagtaccgcctatagagtctataggcccacccccttggcttcttatgcatgctatactgtttttggcttggggtctatacaccccccgnnttcntcatgttataggtgatggtatagcttagcctataggtgtgggttattgaccattattgaccactccccctattggtgacgatactttccattactaatccataacatggctctttgccacaactctctttattggctatatgccaatacactgtccttcagagactgacacggactctgtatttttacaggatggggtctcatttattatttacaaattcacatatacaacaccaccgtccccagtgcccgcagtttttattaaacataacgtgggatctccacgcgaatctcgggtacgtgttccggacatgggctcttctccggtagcggcggagcttctacatccgagccctgctcccatgcctccagcgactcatggtcgctcggcagctccttgctcctaacagtggaggccagacttaggcacagcacgatgcccaccaccaccagtgtgccgcacaaggccgtggcggtagggtatgtgtctgaaaatgagctcggggagcgggcttgcaccgctgacgcatttggaagacttaaggcagcggcagaagaagatgcaggcagctgagttgttgtgttctgataagagtcagaggtaactcccgttgcggtgctgttaacggtggagggcagtgtagtctgagcagtactcgttgctgccgcgcgcgccaccagacataatagctgacagactaacagactgttcctttccatgggtcttttctgcagtcaccgtccttgacacgaagctgctagcgccaccatgagcagcagtagttggcttctcttgagtttggtggcagtgacagcagcccagagtactatcgaggagcaggctaaatactttctggataagtttaacgccgaggccgaagacttgttctatcaatcttctctcgcttcatggaattacaatactaacatcactgaggagaacgtccagaatatgaacaatgctggcgacaaatggagcgccttcttgaaggagcagtctacccttgcacaaatgtatccactgcaggagatacagaaccttacagtaaagttgcagctccaggctctccagcagaacggatctagcgtgctttcagaggataaaagcaaaaggctgaacaccatacttaataccatgtccacaatttactctactggtaaagtatgtaaccccgacaaccctcaagaatgcctccttcttgagccaggcctcaatgagatcatggctaatagtctggactataatgaaagactgtgggcatgggagtcctggagatctgaagtagggaagcaactgaggcccctttatgaagagtacgtcgtacttaagaatgaaatggcccgcgctaaccactacgaggattacggcgattactggcgtggggactatgaagtaaatggtgtagatggatacgactatagtcgtgggcaattgattgaggatgtggagcacacttttgaggagataaaaccactctatgagcatcttcacgcatatgtgagagctaaactgatgaacgcctacccaagttacatcagtccaatcggatgtctcccagctcacctccttggcgacatgtggggacgtttctggaccaatctgtattccctcacagtccctttcgggcaaaagcctaatatagacgtgacagacgcaatggttgatcaggcttgggatgctcaaaggatttttaaggaagctgagaagttttttgtgtcagtcggtttgccaaatatgacacaaggcttctgggaaaatagcatgttgactgatcccggtaatgttcaaaaggctgtgtgtcaccctaccgcttgggaccttgggaaaggtgactttcgaatcttgatgtgtaccaaggtgacaatggatgactttcttacagcccatcatgaaatgggtaatatccagtatgatatggcttatgcagctcaacctttcctcttgagaaatggtgcaaatgaaggttttcatgaagctgtaggggaaataatgtccctgagtgctgcaaccccaaagcatctcaagagtatcggattgttgagcccagattttcaagaagataacgagaccgaaatcaacttccttctgaaacaagccctcacaatagttggtactcttccattcacatacatgctggagaaatggcgttggatggtttttaagggggagatacctaaagatcagtggatgaaaaagtggtgggagatgaagcgtgagatcgtaggggtcgtggagccagtgcctcatgatgagacttactgtgacccagcatcactcttccacgttagcaatgactattcatttatacgttattacactcgcactctttaccagtttcaatttcaggaggctctgtgtcaggctgccaagcatgagggaccccttcacaagtgtgatattagtaacagtactgaggcaggccaaaaactgttcaatatgttgaggcttggcaaaagcgagccatggactctcgccttggaaaatgttgtcggggctaaaaacatgaatgtacgccctctgcttaactattttgagcccctttttacatggctcaaggaccagaataagaactcctttgtcggctggtcaacagactggtctccctatgcagacaaaacacatacttgcccaccttgtcctgcaccagagctgctgggaggtccaagcgtgttcctgtttccacccaagcccaaagacacactgatgatttctcgaactccagaagtgacctgcgtggtcgtggacgtgagccacgaggatcccgaagtgaagttcaactggtacgtggatggcgtggaggtccataatgctaagactaaaccccgggaggaacagtacaacagcacttatagggtcgtgtccgtgctgaccgtcctgcatcaggattggctgaacgggaaggaatataagtgcaaagtgtctaataaggcactgcccgcccctatcgagaaaacaattagcaaggctaagggtcagcctagagaaccacaggtgtacactctgcctccaagtcgcgacgagctgaccaagaaccaggtgtcactgacatgtctggtcaaaggcttttatccctcagatatcgcagtggagtgggaaagcaatggacagcctgagaacaattacaagaccacaccccctgtgctggacagtgatggctcattctttctgtattctaagctgacagtggacaaaagtaggtggcagcagggaaacgtgttctcctgctctgtcatgcacgaagcactgcacaatcattatacccagaagagtctgtcactgagccctggcaaatgagcgataccgattctagaactagatcataatcagccataccacatttgtagaggttttacttgctttaaaaaacctcccacacctccccctgaacctgaaacataaaatgaatgcaattgttgttgttaacttgtttattgcagcttataatggttacaaataaagcaatagcatcacaaatttcacaaataaagcatttttttcactgcattctagttgtggtttgtccaaactcatcaatgtatcttaaggccgcaggtaagccagcccaggcctcgccctccagctcaaggcgggacaggtgccctagagtagcctgcatccagggacaggccccagccgggtgctgacacgtccacctccatctcttcctcaggtctgcccgggtggcatccctgtgacccctccccagtgcctctcctggtcgtggaaggtgctactccagtgcccaccagccttgtcctaataaaattaagttgcatcattttgtttgactaggtgtccttgtataatattatggggtggaggcgggtggtatggagcaaggggcccaagttaacttgtttattgcagcttataatggttacaaataaagcaatagcatcacaaatttcacaaataaagcatttttttcactgcattctagttgtggtttgtccaaactcatcaatgtatcttatcatgtctggatccgcttcaggcaccgggcttgcgggtcatgcaccaggtgcgcggtccttcgggcacctcgacgtcggcggtgacggtgaagccgagccgctcgtagaaggggaggttgcggggcgcggaggtctccaggaaggcgggcaccccggcgcgctcggccgcctccactccggggagcacgacggcgctgcccagacccttgccctggtggtcgggcgagacgccgacggtggccaggaaccacgcgggctccttgggccggtgcggcgccaggaggccttccatctgttgctgcgcggccagcctggaaccgctcaactcggccatgcgcgggccgatctcggcgaacaccgcccccgcttcgacgctctccggcgtggtccagaccgccaccgcggcgccgtcgtccgcgacccacaccttgccgatgtcgagcccgacgcgcgtgaggaagagttcttgcagctcggtgacccgctcgatgtggcggtccgggtcgacggtgtggcgcgtggcggggtagtcggcgaacgcggcggcgagggtgcgtacggcccgggggacgtcgtcgcgggtggcgaggcgcaccgtgggcttgtactcggtcatggtggcctgcagagtcgctctgtgttcgaggccacacgcgtcaccttaatatgcgaagtggacctgggaccgcgccgccccgactgcatctgcgtgttttcgccaatgacaagacgctgggcggggtttgtgtcatcatagaactaaagacatgcaaatatatttcttccggggacaccgccagcaaacgcgagcaacgggccacggggatgaagcagctgcgccactccctgaagatccatcgtctcctaacaagttacatcactcctgcccttcctcaccctcatctccatcacctccttcatctccgtcatctccgtcatcaccctccgcggcagccccttccaccataggtggaaaccagggaggcaaatctactccatcgtcaaagctgcacacagtcaccctgatattgcaggtaggagcgggctttgtcataacaaggtccttaatcgcatccttcaaaacctcagcaaatatatgagtttgtaaaaagaccatgaaataacagacaatggactcccttagcgggccaggttgtgggccgggtccaggggccattccaaaggggagacgactcaatggtgtaagacgacattgtggaatagcaagggcagttcctcgccttaggttgtaaagggaggtcttactacctccatatacgaacacaccggcgacccaagttccttcgtcggtagtcctttctacgtgactcctagccaggagagctcttaaaccttctgcaatgttctcaaatttcgggttggaacctccttgaccacgatgctttccaaaccaccctccttttttgcgcctgcctccatcaccctgacccccgctgcgcgggggcacgtcaggctcaccatctgggccgccttcttggtggtattcaaaataatcggcttcccctacagggtggaaaaatggccttctacctggagggggcctgcgcggtggagacccggatgatgatgactgactactgggactcctgggcctcttttctccacgtccacgacctctccccctggctctttcacgacttccccccctggctctttcacgtcctctaccccggcggcctccactacctcctcgaccccggcctccactacctcctcgaccccggcctccactgcctcctcgaccccggcctccacctcctgctcctgcccctcccgctcctgctcctgctcctgttccaccgtgggtccctttgcagccaatgcaacttggacgtttttggggtctccggacaccatctctatgtcttggccctgatcctgagccgcccggggctcctggtcttccgcctcctcgtcctcgtcctcttccccgtcctcgtccatgtgccatgatggcggcctgcagctgtgttcgaggccgcgcgtgtcaccttaatatgcgaagtggacctgggaccgcgccgccccgactgcatctgcgtgttcgagttcgccaatgacaagacgctgggcggggagatcccccttattaaccctaaacgggtagcatatgcttcccgggtagtagtatatactatccagactaaccctaattcaatagcatatgttacccaacgggaagcatatgctatcgaattagggttagtaaaagggtcctaaggaacagcgatctggatagcatatgctatcctaatctatatctgggtagcatatgctatcctaatctatatctgggtagcataggctatcctaatctatatctgggtagcatatgctatcctaatctatatctgggtagtatatgctatcctaatttatatctgggtagcataggctatcctaatctatatctgggtagcatatgctatcctaatctatatctgggtagtatatgctatcctaatctgtatccgggtagcatatgctatcctcatgcatatacagtcagcatatgatacccagtagtagagtgggagtgctatcctttgcatatgccgccacctcccaaggagatctgtcgacatcgatgggcgcgggtgtacactccgcccatcccgcccctaactccgcccagttccgcccattctccgcctcatggctgactaattttttttatttatgcagaggccgaggccgcctcggcctctgagctattccagaagtagtgaggaggcttttttggaggcctaggcttttgcaaaaagctaattc

SEQ ID NO: 230 - DNA, 38496 bp, synthetic construct
  misc_feature 1..38496: note = vector for IgA against T27Y H34A H345A ACE2 mutant
  source 1..38496: mol_type = other DNA
tattattgatgatgttaattaacatgcatggatcctacgtctcgaccgatgcccttgagagccttcaacccagtcagctccttccggtgggcgcggggcatgactatcgtcgccgcacttatgactgtcttctttatcatgcaactcgtaggacaggtgccggcagcgctctgggtcattttcggcgaggaccgctttcgctggagcgcgacgatgatcggcctgtcgcttgcggtattcggaatcttgcacgccctcgctcaagccttcgtcactggtcccgccaccaaacgtttcggcgagaagcaggccattatcgccggcatggcggccgacgcgctgggctacgtcttgctggcgttcgcgacgcgaggctggatggccttccccattatgattcttctcgcttccggcggcatcgggatgcccgcgttgcaggccatgctgtccaggcaggtagatgacgaccatcagggacagcttcaaggatcgctcgcggctcttaccagcctaacttcgatcattggaccgctgatcgtcacggcgatttatgccgcctcggcgagcacatggaacgggttggcatggattgtaggcgccgccctataccttgtctgcctccccgcgttgcgtcgcggtgcatggagccgggccacctcgacctgaatggaagccggcggcacctcgctaacggattcaccactccaagaattggagccaatcaattcttgcggagaactgtgaatgcgcaaaccaacccttggcagaacatatccatcgcgtccgccatctccagcagccgcacgcggcgcatctcgggcagcgttgggtcctggccacgggtgcgcatgatcgtgctcctgtcgttgaggacccggctaggctggcggggttgccttactggttagcagaatgaatcaccgatacgcgagcgaacgtgaagcgactgctgctgcaaaacgtctgcgacctgagcaacaacatgaatggtcttcggtttccgtgtttcgtaaagtctggaaacgcggaagtcagcgccctgcaccattatgttccggatctgcatcgcaggatgctgctggctaccctgtggaacacctacatctgtattaacgaagcgctggcattgaccctgagtgatttttctctggtcccgccgcatccataccgccagttgtttaccctcacaacgttccagtaaccgggcatgttcatcatcagtaacccgtatcgtgagcatcctctctcgtttcatcggtatcattacccccatgaacagaaatcccccttacacggaggcatcagtgaccaaacaggaaaaaaccgcccttaacatggcccgctttatcagaagccagacattaacgcttctggagaaactcaacgagctggacgcggatgaacaggcagacatctgtgaatcgcttcacgaccacgctgatgagctttaccgcagctgcctcgcgcgtttcggtgatgacggtgaaaacctctgacacatgcagctcccggagacggtcacagcttgtctgtaagcggatgccgggagcagacaagcccgtcagggcgcgtcagcgggtgttggcgggtgtcggggcgcagccatgacccagtcacgtagcgatagcggagtgtatactggcttaactatgcggcatcagagcagattgtactgagagtgcaccatatgcggtgtgaaataccgcacagatgcgtaaggagaaaataccgcatcaggcgctcttccgcttcctcgctcactgactcgctgcgctcggtcgttcggctgcggcgagcggtatcagctcactcaaaggcggtaatacggttatccacagaatcaggggataacgcaggaaagaacatgtgagcaaaaggccagcaaaaggccaggaaccgtaaaaaggccgcgttgctggcgtttttccataggctccgcccccctgacgagcatcacaaaaatcgacgctcaagtcagaggtggcgaaacccgacaggactataaagataccaggcgtttccccctggaagctccctcgtgcgctctcctgttccgaccctgccgcttaccggatacctgtccgcctttctcccttcgggaagcgtggcgctttctcatagctcacgctgtaggtatctcagttcggtgtaggtcgttcgctccaagctgggctgtgtgcacgaaccccccgttcagcccgaccgctgcgccttatccggtaactatcgtcttgagtccaacccggtaagacacgacttatcgccactggcagcagccactggtaacaggattagcagagcgaggtatgtaggcggtgctacagagttcttgaagtggtggcctaactacggctacactagaaggacagtatttggtatctgcgctctgctgaagccagttaccttcggaaaaagagttggtagctcttgatccggcaaacaaaccaccgctggtagcggtggtttttttgtttgcaagcagcagattacgcgcagaaaaaaaggatctcaagaagatcctttgatcttttctacggggtctgacgctcagtggaacgaaaactcacgttaagggattttggtcatgagattatcaaaaaggatcttcacctagatccttttaaattaaaaatgaagttttaaatcaatctaaagtatatatgagtaaacttggtctgacagttaccaatgcttaatcagtgaggcacctatctcagcgatctgtctatttcgttcatccatagttgcctgactccccgtcgtgtagataactacgatacgggagggcttaccatctggccccagtgctgcaatgataccgcgagacccacgctcaccggctccagatttatcagcaataaaccagccagccggaagggccgagcgcagaagtggtcctgcaactttatccgcctccatccagtctattaattgttgccgggaagctagagtaagtagttcgccagttaatagtttgcgcaacgttgttgccattgctgcagccatgagattatcaaaaaggatcttcacctagatccttttcacgtagaaagccagtccgcagaaacggtgctgaccccggatgaatgtcagctactgggctatctggacaagggaaaacgcaagcgcaaagagaaagcaggtagcttgcagtgggcttacatggcgatagctagactgggcggttttatggacagcaagcgaaccggaattgccagctggggcgccctctggtaaggttgggaagccctgcaaagtaaactggatggctttcttgccgccaaggatctgatggcgcaggggatcaagctctgatcaagagacaggatgaggatcgtttcgcatgattgaacaagatggattgcacgcaggttctccggccgcttgggtggagaggctattcggctatgactgggcacaacagacaatcggctgctctgatgccgccgtgttccggctgtcagcgcaggggcgcccggttctttttgtcaagaccgacctgtccggtgccctgaatgaactgcaagacgaggcagcgcggctatcgtggctggccacgacgggcgttccttgcgcagctgtgctcgacgttgtcactgaagcgggaagggactggctgctattgggcgaagtgccggggcaggatctcctgtcatctcaccttgctcctgccgagaaagtatccatcatggctgatgcaatgcggcggctgcatacgcttgatccggctacctgcccattcgaccaccaagcgaaacatcgcatcgagcgagcacgtactcggatggaagccggtcttgtcgatcaggatgatctggacgaagagcatcaggggctcgcgccagccgaactgttcgccaggctcaaggcgagcatgcccgacggcgaggatctcgtcgtgacccatggcgatgcctgcttgccgaatatcatggtggaaaatggccgcttttctggattcatcgactgtggccggctgggtgtggcggaccgctatcaggacatagcgttggctacccgtgatattgctgaagagcttggcggcgaatgggctgaccgcttcctcgtgctttacggtatcgccgctcccgattcgcagcgcatcgccttctatcgccttcttgacgagttcttctgaattttgttaaaatttttgttaaatcagctcattttttaaccaataggccgaaatcggcaaaatcccttataaatcaaaagaatagaccgagatagggttgagtgttgttccagtttggaacaagagtccactattaaagaacgtggactccaacgtcaaagggcgaaaaaccgtctatcagggcgatggcccactacgtgaaccatcaccctaatcaagttttttggggtcgaggtgccgtaaagcactaaatcggaaccctaaagggagcccccgatttagagcttgacggggaaagccggcgaacgtggcgagaaaggaagggaagaaagcgaaaggagcgggcgctagggcgctggcaagtgtagcggtcacgctgcgcgtaaccaccacacccgccgcgcttaatgcgccgctacagggcgcgtccattcgccattcaggatcgaattaattcttaattaacatcatcaataatataccttattttggattgaagccaatatgataatgagggggtggagtttgtgacgtggcgcggggcgtgggaacggggcgggtgacgtagtagtgtggcggaagtgtgatgttgcaagtgtggcggaacacatgtaagcgacggatgtggcaaaagtgacgtttttggtgtgcgccggtgtacacaggaagtgacaattttcgcgcggttttaggcggatgttgtagtaaatttgggcgtaaccgagtaagatttggccattttcgcgggaaaactgaataagaggaagtgaaatctgaataattttgtgttactcatagcgcgtaatactgtaatagtaatcaattacggggtcattagttcatagcccatatatggagttccgcgttacataacttacggtaaatggcccgcctggctgaccgcccaacgacccccgcccattgacgtcaataatgacgtatgttcccatagtaacgccaatagggactttccattgacgtcaatgggtggagtatttacggtaaactgcccacttggcagtacatcaagtgtatcatatgccaagtacgccccctattgacgtcaatgacggtaaatggcccgcctggcattatgcccagtacatgaccttatgggactttcctacttggcagtacatctacgtattagtcatcgctattaccatggtgatgcggttttggcagtacatcaatgggcgtggatagcggtttgactcacggggatttccaagtctccaccccattgacgtcaatgggagtttgttttggcaccaaaatcaacgggactttccaaaatgtcgtaacaactccgccccattgacgcaaatgggcggtaggcgtgtacggtgggaggtctatataagcagagctggtttagtgaaccgtcagatccgctagagatctggtaccgtcgacgcggccgctcgagcctaagcttatgagcagcagtagttggcttctcttgagtttggtggcagtgacagcagcccagagtactatcgaggagcaggctaaatactttctggataagtttaacgccgaggccgaagacttgttctatcaatcttctctcgcttcatggaattacaatactaacatcactgaggagaacgtccagaatatgaacaatgctggcgacaaatggagcgccttcttgaaggagcagtctacccttgcacaaatgtatccactgcaggagatacagaaccttacagtaaagttgcagctccaggctctccagcagaacggatctagcgtgctttcagaggataaaagcaaaaggctgaacaccatacttaataccatgtccacaatttactctactggtaaagtatgtaaccccgacaaccctcaagaatgcctccttcttgagccaggcctcaatgagatcatggctaatagtctggactataatgaaagactgtgggcatgggagtcctggagatctgaagtagggaagcaactgaggcccctttatgaagagtacgtcgtacttaagaatgaaatggcccgcgctaaccactacgaggattacggcgattactggcgtggggactatgaagtaaatggtgtagatggatacgactatagtcgtgggcaattgattgaggatgtggagcacacttttgaggagataaaaccactctatgagcatcttcacgcatatgtgagagctaaactgatgaacgcctacccaagttacatcagtccaatcggatgtctcccagctcacctccttggcgacatgtggggacgtttctggaccaatctgtattccctcacagtccctttcgggcaaaagcctaatatagacgtgacagacgcaatggttgatcaggcttgggatgctcaaaggatttttaaggaagctgagaagttttttgtgtcagtcggtttgccaaatatgacacaaggcttctgggaaaatagcatgttgactgatcccggtaatgttcaaaaggctgtgtgtgcccctaccgcttgggaccttgggaaaggtgactttcgaatcttgatgtgtaccaaggtgacaatggatgactttcttacagcccatcatgaaatgggtcacatccagtatgatatggcttatgcagctcaacctttcctcttgagaaatggtgcaaatgaaggttttcatgaagctgtaggggaaataatgtccctgagtgctgcaaccccaaagcatctcaagagtatcggattgttgagcccagattttcaagaagataacgagaccgaaatcaacttccttctgaaacaagccctcacaatagttggtactcttccattcacatacatgctggagaaatggcgttggatggtttttaagggggagatacctaaagatcagtggatgaaaaagtggtgggagatgaagcgtgagatcgtaggggtcgtggagccagtgcctcatgatgagacttactgtgacccagcatcactcttccacgttagcaatgactattcatttatacgttattacactcgcactctttaccagtttcaatttcaggaggctctgtgtcaggctgccaagcatgagggaccccttcacaagtgtgatattagtaacagtactgaggcaggccaaaaactgttcaatatgttgaggcttggcaaaagcgagccatggactctcgccttggaaaatgttgtcggggctaaaaacatgaatgtacgccctctgcttaactattttgagcccctttttacatggctcaaggaccagaataagaactcctttgtcggctggtcaacagactggtctccctatgcagaccctagtactcctcctactccttctccatcaaccccaccaactccatcccctagctgctgtcacccaaggctgtctctgcaccgacctgcactcgaagaccttctgttgggctctgaagctaacctgacctgtactcttactggcttgcgcgatgctagcggcgtgactttcacctggacacctagtagcggtaaaagtgctgtacaaggacctcctgaacgcgacctgtgtggttgctactctgtgtcttctgtacttcccggctgtgccgagccctggaatcacgggaaaacctttacctgcaccgccgcttaccctgagtcaaaaactcccctcactgccacattgagtaagtcagggaatacattcaggccagaggttcatttgttgcctcctccatctgaagaacttgctttgaacgagctggtcactctgacctgcttggctaggggtttctcccccaaagatgtacttgtacggtggttgcagggcagccaagagttgccccgcgaaaagtatttgacctgggcctcaagacaagaacccagccaggggactaccacatttgccgtgaccagtattctgcgtgtagccgctgaagattggaagaaaggggatacattttcttgcatggtagggcatgaggcccttcccctcgctttcactcagaagacaatagacagactcgccggaaagcctactcacgtgaatgttagcgtagtcatggctgaggttgacggaacttgctactgagatatccgatccaccggatctagataactgatcataatcagccataccacatttgtagaggttttacttgctttaaaaaacctcccacacctccccctgaacctgaaacataaaatgaatgcaattgttgttgttaacttgtttattgcagcttataatggttacaaataaagcaatagcatcacaaatttcacaaataaagcatttttttcactgcattctagttgtggtttgtccaaactcatcaatgtatcttaggtttagtgaaccgtcagatccgctagcgttacataacttacggtaaatggcccgcctggctgaccgcccaacgacccccgcccattgacgtcaataatgacgtatgttcccatagtaacgccaatagggactttccattgacgtcaatgggtggagtatttacggtaaactgcccacttggcagtacatcaagtgtatcatatgccaagtacgccccctattgacgtcaatgacggtaaatggcccgcctggcattatgcccagtacatgaccttatgggactttcctacttggcagtacatctacgtattagtcatcgctattaccatggtgatgcggttttggcagtacatcaatgggcgtggatagcggtttgactcacggggatttccaagtctccaccccattgacgtcaatgggagtttgttttggcaccaaaatcaacgggactttccaaaatgtcgtaacaactccgccccattgacgcaaatgggcggtaggcgtgtacggtgggaggtctatataagcagagctggtttagtgaaccgtcagatccgctagagatctggtaccgtcgacgcggccgctcgagcctaagcttatgaagaaccatctgcttttctggggagtacttgccgttttcataaaagccgtacatgttaaagcacaagaggacgaacgcattgtgttggttgataataaatgcaaatgtgctcggataacatctcggatcattcgtagctcagaggaccccaatgaggatatagtagagcgaaacatcagaattatagtacccctgaacaacagagagaacataagtgatcccacaagtccattgcggacacgctttgtttaccatttgtctgatctgtgtaaaaaatgtgatccaacagaggtggaactcgacaatcagatcgtcaccgccacccagtctaacatctgcgatgaagattcagctacagagacatgctacacatacgaccggaacaagtgctatactgccgttgtgccactcgtttacggtggagaaacaaagatggttgaaactgcacttacaccagatgcctgctatccagattgagatatccgatccaccggatctagataactgatcataatcagccataccacatttgtagaggttttacttgctttaaaaaacctcccacacctccccctgaacctgaaacataaaatgaatgcaattgttgttgttaacttgtttattgcagcttataatggttacaaataaagcaatagcatcacaaatttcacaaataaagcatttttttcactgcattctagttgtggtttgtccaaactcatcaatgtatcttaacgcggatctgggcgtggttaagggtgggaaagaatatataaggtgggggtcttatgtagttttgtatctgttttgcagcagccgccgccgccatgagcaccaactcgtttgatggaagcattgtgagctcatatttgacaacgcgcatgcccccatgggccggggtgcgtcagaatgtgatgggctccagcattgatggtcgccccgtcctgcccgcaaactctactaccttgacctacgagaccgtgtctggaacgccgttggagactgcagcctccgccgccgcttcagccgctgcagccaccgcccgcgggattgtgactgactttgctttcctgagcccgcttgcaagcagtgcagcttcccgttcatccgcccgcgatgacaagttgacggctcttttggcacaattggattctttgacccgggaacttaatgtcgtttctcagcagctgttggatctgcgccagcaggtttctgccctgaaggcttcctcccctcccaatgcggtttaaaacataaataaaaaaccagactctgtttggatttggatcaagcaagtgtcttgctgtctttatttaggggttttgcgcgcgcggtaggcccgggaccagcggtctcggtcgttgagggtcctgtgtattttttccaggacgtggtaaaggtgactctggatgttcagatacatgggcataagcccgtctctggggtggaggtagcaccactgcagagcttcatgctgcggggtggtgttgtagatgatccagtcgtagcaggagcgctgggcgtggtgcctaaaaatgtctttcagtagcaagctgattgccaggggcaggcccttggtgtaagtgtttacaaagcggttaagctgggatgggtgcatacgtggggatatgagatgcatcttggactgtatttttaggttggctatgttcccagccatatccctccggggattcatgttgtgcagaaccaccagcacagtgtatccggtgcacttgggaaatttgtcatgtagcttagaaggaaatgcgtggaagaacttggagacgcccttgtgacctccaagattttccatgcattcgtccataatgatggcaatgggcccacgggcggcggcctgggcgaagatatttctgggatcactaacgtcatagttgtgttccaggatgagatcgtcataggccatttttacaaagcgcgggcggagggtgccagactgcggtataatggttccatccggcccaggggcgtagttaccctcacagatttgcatttcccacgctttgagttcagatggggggatcatgtctacctgcggggcgatgaagaaaacggtttccggggtaggggagatcagctgggaagaaagcaggttcctgagcagctgcgacttaccgcagccggtgggcccgtaaatcacacctattaccggctgcaactggtagttaagagagctgcagctgccgtcatccctgagcaggggggccacttcgttaagcatgtccctgactcgcatgttttccctgaccaaatccgccagaaggcgctcgccgcccagcgatagcagttcttgcaaggaagcaaagtttttcaacggtttgagaccgtccgccgtaggcatgcttttgagcgtttgaccaagcagttccaggcggtcccacagctcggtcacctgctctacggcatctcgatccagcatatctcctcgtttcgcgggttggggcggctttcgctgtacggcagtagtcggtgctcgtccagacgggccagggtcatgtctttccacgggcgcagggtcctcgtcagcgtagtctgggtcacggtgaaggggtgcgctccgggctgcgcgctggccagggtgcgcttgaggctggtcctgctggtgctgaagcgctgccggtcttcgccctgcgcgtcggccaggtagcatttgaccatggtgtcatagtccagcccctccgcggcgtggcccttggcgcgcagcttgcccttggaggaggcgccgcacgaggggcagtgcagacttttgagggcgtagagcttgggcgcgagaaataccgattccggggagtaggcatccgcgccgcaggccccgcagacggtctcgcattccacgagccaggtgagctctggccgttcggggtcaaaaaccaggtttcccccatgctttttgatgcgtttcttacctctggtttccatgagccggtgtccacgctcggtgacgaaaaggctgtccgtgtccccgtatacagacttgagaggcctgtcctcgagcggtgttccgcggtcctcctcgtatagaaactcggaccactctgagacaaaggctcgcgtccaggccagcacgaaggaggctaagtgggaggggtagcggtcgttgtccactagggggtccactcgctccagggtgtgaagacacatgtcgccctcttcggcatcaaggaaggtgattggtttgtaggtgtaggccacgtgaccgggtgttcctgaaggggggctataaaagggggtgggggcgcgttcgtcctcactctcttccgcatcgctgtctgcgagggccagctgttggggtgagtactccctctgaaaagcgggcatgacttctgcgctaagattgtcagtttccaaaaacgaggaggatttgatattcacctggcccgcggtgatgcctttgagggtggccgcatccatctggtcagaaaagacaatctttttgttgtcaagcttggtggcaaacgacccgtagagggcgttggacagcaacttggcgatggagcgcagggtttggtttttgtcgcgatcggcgcgctccttggccgcgatgtttagctgcacgtattcgcgcgcaacgcaccgccattcgggaaagacggtggtgcgctcgtcgggcaccaggtgcacgcgccaaccgcggttgtgcagggtgacaaggtcaacgctggtggctacctctccgcgtaggcgctcgttggtccagcagaggcggccgcccttgcgcgagcagaatggcggtagggggtctagctgcgtctcgtccggggggtctgcgtccacggtaaagaccccgggcagcaggcgcgcgtcgaagtagtctatcttgcatccttgcaagtctagcgcctgctgccatgcgcgggcggcaagcgcgcgctcgtatgggttgagtgggggaccccatggcatggggtgggtgagcgcggaggcgtacatgccgcaaatgtcgtaaacgtagaggggctctctgagtattccaagatatgtagggtagcatcttccaccgcggatgctggcgcgcacgtaatcgtatagttcgtgcgagggagcgaggaggtcgggaccgaggttgctacgggcgggctgctctgctcggaagactatctgcctgaagatggcatgtgagttggatgatatggttggacgctggaagacgttgaagctggcgtctgtgagacctaccgcgtcacgcacgaaggaggcgtaggagtcgcgcagcttgttgaccagctcggcggtgacctgcacgtctagggcgcagtagtccagggtttccttgatgatgtcatacttatcctgtcccttttttttccacagctcgcggttgaggacaaactcttcgcggtctttccagtactcttggatcggaaacccgtcggcctccgaacggtaagagcctagcatgtagaactggttgacggcctggtaggcgcagcatcccttttctacgggtagcgcgtatgcctgcgcggccttccggcatgaccagcatgaagggcacgagctgcttcccaaaggcccccatccaagtataggtctctacatcgtaggtgacaaagagacgctcggtgcgaggatgcgagccgatcgggaagaactggatctcccgccaccaattggaggagtggctattgatgtggtgaaagtagaagtccctgcgacgggccgaacactcgtgctggcttttgtaaaaacgtgcgcagtactggcagcggtgcacgggctgtacatcctgcacgaggttgacctgacgaccgcgcacaaggaagcagagtgggaatttgagcccctcgcctggcgggtttggctggtggtcttctacttcggctgcttgtccttgaccgtctggctgctcgaggggagttacggtggatcggaccaccacgccgcgcgagcccaaagtccagatgtccgcgcgcggcggtcggagcttgatgacaacatcgcgcagatgggagctgtccatggtctggagctcccgcggcgtcaggtcaggcgggagctcctgcaggtttacctcgcatagacgggtcagggcgcgggctagatccaggtgatacctaatttccaggggctggttggtggcggcgtcgatggcttgcaagaggccgcatccccgcggcgcgactacggtaccgcgcggcgggcggtgggccgcgggggtgtccttggatgatgcatctaaaagcggtgacgcgggcgagcccccggaggtagggggggctccggacccgccgggagagggggcaggggcacgtcggcgccgcgcgcgggcaggagctggtgctgcgcgcgtaggttgctggcgaacgcgacgacgcggcggttgatctcctgaatctggcgcctctgcgtgaagacgacgggcccggtgagcttgaacctgaaagagagttcgacagaatcaatttcggtgtcgttgacggcggcctggcgcaaaatctcctgcacgtctcctgagttgtcttgataggcgatctcggccatgaactgctcgatctcttcctcctggagatctccgcgtccggctcgctccacggtggcggcgaggtcgttggaaatgcgggccatgagctgcgagaaggcgttgaggcctccctcgttccagacgcggctgtagaccacgcccccttcggcatcgcgggcgcgcatgaccacctgcgcgagattgagctccacgtgccgggcgaagacggcgtagtttcgcaggcgctgaaagaggtagttgagggtggtggcggtgtgttctgccacgaagaagtacataacccagcgtcgcaacgtggattcgttgataattgttgtgtaggtactccgccgccgagggacctgagcgagtccgcatcgaccggatcggaaaacctctcgagaaaggcgtctaaccagtcacagtcgcaaggtaggctgagcaccgtggcgggcggcagcgggcggcggtcggggttgtttctggcggaggtgctgctgatgatgtaattaaagtaggcggtcttgagacggcggatggtcgacagaagcaccatgtccttgggtccggcctgctgaatgcgcaggcggtcggccatgccccaggcttcgttttgacatcggcgcaggtctttgtagtagtcttgcatgagcctttctaccggcacttcttcttctccttcctcttgtcctgcatctcttgcatctatcgctgcggcggcggcggagtttggccgtaggtggcgccctcttcctcccatgcgtgtgaccccgaagcccctcatcggctgaagcagggctaggtcggcgacaacgcgctcggctaatatggcctgctgcacctgcgtgagggtagactggaagtcatccatgtccacaaagcggtggtatgcgcccgtgttgatggtgtaagtgcagttggccataacggaccagttaacggtctggtgacccggctgcgagagctcggtgtacctgagacgcgagtaagccctcgagtcaaatacgtagtcgttgcaagtccgcaccaggtactggtatcccaccaaaaagtgcggcggcggctggcggtagaggggccagcgtagggtggccggggctccgggggcgagatcttccaacataaggcgatgatatccgtagatgtacctggacatccaggtgatgccggcggcggtggtggaggcgcgcggaaagtcgcggacgcggttccagatgttgcgcagcggcaaaaagtgctccatggtcgggacgctctggccggtcaggcgcgcgcaatcgttgacgctctagcgtgcaaaaggagagcctgtaagcgggcactcttccgtggtctggtggataaattcgcaagggtatcatggcggacgaccggggttcgagccccgtatccggccgtccgccgtgatccatgcggttaccgcccgcgtgtcgaacccaggtgtgcgacgtcagacaacgggggagtgctccttttggcttccttccaggcgcggcggctgctgcgctagcttttttggccactggccgcgcgcagcgtaagcggttaggctggaaagcgaaagcattaagtggctcgctccctgtagccggagggttattttccaagggttgagtcgcgggacccccggttcgagtctcggaccggccggactgcggcgaacgggggtttgcctccccgtcatgcaagaccccgcttgcaaattcctccggaaacagggacgagccccttttttgcttttcccagatgcatccggtgctgcggcagatgcgcccccctcctcagcagcggcaagagcaagagcagcggcagacatgcagggcaccctcccctcctcctaccgcgtcaggaggggcgacatccgcggttgacgcggcagcagatggtgattacgaacccccgcggcgccgggcccggcactacctggacttggaggagggcgagggcctggcgcggctaggagcgccctctcctgagcggcacccaagggtgcagctgaagcgtgatacgcgtgaggcgtacgtgccgcggcagaacctgtttcgcgaccgcgagggagaggagcccgaggagatgcgggatcgaaagttccacgcagggcgcgagctgcggcatggcctgaatcgcgagcggttgctgcgcgaggaggactttgagcccgacgcgcgaaccgggattagtcccgcgcgcgcacacgtggcggccgccgacctggtaaccgcatacgagcagacggtgaaccaggagattaactttcaaaaaagctttaacaaccacgtgcgtacgcttgtggcgcgcgaggaggtggctataggactgatgcatctgtgggactttgtaagcgcgctggagcaaaacccaaatagcaagccgctcatggcgcagctgttccttatagtgcagcacagcagggacaacgaggcattcagggatgcgctgctaaacatagtagagcccgagggccgctggctgctcgatttgataaacatcctgcagagcatagtggtgcaggagcgcagcttgagcctggctgacaaggtggccgccatcaactattccatgcttagcctgggcaagttttacgcccgcaagatataccataccccttacgttcccatagacaaggaggtaaagatcgaggggttctacatgcgcatggcgctgaaggtgcttaccttgagcgacgacctgggcgtttatcgcaacgagcgcatccacaaggccgtgagcgtgagccggcggcgcgagctcagcgaccgcgagctgatgcacagcctgcaaagggccctggctggcacgggcagcggcgatagagaggccgagtcctactttgacgcgggcgctgacctgcgctgggccccaagccgacgcgccctggaggcagctggggccggacctgggctggcggtggcacccgcgcgcgctggcaacgtcggcggcgtggaggaatatgacgaggacgatgagtacgagccagaggacggcgagtactaagcggtgatgtttctgatcagatgatgcaagacgcaacggacccggcggtgcgggcggcgctgcagagccagccgtccggccttaactccacggacgactggcgccaggtcatggaccgcatcatgtcgctgactgcgcgcaatcctgacgcgttccggcagcagccgcaggccaaccggctctccgcaattctggaagcggtggtcccggcgcgcgcaaaccccacgcacgagaaggtgctggcgatcgtaaacgcgctggccgaaaacagggccatccggcccgacgaggccggcctggtctacgacgcgctgcttcagcgcgtggctcgttacaacagcggcaacgtgcagaccaacctggaccggctggtgggggatgtgcgcgaggccgtggcgcagcgtgagcgcgcgcagcagcagggcaacctgggctccatggttgcactaaacgccttcctgagtacacagcccgccaacgtgccgcggggacaggaggactacaccaactttgtgagcgcactgcggctaatggtgactgagacaccgcaaagtgaggtgtaccagtctgggccagactattttttccagaccagtagacaaggcctgcagaccgtaaacctgagccaggctttcaaaaacttgcaggggctgtggggggtgcgggctcccacaggcgaccgcgcgaccgtgtctagcttgctgacgcccaactcgcgcctgttgctgctgctaatagcgcccttcacggacagtggcagcgtgtcccgggacacatacctaggtcacttgctgacactgtaccgcgaggccataggtcaggcgcatgtggacgagcatactttccaggagattacaagtgtcagccgcgcgctggggcaggaggacacgggcagcctggaggcaaccctaaactacctgctgaccaaccggcggcagaagatcccctcgttgcacagtttaaacagcgaggaggagcgcattttgcgctacgtgcagcagagcgtgagccttaacctgatgcgcgacggggtaacgcccagcgtggcgctggacatgaccgcgcgcaacatggaaccgggcatgtatgcctcaaaccggccgtttatcaaccgcctaatggactacttgcatcgcgcggccgccgtgaaccccgagtatttcaccaatgccatcttgaacccgcactggctaccgccccctggtttctacaccgggggattcgaggtgcccgagggtaacgatggattcctctgggacgacatagacgacagcgtgttttccccgcaaccgcagaccctgctagagttgcaacagcgcgagcaggcagaggcggcgctgcgaaaggaaagcttccgcaggccaagcagcttgtccgatctaggcgctgcggccccgcggtcagatgctagtagcccatttccaagcttgatagggtctcttaccagcactcgcaccacccgcccgcgcctgctgggcgaggaggagtacctaaacaactcgctgctgcagccgcagcgcgaaaaaaacctgcctccggcatttcccaacaacgggatagagagcctagtggacaagatgagtagatggaagacgtacgcgcaggagcacagggacgtgccaggcccgcgcccgcccacccgtcgtcaaaggcacgaccgtcagcggggtctggtgtgggaggacgatgactcggcagacgacagcagcgtcctggatttgggagggagtggcaacccgtttgcgcaccttcgccccaggctggggagaatgttttaaaaaaaaaaaagcatgatgcaaaataaaaaactcaccaaggccatggcaccgagcgttggttttcttgtattccccttagtatgcggcgcgcggcgatgtatgaggaaggtcctcctccctcctacgagagtgtggtgagcgcggcgccagtggcggcggcgctgggttctcccttcgatgctcccctggacccgccgtttgtgcctccgcggtacctgcggcctaccggggggagaaacagcatccgttactctgagttggcacccctattcgacaccacccgtgtgtacctggtggacaacaagtcaacggatgtggcatccctgaactaccagaacgaccacagcaactttctgaccacggtcattcaaaacaatgactacagcccgggggaggcaagcacacagaccatcaatcttgacgaccggtcgcactggggcggcgacctgaaaaccatcctgcataccaacatgccaaatgtgaacgagttcatgtttaccaataagtttaaggcgcgggtgatggtgtcgcgcttgcctactaaggacaatcaggtggagctgaaatacgagtgggtggagttcacgctgcccgagggcaactactccgagaccatgaccatagaccttatgaacaacgcgatcgtggagcactacttgaaagtgggcagacagaacggggttctggaaagcgacatcggggtaaagtttgacacccgcaacttcagactggggtttgaccccgtcactggtcttgtcatgcctggggtatatacaaacgaagccttccatccagacatcattttgctgccaggatgcggggtggacttcacccacagccgcctgagcaacttgttgggcatccgcaagcggcaacccttccaggagggctttaggatcacctacgatgatctggagggtggtaacattcccgcactgttggatgtggacgcctaccaggcgagcttgaaagatgacaccgaacagggcgggggtggcgcaggcggcagcaacagcagtggcagcggcgcggaagagaactccaacgcggcagccgcggcaatgcagccggtggaggacatgaacgatcatgccattcgcggcgacacctttgccacacgggctgaggagaagcgcgctgaggccgaagcagcggccgaagctgccgcccccgctgcgcaacccgaggtcgagaagcctcagaagaaaccggtgatcaaacccctgacagaggacagcaagaaacgcagttacaacctaataagcaatgacagcaccttcacccagtaccgcagctggtaccttgcatacaactacggcgaccctcagaccggaatccgctcatggaccctgctttgcactcctgacgtaacctgcggctcggagcaggtctactggtcgttgccagacatgatgcaagaccccgtgaccttccgctccacgcgccagatcagcaactttccggtggtgggcgccgagctgttgcccgtgcactccaagagcttctacaacgaccaggccgtctactcccaactcatccgccagtttacctctctgacccacgtgttcaatcgctttcccgagaaccagattttggcgcgcccgccagcccccaccatcaccaccgtcagtgaaaacgttcctgctctcacagatcacgggacgctaccgctgcgcaacagcatcggaggagtccagcgagtgaccattactgacgccagacgccgcacctgcccctacgtttacaaggccctgggcatagtctcgccgcgcgtcctatcgagccgcactttttgagcaagcatgtccatccttatatcgcccagcaataacacaggctggggcctgcgcttcccaagcaagatgtttggcggggccaagaagcgctccgaccaacacccagtgcgcgtgcgcgggcactaccgcgcgccctggggcgcgcacaaacgcggccgcactgggcgcaccaccgtcgatgacgccatcgacgcggtggtggaggaggcgcgcaactacacgcccacgccgccaccagtgtccacagtggacgcggccattcagaccgtggtgcgcggagcccggcgctatgctaaaatgaagagacggcggaggcgcgtagcacgtcgccaccgccgccgacccggcactgccgcccaacgcgcggcggcggccctgcttaaccgcgcacgtcgcaccggccgacgggcggccatgcgggccgctcgaaggctggccgcgggtattgtcactgtgccccccaggtccaggcgacgagcggccgccgcagcagccgcggccattagtgctatgactcagggtcgcaggggcaacgtgtattgggtgcgcgactcggttagcggcctgcgcgtgcccgtgcgcacccgccccccgcgcaactagattgcaagaaaaaactacttagactcgtactgttgtatgtatccagcggcggcggcgcgcaacgaagctatgtccaagcgcaaaatcaaagaagagatgctccaggtcatcgcgccggagatctatggccccccgaagaaggaagagcaggattacaagccccgaaagctaaagcgggtcaaaaagaaaaagaaagatgatgatgatgaacttgacgacgaggtggaactgctgcacgctaccgcgcccaggcgacgggtacagtggaaaggtcgacgcgtaaaacgtgttttgcgacccggcaccaccgtagtctttacgcccggtgagcgctccacccgcacctacaagcgcgtgtatgatgaggtgtacggcgacgaggacctgcttgagcaggccaacgagcgcctcggggagtttgcctacggaaagcggcataaggacatgctggcgttgccgctggacgagggcaacccaacacctagcctaaagcccgtaacactgcagcaggtgctgcccgcgcttgcaccgtccgaagaaaagcgcggcctaaagcgcgagtctggtgacttggcacccaccgtgcagctgatggtacccaagcgccagcgactggaagatgtcttggaaaaaatgaccgtggaacctgggctggagcccgaggtccgcgtgcggccaatcaagcaggtggcgccgggactgggcgtgcagaccgtggacgttcagatacccactaccagtagcaccagtattgccaccgccacagagggcatggagacacaaacgtccccggttgcctcagcggtggcggatgccgcggtgcaggcggtcgctgcggccgcgtccaagacctctacggaggtgcaaacggacccgtggatgtttcgcgtttcagccccccggcgcccgcgccgttcgaggaagtacggcgccgccagcgcgctactgcccgaatatgccctacatccttccattgcgcctacccccggctatcgtggctacacctaccgccccagaagacgagcaactacccgacgccgaaccaccactggaacccgccgccgccgtcgccgtcgccagcccgtgctggccccgatttccgtgcgcagggtggctcgcgaaggaggcaggaccctggtgctgccaacagcgcgctaccaccccagcatcgtttaaaagccggtctttgtggttcttgcagatatggccctcacctgccgcctccgtttcccggtgccgggattccgaggaagaatgcaccgtaggaggggcatggccggccacggcctgacgggcggcatgcgtcgtgcgcaccaccggcggcggcgcgcgtcgcaccgtcgcatgcgcggcggtatcctgcccctccttattccactgatcgccgcggcgattggcgccgtgcccggaattgcatccgtggccttgcaggcgcagagacactgattaaaaacaagttgcatgtggaaaaatcaaaataaaaagtctggactctcacgctcgcttggtcctgtaactattttgtagaatggaagacatcaactttgcgtctctggccccgcgacacggctcgcgcccgttcatgggaaactggcaagatatcggcaccagcaatatgagcggtggcgccttcagctggggctcgctgtggagcggcattaaaaatttcggttccaccgttaagaactatggcagcaaggcctggaacagcagcacaggccagatgctgagggataagttgaaagagcaaaatttccaacaaaaggtggtagatggcctggcctctggcattagcggggtggtggacctggccaaccaggcagtgcaaaataagattaacagtaagcttgatccccgccctcccgtagaggagcctccaccggccgtggagacagtgtctccagaggggcgtggcgaaaagcgtccgcgccccgacagggaagaaactctggtgacgcaaatagacgagcctccctcgtacgaggaggcactaaagcaaggcctgcccaccacccgtcccatcgcgcccatggctaccggagtgctgggccagcacacacccgtaacgctggacctgcctccccccgccgacacccagcagaaacctgtgctgccaggcccgaccgccgttgttgtaacccgtcctagccgcgcgtccctgcgccgcgccgccagcggtccgcgatcgttgcggcccgtagccagtggcaactggcaaagcacactgaacagcatcgtgggtctgggggtgcaatccctgaagcgccgacgatgcttctgatagctaacgtgtcgtatgtgtgtcatgtatgcgtccatgtcgccgccagaggagctgctgagccgccgcgcgcccgctttccaagatggctaccccttcgatgatgccgcagtggtcttacatgcacatctcgggccaggacgcctcggagtacctgagccccgggctggtgcagtttgcccgcgccaccgagacgtacttcagcctgaataacaagtttagaaaccccacggtggcgcctacgcacgacgtgaccacagaccggtcccagcgtttgacgctgcggttcatccctgtggaccgtgaggatactgcgtactcgtacaaggcgcggttcaccctagctgtgggtgataaccgtgtgctggacatggcttccacgtactttgacatccgcggcgtgctggacaggggccctacttttaagccctactctggcactgcctacaacgccctggctcccaagggtgccccaaatccttgcgaatgggatgaagctgctactgctcttgaaataaacctagaagaagaggacgatgacaacgaagacgaagtagacgagcaagctgagcagcaaaaaactcacgtatttgggcaggcgccttattctggtataaatattacaaaggagggtattcaaataggtgtcgaaggtcaaacacctaaatatgccgataaaacatttcaacctgaacctcaaataggagaatctcagtggtacgaaacagaaattaatcatgcagctgggagagtcctaaaaaagactaccccaatgaaaccatgttacggttcatatgcaaaacccacaaatgaaaatggagggcaaggcattcttgtaaagcaacaaaatggaaagctagaaagtcaagtggaaatgcaatttttctcaactactgaggcagccgcaggcaatggtgataacttgactcctaaagtggtattgtacagtgaagatgtagatatagaaaccccagacactcatatttcttacatgcccactattaaggaaggtaactcacgagaactaatgggccaacaatctatgcccaacaggcctaattacattgcttttagggacaattttattggtctaatgtattacaacagcacgggtaatatgggtgttctggcgggccaagcatcgcagttgaatgctgttgtagatttgcaagacagaaacacagagctttcataccagcttttgcttgattccattggtgatagaaccaggtacttttctatgtggaatcaggctgttgacagctatgatccagatgttagaattattgaaaatcatggaactgaagatgaacttccaaattactgctttccactgggaggtgtgattaatacagagactcttaccaaggtaaaacctaaaacaggtcaggaaaatggatgggaaaaagatgctacagaattttcagataaaaatgaaataagagttggaaataattttgccatggaaatcaatctaaatgccaacctgtggagaaatttcctgtactccaacatagcgctgtatttgcccgacaagctaaagtacagtccttccaacgtaaaaatttctgataacccaaacacctacgactacatgaacaagcgagtggtggctcccgggctagtggactgctacattaaccttggagcacgctggtcccttgactatatggacaacgtcaacccatttaaccaccaccgcaatgctggcctgcgctaccgctcaatgttgctgggcaatggtcgctatgtgcccttccacatccaggtgcctcagaagttctttgccattaaaaacctccttctcctgccgggctcatacacctacgagtggaacttcaggaaggatgttaacatggttctgcagagctccctaggaaatgacctaagggttgacggagccagcattaagtttgatagcatttgcctttacgccaccttcttccccatggcccacaacaccgcctccacgcttgaggccatgcttagaaacgacaccaacgaccagtcctttaacgactatctctccgccgccaacatgctctaccctatacccgccaacgctaccaacgtgcccatatccatcccctcccgcaactgggcggctttccgcggctgggccttcacgcgccttaagactaaggaaaccccatcactgggctcgggctacgacccttattacacctactctggctctataccctacctagatggaaccttttacctcaaccacacctttaagaaggtggccattacctttgactcttctgtcagctggcctggcaatgaccgcctgcttacccccaacgagtttgaaattaagcgctcagttgacggggagggttacaacgttgcccagtgtaacatgaccaaagactggttcctggtacaaatgctagctaactataacattggctaccagggcttctatatcccagagagctacaaggaccgcatgtactccttctttagaaacttccagcccatgagccgtcaggtggtggatgatactaaatacaaggactaccaacaggtgggcatcctacaccaacacaacaactctggatttgttggctaccttgcccccaccatgcgcgaaggacaggcctaccctgctaacttcccctatccgcttataggcaagaccgcagttgacagcattacccagaaaaagtttctttgcgatcgcaccctttggcgcatcccattctccagtaactttatgtccatgggcgcactcacagacctgggccaaaaccttctctacgccaactccgcccacgcgctagacatgacttttgaggtggatcccatggacgagcccacccttctttatgttttgtttgaagtctttgacgtggtccgtgtgcaccagccgcaccgcggcgtcatcgaaaccgtgtacctgcgcacgcccttctcggccggcaacgccacaacataaagaagcaagcaacatcaacaacagctgccgccatgggctccagtgagcaggaactgaaagccattgtcaaagatcttggttgtgggccatattttttgggcacctatgacaagcgctttccaggctttgtttctccacacaagctcgcctgcgccatagtcaatacggccggtcgcgagactgggggcgtacactggatggcctttgcctggaacccgcactcaaaaacatgctacctctttgagccctttggcttttctgaccagcgactcaagcaggtttaccagtttgagtacgagtcactcctgcgccgtagcgccattgcttcttcccccgaccgctgtataacgctggaaaagtccacccaaagcgtacaggggcccaactcggccgcctgtggactattctgctgcatgtttctccacgcctttgccaactggccccaaactcccatggatcacaaccccaccatgaaccttattaccggggtacccaactccatgctcaacagtccccaggtacagcccaccctgcgtcgcaaccaggaacagctctacagcttcctggagcgccactcgccctacttccgcagccacagtgcgcagattaggagcgccacttctttttgtcacttgaaaaacatgtaaaaataatgtactagagacactttcaataaaggcaaatgcttttatttgtacactctcgggtgattatttacccccacccttgccgtctgcgccgtttaaaaatcaaaggggttctgccgcgcatcgctatgcgccactggcagggacacgttgcgatactggtgtttagtgctccacttaaactcaggcacaaccatccgcggcagctcggtgaagttttcactccacaggctgcgcaccatcaccaacgcgtttagcaggtcgggcgccgatatcttgaagtcgcagttggggcctccgccctgcgcgcgcgagttgcgatacacagggttgcagcactggaacactatcagcgccgggtggtgcacgctggccagcacgctcttgtcggagatcagatccgcgtccaggtcctccgcgttgctcagggcgaacggagtcaactttggtagctgccttcccaaaaagggcgcgtgcccaggctttgagttgcactcgcaccgtagtggcatcaaaaggtgaccgtgcccggtctgggcgttaggatacagcgcctgcataaaagccttgatctgcttaaaagccacctgagcctttgcgccttcagagaagaacatgccgcaagacttgccggaaaactgattggccggacaggccgcgtcgtgcacgcagcaccttgcgtcggtgttggagatctgcaccacatttcggccccaccggttcttcacgatcttggccttgctagactgctccttcagcgcgcgctgcccgttttcgctcgtcacatccatttcaatcacgtgctccttatttatcataatgcttccgtgtagacacttaagctcgccttcgatctcagcgcagcggtgcagccacaacgcgcagcccgtgggctcgtgatgcttgtaggtcacctctgcaaacgactgcaggtacgcctgcaggaatcgccccatcatcgtcacaaaggtcttgttgctggtgaaggtcagctgcaacccgcggtgctcctcgttcagccaggtcttgcatacggccgccagagcttccacttggtcaggcagtagtttgaagttcgcctttagatcgttatccacgtggtacttgtccatcagcgcgcgcgcagcctccatgcccttctcccacgcagacacgatcggcacactcagcgggttcatcaccgtaatttcactttccgcttcgctgggctcttcctcttcctcttgcgtccgcataccacgcgccactgggtcgtcttcattcagccgccgcactgtgcgcttacctcctttgccatgcttgattagcaccggtgggttgctgaaacccaccatttgtagcgccacatcttctctttcttcctcgctgtccacgattacctctggtgatggcgggcgctcgggcttgggagaagggcgcttctttttcttcttgggcgcaatggccaaatccgccgccgaggtcgatggccgcgggctgggtgtgcgcggcaccagcgcgtcttgtgatgagtcttcctcgtcctcggactcgatacgccgcctcatccgcttttttgggggcgcccggggaggcggcggcgacggggacggggacgacacgtcctccatggttgggggacgtcgcgccgcaccgcgtccgcgctcgggggtggtttcgcgctgctcctcttcccgactggccatttccttctcctataggcagaaaaagatcatggagtcagtcgagaagaaggacagcctaaccgccccctctgagttcgccaccaccgcctccaccgatgccgccaacgcgcctaccaccttccccgtcgaggcacccccgcttgaggaggaggaagtgattatcgagcaggacccaggttttgtaagcgaagacgacgaggaccgctcagtaccaacagaggataaaaagcaagaccaggacaacgcagaggcaaacgaggaacaagtcgggcggggggacgaaaggcatggcgactacctagatgtgggagacgacgtgctgttgaagcatctgcagcgccagtgcgccattatctgcgacgcgttgcaagagcgcagcgatgtgcccctcgccatagcggatgtcagccttgcctacgaacgccacctattctcaccgcgcgtaccccccaaacgccaagaaaacggcacatgcgagcccaacccgcgcctcaacttctaccccgtatttgccgtgccagaggtgcttgccacctatcacatctttttccaaaactgcaagatacccctatcctgccgtgccaaccgcagccgagcggacaagcagctggccttgcggcagggcgctgtcatacctgatatcgcctcgctcaacgaagtgccaaaaatctttgagggtcttggacgcgacgagaagcgcgcggcaaacgctctgcaacaggaaaacagcgaaaatgaaagtcactctggagtgttggtggaactcgagggtgacaacgcgcgcctagccgtactaaaacgcagcatcgaggtcacccactttgcctacccggcacttaacctaccccccaaggtcatgagcacagtcatgagtgagctgatcgtgcgccgtgcgcagcccctggagagggatgcaaatttgcaagaacaaacagaggagggcctacccgcagttggcgacgagcagctagcgcgctggcttcaaacgcgcgagcctgccgacttggaggagcgacgcaaactaatgatggccgcagtgctcgttaccgtggagcttgagtgcatgcagcggttctttgctgacccggagatgcagcgcaagctagaggaaacattgcactacacctttcgacagggctacgtacgccaggcctgcaagatctccaacgtggagctctgcaacctggtctcctaccttggaattttgcacgaaaaccgccttgggcaaaacgtgcttcattccacgctcaagggcgaggcgcgccgcgactacgtccgcgactgcgtttacttatttctatgctacacctggcagacggccatgggcgtttggcagcagtgcttggaggagtgcaacctcaaggagctgcagaaactgctaaagcaaaacttgaaggacctatggacggccttcaacgagcgctccgtggccgcgcacctggcggacatcattttccccgaacgcctgcttaaaaccctgcaacagggtctgccagacttcaccagtcaaagcatgttgcagaactttaggaactttatcctagagcgctcaggaatcttgcccgccacctgctgtgcacttcctagcgactttgtgcccattaagtaccgcgaatgccctccgccgctttggggccactgctaccttctgcagctagccaactaccttgcctaccactctgacataatggaagacgtgagcggtgacggtctactggagtgtcactgtcgctgcaacctatgcaccccgcaccgctccctggtttgcaattcgcagctgcttaacgaaagtcaaattatcggtacctttgagctgcagggtccctcgcctgacgaaaagtccgcggctccggggttgaaactcactccggggctgtggacgtcggcttaccttcgcaaatttgtacctgaggactaccacgcccacgagattaggttctacgaagaccaatcccgcccgcctaatgcggagcttaccgcctgcgtcattacccagggccacattcttggccaattgcaagccatcaacaaagcccgccaagagtttctgctacgaaagggacggggggtttacttggacccccagtccggcgaggagctcaacccaatccccccgccgccgcagccctatcagcagcagccgcgggcccttgcttcccaggatggcacccaaaaagaagctgcagctgccgccgccacccacggacgaggaggaatactgggacagtcaggcagaggaggttttggacgaggaggaggaggacatgatggaagactgggagagcctagacgaggaagcttccgaggtcgaagaggtgtcagacgaaacaccgtcaccctcggtcgcattcccctcgccggcgccccagaaatcggcaaccggttccagcatggctacaacctccgctcctcaggcgccgccggcactgcccgttcgccgacccaaccgtagatgggacaccactggaaccagggccggtaagtccaagcagccgccgccgttagcccaagagcaacaacagcgccaaggctaccgctcatggcgcgggcacaagaacgccatagttgcttgcttgcaagactgtgggggcaacatctccttcgcccgccgctttcttctctaccatcacggcgtggccttcccccgtaacatcctgcattactaccgtcatctctacagcccatactgcaccggcggcagcggcagcaacagcagcggccacacagaagcaaaggcgaccggatagcaagactctgacaaagcccaagaaatccacagcggcggcagcagcaggaggaggagcgctgcgtctggcgcccaacgaacccgtatcgacccgcgagcttagaaacaggatttttcccactctgtatgctatatttcaacagagcaggggccaagaacaagagctgaaaataaaaaacaggtctctgcgatccctcacccgcagctgcctgtatcacaaaagcgaagatcagcttcggcgcacgctggaagacgcggaggctctcttcagtaaatactgcgcgctgactcttaaggactagtttcgcgccctttctcaaatttaagcgcgaaaactacgtcatctccagcggccacacccggcgccagcacctgttgtcagcgccattatgagcaaggaaattcccacgccctacatgtggagttaccagccacaaatgggacttgcggctggagctgcccaagactactcaacccgaataaactacatgagcgcgggaccccacatgatatcccgggtcaacggaatacgcgcccaccgaaaccgaattctcctggaacaggcggctattaccaccacacctcgtaataaccttaatccccgtagttggcccgctgccctggtgtaccaggaaagtcccgctcccaccactgtggtacttcccagagacgcccaggccgaagttcagatgactaactcaggggcgcagcttgcgggcggctttcgtcacagggtgcggtcgcccgggcagggtataactcacctgacaatcagagggcgaggtattcagctcaacgacgagtcggtgagctcctcgcttggtctccgtccggacgggacatttcagatcggcggcgccggccgctcttcattcacgcctcgtcaggcaatcctaactctgcagacctcgtcctctgagccgcgctctggaggcattggaactctgcaatttattgaggagtttgtgccatcggtctactttaaccccttctcgggacctcccggccactatccggatcaatttattcctaactttgacgcggtaaaggactcggcggacggctacgactgaatgttaagtggagaggcagagcaactgcgcctgaaacacctggtccactgtcgccgccacaagtgctttgcccgcgactccggtgagttttgctactttgaattgcccgaggatcatatcgagggcccggcgcacggcgtccggcttaccgcccagggagagcttgcccgtagcctgattcgggagtttacccagcgccccctgctagttgagcgggacaggggaccctgtgttctcactgtgatttgcaactgtcctaaccctggattacatcaagatcctctagttaatgtcaggtcgcctaagtcgattaactagagtacccggggatcttattccctttaactaataaaaaaaaataataaagcatcacttacttaaaatcagttagcaaatttctgtccagtttattcagcagcacctccttgccctcctcccagctctggtattgcagcttcctcctggctgcaaactttctccacaatctaaatggaatgtcagtttcctcctgttcctgtccatccgcacccactatcttcatgttgttgcagatgaagcgcgcaagaccgtctgaagataccttcaaccccgtgtatccatatgacacggaaaccggtcctccaactgtgccttttcttactcctccctttgtatcccccaatgggtttcaagagagtccccctggggtactctctttgcgcctatccgaacctctagttacctccaatggcatgcttgcgctcaaaatgggcaacggcctctctctggacgaggccggcaaccttacctcccaaaatgtaaccactgtgagcccacctctcaaaaaaaccaagtcaaacataaacctggaaatatctgcacccctcacagttacctcagaagccctaactgtggctgccgccgcacctctaatggtcgcgggcaacacactcaccatgcaatcacaggccccgctaaccgtgcacgactccaaacttagcattgccacccaaggacccctcacagtgtcagaaggaaagctagccctgcaaacatcaggccccctcaccaccaccgatagcagtacccttactatcactgcctcaccccctctaactactgccactggtagcttgggcattgacttgaaagagcccatttatacacaaaatggaaaactaggactaaagtacggggctcctttgcatgtaacagacgacctaaacactttgaccgtagcaactggtccaggtgtgactattaataatacttccttgcaaactaaagttactggagccttgggttttgattcacaaggcaatatgcaacttaatgtagcaggaggactaaggattgattctcaaaacagacgccttatacttgatgttagttatccgtttgatgctcaaaaccaactaaatctaagactaggacagggccctctttttataaactcagcccacaacttggatattaactacaacaaaggcctttacttgtttacagcttcaaacaattccaaaaagcttgaggttaacctaagcactgccaaggggttgatgtttgacgctacagccatagccattaatgcaggagatgggcttgaatttggttcacctaatgcaccaaacacaaatcccctcaaaacaaaaattggccatggcctagaatttgattcaaacaaggctatggttcctaaactaggaactggccttagttttgacagcacaggtgccattacagtaggaaacaaaaataatgataagctaactttgtggaccacaccagctccatctcctaactgtagactaaatgcagagaaagatgctaaactcactttggtcttaacaaaatgtggcagtcaaatacttgctacagtttcagttttggctgttaaaggcagtttggctccaatatctggaacagttcaaagtgctcatcttattataagatttgacgaaaatggagtgctactaaacaattccttcctggacccagaatattggaactttagaaatggagatcttactgaaggcacagcctatacaaacgctgttggatttatgcctaacctatcagcttatccaaaatctcacggtaaaactgccaaaagtaacattgtcagtcaagtttacttaaacggagacaaaactaaacctgtaacactaaccattacactaaacggtacacaggaaacaggagacacaactccaagtgcatactctatgtcattttcatgggactggtctggccacaactacattaatgaaatatttgccacatcctcttacactttttcatacattgcccaagaataaagaatcgtttgtgttatgtttcaacgtgtttatttttcaattgcagaaaatttcaagtcatttttcattcagtagtatagccccaccaccacatagcttatacagatcaccgtaccttaatcaaactcacagaaccctagtattcaacctgccacctccctcccaacacacagagtacacagtcctttctccccggctggccttaaaaagcatcatatcatgggtaacagacatattcttaggtgttatattccacacggtttcctgtcgagccaaacgctcatcagtgatattaataaactccccgggcagctcacttaagttcatgtcgctgtccagctgctgagccacaggctgctgtccaacttgcggttgcttaacgggcggcgaaggagaagtccacgcctacatgggggtagagtcataatcgtgcatcaggatagggcggtggtgctgcagcagcgcgcgaataaactgctgccgccgccgctccgtcctgcaggaatacaacatggcagtggtctcctcagcgatgattcgcaccgcccgcagcataaggcgccttgtcctccgggcacagcagcgcaccctgatctcacttaaatcagcacagtaactgcagcacagcaccacaatattgttcaaaatcccacagtgcaaggcgctgtatccaaagctcatggcggggaccacagaacccacgtggccatcataccacaagcgcaggtagattaagtggcgacccctcataaacacgctggacataaacattacctcttttggcatgttgtaattcaccacctcccggtaccatataaacctctgattaaacatggcgccatccaccaccatcctaaaccagctggccaaaacctgcccgccggctatacactgcagggaaccgggactggaacaatgacagtggagagcccaggactcgtaaccatggatcatcatgctcgtcatgatatcaatgttggcacaacacaggcacacgtgcatacacttcctcaggattacaagctcctcccgcgttagaaccatatcccagggaacaacccattcctgaatcagcgtaaatcccacactgcagggaagacctcgcacgtaactcacgttgtgcattgtcaaagtgttacattcgggcagcagcggatgatcctccagtatggtagcgcgggtttctgtctcaaaaggaggtagacgatccctactgtacggagtgcgccgagacaaccgagatcgtgttggtcgtagtgtcatgccaaatggaacgccggacgtagtcatatttcctgaagcaaaaccaggtgcgggcgtgacaaacagatctgcgtctccggtctcgccgcttagatcgctctgtgtagtagttgtagtatatccactctctcaaagcatccaggcgccccctggcttcgggttctatgtaaactccttcatgcgccgctgccctgataacatccaccaccgcagaataagccacacccagccaacctacacattcgttctgcgagtcacacacgggaggagcgggaagagctggaagaaccatgtttttttttttattccaaaagattatccaaaacctcaaaatgaagatctattaagtgaacgcgctcccctccggtggcgtggtcaaactctacagccaaagaacagataatggcatttgtaagatgttgcacaatggcttccaaaaggcaaacggccctcacgtccaagtggacgtaaaggctaaacccttcagggtgaatctcctctataaacattccagcaccttcaaccatgcccaaataattctcatctcgccaccttctcaatatatctctaagcaaatcccgaatattaagtccggccattgtaaaaatctgctccagagcgccctccaccttcagcctcaagcagcgaatcatgattgcaaaaattcaggttcctcacagacctgtataagattcaaaagcggaacattaacaaaaataccgcgatcccgtaggtcccttcgcagggccagctgaacataatcgtgcaggtctgcacggaccagcgcggccacttccccgccaggaaccatgacaaaagaacccacactgattatgacacgcatactcggagctatgctaaccagcgtagccccgatgtaagcttgttgcatgggcggcgatataaaatgcaaggtgctgctcaaaaaatcaggcaaagcctcgcgcaaaaaagaaagcacatcgtagtcatgctcatgcagataaaggcaggtaagctccggaaccaccacagaaaaagacaccatttttctctcaaacatgtctgcgggtttctgcataaacacaaaataaaataacaaaaaaacatttaaacattagaagcctgtcttacaacaggaaaaacaacccttataagcataagacggactacggccatgccggcgtgaccgtaaaaaaactggtcaccgtgattaaaaagcaccaccgacagctcctcggtcatgtccggagtcataatgtaagactcggtaaacacatcaggttgattcacatcggtcagtgctaaaaagcgaccgaaatagcccgggggaatacatacccgcaggcgtagagacaacattacagcccccataggaggtataacaaaattaataggagagaaaaacacataaacacctgaaaaaccctcctgcctaggcaaaatagcaccctcccgctccagaacaacatacagcgcttccacagcggcagccataacagtcagccttaccagtaaaaaagaaaacctattaaaaaaacaccactcgacacggcaccagctcaatcagtcacagtgtaaaaaagggccaagtgcagagcgagtatatataggactaaaaaatgacgtaacggttaaagtccacaaaaaacacccagaaaaccgcacgcgaacctacgcccagaaacgaaagccaaaaaacccacaacttcctcaaatcgtcacttccgttttcccacgttacgtcacttcccattttaagaaaactacaattcccaacacatacaagttactccgccctaaaacctacgtcacccgccccgttcccacgccccgcgccacgtcacaaactccaccccctcattatcatattggcttcaatccaaaataaggta

SEQ ID NO: 231 - DNA, 9701 bp, synthetic construct
  misc_feature 1..9701: note = vector for IgG1 against T27Y H34A H345A ACE2 mutant
  misc_feature 2929..2930: note = n is a, c, g, or t
  misc_feature 2934: note = n is a, c, g, or t
  source 1..9701: mol_type = other DNA
ggcgtaatctgctgcttgcaaacaaaaaaaccaccgctaccagcggtggtttgtttgccggatcaagagctaccaactctttttccgaaggtaactggcttcagcagagcgcagataccaaatactgtccttctagtgtagccgtagttaggccaccacttcaagaactctgtagcaccgcctacatacctcgctctgctgaagccagttaccagtggctgctgccagtggcgataagtcgtgtcttaccgggttggactcaagagatagttaccggataaggcgcagcggtcgggctgaacggggggttcgtgcacacagcccagcttggagcgaacgacctacaccgaactgagatacctacagcgtgagctatgagaaagcgccacgcttcccgaagggagaaaggcggacaggtatccggtaagcggcagggtcggaacaggagagcgcacgagggagcttccagggggaaacgcctggtatctttatagtcctgtcgggtttcgccacctctgacttgagcgtcgatttttgtgatgctcgtcaggggggcggagcctatggaaaaacgccagcaacgcaagctagagtttaaacttgacagatgagacaataaccctgataaatgcttcaataatattgaaaaaggaaaagtatgagtattcaacatttccgtgtcgcccttattcccttttttgcggcattttgccttcctgtttttgctcacccagaaacgctggtgaaagtaaaagatgcagaagatcacttgggtgcgcgagtgggttacatcgaactggatctcaacagcggtaagatccttgagagttttcgccccgaagaacgtttcccaatgatgagcacttttaaagttctgctatgtggcgcggtattatcccgtattgatgccgggcaagagcaactcggtcgccgcatacactattctcagaatgacttggttgaatactcaccagtcacagaaaagcatcttacggatggcatgacagtaagagaattatgcagtgctgccataaccatgagtgataacactgcggccaacttacttctgacaactatcggaggaccgaaggagctaaccgcttttttgcacaacatgggggatcatgtaactcgccttgatcgttgggaaccggagctgaatgaagccataccaaacgacgagcgtgacaccacgatgcctgtagcaatggcaacaacgttgcgaaaactattaactggcgaactacttactctagcttcccggcaacaactaatagactggatggaggcggataaagttgcaggaccacttctgcgctcggcacttccggctggctggtttattgctgataaatcaggagccggtgagcgtgggtcacgcggtatcattgcagcactggggccggatggtaagccctcccgtatcgtagttatctacactacggggagtcaggcaactatggatgaacgaaatagacagatcgctgagataggtgcctcactgattaagcattggtaaggataaatttctggtaaggaggacacgtatggaagtgggcaagttggggaagccgtatccgttgctgaatctggcatatgtgggagtataagacgcgcagcgtcgcatcaggcatttttttctgcgccaatgcaaaaaggccatccgtcaggatggcctttcggcataactagggccgccgatatttgaaaatatggcatattgaaaatgtcgccgatgtgagtttctgtgtaactgatatcgccatttttccaaaagtgatttttgggcatacgcgatatctggcgatagcgcttatatcgtttacgggggatggcgatagacgactttggtgacttgggcgattctgtgtgtcgcaaatatcgcagtttcgatataggtgacagacgatatgaggctatatcgccgatagaggcgacatcaagctggcacatggccaatgcatatcgatctatacattgaatcaatattggccattagccatattattcattggttatatagcataaatcaatattggctattggccattgcatacgttgtatccatatcataatatgtacatttatattggctcatgtccaacattaccgccatgttgacattgattattgactagttattaatagtaatcaattacggggtcattagttcatagcccatatatggagttccgcgttacataacttacggtaaatggcccgcctggctgaccgcccaacgacccccgcccattgacgtcaataatgacgtatgttcccatagtaacgccaatagggactttccattgacgtcaatgggtggagtatttacggtaaactgcccacttggcagtacatcaagtgtatcatatgccaagtacgccccctattgacgtcaatgacggtaaatggcccgcctggcattatgcccagtacatgaccttatgggactttcctacttggcagtacatctacgtattagtcatcgctattaccatggtgatgcggttttggcagtacatcaatgggcgtggatagcggtttgactcacggggatttccaagtctccaccccattgacgtcaatgggagtttgttttggcaccaaaatcaacgggactttccaaaatgtcgtaacaactccgccccattgacgcaaatgggcggtaggcgtgtacggtgggaggtctatataagcagagctcgtttagtgaaccgtcagatcgcctggagacgccatccacgctgttttgacctccatagaagacaccgggaccgatccagcctccgcggccgggaacggtgcattggaacgcggattccccgtgccaagagtgacgtaagtaccgcctatagagtctataggcccacccccttggcttcttatgcatgctatactgtttttggcttggggtctatacaccccccgnnttcntcatgttataggtgatggtatagcttagcctataggtgtgggttattgaccattattgaccactccccctattggtgacgatactttccattactaatccataacatggctctttgccacaactctctttattggctatatgccaatacactgtccttcagagactgacacggactctgtatttttacaggatggggtctcatttattatttacaaattcacatatacaacaccaccgtccccagtgcccgcagtttttattaaacataacgtgggatctccacgcgaatctcgggtacgtgttccggacatgggctcttctccggtagcggcggagcttctacatccgagccctgctcccatgcctccagcgactcatggtcgctcggcagctccttgctcctaacagtggaggccagacttaggcacagcacgatgcccaccaccaccagtgtgccgcacaaggccgtggcggtagggtatgtgtctgaaaatgagctcggggagcgggcttgcaccgctgacgcatttggaagacttaaggcagcggcagaagaagatgcaggcagctgagttgttgtgttctgataagagtcagaggtaactcccgttgcggtgctgttaacggtggagggcagtgtagtctgagcagtactcgttgctgccgcgcgcgccaccagacataatagctgacagactaacagactgttcctttccatgggtcttttctgcagtcaccgtccttgacacgaagctgctagcgccaccatgagcagcagtagttggcttctcttgagtttggtggcagtgacagcagcccagagtactatcgaggagcaggctaaatactttctggataagtttaacgccgaggccgaagacttgttctatcaatcttctctcgcttcatggaattacaatactaacatcactgaggagaacgtccagaatatgaacaatgctggcgacaaatggagcgccttcttgaaggagcagtctacccttgcacaaatgtatccactgcaggagatacagaaccttacagtaaagttgcagctccaggctctccagcagaacggatctagcgtgctttcagaggataaaagcaaaaggctgaacaccatacttaataccatgtccacaatttactctactggtaaagtatgtaaccccgacaaccctcaagaatgcctccttcttgagccaggcctcaatgagatcatggctaatagtctggactataatgaaagactgtgggcatgggagtcctggagatctgaagtagggaagcaactgaggcccctttatgaagagtacgtcgtacttaagaatgaaatggcccgcgctaaccactacgaggattacggcgattactggcgtggggactatgaagtaaatggtgtagatggatacgactatagtcgtgggcaattgattgaggatgtggagcacacttttgaggagataaaaccactctatgagcatcttcacgcatatgtgagagctaaactgatgaacgcctacccaagttacatcagtccaatcggatgtctcccagctcacctccttggcgacatgtggggacgtttctggaccaatctgtattccctcacagtccctttcgggcaaaagcctaatatagacgtgacagacgcaatggttgatcaggcttgggatgctcaaaggatttttaaggaagctgagaagttttttgtgtcagtcggtttgccaaatatgacacaaggcttctgggaaaatagcatgttgactgatcccggtaatgttcaaaaggctgtgtgtgcccctaccgcttgggaccttgggaaaggtgactttcgaatcttgatgtgtaccaaggtgacaatggatgactttcttacagcccatcatgaaatgggtcacatccagtatgatatggcttatgcagctcaacctttcctcttgagaaatggtgcaaatgaaggttttcatgaagctgtaggggaaataatgtccctgagtgctgcaaccccaaagcatctcaagagtatcggattgttgagcccagattttcaagaagataacgagaccgaaatcaacttccttctgaaacaagccctcacaatagttggtactcttccattcacatacatgctggagaaatggcgttggatggtttttaagggggagatacctaaagatcagtggatgaaaaagtggtgggagatgaagcgtgagatcgtaggggtcgtggagccagtgcctcatgatgagacttactgtgacccagcatcactcttccacgttagcaatgactattcatttatacgttattacactcgcactctttaccagtttcaatttcaggaggctctgtgtcaggctgccaagcatgagggaccccttcacaagtgtgatattagtaacagtactgaggcaggccaaaaactgttcaatatgttgaggcttggcaaaagcgagccatggactctcgccttggaaaatgttgtcggggctaaaaacatgaatgtacgccctctgcttaactattttgagcccctttttacatggctcaaggaccagaataagaactcctttgtcggctggtcaacagactggtctccctatgcagacaaaacacatacttgcccaccttgtcctgcaccagagctgctgggaggtccaagcgtgttcctgtttccacccaagcccaaagacacactgatgatttctcgaactccagaagtgacctgcgtggtcgtggacgtgagccacgaggatcccgaagtgaagttcaactggtacgtggatggcgtggaggtccataatgctaagactaaaccccgggaggaacagtacaacagcacttatagggtcgtgtccgtgctgaccgtcctgcatcaggattggctgaacgggaaggaatataagtgcaaagtgtctaataaggcactgcccgcccctatcgagaaaacaattagcaaggctaagggtcagcctagagaaccacaggtgtacactctgcctccaagtcgcgacgagctgaccaagaaccaggtgtcactgacatgtctggtcaaaggcttttatccctcagatatcgcagtggagtgggaaagcaatggacagcctgagaacaattacaagaccacaccccctgtgctggacagtgatggctcattctttctgtattctaagctgacagtggacaaaagtaggtggcagcagggaaacgtgttctcctgctctgtcatgcacgaagcactgcacaatcattatacccagaagagtctgtcactgagccctggcaaatgagcgataccgattctagaactagatcataatcagccataccacatttgtagaggttttacttgctttaaaaaacctcccacacctccccctgaacctgaaacataaaatgaatgcaattgttgttgttaacttgtttattgcagcttataatggttacaaataaagcaatagcatcacaaatttcacaaataaagcatttttttcactgcattctagttgtggtttgtccaaactcatcaatgtatcttaaggccgcaggtaagccagcccaggcctcgccctccagctcaaggcgggacaggtgccctagagtagcctgcatccagggacaggccccagccgggtgctgacacgtccacctccatctcttcctcaggtctgcccgggtggcatccctgtgacccctccccagtgcctctcctggtcgtggaaggtgctactccagtgcccaccagccttgtcctaataaaattaagttgcatcattttgtttgactaggtgtccttgtataatattatggggtggaggcgggtggtatggagcaaggggcccaagttaacttgtttattgcagcttataatggttacaaataaagcaatagcatcacaaatttcacaaataaagcatttttttcactgcattctagttgtggtttgtccaaactcatcaatgtatcttatcatgtctggatccgcttcaggcaccgggcttgcgggtcatgcaccaggtgcgcggtccttcgggcacctcgacgtcggcggtgacggtgaagccgagccgctcgtagaaggggaggttgcggggcgcggaggtctccaggaaggcgggcaccccggcgcgctcggccgcctccactccggggagcacgacggcgctgcccagacccttgccctggtggtcgggcgagacgccgacggtggccaggaaccacgcgggctccttgggccggtgcggcgccaggaggccttccatctgttgctgcgcggccagcctggaaccgctcaactcggccatgcgcgggccgatctcggcgaacaccgcccccgcttcgacgctctccggcgtggtccagaccgccaccgcggcgccgtcgtccgcgacccacaccttgccgatgtcgagcccgacgcgcgtgaggaagagttcttgcagctcggtgacccgctcgatgtggcggtccgggtcgacggtgtggcgcgtggcggggtagtcggcgaacgcggcggcgagggtgcgtacggcccgggggacgtcgtcgcgggtggcgaggcgcaccgtgggcttgtactcggtcatggtggcctgcagagtcgctctgtgttcgaggccacacgcgtcaccttaatatgcgaagtggacctgggaccgcgccgccccgactgcatctgcgtgttttcgccaatgacaagacgctgggcggggtttgtgtcatcatagaactaaagacatgcaaatatatttcttccggggacaccgccagcaaacgcgagcaacgggccacggggatgaagcagctgcgccactccctgaagatccatcgtctcctaacaagttacatcactcctgcccttcctcaccctcatctccatcacctccttcatctccgtcatctccgtcatcaccctccgcggcagccccttccaccataggtggaaaccagggaggcaaatctactccatcgtcaaagctgcacacagtcaccctgatattgcaggtaggagcgggctttgtcataacaaggtccttaatcgcatccttcaaaacctcagcaaatatatgagtttgtaaaaagaccatgaaataacagacaatggactcccttagcgggccaggttgtgggccgggtccaggggccattccaaaggggagacgactcaatggtgtaagacgacattgtggaatagcaagggcagttcctcgccttaggttgtaaagggaggtcttactacctccatatacgaacacaccggcgacccaagttccttcgtcggtagtcctttctacgtgactcctagccaggagagctcttaaaccttctgcaatgttctcaaatttcgggttggaacctccttgaccacgatgctttccaaaccaccctccttttttgcgcctgcctccatcaccctgacccccgctgcgcgggggcacgtcaggctcaccatctgggccgccttcttggtggtattcaaaataatcggcttcccctacagggtggaaaaatggccttctacctggagggggcctgcgcggtggagacccggatgatgatgactgactactgggactcctgggcctcttttctccacgtccacgacctctccccctggctctttcacgacttccccccctggctctttcacgtcctctaccccggcggcctccactacctcctcgaccccggcctccactacctcctcgaccccggcctccactgcctcctcgaccccggcctccacctcctgctcctgcccctcccgctcctgctcctgctcctgttccaccgtgggtccctttgcagccaatgcaacttggacgtttttggggtctccggacaccatctctatgtcttggccctgatcctgagccgcccggggctcctggtcttccgcctcctcgtcctcgtcctcttccccgtcctcgtccatgtgccatgatggcggcctgcagctgtgttcgaggccgcgcgtgtcaccttaatatgcgaagtggacctgggaccgcgccgccccgactgcatctgcgtgttcgagttcgccaatgacaagacgctgggcggggagatcccccttattaaccctaaacgggtagcatatgcttcccgggtagtagtatatactatccagactaaccctaattcaatagcatatgttacccaacgggaagcatatgctatcgaattagggttagtaaaagggtcctaaggaacagcgatctggatagcatatgctatcctaatctatatctgggtagcatatgctatcctaatctatatctgggtagcataggctatcctaatctatatctgggtagcatatgctatcctaatctatatctgggtagtatatgctatcctaatttatatctgggtagcataggctatcctaatctatatctgggtagcatatgctatcctaatctatatctgggtagtatatgctatcctaatctgtatccgggtagcatatgctatcctcatgcatatacagtcagcatatgatacccagtagtagagtgggagtgctatcctttgcatatgccgccacctcccaaggagatctgtcgacatcgatgggcgcgggtgtacactccgcccatcccgcccctaactccgcccagttccgcccattctccgcctcatggctgactaattttttttatttatgcagaggccgaggccgcctcggcctctgagctattccagaagtagtgaggaggcttttttggaggcctaggcttttgcaaaaagctaattc

SEQ ID NO: 232 - DNA, 38496 bp, synthetic construct
  misc_feature 1..38496: note = vector for IgA against T27Y H34A R273Q ACE2 mutant
  source 1..38496: mol_type = other DNA
tattattgatgatgttaattaacatgcatggatcctacgtctcgaccgatgcccttgagagccttcaacccagtcagctccttccggtgggcgcggggcatgactatcgtcgccgcacttatgactgtcttctttatcatgcaactcgtaggacaggtgccggcagcgctctgggtcattttcggcgaggaccgctttcgctggagcgcgacgatgatcggcctgtcgcttgcggtattcggaatcttgcacgccctcgctcaagccttcgtcactggtcccgccaccaaacgtttcggcgagaagcaggccattatcgccggcatggcggccgacgcgctgggctacgtcttgctggcgttcgcgacgcgaggctggatggccttccccattatgattcttctcgcttccggcggcatcgggatgcccgcgttgcaggccatgctgtccaggcaggtagatgacgaccatcagggacagcttcaaggatcgctcgcggctcttaccagcctaacttcgatcattggaccgctgatcgtcacggcgatttatgccgcctcggcgagcacatggaacgggttggcatggattgtaggcgccgccctataccttgtctgcctccccgcgttgcgtcgcggtgcatggagccgggccacctcgacctgaatggaagccggcggcacctcgctaacggattcaccactccaagaattggagccaatcaattcttgcggagaactgtgaatgcgcaaaccaacccttggcagaacatatccatcgcgtccgccatctccagcagccgcacgcggcgcatctcgggcagcgttgggtcctggccacgggtgcgcatgatcgtgctcctgtcgttgaggacccggctaggctggcggggttgccttactggttagcagaatgaatcaccgatacgcgagcgaacgtgaagcgactgctgctgcaaaacgtctgcgacctgagcaacaacatgaatggtcttcggtttccgtgtttcgtaaagtctggaaacgcggaagtcagcgccctgcaccattatgttccggatctgcatcgcaggatgctgctggctaccctgtggaacacctacatctgtattaacgaagcgctggcattgaccctgagtgatttttctctggtcccgccgcatccataccgccagttgtttaccctcacaacgttccagtaaccgggcatgttcatcatcagtaacccgtatcgtgagcatcctctctcgtttcatcggtatcattacccccatgaacagaaatcccccttacacggaggcatcagtgaccaaacaggaaaaaaccgcccttaacatggcccgctttatcagaagccagacattaacgcttctggagaaactcaacgagctggacgcggatgaacaggcagacatctgtgaatcgcttcacgaccacgctgatgagctttaccgcagctgcctcgcgcgtttcggtgatgacggtgaaaacctctgacacatgcagctcccggagacggtcacagcttgtctgtaagcggatgccgggagcagacaagcccgtcagggcgcgtcagcgggtgttggcgggtgtcggggcgcagccatgacccagtcacgtagcgatagcggagtgtatactggcttaactatgcggcatcagagcagattgtactgagagtgcaccatatgcggtgtgaaataccgcacagatgcgtaaggagaaaataccgcatcaggcgctcttccgcttcctcgctcactgactcgctgcgctcggtcgttcggctgcggcgagcggtatcagctcactcaaaggcggtaatacggttatccacagaatcaggggataacgcaggaaagaacatgtgagcaaaaggccagcaaaaggccaggaaccgtaaaaaggccgcgttgctggcgtttttccataggctccgcccccctgacgagcatcacaaaaatcgacgctcaagtcagaggtggcgaaacccgacaggactataaagataccaggcgtttccccctggaagctccctcgtgcgctctcctgttccgaccctgccgcttaccggatacctgtccgcctttctcccttcgggaagcgtggcgctttctcatagctcacgctgtaggtatctcagttcggtgtaggtcgttcgctccaagctgggctgtgtgcacgaaccccccgttcagcccgaccgctgcgccttatccggtaactatcgtcttgagtccaacccggtaagacacgacttatcgccactggcagcagccactggtaacaggattagcagagcgaggtatgtaggcggtgctacagagttcttgaagtggtggcctaactacggctacactagaaggacagtatttggtatctgcgctctgctgaagccagttaccttcggaaaaagagttggtagctcttgatccggcaaacaaaccaccgctggtagcggtggtttttttgtttgcaagcagcagattacgcgcagaaaaaaaggatctcaagaagatcctttgatcttttctacggggtctgacgctcagtggaacgaaaactcacgttaagggattttggtcatgagattatcaaaaaggatcttcacctagatccttttaaattaaaaatgaagttttaaatcaatctaaagtatatatgagtaaacttggtctgacagttaccaatgcttaatcagtgaggcacctatctcagcgatctgtctatttcgttcatccatagttgcctgactccccgtcgtgtagataactacgatacgggagggcttaccatctggccccagtgctgcaatgataccgcgagacccacgctcaccggctccagatttatcagcaataaaccagccagccggaagggccgagcgcagaagtggtcctgcaactttatccgcctccatccagtctattaattgttgccgggaagctagagtaagtagttcgccagttaatagtttgcgcaacgttgttgccattgctgcagccatgagattatcaaaaaggatcttcacctagatccttttcacgtagaaagccagtccgcagaaacggtgctgaccccggatgaatgtcagctactgggctatctggacaagggaaaacgcaagcgcaaagagaaagcaggtagcttgcagtgggcttacatggcgatagctagactgggcggttttatggacagcaagcgaaccggaattgccagctggggcgccctctggtaaggttgggaagccctgcaaagtaaactggatggctttcttgccgccaaggatctgatggcgcaggggatcaagctctgatcaagagacaggatgaggatcgtttcgcatgattgaacaagatggattgcacgcaggttctccggccgcttgggtggagaggctattcggctatgactgggcacaacagacaatcggctgctctgatgccgccgtgttccggctgtcagcgcaggggcgcccggttctttttgtcaagaccgacctgtccggtgccctgaatgaactgcaagacgaggcagcgcggctatcgtggctggccacgacgggcgttccttgcgcagctgtgctcgacgttgtcactgaagcgggaagggactggctgctattgggcgaagtgccggggcaggatctcctgtcatctcaccttgctcctgccgagaaagtatccatcatggctgatgcaatgcggcggctgcatacgcttgatccggctacctgcccattcgaccaccaagcgaaacatcgcatcgagcgagcacgtactcggatggaagccggtcttgtcgatcaggatgatctggacgaagagcatcaggggctcgcgccagccgaactgttcgccaggctcaaggcgagcatgcccgacggcgaggatctcgtcgtgacccatggcgatgcctgcttgccgaatatcatggtggaaaatggccgcttttctggattcatcgactgtggccggctgggtgtggcggaccgctatcaggacatagcgttggctacccgtgatattgctgaagagcttggcggcgaatgggctgaccgcttcctcgtgctttacggtatcgccgctcccgattcgcagcgcatcgccttctatcgccttcttgacgagttcttctgaattttgttaaaatttttgttaaatcagctcattttttaaccaataggccgaaatcggcaaaatcccttataaatcaaaagaatagaccgagatagggttgagtgttgttccagtttggaacaagagtccactattaaagaacgtggactccaacgtcaaagggcgaaaaaccgtctatcagggcgatggcccactacgtgaaccatcaccctaatcaagttttttggggtcgaggtgccgtaaagcactaaatcggaaccctaaagggagcccccgatttagagcttgacggggaaagccggcgaacgtggcgagaaaggaagggaagaaagcgaaaggagcgggcgctagggcgctggcaagtgtagcggtcacgctgcgcgtaaccaccacacccgccgcgcttaatgcgccgctacagggcgcgtccattcgccattcaggatcgaattaattcttaattaacatcatcaataatataccttattttggattgaagccaatatgataatgagggggtggagtttgtgacgtggcgcggggcgtgggaacggggcgggtgacgtagtagtgtggcggaagtgtgatgttgcaagtgtggcggaacacatgtaagcgacggatgtggcaaaagtgacgtttttggtgtgcgccggtgtacacaggaagtgacaattttcgcgcggttttaggcggatgttgtagtaaatttgggcgtaaccgagtaagatttggccattttcgcgggaaaactgaataagaggaagtgaaatctgaataattttgtgttactcatagcgcgtaatactgtaatagtaatcaattacggggtcattagttcatagcccatatatggagttccgcgttacataacttacggtaaatggcccgcctggctgaccgcccaacgacccccgcccattgacgtcaataatgacgtatgttcccatagtaacgccaatagggactttccattgacgtcaatgggtggagtatttacggtaaactgcccacttggcagtacatcaagtgtatcatatgccaagtacgccccctattgacgtcaatgacggtaaatggcccgcctggcattatgcccagtacatgaccttatgggactttcctacttggcagtacatctacgtattagtcatcgctattaccatggtgatgcggttttggcagtacatcaatgggcgtggatagcggtttgactcacggggatttccaagtctccaccccattgacgtcaatgggagtttgttttggcaccaaaatcaacgggactttccaaaatgtcgtaacaactccgccccattgacgcaaatgggcggtaggcgtgtacggtgggaggtctatataagcagagctggtttagtgaaccgtcagatccgctagagatctggtaccgtcgacgcggccgctcgagcctaagcttatgagcagcagtagttggcttctcttgagtttggtggcagtgacagcagcccagagtactatcgaggagcaggctaaatactttctggataagtttaacgccgaggccgaagacttgttctatcaatcttctctcgcttcatggaattacaatactaacatcactgaggagaacgtccagaatatgaacaatgctggcgacaaatggagcgccttcttgaaggagcagtctacccttgcacaaatgtatccactgcaggagatacagaaccttacagtaaagttgcagctccaggctctccagcagaacggatctagcgtgctttcagaggataaaagcaaaaggctgaacaccatacttaataccatgtccacaatttactctactggtaaagtatgtaaccccgacaaccctcaagaatgcctccttcttgagccaggcctcaatgagatcatggctaatagtctggactataatgaaagactgtgggcatgggagtcctggagatctgaagtagggaagcaactgaggcccctttatgaagagtacgtcgtacttaagaatgaaatggcccgcgctaaccactacgaggattacggcgattactggcgtggggactatgaagtaaatggtgtagatggatacgactatagtcgtgggcaattgattgaggatgtggagcacacttttgaggagataaaaccactctatgagcatcttcacgcatatgtgagagctaaactgatgaacgcctacccaagttacatcagtccaatcggatgtctcccagctcacctccttggcgacatgtggggacagttctggaccaatctgtattccctcacagtccctttcgggcaaaagcctaatatagacgtgacagacgcaatggttgatcaggcttgggatgctcaaaggatttttaaggaagctgagaagttttttgtgtcagtcggtttgccaaatatgacacaaggcttctgggaaaatagcatgttgactgatcccggtaatgttcaaaaggctgtgtgtcaccctaccgcttgggaccttgggaaaggtgactttcgaatcttgatgtgtaccaaggtgacaatggatgactttcttacagcccatcatgaaatgggtcacatccagtatgatatggcttatgcagctcaacctttcctcttgagaaatggtgcaaatgaaggttttcatgaagctgtaggggaaataatgtccctgagtgctgcaaccccaaagcatctcaagagtatcggattgttgagcccagattttcaagaagataacgagaccgaaatcaacttccttctgaaacaagccctcacaatagttggtactcttccattcacatacatgctggagaaatggcgttggatggtttttaagggggagatacctaaagatcagtggatgaaaaagtggtgggagatgaagcgtgagatcgtaggggtcgtggagccagtgcctcatgatgagacttactgtgacccagcatcactcttccacgttagcaatgactattcatttatacgttattacactcgcactctttaccagtttcaatttcaggaggctctgtgtcaggctgccaagcatgagggaccccttcacaagtgtgatattagtaacagtactgaggcaggccaaaaactgttcaatatgttgaggcttggcaaaagcgagccatggactctcgccttggaaaatgttgtcggggctaaaaacatgaatgtacgccctctgcttaactattttgagcccctttttacatggctcaaggaccagaataagaactcctttgtcggctggtcaacagactggtctccctatgcagaccctagtactcctcctactccttctccatcaaccccaccaactccatcccctagctgctgtcacccaaggctgtctctgcaccgacctgcactcgaagaccttctgttgggctctgaagctaacctgacctgtactcttactggcttgcgcgatgctagcggcgtgactttcacctggacacctagtagcggtaaaagtgctgtacaaggacctcctgaacgcgacctgtgtggttgctactctgtgtcttctgtacttcccggctgtgccgagccctggaatcacgggaaaacctttacctgcaccgccgcttaccctgagtcaaaaactcccctcactgccacattgagtaagtcagggaatacattcaggccagaggttcatttgttgcctcctccatctgaagaacttgctttgaacgagctggtcactctgacctgcttggctaggggtttctcccccaaagatgtacttgtacggtggttgcagggcagccaagagttgccccgcgaaaagtatttgacctgggcctcaagacaagaacccagccaggggactaccacatttgccgtgaccagtattctgcgtgtagccgctgaagattggaagaaaggggatacattttcttgcatggtagggcatgaggcccttcccctcgctttcactcagaagacaatagacagactcgccggaaagcctactcacgtgaatgttagcgtagtcatggctgaggttgacggaacttgctactgagatatccgatccaccggatctagataactgatcataatcagccataccacatttgtagaggttttacttgctttaaaaaacctcccacacctccccctgaacctgaaacataaaatgaatgcaattgttgttgttaacttgtttattgcagcttataatggttacaaataaagcaatagcatcacaaatttcacaaataaagcatttttttcactgcattctagttgtggtttgtccaaactcatcaatgtatcttaggtttagtgaaccgtcagatccgctagcgttacataacttacggtaaatggcccgcctggctgaccgcccaacgacccccgcccattgacgtcaataatgacgtatgttcccatagtaacgccaatagggactttccattgacgtcaatgggtggagtatttacggtaaactgcccacttggcagtacatcaagtgtatcatatgccaagtacgccccctattgacgtcaatgacggtaaatggcccgcctggcattatgcccagtacatgaccttatgggactttcctacttggcagtacatctacgtattagtcatcgctattaccatggtgatgcggttttggcagtacatcaatgggcgtggatagcggtttgactcacggggatttccaagtctccaccccattgacgtcaatgggagtttgttttggcaccaaaatcaacgggactttccaaaatgtcgtaacaactccgccccattgacgcaaatgggcggtaggcgtgtacggtgggaggtctatataagcagagctggtttagtgaaccgtcagatccgctagagatctggtaccgtcgacgcggccgctcgagcctaagcttatgaagaaccatctgcttttctggggagtacttgccgttttcataaaagccgtacatgttaaagcacaagaggacgaacgcattgtgttggttgataataaatgcaaatgtgctcggataacatctcggatcattcgtagctcagaggaccccaatgaggatatagtagagcgaaacatcagaattatagtacccctgaacaacagagagaacataagtgatcccacaagtccattgcggacacgctttgtttaccatttgtctgatctgtgtaaaaaatgtgatccaacagaggtggaactcgacaatcagatcgtcaccgccacccagtctaacatctgcgatgaagattcagctacagagacatgctacacatacgaccggaacaagtgctatactgccgttgtgccactcgtttacggtggagaaacaaagatggttgaaactgcacttacaccagatgcctgctatccagattgagatatccgatccaccggatctagataactgatcataatcagccataccacatttgtagaggttttacttgctttaaaaaacctcccacacctccccctgaacctgaaacataaaatgaatgcaattgttgttgttaacttgtttattgcagcttataatggttacaaataaagcaatagcatcacaaatttcacaaataaagcatttttttcactgcattctagttgtggtttgtccaaactcatcaatgtatcttaacgcggatctgggcgtggttaagggtgggaaagaatatataaggtgggggtcttatgtagttttgtatctgttttgcagcagccgccgccgccatgagcaccaactcgtttgatggaagcattgtgagctcatatttgacaacgcgcatgcccccatgggccggggtgcgtcagaatgtgatgggctccagcattgatggtcgccccgtcctgcccgcaaactctactaccttgacctacgagaccgtgtctggaacgccgttggagactgcagcctccgccgccgcttcagccgctgcagccaccgcccgcgggattgtgactgactttgctttcctgagcccgcttgcaagcagtgcagcttcccgttcatccgcccgcgatgacaagttgacggctcttttggcacaattggattctttgacccgggaacttaatgtcgtttctcagcagctgttggatctgcgccagcaggtttctgccctgaaggcttcctcccctcccaatgcggtttaaaacataaataaaaaaccagactctgtttggatttggatcaagcaagtgtcttgctgtctttatttaggggttttgcgcgcgcggtaggcccgggaccagcggtctcggtcgttgagggtcctgtgtattttttccaggacgtggtaaaggtgactctggatgttcagatacatgggcataagcccgtctctggggtggaggtagcaccactgcagagcttcatgctgcggggtggtgttgtagatgatccagtcgtagcaggagcgctgggcgtggtgcctaaaaatgtctttcagtagcaagctgattgccaggggcaggcccttggtgtaagtgtttacaaagcggttaagctgggatgggtgcatacgtggggatatgagatgcatcttggactgtatttttaggttggctatgttcccagccatatccctccggggattcatgttgtgcagaaccaccagcacagtgtatccggtgcacttgggaaatttgtcatgtagcttagaaggaaatgcgtggaagaacttggagacgcccttgtgacctccaagattttccatgcattcgtccataatgatggcaatgggcccacgggcggcggcctgggcgaagatatttctgggatcactaacgtcatagttgtgttccaggatgagatcgtcataggccatttttacaaagcgcgggcggagggtgccagactgcggtataatggttccatccggcccaggggcgtagttaccctcacagatttgcatttcccacgctttgagttcagatggggggatcatgtctacctgcggggcgatgaagaaaacggtttccggggtaggggagatcagctgggaagaaagcaggttcctgagcagctgcgacttaccgcagccggtgggcccgtaaatcacacctattaccggctgcaactggtagttaagagagctgcagctgccgtcatccctgagcaggggggccacttcgttaagcatgtccctgactcgcatgttttccctgaccaaatccgccagaaggcgctcgccgcccagcgatagcagttcttgcaaggaagcaaagtttttcaacggtttgagaccgtccgccgtaggcatgcttttgagcgtttgaccaagcagttccaggcggtcccacagctcggtcacctgctctacggcatctcgatccagcatatctcctcgtttcgcgggttggggcggctttcgctgtacggcagtagtcggtgctcgtccagacgggccagggtcatgtctttccacgggcgcagggtcctcgtcagcgtagtctgggtcacggtgaaggggtgcgctccgggctgcgcgctggccagggtgcgcttgaggctggtcctgctggtgctgaagcgctgccggtcttcgccctgcgcgtcggccaggtagcatttgaccatggtgtcatagtccagcccctccgcggcgtggcccttggcgcgcagcttgcccttggaggaggcgccgcacgaggggcagtgcagacttttgagggcgtagagcttgggcgcgagaaataccgattccggggagtaggcatccgcgccgcaggccccgcagacggtctcgcattccacgagccaggtgagctctggccgttcggggtcaaaaaccaggtttcccccatgctttttgatgcgtttcttacctctggtttccatgagccggtgtccacgctcggtgacgaaaaggctgtccgtgtccccgtatacagacttgagaggcctgtcctcgagcggtgttccgcggtcctcctcgtatagaaactcggaccactctgagacaaaggctcgcgtccaggccagcacgaaggaggctaagtgggaggggtagcggtcgttgtccactagggggtccactcgctccagggtgtgaagacacatgtcgccctcttcggcatcaaggaaggtgattggtttgtaggtgtaggccacgtgaccgggtgttcctgaaggggggctataaaagggggtgggggcgcgttcgtcctcactctcttccgcatcgctgtctgcgagggccagctgttggggtgagtactccctctgaaaagcgggcatgacttctgcgctaagattgtcagtttccaaaaacgaggaggatttgatattcacctggcccgcggtgatgcctttgagggtggccgcatccatctggtcagaaaagacaatctttttgttgtcaagcttggtggcaaacgacccgtagagggcgttggacagcaacttggcgatggagcgcagggtttggtttttgtcgcgatcggcgcgctccttggccgcgatgtttagctgcacgtattcgcgcgcaacgcaccgccattcgggaaagacggtggtgcgctcgtcgggcaccaggtgcacgcgccaaccgcggttgtgcagggtgacaaggtcaacgctggtggctacctctccgcgtaggcgctcgttggtccagcagaggcggccgcccttgcgcgagcagaatggcggtagggggtctagctgcgtctcgtccggggggtctgcgtccacggtaaagaccccgggcagcaggcgcgcgtcgaagtagtctatcttgcatccttgcaagtctagcgcctgctgccatgcgcgggcggcaagcgcgcgctcgtatgggttgagtgggggaccccatggcatggggtgggtgagcgcggaggcgtacatgccgcaaatgtcgtaaacgtagaggggctctctgagtattccaagatatgtagggtagcatcttccaccgcggatgctggcgcgcacgtaatcgtatagttcgtgcgagggagcgaggaggtcgggaccgaggttgctacgggcgggctgctctgctcggaagactatctgcctgaagatggcatgtgagttggatgatatggttggacgctggaagacgttgaagctggcgtctgtgagacctaccgcgtcacgcacgaaggaggcgtaggagtcgcgcagcttgttgaccagctcggcggtgacctgcacgtctagggcgcagtagtccagggtttccttgatgatgtcatacttatcctgtcccttttttttccacagctcgcggttgaggacaaactcttcgcggtctttccagtactcttggatcggaaacccgtcggcctccgaacggtaagagcctagcatgtagaactggttgacggcctggtaggcgcagcatcccttttctacgggtagcgcgtatgcctgcgcggccttccggcatgaccagcatgaagggcacgagctgcttcccaaaggcccccatccaagtataggtctctacatcgtaggtgacaaagagacgctcggtgcgaggatgcgagccgatcgggaagaactggatctcccgccaccaattggaggagtggctattgatgtggtgaaagtagaagtccctgcgacgggccgaacactcgtgctggcttttgtaaaaacgtgcgcagtactggcagcggtgcacgggctgtacatcctgcacgaggttgacctgacgaccgcgcacaaggaagcagagtgggaatttgagcccctcgcctggcgggtttggctggtggtcttctacttcggctgcttgtccttgaccgtctggctgctcgaggggagttacggtggatcggaccaccacgccgcgcgagcccaaagtccagatgtccgcgcgcggcggtcggagcttgatgacaacatcgcgcagatgggagctgtccatggtctggagctcccgcggcgtcaggtcaggcgggagctcctgcaggtttacctcgcatagacgggtcagggcgcgggctagatccaggtgatacctaatttccaggggctggttggtggcggcgtcgatggcttgcaagaggccgcatccccgcggcgcgactacggtaccgcgcggcgggcggtgggccgcgggggtgtccttggatgatgcatctaaaagcggtgacgcgggcgagcccccggaggtagggggggctccggacccgccgggagagggggcaggggcacgtcggcgccgcgcgcgggcaggagctggtgctgcgcgcgtaggttgctggcgaacgcgacgacgcggcggttgatctcctgaatctggcgcctctgcgtgaagacgacgggcccggtgagcttgaacctgaaagagagttcgacagaatcaatttcggtgtcgttgacggcggcctggcgcaaaatctcctgcacgtctcctgagttgtcttgataggcgatctcggccatgaactgctcgatctcttcctcctggagatctccgcgtccggctcgctccacggtggcggcgaggtcgttggaaatgcgggccatgagctgcgagaaggcgttgaggcctccctcgttccagacgcggctgtagaccacgcccccttcggcatcgcgggcgcgcatgaccacctgcgcgagattgagctccacgtgccgggcgaagacggcgtagtttcgcaggcgctgaaagaggtagttgagggtggtggcggtgtgttctgccacgaagaagtacataacccagcgtcgcaacgtggattcgttgataattgttgtgtaggtactccgccgccgagggacctgagcgagtccgcatcgaccggatcggaaaacctctcgagaaaggcgtctaaccagtcacagtcgcaaggtaggctgagcaccgtggcgggcggcagcgggcggcggtcggggttgtttctggcggaggtgctgctgatgatgtaattaaagtaggcggtcttgagacggcggatggtcgacagaagcaccatgtccttgggtccggcctgctgaatgcgcaggcggtcggccatgccccaggcttcgttttgacatcggcgcaggtctttgtagtagtcttgcatgagcctttctaccggcacttcttcttctccttcctcttgtcctgcatctcttgcatctatcgctgcggcggcggcggagtttggccgtaggtggcgccctcttcctcccatgcgtgtgaccccgaagcccctcatcggctgaagcagggctaggtcggcgacaacgcgctcggctaatatggcctgctgcacctgcgtgagggtagactggaagtcatccatgtccacaaagcggtggtatgcgcccgtgttgatggtgtaagtgcagttggccataacggaccagttaacggtctggtgacccggctgcgagagctcggtgtacctgagacgcgagtaagccctcgagtcaaatacgtagtcgttgcaagtccgcaccaggtactggtatcccaccaaaaagtgcggcggcggctggcggtagaggggccagcgtagggtggccggggctccgggggcgagatcttccaacataaggcgatgatatccgtagatgtacctggacatccaggtgatgccggcggcggtggtggaggcgcgcggaaagtcgcggacgcggttccagatgttgcgcagcggcaaaaagtgctccatggtcgggacgctctggccggtcaggcgcgcgcaatcgttgacgctctagcgtgcaaaaggagagcctgtaagcgggcactcttccgtggtctggtggataaattcgcaagggtatcatggcggacgaccggggttcgagccccgtatccggccgtccgccgtgatccatgcggttaccgcccgcgtgtcgaacccaggtgtgcgacgtcagacaacgggggagtgctccttttggcttccttccaggcgcggcggctgctgcgctagcttttttggccactggccgcgcgcagcgtaagcggttaggctggaaagcgaaagcattaagtggctcgctccctgtagccggagggttattttccaagggttgagtcgcgggacccccggttcgagtctcggaccggccggactgcggcgaacgggggtttgcctccccgtcatgcaagaccccgcttgcaaattcctccggaaacagggacgagccccttttttgcttttcccagatgcatccggtgctgcggcagatgcgcccccctcctcagcagcggcaagagcaagagcagcggcagacatgcagggcaccctcccctcctcctaccgcgtcaggaggggcgacatccgcggttgacgcggcagcagatggtgattacgaacccccgcggcgccgggcccggcactacctggacttggaggagggcgagggcctggcgcggctaggagcgccctctcctgagcggcacccaagggtgcagctgaagcgtgatacgcgtgaggcgtacgtgccgcggcagaacctgtttcgcgaccgcgagggagaggagcccgaggagatgcgggatcgaaagttccacgcagggcgcgagctgcggcatggcctgaatcgcgagcggttgctgcgcgaggaggactttgagcccgacgcgcgaaccgggattagtcccgcgcgcgcacacgtggcggccgccgacctggtaaccgcatacgagcagacggtgaaccaggagattaactttcaaaaaagctttaacaaccacgtgcgtacgcttgtggcgcgcgaggaggtggctataggactgatgcatctgtgggactttgtaagcgcgctggagcaaaacccaaatagcaagccgctcatggcgcagctgttccttatagtgcagcacagcagggacaacgaggcattcagggatgcgctgctaaacatagtagagcccgagggccgctggctgctcgatttgataaacatcctgcagagcatagtggtgcaggagcgcagcttgagcctggctgacaaggtggccgccatcaactattccatgcttagcctgggcaagttttacgcccgcaagatataccataccccttacgttcccatagacaaggaggtaaagatcgaggggttctacatgcgcatggcgctgaaggtgcttaccttgagcgacgacctgggcgtttatcgcaacgagcgcatccacaaggccgtgagcgtgagccggcggcgcgagctcagcgaccgcgagctgatgcacagcctgcaaagggccctggctggcacgggcagcggcgatagagaggccgagtcctactttgacgcgggcgctgacctgcgctgggccccaagccgacgcgccctggaggcagctggggccggacctgggctggcggtggcacccgcgcgcgctggcaacgtcggcggcgtggaggaatatgacgaggacgatgagtacgagccagaggacggcgagtactaagcggtgatgtttctgatcagatgatgcaagacgcaacggacccggcggtgcgggcggcgctgcagagccagccgtccggccttaactccacggacgactggcgccaggtcatggaccgcatcatgtcgctgactgcgcgcaatcctgacgcgttccggcagcagccgcaggccaaccggctctccgcaattctggaagcggtggtcccggcgcgcgcaaaccccacgcacgagaaggtgctggcgatcgtaaacgcgctggccgaaaacagggccatccggcccgacgaggccggcctggtctacgacgcgctgcttcagcgcgtggctcgttacaacagcggcaacgtgcagaccaacctggaccggctggtgggggatgtgcgcgaggccgtggcgcagcgtgagcgcgcgcagcagcagggcaacctgggctccatggttgcactaaacgccttcctgagtacacagcccgccaacgtgccgcggggacaggaggactacaccaactttgtgagcgcactgcggctaatggtgactgagacaccgcaaagtgaggtgtaccagtctgggccagactattttttccagaccagtagacaaggcctgcagaccgtaaacctgagccaggctttcaaaaacttgcaggggctgtggggggtgcgggctcccacaggcgaccgcgcgaccgtgtctagcttgctgacgcccaactcgcgcctgttgctgctgctaatagcgcccttcacggacagtggcagcgtgtcccgggacacatacctaggtcacttgctgacactgtaccgcgaggccataggtcaggcgcatgtggacgagcatactttccaggagattacaagtgtcagccgcgcgctggggcaggaggacacgggcagcctggaggcaaccctaaactacctgctgaccaaccggcggcagaagatcccctcgttgcacagtttaaacagcgaggaggagcgcattttgcgctacgtgcagcagagcgtgagccttaacctgatgcgcgacggggtaacgcccagcgtggcgctggacatgaccgcgcgcaacatggaaccgggcatgtatgcctcaaaccggccgtttatcaaccgcctaatggactacttgcatcgcgcggccgccgtgaaccccgagtatttcaccaatgccatcttgaacccgcactggctaccgccccctggtttctacaccgggggattcgaggtgcccgagggtaacgatggattcctctgggacgacatagacgacagcgtgttttccccgcaaccgcagaccctgctagagttgcaacagcgcgagcaggcagaggcggcgctgcgaaaggaaagcttccgcaggccaagcagcttgtccgatctaggcgctgcggccccgcggtcagatgctagtagcccatttccaagcttgatagggtctcttaccagcactcgcaccacccgcccgcgcctgctgggcgaggaggagtacctaaacaactcgctgctgcagccgcagcgcgaaaaaaacctgcctccggcatttcccaacaacgggatagagagcctagtggacaagatgagtagatggaagacgtacgcgcaggagcacagggacgtgccaggcccgcgcccgcccacccgtcgtcaaaggcacgaccgtcagcggggtctggtgtgggaggacgatgactcggcagacgacagcagcgtcctggatttgggagggagtggcaacccgtttgcgcaccttcgccccaggctggggagaatgttttaaaaaaaaaaaagcatgatgcaaaataaaaaactcaccaaggccatggcaccgagcgttggttttcttgtattccccttagtatgcggcgcgcggcgatgtatgaggaaggtcctcctccctcctacgagagtgtggtgagcgcggcgccagtggcggcggcgctgggttctcccttcgatgctcccctggacccgccgtttgtgcctccgcggtacctgcggcctaccggggggagaaacagcatccgttactctgagttggcacccctattcgacaccacccgtgtgtacctggtggacaacaagtcaacggatgtggcatccctgaactaccagaacgaccacagcaactttctgaccacggtcattcaaaacaatgactacagcccgggggaggcaagcacacagaccatcaatcttgacgaccggtcgcactggggcggcgacctgaaaaccatcctgcataccaacatgccaaatgtgaacgagttcatgtttaccaataagtttaaggcgcgggtgatggtgtcgcgcttgcctactaaggacaatcaggtggagctgaaatacgagtgggtggagttcacgctgcccgagggcaactactccgagaccatgaccatagaccttatgaacaacgcgatcgtggagcactacttgaaagtgggcagacagaacggggttctggaaagcgacatcggggtaaagtttgacacccgcaacttcagactggggtttgaccccgtcactggtcttgtcatgcctggggtatatacaaacgaagccttccatccagacatcattttgctgccaggatgcggggtggacttcacccacagccgcctgagcaacttgttgggcatccgcaagcggcaacccttccaggagggctttaggatcacctacgatgatctggagggtggtaacattcccgcactgttggatgtggacgcctaccaggcgagcttgaaagatgacaccgaacagggcgggggtggcgcaggcggcagcaacagcagtggcagcggcgcggaagagaactccaacgcggcagccgcggcaatgcagccggtggaggacatgaacgatcatgccattcgcggcgacacctttgccacacgggctgaggagaagcgcgctgaggccgaagcagcggccgaagctgccgcccccgctgcgcaacccgaggtcgagaagcctcagaagaaaccggtgatcaaacccctgacagaggacagcaagaaacgcagttacaacctaataagcaatgacagcaccttcacccagtaccgcagctggtaccttgcatacaactacggcgaccctcagaccggaatccgctcatggaccctgctttgcactcctgacgtaacctgcggctcggagcaggtctactggtcgttgccagacatgatgcaagaccccgtgaccttccgctccacgcgccagatcagcaactttccggtggtgggcgccgagctgttgcccgtgcactccaagagcttctacaacgaccaggccgtctactcccaactcatccgccagtttacctctctgacccacgtgttcaatcgctttcccgagaaccagattttggcgcgcccgccagcccccaccatcaccaccgtcagtgaaaacgttcctgctctcacagatcacgggacgctaccgctgcgcaacagcatcggaggagtccagcgagtgaccattactgacgccagacgccgcacctgcccctacgtttacaaggccctgggcatagtctcgccgcgcgtcctatcgagccgcactttttgagcaagcatgtccatccttatatcgcccagcaataacacaggctggggcctgcgcttcccaagcaagatgtttggcggggccaagaagcgctccgaccaacacccagtgcgcgtgcgcgggcactaccgcgcgccctggggcgcgcacaaacgcggccgcactgggcgcaccaccgtcgatgacgccatcgacgcggtggtggaggaggcgcgcaactacacgcccacgccgccaccagtgtccacagtggacgcggccattcagaccgtggtgcgcggagcccggcgctatgctaaaatgaagagacggcggaggcgcgtagcacgtcgccaccgccgccgacccggcactgccgcccaacgcgcggcggcggccctgcttaaccgcgcacgtcgcaccggccgacgggcggccatgcgggccgctcgaaggctggccgcgggtattgtcactgtgccccccaggtccaggcgacgagcggccgccgcagcagccgcggccattagtgctatgactcagggtcgcaggggcaacgtgtattgggtgcgcgactcggttagcggcctgcgcgtgcccgtgcgcacccgccccccgcgcaactagattgcaagaaaaaactacttagactcgtactgttgtatgtatccagcggcggcggcgcgcaacgaagctatgtccaagcgcaaaatcaaagaagagatgctccaggtcatcgcgccggagatctatggccccccgaagaaggaagagcaggattacaagccccgaaagctaaagcgggtcaaaaagaaaaagaaagatgatgatgatgaacttgacgacgaggtggaactgctgcacgctaccgcgcccaggcgacgggtacagtggaaaggtcgacgcgtaaaacgtgttttgcgacccggcaccaccgtagtctttacgcccggtgagcgctccacccgcacctacaagcgcgtgtatgatgaggtgtacggcgacgaggacctgcttgagcaggccaacgagcgcctcggggagtttgcctacggaaagcggcataaggacatgctggcgttgccgctggacgagggcaacccaacacctagcctaaagcccgtaacactgcagcaggtgctgcccgcgcttgcaccgtccgaagaaaagcgcggcctaaagcgcgagtctggtgacttggcacccaccgtgcagctgatggtacccaagcgccagcgactggaagatgtcttggaaaaaatgaccgtggaacctgggctggagcccgaggtccgcgtgcggccaatcaagcaggtggcgccgggactgggcgtgcagaccgtggacgttcagatacccactaccagtagcaccagtattgccaccgccacagagggcatggagacacaaacgtccccggttgcctcagcggtggcggatgccgcggtgcaggcggtcgctgcggccgcgtccaagacctctacggaggtgcaaacggacccgtggatgtttcgcgtttcagccccccggcgcccgcgccgttcgaggaagtacggcgccgccagcgcgctactgcccgaatatgccctacatccttccattgcgcctacccccggctatcgtggctacacctaccgccccagaagacgagcaactacccgacgccgaaccaccactggaacccgccgccgccgtcgccgtcgccagcccgtgctggccccgatttccgtgcgcagggtggctcgcgaaggaggcaggaccctggtgctgccaacagcgcgctaccaccccagcatcgtttaaaagccggtctttgtggttcttgcagatatggccctcacctgccgcctccgtttcccggtgccgggattccgaggaagaatgcaccgtaggaggggcatggccggccacggcctgacgggcggcatgcgtcgtgcgcaccaccggcggcggcgcgcgtcgcaccgtcgcatgcgcggcggtatcctgcccctccttattccactgatcgccgcggcgattggcgccgtgcccggaattgcatccgtggccttgcaggcgcagagacactgattaaaaacaagttgcatgtggaaaaatcaaaataaaaagtctggactctcacgctcgcttggtcctgtaactattttgtagaatggaagacatcaactttgcgtctctggccccgcgacacggctcgcgcccgttcatgggaaactggcaagatatcggcaccagcaatatgagcggtggcgccttcagctggggctcgctgtggagcggcattaaaaatttcggttccaccgttaagaactatggcagcaaggcctggaacagcagcacaggccagatgctgagggataagttgaaagagcaaaatttccaacaaaaggtggtagatggcctggcctctggcattagcggggtggtggacctggccaaccaggcagtgcaaaataagattaacagtaagcttgatccccgccctcccgtagaggagcctccaccggccgtggagacagtgtctccagaggggcgtggcgaaaagcgtccgcgccccgacagggaagaaactctggtgacgcaaatagacgagcctccctcgtacgaggaggcactaaagcaaggcctgcccaccacccgtcccatcgcgcccatggctaccggagtgctgggccagcacacacccgtaacgctggacctgcctccccccgccgacacccagcagaaacctgtgctgccaggcccgaccgccgttgttgtaacccgtcctagccgcgcgtccctgcgccgcgccgccagcggtccgcgatcgttgcggcccgtagccagtggcaactggcaaagcacactgaacagcatcgtgggtctgggggtgcaatccctgaagcgccgacgatgcttctgatagctaacgtgtcgtatgtgtgtcatgtatgcgtccatgtcgccgccagaggagctgctgagccgccgcgcgcccgctttccaagatggctaccccttcgatgatgccgcagtggtcttacatgcacatctcgggccaggacgcctcggagtacctgagccccgggctggtgcagtttgcccgcgccaccgagacgtacttcagcctgaataacaagtttagaaaccccacggtggcgcctacgcacgacgtgaccacagaccggtcccagcgtttgacgctgcggttcatccctgtggaccgtgaggatactgcgtactcgtacaaggcgcggttcaccctagctgtgggtgataaccgtgtgctggacatggcttccacgtactttgacatccgcggcgtgctggacaggggccctacttttaagccctactctggcactgcctacaacgccctggctcccaagggtgccccaaatccttgcgaatgggatgaagctgctactgctcttgaaataaacctagaagaagaggacgatgacaacgaagacgaagtagacgagcaagctgagcagcaaaaaactcacgtatttgggcaggcgccttattctggtataaatattacaaaggagggtattcaaataggtgtcgaaggtcaaacacctaaatatgccgataaaacatttcaacctgaacctcaaataggagaatctcagtggtacgaaacagaaattaatcatgcagctgggagagtcctaaaaaagactaccccaatgaaaccatgttacggttcatatgcaaaacccacaaatgaaaatggagggcaaggcattcttgtaaagcaacaaaatggaaagctagaaagtcaagtggaaatgcaatttttctcaactactgaggcagccgcaggcaatggtgataacttgactcctaaagtggtattgtacagtgaagatgtagatatagaaaccccagacactcatatttcttacatgcccactattaaggaaggtaactcacgagaactaatgggccaacaatctatgcccaacaggcctaattacattgcttttagggacaattttattggtctaatgtattacaacagcacgggtaatatgggtgttctggcgggccaagcatcgcagttgaatgctgttgtagatttgcaagacagaaacacagagctttcataccagcttttgcttgattccattggtgatagaaccaggtacttttctatgtggaatcaggctgttgacagctatgatccagatgttagaattattgaaaatcatggaactgaagatgaacttccaaattactgctttccactgggaggtgtgattaatacagagactcttaccaaggtaaaacctaaaacaggtcaggaaaatggatgggaaaaagatgctacagaattttcagataaaaatgaaataagagttggaaataattttgccatggaaatcaatctaaatgccaacctgtggagaaatttcctgtactccaacatagcgctgtatttgcccgacaagctaaagtacagtccttccaacgtaaaaatttctgataacccaaacacctacgactacatgaacaagcgagtggtggctcccgggctagtggactgctacattaaccttggagcacgctggtcccttgactatatggacaacgtcaacccatttaaccaccaccgcaatgctggcctgcgctaccgctcaatgttgctgggcaatggtcgctatgtgcccttccacatccaggtgcctcagaagttctttgccattaaaaacctccttctcctgccgggctcatacacctacgagtggaacttcaggaaggatgttaacatggttctgcagagctccctaggaaatgacctaagggttgacggagccagcattaagtttgatagcatttgcctttacgccaccttcttccccatggcccacaacaccgcctccacgcttgaggccatgcttagaaacgacaccaacgaccagtcctttaacgactatctctccgccgccaacatgctctaccctatacccgccaacgctaccaacgtgcccatatccatcccctcccgcaactgggcggctttccgcggctgggccttcacgcgccttaagactaaggaaaccccatcactgggctcgggctacgacccttattacacctactctggctctataccctacctagatggaaccttttacctcaaccacacctttaagaaggtggccattacctttgactcttctgtcagctggcctggcaatgaccgcctgcttacccccaacgagtttgaaattaagcgctcagttgacggggagggttacaacgttgcccagtgtaacatgaccaaagactggttcctggtacaaatgctagctaactataacattggctaccagggcttctatatcccagagagctacaaggaccgcatgtactccttctttagaaacttccagcccatgagccgtcaggtggtggatgatactaaatacaaggactaccaacaggtgggcatcctacaccaacacaacaactctggatttgttggctaccttgcccccaccatgcgcgaaggacaggcctaccctgctaacttcccctatccgcttataggcaagaccgcagttgacagcattacccagaaaaagtttctttgcgatcgcaccctttggcgcatcccattctccagtaactttatgtccatgggcgcactcacagacctgggccaaaaccttctctacgccaactccgcccacgcgctagacatgacttttgaggtggatcccatggacgagcccacccttctttatgttttgtttgaagtctttgacgtggtccgtgtgcaccagccgcaccgcggcgtcatcgaaaccgtgtacctgcgcacgcccttctcggccggcaacgccacaacataaagaagcaagcaacatcaacaacagctgccgccatgggctccagtgagcaggaactgaaagccattgtcaaagatcttggttgtgggccatattttttgggcacctatgacaagcgctttccaggctttgtttctccacacaagctcgcctgcgccatagtcaatacggccggtcgcgagactgggggcgtacactggatggcctttgcctggaacccgcactcaaaaacatgctacctctttgagccctttggcttttctgaccagcgactcaagcaggtttaccagtttgagtacgagtcactcctgcgccgtagcgccattgcttcttcccccgaccgctgtataacgctggaaaagtccacccaaagcgtacaggggcccaactcggccgcctgtggactattctgctgcatgtttctccacgcctttgccaactggccccaaactcccatggatcacaaccccaccatgaaccttattaccggggtacccaactccatgctcaacagtccccaggtacagcccaccctgcgtcgcaaccaggaacagctctacagcttcctggagcgccactcgccctacttccgcagccacagtgcgcagattaggagcgccacttctttttgtcacttgaaaaacatgtaaaaataatgtactagagacactttcaataaaggcaaatgcttttatttgtacactctcgggtgattatttacccccacccttgccgtctgcgccgtttaaaaatcaaaggggttctgccgcgcatcgctatgcgccactggcagggacacgttgcgatactggtgtttagtgctccacttaaactcaggcacaaccatccgcggcagctcggtgaagttttcactccacaggctgcgcaccatcaccaacgcgtttagcaggtcgggcgccgatatcttgaagtcgcagttggggcctccgccctgcgcgcgcgagttgcgatacacagggttgcagcactggaacactatcagcgccgggtggtgcacgctggccagcacgctcttgtcggagatcagatccgcgtccaggtcctccgcgttgctcagggcgaacggagtcaactttggtagctgccttcccaaaaagggcgcgtgcccaggctttgagttgcactcgcaccgtagtggcatcaaaaggtgaccgtgcccggtctgggcgttaggatacagcgcctgcataaaagccttgatctgcttaaaagccacctgagcctttgcgccttcagagaagaacatgccgcaagacttgccggaaaactgattggccggacaggccgcgtcgtgcacgcagcaccttgcgtcggtgttggagatctgcaccacatttcggccccaccggttcttcacgatcttggccttgctagactgctccttcagcgcgcgctgcccgttttcgctcgtcacatccatttcaatcacgtgctccttatttatcataatgcttccgtgtagacacttaagctcgccttcgatctcagcgcagcggtgcagccacaacgcgcagcccgtgggctcgtgatgcttgtaggtcacctctgcaaacgactgcaggtacgcctgcaggaatcgccccatcatcgtcacaaaggtcttgttgctggtgaaggtcagctgcaacccgcggtgctcctcgttcagccaggtcttgcatacggccgccagagcttccacttggtcaggcagtagtttgaagttcgcctttagatcgttatccacgtggtacttgtccatcagcgcgcgcgcagcctccatgcccttctcccacgcagacacgatcggcacactcagcgggttcatcaccgtaatttcactttccgcttcgctgggctcttcctcttcctcttgcgtccgcataccacgcgccactgggtcgtcttcattcagccgccgcactgtgcgcttacctcctttgccatgcttgattagcaccggtgggttgctgaaacccaccatttgtagcgccacatcttctctttcttcctcgctgtccacgattacctctggtgatggcgggcgctcgggcttgggagaagggcgcttctttttcttcttgggcgcaatggccaaatccgccgccgaggtcgatggccgcgggctgggtgtgcgcggcaccagcgcgtcttgtgatgagtcttcctcgtcctcggactcgatacgccgcctcatccgcttttttgggggcgcccggggaggcggcggcgacggggacggggacgacacgtcctccatggttgggggacgtcgcgccgcaccgcgtccgcgctcgggggtggtttcgcgctgctcctcttcccgactggccatttccttctcctataggcagaaaaagatcatggagtcagtcgagaagaaggacagcctaaccgccccctctgagttcgccaccaccgcctccaccgatgccgccaacgcgcctaccaccttccccgtcgaggcacccccgcttgaggaggaggaagtgattatcgagcaggacccaggttttgtaagcgaagacgacgaggaccgctcagtaccaacagaggataaaaagcaagaccaggacaacgcagaggcaaacgaggaacaagtcgggcggggggacgaaaggcatggcgactacctagatgtgggagacgacgtgctgttgaagcatctgcagcgccagtgcgccattatctgcgacgcgttgcaagagcgcagcgatgtgcccctcgccatagcggatgtcagccttgcctacgaacgccacctattctcaccgcgcgtaccccccaaacgccaagaaaacggcacatgcgagcccaacccgcgcctcaacttctaccccgtatttgccgtgccagaggtgcttgccacctatcacatctttttccaaaactgcaagatacccctatcctgccgtgccaaccgcagccgagcggacaagcagctggccttgcggcagggcgctgtcatacctgatatcgcctcgctcaacgaagtgccaaaaatctttgagggtcttggacgcgacgagaagcgcgcggcaaacgctctgcaacaggaaaacagcgaaaatgaaagtcactctggagtgttggtggaactcgagggtgacaacgcgcgcctagccgtactaaaacgcagcatcgaggtcacccactttgcctacccggcacttaacctaccccccaaggtcatgagcacagtcatgagtgagctgatcgtgcgccgtgcgcagcccctggagagggatgcaaatttgcaagaacaaacagaggagggcctacccgcagttggcgacgagcagctagcgcgctggcttcaaacgcgcgagcctgccgacttggaggagcgacgcaaactaatgatggccgcagtgctcgttaccgtggagcttgagtgcatgcagcggttctttgctgacccggagatgcagcgcaagctagaggaaacattgcactacacctttcgacagggctacgtacgccaggcctgcaagatctccaacgtggagctctgcaacctggtctcctaccttggaattttgcacgaaaaccgccttgggcaaaacgtgcttcattccacgctcaagggcgaggcgcgccgcgactacgtccgcgactgcgtttacttatttctatgctacacctggcagacggccatgggcgtttggcagcagtgcttggaggagtgcaacctcaaggagctgcagaaactgctaaagcaaaacttgaaggacctatggacggccttcaacgagcgctccgtggccgcgcacctggcggacatcattttccccgaacgcctgcttaaaaccctgcaacagggtctgccagacttcaccagtcaaagcatgttgcagaactttaggaactttatcctagagcgctcaggaatcttgcccgccacctgctgtgcacttcctagcgactttgtgcccattaagtaccgcgaatgccctccgccgctttggggccactgctaccttctgcagctagccaactaccttgcctaccactctgacataatggaagacgtgagcggtgacggtctactggagtgtcactgtcgctgcaacctatgcaccccgcaccgctccctggtttgcaattcgcagctgcttaacgaaagtcaaattatcggtacctttgagctgcagggtccctcgcctgacgaaaagtccgcggctccggggttgaaactcactccggggctgtggacgtcggcttaccttcgcaaatttgtacctgaggactaccacgcccacgagattaggttctacgaagaccaatcccgcccgcctaatgcggagcttaccgcctgcgtcattacccagggccacattcttggccaattgcaagccatcaacaaagcccgccaagagtttctgctacgaaagggacggggggtttacttggacccccagtccggcgaggagctcaacccaatccccccgccgccgcagccctatcagcagcagccgcgggcccttgcttcccaggatggcacccaaaaagaagctgcagctgccgccgccacccacggacgaggaggaatactgggacagtcaggcagaggaggttttggacgaggaggaggaggacatgatggaagactgggagagcctagacgaggaagcttccgaggtcgaagaggtgtcagacgaaacaccgtcaccctcggtcgcattcccctcgccggcgccccagaaatcggcaaccggttccagcatggctacaacctccgctcctcaggcgccgccggcactgcccgttcgccgacccaaccgtagatgggacaccactggaaccagggccggtaagtccaagcagccgccgccgttagcccaagagcaacaacagcgccaaggctaccgctcatggcgcgggcacaagaacgccatagttgcttgcttgcaagactgtgggggcaacatctccttcgcccgccgctttcttctctaccatcacggcgtggccttcccccgtaacatcctgcattactaccgtcatctctacagcccatactgcaccggcggcagcggcagcaacagcagcggccacacagaagcaaaggcgaccggatagcaagactctgacaaagcccaagaaatccacagcggcggcagcagcaggaggaggagcgctgcgtctggcgcccaacgaacccgtatcgacccgcgagcttagaaacaggatttttcccactctgtatgctatatttcaacagagcaggggccaagaacaagagctgaaaataaaaaacaggtctctgcgatccctcacccgcagctgcctgtatcacaaaagcgaagatcagcttcggcgcacgctggaagacgcggaggctctcttcagtaaatactgcgcgctgactcttaaggactagtttcgcgccctttctcaaatttaagcgcgaaaactacgtcatctccagcggccacacccggcgccagcacctgttgtcagcgccattatgagcaaggaaattcccacgccctacatgtggagttaccagccacaaatgggacttgcggctggagctgcccaagactactcaacccgaataaactacatgagcgcgggaccccacatgatatcccgggtcaacggaatacgcgcccaccgaaaccgaattctcctggaacaggcggctattaccaccacacctcgtaataaccttaatccccgtagttggcccgctgccctggtgtaccaggaaagtcccgctcccaccactgtggtacttcccagagacgcccaggccgaagttcagatgactaactcaggggcgcagcttgcgggcggctttcgtcacagggtgcggtcgcccgggcagggtataactcacctgacaatcagagggcgaggtattcagctcaacgacgagtcggtgagctcctcgcttggtctccgtccggacgggacatttcagatcggcggcgccggccgctcttcattcacgcctcgtcaggcaatcctaactctgcagacctcgtcctctgagccgcgctctggaggcattggaactctgcaatttattgaggagtttgtgccatcggtctactttaaccccttctcgggacctcccggccactatccggatcaatttattcctaactttgacgcggtaaaggactcggcggacggctacgactgaatgttaagtggagaggcagagcaactgcgcctgaaacacctggtccactgtcgccgccacaagtgctttgcccgcgactccggtgagttttgctactttgaattgcccgaggatcatatcgagggcccggcgcacggcgtccggcttaccgcccagggagagcttgcccgtagcctgattcgggagtttacccagcgccccctgctagttgagcgggacaggggaccctgtgttctcactgtgatttgcaactgtcctaaccctggattacatcaagatcctctagttaatgtcaggtcgcctaagtcgattaactagagtacccggggatcttattccctttaactaataaaaaaaaataataaagcatcacttacttaaaatcagttagcaaatttctgtccagtttattcagcagcacctccttgccctcctcccagctctggtattgcagcttcctcctggctgcaaactttctccacaatctaaatggaatgtcagtttcctcctgttcctgtccatccgcacccactatcttcatgttgttgcagatgaagcgcgcaagaccgtctgaagataccttcaaccccgtgtatccatatgacacggaaaccggtcctccaactgtgccttttcttactcctccctttgtatcccccaatgggtttcaagagagtccccctggggtactctctttgcgcctatccgaacctctagttacctccaatggcatgcttgcgctcaaaatgggcaacggcctctctctggacgaggccggcaaccttacctcccaaaatgtaaccactgtgagcccacctctcaaaaaaaccaagtcaaacataaacctggaaatatctgcacccctcacagttacctcagaagccctaactgtggctgccgccgcacctctaatggtcgcgggcaacacactcaccatgcaatcacaggccccgctaaccgtgcacgactccaaacttagcattgccacccaaggacccctcacagtgtcagaaggaaagctagccctgcaaacatcaggccccctcaccaccaccgatagcagtacccttactatcactgcctcaccccctctaactactgccactggtagcttgggcattgacttgaaagagcccatttatacacaaaatggaaaactaggactaaagtacggggctcctttgcatgtaacagacgacctaaacactttgaccgtagcaactggtccaggtgtgactattaataatacttccttgcaaactaaagttactggagccttgggttttgattcacaaggcaatatgcaacttaatgtagcaggaggactaaggattgattctcaaaacagacgccttatacttgatgttagttatccgtttgatgctcaaaaccaactaaatctaagactaggacagggccctctttttataaactcagcccacaacttggatattaactacaacaaaggcctttacttgtttacagcttcaaacaattccaaaaagcttgaggttaacctaagcactgccaaggggttgatgtttgacgctacagccatagccattaatgcaggagatgggcttgaatttggttcacctaatgcaccaaacacaaatcccctcaaaacaaaaattggccatggcctagaatttgattcaaacaaggctatggttcctaaactaggaactggccttagttttgacagcacaggtgccattacagtaggaaacaaaaataatgataagctaactttgtggaccacaccagctccatctcctaactgtagactaaatgcagagaaagatgctaaactcactttggtcttaacaaaatgtggcagtcaaatacttgctacagtttcagttttggctgttaaaggcagtttggctccaatatctggaacagttcaaagtgctcatcttattataagatttgacgaaaatggagtgctactaaacaattccttcctggacccagaatattggaactttagaaatggagatcttactgaaggcacagcctatacaaacgctgttggatttatgcctaacctatcagcttatccaaaatctcacggtaaaactgccaaaagtaacattgtcagtcaagtttacttaaacggagacaaaactaaacctgtaacactaaccattacactaaacggtacacaggaaacaggagacacaactccaagtgcatactctatgtcattttcatgggactggtctggccacaactacattaatgaaatatttgccacatcctcttacactttttcatacattgcccaagaataaagaatcgtttgtgttatgtttcaacgtgtttatttttcaattgcagaaaatttcaagtcatttttcattcagtagtatagccccaccaccacatagcttatacagatcaccgtaccttaatcaaactcacagaaccctagtattcaacctgccacctccctcccaacacacagagtacacagtcctttctccccggctggccttaaaaagcatcatatcatgggtaacagacatattcttaggtgttatattccacacggtttcctgtcgagccaaacgctcatcagtgatattaataaactccccgggcagctcacttaagttcatgtcgctgtccagctgctgagccacaggctgctgtccaacttgcggttgcttaacgggcggcgaaggagaagtccacgcctacatgggggtagagtcataatcgtgcatcaggatagggcggtggtgctgcagcagcgcgcgaataaactgctgccgccgccgctccgtcctgcaggaatacaacatggcagtggtctcctcagcgatgattcgcaccgcccgcagcataaggcgccttgtcctccgggcacagcagcgcaccctgatctcacttaaatcagcacagtaactgcagcacagcaccacaatattgttcaaaatcccacagtgcaaggcgctgtatccaaagctcatggcggggaccacagaacccacgtggccatcataccacaagcgcaggtagattaagtggcgacccctcataaacacgctggacataaacattacctcttttggcatgttgtaattcaccacctcccggtaccatataaacctctgattaaacatggcgccatccaccaccatcctaaaccagctggccaaaacctgcccgccggctatacactgcagggaaccgggactggaacaatgacagtggagagcccaggactcgtaaccatggatcatcatgctcgtcatgatatcaatgttggcacaacacaggcacacgtgcatacacttcctcaggattacaagctcctcccgcgttagaaccatatcccagggaacaacccattcctgaatcagcgtaaatcccacactgcagggaagacctcgcacgtaactcacgttgtgcattgtcaaagtgttacattcgggcagcagcggatgatcctccagtatggtagcgcgggtttctgtctcaaaaggaggtagacgatccctactgtacggagtgcgccgagacaaccgagatcgtgttggtcgtagtgtcatgccaaatggaacgccggacgtagtcatatttcctgaagcaaaaccaggtgcgggcgtgacaaacagatctgcgtctccggtctcgccgcttagatcgctctgtgtagtagttgtagtatatccactctctcaaagcatccaggcgccccctggcttcgggttctatgtaaactccttcatgcgccgctgccctgataacatccaccaccgcagaataagccacacccagccaacctacacattcgttctgcgagtcacacacgggaggagcgggaagagctggaagaaccatgtttttttttttattccaaaagattatccaaaacctcaaaatgaagatctattaagtgaacgcgctcccctccggtggcgtggtcaaactctacagccaaagaacagataatggcatttgtaagatgttgcacaatggcttccaaaaggcaaacggccctcacgtccaagtggacgtaaaggctaaacccttcagggtgaatctcctctataaacattccagcaccttcaaccatgcccaaataattctcatctcgccaccttctcaatatatctctaagcaaatcccgaatattaagtccggccattgtaaaaatctgctccagagcgccctccaccttcagcctcaagcagcgaatcatgattgcaaaaattcaggttcctcacagacctgtataagattcaaaagcggaacattaacaaaaataccgcgatcccgtaggtcccttcgcagggccagctgaacataatcgtgcaggtctgcacggaccagcgcggccacttccccgccaggaaccatgacaaaagaacccacactgattatgacacgcatactcggagctatgctaaccagcgtagccccgatgtaagcttgttgcatgggcggcgatataaaatgcaaggtgctgctcaaaaaatcaggcaaagcctcgcgcaaaaaagaaagcacatcgtagtcatgctcatgcagataaaggcaggtaagctccggaaccaccacagaaaaagacaccatttttctctcaaacatgtctgcgggtttctgcataaacacaaaataaaataacaaaaaaacatttaaacattagaagcctgtcttacaacaggaaaaacaacccttataagcataagacggactacggccatgccggcgtgaccgtaaaaaaactggtcaccgtgattaaaaagcaccaccgacagctcctcggtcatgtccggagtcataatgtaagactcggtaaacacatcaggttgattcacatcggtcagtgctaaaaagcgaccgaaatagcccgggggaatacatacccgcaggcgtagagacaacattacagcccccataggaggtataacaaaattaataggagagaaaaacacataaacacctgaaaaaccctcctgcctaggcaaaatagcaccctcccgctccagaacaacatacagcgcttccacagcggcagccataacagtcagccttaccagtaaaaaagaaaacctattaaaaaaacaccactcgacacggcaccagctcaatcagtcacagtgtaaaaaagggccaagtgcagagcgagtatatataggactaaaaaatgacgtaacggttaaagtccacaaaaaacacccagaaaaccgcacgcgaacctacgcccagaaacgaaagccaaaaaacccacaacttcctcaaatcgtcacttccgttttcccacgttacgtcacttcccattttaagaaaactacaattcccaacacatacaagttactccgccctaaaacctacgtcacccgccccgttcccacgccccgcgccacgtcacaaactccaccccctcattatcatattggcttcaatccaaaataaggta

SEQ ID NO: 233 - DNA, 9701 bp, synthetic construct
  misc_feature 1..9701: note = vector for IgG1 against T27Y H34A R273Q ACE2 mutant
  misc_feature 2929..2930: note = n is a, c, g, or t
  misc_feature 2934: note = n is a, c, g, or t
  source 1..9701: mol_type = other DNA
ggcgtaatctgctgcttgcaaacaaaaaaaccaccgctaccagcggtggtttgtttgccggatcaagagctaccaactctttttccgaaggtaactggcttcagcagagcgcagataccaaatactgtccttctagtgtagccgtagttaggccaccacttcaagaactctgtagcaccgcctacatacctcgctctgctgaagccagttaccagtggctgctgccagtggcgataagtcgtgtcttaccgggttggactcaagagatagttaccggataaggcgcagcggtcgggctgaacggggggttcgtgcacacagcccagcttggagcgaacgacctacaccgaactgagatacctacagcgtgagctatgagaaagcgccacgcttcccgaagggagaaaggcggacaggtatccggtaagcggcagggtcggaacaggagagcgcacgagggagcttccagggggaaacgcctggtatctttatagtcctgtcgggtttcgccacctctgacttgagcgtcgatttttgtgatgctcgtcaggggggcggagcctatggaaaaacgccagcaacgcaagctagagtttaaacttgacagatgagacaataaccctgataaatgcttcaataatattgaaaaaggaaaagtatgagtattcaacatttccgtgtcgcccttattcccttttttgcggcattttgccttcctgtttttgctcacccagaaacgctggtgaaagtaaaagatgcagaagatcacttgggtgcgcgagtgggttacatcgaactggatctcaacagcggtaagatccttgagagttttcgccccgaagaacgtttcccaatgatgagcacttttaaagttctgctatgtggcgcggtattatcccgtattgatgccgggcaagagcaactcggtcgccgcatacactattctcagaatgacttggttgaatactcaccagtcacagaaaagcatcttacggatggcatgacagtaagagaattatgcagtgctgccataaccatgagtgataacactgcggccaacttacttctgacaactatcggaggaccgaaggagctaaccgcttttttgcacaacatgggggatcatgtaactcgccttgatcgttgggaaccggagctgaatgaagccataccaaacgacgagcgtgacaccacgatgcctgtagcaatggcaacaacgttgcgaaaactattaactggcgaactacttactctagcttcccggcaacaactaatagactggatggaggcggataaagttgcaggaccacttctgcgctcggcacttccggctggctggtttattgctgataaatcaggagccggtgagcgtgggtcacgcggtatcattgcagcactggggccggatggtaagccctcccgtatcgtagttatctacactacggggagtcaggcaactatggatgaacgaaatagacagatcgctgagataggtgcctcactgattaagcattggtaaggataaatttctggtaaggaggacacgtatggaagtgggcaagttggggaagccgtatccgttgctgaatctggcatatgtgggagtataagacgcgcagcgtcgcatcaggcatttttttctgcgccaatgcaaaaaggccatccgtcaggatggcctttcggcataactagggccgccgatatttgaaaatatggcatattgaaaatgtcgccgatgtgagtttctgtgtaactgatatcgccatttttccaaaagtgatttttgggcatacgcgatatctggcgatagcgcttatatcgtttacgggggatggcgatagacgactttggtgacttgggcgattctgtgtgtcgcaaatatcgcagtttcgatataggtgacagacgatatgaggctatatcgccgatagaggcgacatcaagctggcacatggccaatgcatatcgatctatacattgaatcaatattggccattagccatattattcattggttatatagcataaatcaatattggctattggccattgcatacgttgtatccatatcataatatgtacatttatattggctcatgtccaacattaccgccatgttgacattgattattgactagttattaatagtaatcaattacggggtcattagttcatagcccatatatggagttccgcgttacataacttacggtaaatggcccgcctggctgaccgcccaacgacccccgcccattgacgtcaataatgacgtatgttcccatagtaacgccaatagggactttccattgacgtcaatgggtggagtatttacggtaaactgcccacttggcagtacatcaagtgtatcatatgccaagtacgccccctattgacgtcaatgacggtaaatggcccgcctggcattatgcccagtacatgaccttatgggactttcctacttggcagtacatctacgtattagtcatcgctattaccatggtgatgcggttttggcagtacatcaatgggcgtggatagcggtttgactcacggggatttccaagtctccaccccattgacgtcaatgggagtttgttttggcaccaaaatcaacgggactttccaaaatgtcgtaacaactccgccccattgacgcaaatgggcggtaggcgtgtacggtgggaggtctatataagcagagctcgtttagtgaaccgtcagatcgcctggagacgccatccacgctgttttgacctccatagaagacaccgggaccgatccagcctccgcggccgggaacggtgcattggaacgcggattccccgtgccaagagtgacgtaagtaccgcctatagagtctataggcccacccccttggcttcttatgcatgctatactgtttttggcttggggtctatacaccccccgnnttcntcatgttataggtgatggtatagcttagcctataggtgtgggttattgaccattattgaccactccccctattggtgacgatactttccattactaatccataacatggctctttgccacaactctctttattggctatatgccaatacactgtccttcagagactgacacggactctgtatttttacaggatggggtctcatttattatttacaaattcacatatacaacaccaccgtccccagtgcccgcagtttttattaaacataacgtgggatctccacgcgaatctcgggtacgtgttccggacatgggctcttctccggtagcggcggagcttctacatccgagccctgctcccatgcctccagcgactcatggtcgctcggcagctccttgctcctaacagtggaggccagacttaggcacagcacgatgcccaccaccaccagtgtgccgcacaaggccgtggcggtagggtatgtgtctgaaaatgagctcggggagcgggcttgcaccgctgacgcatttggaagacttaaggcagcggcagaagaagatgcaggcagctgagttgttgtgttctgataagagtcagaggtaactcccgttgcggtgctgttaacggtggagggcagtgtagtctgagcagtactcgttgctgccgcgcgcgccaccagacataatagctgacagactaacagactgttcctttccatgggtcttttctgcagtcaccgtccttgacacgaagctgctagcgccaccatgagcagcagtagttggcttctcttgagtttggtggcagtgacagcagcccagagtactatcgaggagcaggctaaatactttctggataagtttaacgccgaggccgaagacttgttctatcaatcttctctcgcttcatggaattacaatactaacatcactgaggagaacgtccagaatatgaacaatgctggcgacaaatggagcgccttcttgaaggagcagtctacccttgcacaaatgtatccactgcaggagatacagaaccttacagtaaagttgcagctccaggctctccagcagaacggatctagcgtgctttcagaggataaaagcaaaaggctgaacaccatacttaataccatgtccacaatttactctactggtaaagtatgtaaccccgacaaccctcaagaatgcctccttcttgagccaggcctcaatgagatcatggctaatagtctggactataatgaaagactgtgggcatgggagtcctggagatctgaagtagggaagcaactgaggcccctttatgaagagtacgtcgtacttaagaatgaaatggcccgcgctaaccactacgaggattacggcgattactggcgtggggactatgaagtaaatggtgtagatggatacgactatagtcgtgggcaattgattgaggatgtggagcacacttttgaggagataaaaccactctatgagcatcttcacgcatatgtgagagctaaactgatgaacgcctacccaagttacatcagtccaatcggatgtctcccagctcacctccttggcgacatgtggggacagttctggaccaatctgtattccctcacagtccctttcgggcaaaagcctaatatagacgtgacagacgcaatggttgatcaggcttgggatgctcaaaggatttttaaggaagctgagaagttttttgtgtcagtcggtttgccaaatatgacacaaggcttctgggaaaatagcatgttgactgatcccggtaatgttcaaaaggctgtgtgtcaccctaccgcttgggaccttgggaaaggtgactttcgaatcttgatgtgtaccaaggtgacaatggatgactttcttacagcccatcatgaaatgggtcacatccagtatgatatggcttatgcagctcaacctttcctcttgagaaatggtgcaaatgaaggttttcatgaagctgtaggggaaataatgtccctgagtgctgcaaccccaaagcatctcaagagtatcggattgttgagcccagattttcaagaagataacgagaccgaaatcaacttccttctgaaacaagccctcacaatagttggtactcttccattcacatacatgctggagaaatggcgttggatggtttttaagggggagatacctaaagatcagtggatgaaaaagtggtgggagatgaagcgtgagatcgtaggggtcgtggagccagtgcctcatgatgagacttactgtgacccagcatcactcttccacgttagcaatgactattcatttatacgttattacactcgcactctttaccagtttcaatttcaggaggctctgtgtcaggctgccaagcatgagggaccccttcacaagtgtgatattagtaacagtactgaggcaggccaaaaactgttcaatatgttgaggcttggcaaaagcgagccatggactctcgccttggaaaatgttgtcggggctaaaaacatgaatgtacgccctctgcttaactattttgagcccctttttacatggctcaaggaccagaataagaactcctttgtcggctggtcaacagactggtctccctatgcagacaaaacacatacttgcccaccttgtcctgcaccagagctgctgggaggtccaagcgtgttcctgtttccacccaagcccaaagacacactgatgatttctcgaactccagaagtgacctgcgtggtcgtggacgtgagccacgaggatcccgaagtgaagttcaactggtacgtggatggcgtggaggtccataatgctaagactaaaccccgggaggaacagtacaacagcacttatagggtcgtgtccgtgctgaccgtcctgcatcaggattggctgaacgggaaggaatataagtgcaaagtgtctaataaggcactgcccgcccctatcgagaaaacaattagcaaggctaagggtcagcctagagaaccacaggtgtacactctgcctccaagtcgcgacgagctgaccaagaaccaggtgtcactgacatgtctggtcaaaggcttttatccctcagatatcgcagtggagtgggaaagcaatggacagcctgagaacaattacaagaccacaccccctgtgctggacagtgatggctcattctttctgtattctaagctgacagtggacaaaagtaggtggcagcagggaaacgtgttctcctgctctgtcatgcacgaagcactgcacaatcattatacccagaagagtctgtcactgagccctggcaaatgagcgataccgattctagaactagatcataatcagccataccacatttgtagaggttttacttgctttaaaaaacctcccacacctccccctgaacctgaaacataaaatgaatgcaattgttgttgttaacttgtttattgcagcttataatggttacaaataaagcaatagcatcacaaatttcacaaataaagcatttttttcactgcattctagttgtggtttgtccaaactcatcaatgtatcttaaggccgcaggtaagccagcccaggcctcgccctccagctcaaggcgggacaggtgccctagagtagcctgcatccagggacaggccccagccgggtgctgacacgtccacctccatctcttcctcaggtctgcccgggtggcatccctgtgacccctccccagtgcctctcctggtcgtggaaggtgctactccagtgcccaccagccttgtcctaataaaattaagttgcatcattttgtttgactaggtgtccttgtataatattatggggtggaggcgggtggtatggagcaaggggcccaagttaacttgtttattgcagcttataatggttacaaataaagcaatagcatcacaaatttcacaaataaagcatttttttcactgcattctagttgtggtttgtccaaactcatcaatgtatcttatcatgtctggatccgcttcaggcaccgggcttgcgggtcatgcaccaggtgcgcggtccttcgggcacctcgacgtcggcggtgacggtgaagccgagccgctcgtagaaggggaggttgcggggcgcggaggtctccaggaaggcgggcaccccggcgcgctcggccgcctccactccggggagcacgacggcgctgcccagacccttgccctggtggtcgggcgagacgccgacggtggccaggaaccacgcgggctccttgggccggtgcggcgccaggaggccttccatctgttgctgcgcggccagcctggaaccgctcaactcggccatgcgcgggccgatctcggcgaacaccgcccccgcttcgacgctctccggcgtggtccagaccgccaccgcggcgccgtcgtccgcgacccacaccttgccgatgtcgagcccgacgcgcgtgaggaagagttcttgcagctcggtgacccgctcgatgtggcggtccgggtcgacggtgtggcgcgtggcggggtagtcggcgaacgcggcggcgagggtgcgtacggcccgggggacgtcgtcgcgggtggcgaggcgcaccgtgggcttgtactcggtcatggtggcctgcagagtcgctctgtgttcgaggccacacgcgtcaccttaatatgcgaagtggacctgggaccgcgccgccccgactgcatctgcgtgttttcgccaatgacaagacgctgggcggggtttgtgtcatcatagaactaaagacatgcaaatatatttcttccggggacaccgccagcaaacgcgagcaacgggccacggggatgaagcagctgcgccactccctgaagatccatcgtctcctaacaagttacatcactcctgcccttcctcaccctcatctccatcacctccttcatctccgtcatctccgtcatcaccctccgcggcagccccttccaccataggtggaaaccagggaggcaaatctactccatcgtcaaagctgcacacagtcaccctgatattgcaggtaggagcgggctttgtcataacaaggtccttaatcgcatccttcaaaacctcagcaaatatatgagtttgtaaaaagaccatgaaataacagacaatggactcccttagcgggccaggttgtgggccgggtccaggggccattccaaaggggagacgactcaatggtgtaagacgacattgtggaatagcaagggcagttcctcgccttaggttgtaaagggaggtcttactacctccatatacgaacacaccggcgacccaagttccttcgtcggtagtcctttctacgtgactcctagccaggagagctcttaaaccttctgcaatgttctcaaatttcgggttggaacctccttgaccacgatgctttccaaaccaccctccttttttgcgcctgcctccatcaccctgacccccgctgcgcgggggcacgtcaggctcaccatctgggccgccttcttggtggtattcaaaataatcggcttcccctacagggtggaaaaatggccttctacctggagggggcctgcgcggtggagacccggatgatgatgactgactactgggactcctgggcctcttttctccacgtccacgacctctccccctggctctttcacgacttccccccctggctctttcacgtcctctaccccggcggcctccactacctcctcgaccccggcctccactacctcctcgaccccggcctccactgcctcctcgaccccggcctccacctcctgctcctgcccctcccgctcctgctcctgctcctgttccaccgtgggtccctttgcagccaatgcaacttggacgtttttggggtctccggacaccatctctatgtcttggccctgatcctgagccgcccggggctcctggtcttccgcctcctcgtcctcgtcctcttccccgtcctcgtccatgtgccatgatggcggcctgcagctgtgttcgaggccgcgcgtgtcaccttaatatgcgaagtggacctgggaccgcgccgccccgactgcatctgcgtgttcgagttcgccaatgacaagacgctgggcggggagatcccccttattaaccctaaacgggtagcatatgcttcccgggtagtagtatatactatccagactaaccctaattcaatagcatatgttacccaacgggaagcatatgctatcgaattagggttagtaaaagggtcctaaggaacagcgatctggatagcatatgctatcctaatctatatctgggtagcatatgctatcctaatctatatctgggtagcataggctatcctaatctatatctgggtagcatatgctatcctaatctatatctgggtagtatatgctatcctaatttatatctgggtagcataggctatcctaatctatatctgggtagcatatgctatcctaatctatatctgggtagtatatgctatcctaatctgtatccgggtagcatatgctatcctcatgcatatacagtcagcatatgatacccagtagtagagtgggagtgctatcctttgcatatgccgccacctcccaaggagatctgtcgacatcgatgggcgcgggtgtacactccgcccatcccgcccctaactccgcccagttccgcccattctccgcctcatggctgactaattttttttatttatgcagaggccgaggccgcctcggcctctgagctattccagaagtagtgaggaggcttttttggaggcctaggcttttgcaaaaagctaattc

SEQ ID NO: 234 - protein, 841 aa, synthetic construct
  REGION 1..841: note = ACE2-Fc IgG Hybrid Protein
  REGION 1..776: note = misc_feature - ACE2 Portion
  REGION 777..841: note = misc_feature - IgG Fc Portion
MSSSSWLLLSLVAVTAAQSTIEEQAKTFLDKFNHEAEDLFYQSSLASWNYNTNITEENVQNMNNAGDKWSAFLKEQSTLAQMYPLQEIQNLTVKLQLQALQQNGSSVLSEDKSKRLNTILNTMSTIYSTGKVCNPDNPQECLLLEPGLNEIMANSLDYNERLWAWESWRSEVGKQLRPLYEEYVVLKNEMARANHYEDYGDYWRGDYEVNGVDGYDYSRGQLIEDVEHTFEEIKPLYEHLHAYVRAKLMNAYPSYISPIGCLPAHLLGDMWGRFWTNLYSLTVPFGQKPNIDVTDAMVDQAWDAQRIFKEAEKFFVSVGLPNMTQGFWENSMLTDPGNVQKAVCHPTAWDLGKGDFRILMCTKVTMDDFLTAHHEMGHIQYDMAYAAQPFLLRNGANEGFHEAVGEIMSLSAATPKHLKSIGLLSPDFQEDNETEINFLLKQALTIVGTLPFTYMLEKWRWMVFKGEIPKDQWMKKWWEMKREIVGVVEPVPHDETYCDPASLFHVSNDYSFIRYYTRTLYQFQFQEALCQAAKHEGPLHKCDISNSTEAGQKLFNMLRLGKSEPWTLALENVVGAKNMNVRPLLNYFEPLFTWLKDQNKNSFVGWSTDWSPYADKTHTCPPCPAPELLGGPSVFLFPPKPKDTLMISRTPEVTCVVVDVSHEDPEVKFNWYVDGVEVHNAKTKPREEQYNSTYRVVSVLTVLHQDWLNGKEYKCKVSNKALPAPIEKTISKAKGQPREPQVYTLPPSRDELTKNQVSLTCLVKGFYPSDIAVEWESNGQPENNYKTTPPVLDSDGSFFLYSKLTVDKSRWQQGNVFSCSVMHEALHNHYTQKSLSLSPGK

SEQ ID NO: 235 - protein, 841 aa, synthetic construct
  REGION 1..841: note = ACE2-Fc IgG R273Q Hybrid Protein
  REGION 1..776: note = misc_feature - ACE2 Portion with R273Q mutation
  REGION 777..841: note = misc_feature - IgG Fc Portion
MSSSSWLLLSLVAVTAAQSTIEEQAKTFLDKFNHEAEDLFYQSSLASWNYNTNITEENVQNMNNAGDKWSAFLKEQSTLAQMYPLQEIQNLTVKLQLQALQQNGSSVLSEDKSKRLNTILNTMSTIYSTGKVCNPDNPQECLLLEPGLNEIMANSLDYNERLWAWESWRSEVGKQLRPLYEEYVVLKNEMARANHYEDYGDYWRGDYEVNGVDGYDYSRGQLIEDVEHTFEEIKPLYEHLHAYVRAKLMNAYPSYISPIGCLPAHLLGDMWGQFWTNLYSLTVPFGQKPNIDVTDAMVDQAWDAQRIFKEAEKFFVSVGLPNMTQGFWENSMLTDPGNVQKAVCHPTAWDLGKGDFRILMCTKVTMDDFLTAHHEMGHIQYDMAYAAQPFLLRNGANEGFHEAVGEIMSLSAATPKHLKSIGLLSPDFQEDNETEINFLLKQALTIVGTLPFTYMLEKWRWMVFKGEIPKDQWMKKWWEMKREIVGVVEPVPHDETYCDPASLFHVSNDYSFIRYYTRTLYQFQFQEALCQAAKHEGPLHKCDISNSTEAGQKLFNMLRLGKSEPWTLALENVVGAKNMNVRPLLNYFEPLFTWLKDQNKNSFVGWSTDWSPYADKTHTCPPCPAPELLGGPSVFLFPPKPKDTLMISRTPEVTCVVVDVSHEDPEVKFNWYVDGVEVHNAKTKPREEQYNSTYRVVSVLTVLHQDWLNGKEYKCKVSNKALPAPIEKTISKAKGQPREPQVYTLPPSRDELTKNQVSLTCLVKGFYPSDIAVEWESNGQPENNYKTTPPVLDSDGSFFLYSKLTVDKSRWQQGNVFSCSVMHEALHNHYTQKSLSLSPGK

SEQ ID NO: 236 - protein, 865 aa, synthetic construct
  REGION 1..865: note = ACE2-Fc IgA Hybrid Protein
  REGION 1..776: note = misc_feature - ACE2 Portion
  REGION 777..865: note = misc_feature - IgA Fc Portion
MSSSSWLLLSLVAVTAAQSTIEEQAKTFLDKFNHEAEDLFYQSSLASWNYNTNITEENVQNMNNAGDKWSAFLKEQSTLAQMYPLQEIQNLTVKLQLQALQQNGSSVLSEDKSKRLNTILNTMSTIYSTGKVCNPDNPQECLLLEPGLNEIMANSLDYNERLWAWESWRSEVGKQLRPLYEEYVVLKNEMARANHYEDYGDYWRGDYEVNGVDGYDYSRGQLIEDVEHTFEEIKPLYEHLHAYVRAKLMNAYPSYISPIGCLPAHLLGDMWGRFWTNLYSLTVPFGQKPNIDVTDAMVDQAWDAQRIFKEAEKFFVSVGLPNMTQGFWENSMLTDPGNVQKAVCHPTAWDLGKGDFRILMCTKVTMDDFLTAHHEMGHIQYDMAYAAQPFLLRNGANEGFHEAVGEIMSLSAATPKHLKSIGLLSPDFQEDNETEINFLLKQALTIVGTLPFTYMLEKWRWMVFKGEIPKDQWMKKWWEMKREIVGVVEPVPHDETYCDPASLFHVSNDYSFIRYYTRTLYQFQFQEALCQAAKHEGPLHKCDISNSTEAGQKLFNMLRLGKSEPWTLALENVVGAKNMNVRPLLNYFEPLFTWLKDQNKNSFVGWSTDWSPYADPSTPPTPSPSTPPTPSPSCCHPRLSLHRPALEDLLLGSEANLTCTLTGLRDASGVTFTWTPSSGKSAVQGPPERDLCGCYSVSSVLPGCAEPWNHGKTFTCTAAYPESKTPLTATLSKSGNTFRPEVHLLPPPSEELALNELVTLTCLARGFSPKDVLVRWLQGSQELPREKYLTWASRQEPSQGTTTFAVTSILRVAAEDWKKGDTFSCMVGHEALPLAFTQKTIDRLAGKPTHVNVSVVMAEVDGTCY

SEQ ID NO: 237 - protein, 865 aa, synthetic construct
  REGION 1..865: note = ACE2-Fc IgA R273Q Hybrid Protein
  REGION 1..776: note = misc_feature - ACE2 Portion with R273Q mutation
  REGION 777..865: note = misc_feature - IgA Fc Portion
MSSSSWLLLSLVAVTAAQSTIEEQAKTFLDKFNHEAEDLFYQSSLASWNYNTNITEENVQNMNNAGDKWSAFLKEQSTLAQMYPLQEIQNLTVKLQLQALQQNGSSVLSEDKSKRLNTILNTMSTIYSTGKVCNPDNPQECLLLEPGLNEIMANSLDYNERLWAWESWRSEVGKQLRPLYEEYVVLKNEMARANHYEDYGDYWRGDYEVNGVDGYDYSRGQLIEDVEHTFEEIKPLYEHLHAYVRAKLMNAYPSYISPIGCLPAHLLGDMWGQFWTNLYSLTVPFGQKPNIDVTDAMVDQAWDAQRIFKEAEKFFVSVGLPNMTQGFWENSMLTDPGNVQKAVCHPTAWDLGKGDFRILMCTKVTMDDFLTAHHEMGHIQYDMAYAAQPFLLRNGANEGFHEAVGEIMSLSAATPKHLKSIGLLSPDFQEDNETEINFLLKQALTIVGTLPFTYMLEKWRWMVFKGEIPKDQWMKKWWEMKREIVGVVEPVPHDETYCDPASLFHVSNDYSFIRYYTRTLYQFQFQEALCQAAKHEGPLHKCDISNSTEAGQKLFNMLRLGKSEPWTLALENVVGAKNMNVRPLLNYFEPLFTWLKDQNKNSFVGWSTDWSPYADPSTPPTPSPSTPPTPSPSCCHPRLSLHRPALEDLLLGSEANLTCTLTGLRDASGVTFTWTPSSGKSAVQGPPERDLCGCYSVSSVLPGCAEPWNHGKTFTCTAAYPESKTPLTATLSKSGNTFRPEVHLLPPPSEELALNELVTLTCLARGFSPKDVLVRWLQGSQELPREKYLTWASRQEPSQGTTTFAVTSILRVAAEDWKKGDTFSCMVGHEALPLAFTQKTIDRLAGKPTHVNVSVVMAEVDGTCY

SEQ ID NO: 238 - protein, 6 aa, synthetic construct
SPYVMH

SEQ ID NO: 239 - protein, 6 aa, synthetic construct
SSYVMH

SEQ ID NO: 240 - protein, 9 aa, synthetic construct
AIWGWTNTY

SEQ ID NO: 241 - protein, 11 aa, synthetic construct
GRELAAFTKTA

SEQ ID NO: 242 - protein, 11 aa, synthetic construct
GEELAAFTKTA

SEQ ID NO: 243 - protein, 9 aa, synthetic construct
DLWGPGFFA

SEQ ID NO: 244 - protein, 39 aa, synthetic construct
YADSVKGRFTISSDNSKNTLYLQMNSLRAEDTAVYYCAR

SEQ ID NO: 245 - protein, 39 aa, synthetic construct
YADSVKGRFTISVDNSKNTLYLQMNSLRAEDTAVYYCAR